European Patent Application EP 4 660 306 A1, published December 10, 2025. Title: Artificial Synthetic Nucleic Acids For Enhancing Protein Expression. Applicant: 株式会社シンプロジェン. The sequence listing filed with the application follows.

SEQUENCE LISTING (339 sequences)

SEQ ID NO: 1 - DNA, 156 bp, synthetic construct
  source 1..156: mol_type = other DNA
tagaggcaagggttgtttttattgactataatacgactcactataaggcgagaccaataataataggtctccgccaccatgcgaagagcacaagtttaagctcttcctgataatagccccgcaggtgatgtcaataacacctgcccccaaaaaaaa

SEQ ID NO: 2 - DNA, 154 bp, synthetic construct
  source 1..154: mol_type = other DNA
tactggttggaagaaagacctctatcgtctctttttttttttttttttttttttttttttttttttttttttttttttttttttttttttttttttttttttttttttttttttttttttttttttttttttgggggcaggtgttattgacatc

SEQ ID NO: 3 - DNA, 28 bp, synthetic construct
  source 1..28: mol_type = other DNA
tagaggcaagggttgtttttattgacta

SEQ ID NO: 4 - DNA, 25 bp, synthetic construct
  source 1..25: mol_type = other DNA
tactggttggaagaaagacctctat

SEQ ID NO: 5 - DNA, 150 bp, synthetic construct
  source 1..150: mol_type = other DNA
tagaggcaagggttgtttttattgactagctcttccatggatagcactgagaacgtcatcaagcccttcatgcgcttcaaggtgcacatggagggctccgtgaacggccacgagttcgagatcgagggcgtgggcgagggcaagccctac

SEQ ID NO: 6 - DNA, 150 bp, synthetic construct
  source 1..150: mol_type = other DNA
gtcggcggggtgcttgatgtacgccttggagccgtagaagaactggggggacaggatgtcccaggcgaagggcagggggccgcccttggtcacttgcagcttggcggtctgggtgccctcgtagggcttgccctcgcccacgccctcgat

SEQ ID NO: 7 - DNA, 150 bp, synthetic construct
  source 1..150: mol_type = other DNA
tccaaggcgtacatcaagcaccccgccgacatccccgactacctcaagcagtccttccccgagggcttcaagtgggagcgcgtgatgaacttcgaggacggcggcgtggtgaccgtgacccaggactcctccctgcaggacggcaccctc

SEQ ID NO: 8 - DNA, 150 bp, synthetic construct
  source 1..150: mol_type = other DNA
cttcagcacgccgtcgcgggggtagttgcgctcagtggagggctcccagcccagagttttcttctgcattacggggccgtcggaggggaagttcacgccgatgaacttcacgtggtagatgagggtgccgtcctgcagggaggagtcctg

SEQ ID NO: 9 - DNA, 150 bp, synthetic construct
  source 1..150: mol_type = other DNA
cgcaactacccccgcgacggcgtgctgaagggcgagaaccacatggcgctgaagctgaagggcggcggccactacctgtgtgagttcaagtccatctacatggccaagaagcccgtgaagctgcccggctaccactacgtggactacaag

SEQ ID NO: 10 - DNA, 147 bp, synthetic construct
  source 1..147: mol_type = other DNA
tactggttggaagaaagacctctatgctcttcgtcactggaacaggtggtggcgggcctcggcgcgctcgtactgctccaccacggtgtagtcctcgttgtgggaggtgatgtcgagcttgtagtccacgtagtggtagccgggcag

SEQ ID NO: 11 - DNA, 200 bp, synthetic construct
  source 1..200: mol_type = other DNA
tagaggcaagggttgtttttattgactaggtctccatagctcgagctggtactgcatgcacgcaatgctagctgcccctttcccgtcctgggtaccccgagtctcccccgacctcgggtcccaggtatgctcccacctccacctgccccactcaccacctctgctagttccagacacctcccaagcacgcagcaatgcag

SEQ ID NO: 12 - DNA, 200 bp, synthetic construct
  source 1..200: mol_type = other DNA
tactggttggaagaaagacctctatggtctcgttttgctagctccagggtgtggctggcacgaaattgaccaaccctggggttagtatagcttagttaaactttcgtttattgctaaaggttaatcactgctgtttcccgtgggggtgtggctaggctaagcgttttgagctgcattgctgcgtgcttgggaggtgtctg

SEQ ID NO: 13 - DNA, 52 bp, synthetic construct
  source 1..52: mol_type = other DNA
aagggagaataaactagtattcttctggtccccacagactcagagagaaccc

SEQ ID NO: 14 - DNA, 52 bp, synthetic construct
  source 1..52: mol_type = other DNA
tggcgggttctctctgagtctgtggggaccagaagaatactagtttattctc

SEQ ID NO: 15 - DNA, 74 bp, synthetic construct
  source 1..74: mol_type = other DNA
aagggctctctgctcctcctgttcgacagtcagccgcatcttcttttgcgtcgccagccgagccacatcgctca

SEQ ID NO: 16 - DNA, 74 bp, synthetic construct
  source 1..74: mol_type = other DNA
tggctgagcgatgtggctcggctggcgacgcaaaagaagatgcggctgactgtcgaacaggaggagcagagagc

SEQ ID NO: 17 - DNA, 68 bp, synthetic construct
  source 1..68: mol_type = other DNA
atagatgtggctcggctggcgacgcaaaagaagatgcggctgactgtcgaacaggaggagcagagagc

SEQ ID NO: 18 - DNA, 68 bp, synthetic construct
  source 1..68: mol_type = other DNA
ttttgctctctgctcctcctgttcgacagtcagccgcatcttcttttgcgtcgccagccgagccacat

SEQ ID NO: 19 - DNA, 68 bp, synthetic construct
  source 1..68: mol_type = other DNA
atagatgtggctcggctggggacgcaaaagaagatccggctgactgtcgaagaggaggagcagagagg

SEQ ID NO: 20 - DNA, 68 bp, synthetic construct
  source 1..68: mol_type = other DNA
ttttcctctctgctcctcctcttcgacagtcagccggatcttcttttgcgtccccagccgagccacat

SEQ ID NO: 21 - DNA, 68 bp, synthetic construct
  source 1..68: mol_type = other DNA
atagatgaggcacgggtggggacccaatagatgatccgggtgagtgtggaagaggtggaccagtgagg

SEQ ID NO: 22 - DNA, 68 bp, synthetic construct
  source 1..68: mol_type = other DNA
ttttcctcactggtccacctcttccacactcacccggatcatctattgggtccccacccgtgcctcat

SEQ ID NO: 23 - DNA, 68 bp, synthetic construct
  source 1..68: mol_type = other DNA
atagatgtgggacggctgcggacgcattagaagaaccggctgtgtgtcgatgaggaggcccagagatg

SEQ ID NO: 24 - DNA, 68 bp, synthetic construct
  source 1..68: mol_type = other DNA
ttttcatctctgggcctcctcatcgacacacagccggttcttctaatgcgtccgcagccgtcccacat

SEQ ID NO: 25 - DNA, 68 bp, synthetic construct
  source 1..68: mol_type = other DNA
atagatgtggctcggcaccggacgcaaaagaactaccggctgactgtccttgaggaggagcagactcg

SEQ ID NO: 26 - DNA, 68 bp, synthetic construct
  source 1..68: mol_type = other DNA
ttttcgagtctgctcctcctcaaggacagtcagccggtagttcttttgcgtccggtgccgagccacat

SEQ ID NO: 27 - DNA, 68 bp, synthetic construct
  source 1..68: mol_type = other DNA
atagtacaccgacggctggcgacgcaaaagaagatgcggctgactgtcgaacaggaggaggtctctcg

SEQ ID NO: 28 - DNA, 68 bp, synthetic construct
  source 1..68: mol_type = other DNA
ttttcgagagacctcctcctgttcgacagtcagccgcatcttcttttgcgtcgccagccgtcggtgta

SEQ ID NO: 29 - DNA, 68 bp, synthetic construct
  source 1..68: mol_type = other DNA
atagatgtggctccgctggcgacggaaaagaagatccggctgactgacgaacaggagcagcagagagc

SEQ ID NO: 30 - DNA, 68 bp, synthetic construct
  source 1..68: mol_type = other DNA
ttttgctctctgctgctcctgttcgtcagtcagccggatcttcttttccgtcgccagcggagccacat

SEQ ID NO: 31 - DNA, 68 bp, synthetic construct
  source 1..68: mol_type = other DNA
atagatgtgcctcggctggggacgcaaaacaagatgcgggtgactgtcgtacaggaggtgcagagagc

SEQ ID NO: 32 - DNA, 68 bp, synthetic construct
  source 1..68: mol_type = other DNA
ttttgctctctgcacctcctgtacgacagtcacccgcatcttgttttgcgtccccagccgaggcacat

SEQ ID NO: 33 - DNA, 68 bp, synthetic construct
  source 1..68: mol_type = other DNA
atagaagtggctcgcctggcgacccaaaagaacatgcggctcactgtcgatcaggaggaccagagagc

SEQ ID NO: 34 - DNA, 68 bp, synthetic construct
  source 1..68: mol_type = other DNA
ttttgctctctggtcctcctgatcgacagtgagccgcatgttcttttgggtcgccaggcgagccactt

SEQ ID NO: 35 - DNA, 68 bp, synthetic construct
  source 1..68: mol_type = other DNA
atagaagtggctccgctggcgtcgcaaaacaagatgccgctgactctcgaacacgaggagctgagagc

SEQ ID NO: 36 - DNA, 68 bp, synthetic construct
  source 1..68: mol_type = other DNA
ttttgctctcagctcctcgtgttcgagagtcagcggcatcttgttttgcgacgccagcggagccactt

SEQ ID NO: 37 - DNA, 68 bp, synthetic construct
  source 1..68: mol_type = other DNA
atagaagtggctgggctggggacgcataagaagttgcggcagactgtggaacagcaggagctgagagc

SEQ ID NO: 38 - DNA, 68 bp, synthetic construct
  source 1..68: mol_type = other DNA
ttttgctctcagctcctgctgttccacagtctgccgcaacttcttatgcgtccccagcccagccactt

SEQ ID NO: 39 - DNA, 68 bp, synthetic construct
  source 1..68: mol_type = other DNA
atagatgtcgctcgcctggccacgcataagaacatgcgcctgacagtcgatcaggacgagcacagagc

SEQ ID NO: 40 - DNA, 68 bp, synthetic construct
  source 1..68: mol_type = other DNA
ttttgctctgtgctcgtcctgatcgactgtcaggcgcatgttcttatgcgtggccaggcgagcgacat

SEQ ID NO: 41 - DNA, 68 bp, synthetic construct
  source 1..68: mol_type = other DNA
atagatgtcgctccgctgccgacccaaatgaagttgcgcctgagtgtccaacacgaggtgcagtgagc

SEQ ID NO: 42 - DNA, 68 bp, synthetic construct
  source 1..68: mol_type = other DNA
ttttgctcactgcacctcgtgttggacactcaggcgcaacttcatttgggtcggcagcggagcgacat

SEQ ID NO: 43 - DNA, 68 bp, synthetic construct
  source 1..68: mol_type = other DNA
atagaagtgcctccgctcgcgtcgctaaacaagttgccgctcactctcgtacacgagcagctgagtgc

SEQ ID NO: 44 - DNA, 68 bp, synthetic construct
  source 1..68: mol_type = other DNA
ttttgcactcagctgctcgtgtacgagagtgagcggcaacttgtttagcgacgcgagcggaggcactt

SEQ ID NO: 45 - DNA, 68 bp, synthetic construct
  source 1..68: mol_type = other DNA
atagatgtccctcggctggcgaccgaaaagaagatgcgcgtgactgtcgaacaccaggagcagagagc

SEQ ID NO: 46 - DNA, 68 bp, synthetic construct
  source 1..68: mol_type = other DNA
ttttgctctctgctcctggtgttcgacagtcacgcgcatcttcttttcggtcgccagccgagggacat

SEQ ID NO: 47 - DNA, 68 bp, synthetic construct
  source 1..68: mol_type = other DNA
atagatgtccctcggctggcctcgcaaaagaacttgcggctgacactcgaacaggaccagcagagagc

SEQ ID NO: 48 - DNA, 68 bp, synthetic construct
  source 1..68: mol_type = other DNA
ttttgctctctgctggtcctgttcgagtgtcagccgcaagttcttttgcgaggccagccgagggacat

SEQ ID NO: 49 - DNA, 68 bp, synthetic construct
  source 1..68: mol_type = other DNA
atagatgtggctcccctggcgacggtaaagaagatcgggctgactgaggaacaggagctgcagagagc

SEQ ID NO: 50 - DNA, 68 bp, synthetic construct
  source 1..68: mol_type = other DNA
ttttgctctctgcagctcctgttcctcagtcagcccgatcttctttaccgtcgccaggggagccacat

SEQ ID NO: 51 - DNA, 68 bp, synthetic construct
  source 1..68: mol_type = other DNA
atagatgtccctcggctgcggacgcaaatcaagatgcgcgtgactgtcctacaggaggtccagagagc

SEQ ID NO: 52 - DNA, 68 bp, synthetic construct
  source 1..68: mol_type = other DNA
ttttgctctctggacctcctgtaggacagtcacgcgcatcttgatttgcgtccgcagccgagggacat

SEQ ID NO: 53 - DNA, 68 bp, synthetic construct
  source 1..68: mol_type = other DNA
atagaactggctcccctggcgtggcaaaactagatgcccctgactcacgaacaccaggagctcagagc

SEQ ID NO: 54 - DNA, 68 bp, synthetic construct
  source 1..68: mol_type = other DNA
ttttgctctgagctcctggtgttcgtgagtcaggggcatctagttttgccacgccaggggagccagtt

SEQ ID NO: 55 - DNA, 68 bp, synthetic construct
  source 1..68: mol_type = other DNA
atagatgtggctcggctggcgagcgaaaagaagatgcggctgactcaggaacaggaggagcagagagc

SEQ ID NO: 56 - DNA, 68 bp, synthetic construct
  source 1..68: mol_type = other DNA
ttttgctctctgctcctcctgttcctgagtcagccgcatcttcttttcgctcgccagccgagccacat

SEQ ID NO: 57 - DNA, 68 bp, synthetic construct
  source 1..68: mol_type = other DNA
atagatgtggctcggctccggacgcaaaagaagaacgggctgactgtcgaagtcgaggagcagagagc

SEQ ID NO: 58 - DNA, 68 bp, synthetic construct
  source 1..68: mol_type = other DNA
ttttgctctctgctcctcgacttcgacagtcagcccgttcttcttttgcgtccggagccgagccacat

SEQ ID NO: 59 - DNA, 68 bp, synthetic construct
  source 1..68: mol_type = other DNA
atagatgtggctgccctggcgacgcatttgaagatgcggcactctgtcgaacagctcgagcagagagc

SEQ ID NO: 60 - DNA, 68 bp, synthetic construct
  source 1..68: mol_type = other DNA
ttttgctctctgctcgagctgttcgacagagtgccgcatcttcaaatgcgtcgccagggcagccacat

SEQ ID NO: 61 - DNA, 52 bp, synthetic construct
  source 1..52: mol_type = other DNA
ataggggttctctctgagtctgtggggaccagaagaatactagtttattctc

SEQ ID NO: 62 - DNA, 52 bp, synthetic construct
  source 1..52: mol_type = other DNA
ttttgagaataaactagtattcttctggtccccacagactcagagagaaccc

SEQ ID NO: 63 - DNA, 52 bp, synthetic construct
  source 1..52: mol_type = other DNA
ataggggttctcactgagtctgaggggaccagtagaatactactttattctc

SEQ ID NO: 64 - DNA, 52 bp, synthetic construct
  source 1..52: mol_type = other DNA
ttttgagaataaagtagtattctactggtcccctcagactcagtgagaaccc

SEQ ID NO: 65 - DNA, 52 bp, synthetic construct
  source 1..52: mol_type = other DNA
ataggggatctctctgtgtctgtggcgaccagaacaatactagattattctc

SEQ ID NO: 66 - DNA, 52 bp, synthetic construct
  source 1..52: mol_type = other DNA
ttttgagaataatctagtattgttctggtcgccacagacacagagagatccc

SEQ ID NO: 67 - DNA, 52 bp, synthetic construct
  source 1..52: mol_type = other DNA
ataggcgttctctgtgagtctctggggacgagaagaaaactagttaattctc

SEQ ID NO: 68 - DNA, 52 bp, synthetic construct
  source 1..52: mol_type = other DNA
ttttgagaattaactagttttcttctcgtccccagagactcacagagaacgc

SEQ ID NO: 69 - DNA, 52 bp, synthetic construct
  source 1..52: mol_type = other DNA
ataggggttcactctgactctgtgcggaccacaagaattctagttaattctc

SEQ ID NO: 70 - DNA, 52 bp, synthetic construct
  source 1..52: mol_type = other DNA
ttttgagaattaactagaattcttgtggtccgcacagagtcagagtgaaccc

SEQ ID NO: 71 - DNA, 52 bp, synthetic construct
  source 1..52: mol_type = other DNA
ataggcgttctgtctgactctgtcgggacgagaagtatacttgtttaatctc

SEQ ID NO: 72 - DNA, 52 bp, synthetic construct
  source 1..52: mol_type = other DNA
ttttgagattaaacaagtatacttctcgtcccgacagagtcagacagaacgc

SEQ ID NO: 73 - DNA, 52 bp, synthetic construct
  source 1..52: mol_type = other DNA
ataggggatctcactgactctgaggggtccagtagaaaactactttaatctc

SEQ ID NO: 74 - DNA, 52 bp, synthetic construct
  source 1..52: mol_type = other DNA
ttttgagattaaagtagttttctactggacccctcagagtcagtgagatccc

SEQ ID NO: 75 - DNA, 52 bp, synthetic construct
  source 1..52: mol_type = other DNA
ataggcgttgtctgtgactctctggcgacgagatgaaaacttgttaattgtc

SEQ ID NO: 76 - DNA, 52 bp, synthetic construct
  source 1..52: mol_type = other DNA
ttttgacaattaacaagttttcatctcgtcgccagagagtcacagacaacgc

SEQ ID NO: 77 - DNA, 52 bp, synthetic construct
  source 1..52: mol_type = other DNA
ataggggttctctgagagtctgtgggctccagaagaatagaagtttattctc

SEQ ID NO: 78 - DNA, 52 bp, synthetic construct
  source 1..52: mol_type = other DNA
ttttgagaataaacttctattcttctggagcccacagactctcagagaaccc

SEQ ID NO: 79 - DNA, 52 bp, synthetic construct
  source 1..52: mol_type = other DNA
ataggccttctctctgacactgtggggacgtgaagaatacttctttattctc

SEQ ID NO: 80 - DNA, 52 bp, synthetic construct
  source 1..52: mol_type = other DNA
ttttgagaataaagaagtattcttcacgtccccacagtgtcagagagaaggc

SEQ ID NO: 81 - DNA, 52 bp, synthetic construct
  source 1..52: mol_type = other DNA
ataggggtagtctctgagtgagtggggacctcaagaatacttctttattctc

SEQ ID NO: 82 - DNA, 52 bp, synthetic construct
  source 1..52: mol_type = other DNA
ttttgagaataaagaagtattcttgaggtccccactcactcagagactaccc

SEQ ID NO: 83 - DNA, 52 bp, synthetic construct
  source 1..52: mol_type = other DNA
ataggggttctcagtgagtctgacgggaccagttgaatactacattattctc

SEQ ID NO: 84 - DNA, 52 bp, synthetic construct
  source 1..52: mol_type = other DNA
ttttgagaataatgtagtattcaactggtcccgtcagactcactgagaaccc

SEQ ID NO: 85 - DNA, 52 bp, synthetic construct
  source 1..52: mol_type = other DNA
ataggggaactctctgtctctgtggccaccagaactatactagaatattctc

SEQ ID NO: 86 - DNA, 52 bp, synthetic construct
  source 1..52: mol_type = other DNA
ttttgagaatattctagtatagttctggtggccacagagacagagagttccc

SEQ ID NO: 87 - DNA, 52 bp, synthetic construct
  source 1..52: mol_type = other DNA
ataggccttctctgagagtctcaggggacgtgaagaaatctagttatttctc

SEQ ID NO: 88 - DNA, 52 bp, synthetic construct
  source 1..52: mol_type = other DNA
ttttgagaaataactagatttcttcacgtcccctgagactctcagagaaggc

SEQ ID NO: 89 - DNA, 52 bp, synthetic construct
  source 1..52: mol_type = other DNA
ataggccttctcagtgagtgagtgggctccagatcaatacatgtttaaactc

SEQ ID NO: 90 - DNA, 52 bp, synthetic construct
  source 1..52: mol_type = other DNA
ttttgagtttaaacatgtattgatctggagcccactcactcactgagaaggc

SEQ ID NO: 91 - DNA, 52 bp, synthetic construct
  source 1..52: mol_type = other DNA
ataggggaagtctctgagtctgaccggaccagaagaaatgtagtttattctc

SEQ ID NO: 92 - DNA, 52 bp, synthetic construct
  source 1..52: mol_type = other DNA
ttttgagaataaactacatttcttctggtccggtcagactcagagacttccc

SEQ ID NO: 93 - DNA, 52 bp, synthetic construct
  source 1..52: mol_type = other DNA
ataggggttctctgacagtctgtgggctgcagaagaatagatgtttattctc

SEQ ID NO: 94 - DNA, 52 bp, synthetic construct
  source 1..52: mol_type = other DNA
ttttgagaataaacatctattcttctgcagcccacagactgtcagagaaccc

SEQ ID NO: 95 - DNA, 52 bp, synthetic construct
  source 1..52: mol_type = other DNA
ataggccatctctctgacagtgtggggacgtcaagaatacttcattattctc

SEQ ID NO: 96 - DNA, 52 bp, synthetic construct
  source 1..52: mol_type = other DNA
ttttgagaataatgaagtattcttgacgtccccacactgtcagagagatggc

SEQ ID NO: 97 - DNA, 52 bp, synthetic construct
  source 1..52: mol_type = other DNA
ataggggtagactctgagtgactggggacctctagaatacttcattattctc

SEQ ID NO: 98 - DNA, 52 bp, synthetic construct
  source 1..52: mol_type = other DNA
ttttgagaataatgaagtattctagaggtccccagtcactcagagtctaccc

SEQ ID NO: 99 - DNA, 65 bp, synthetic construct
  source 1..65: mol_type = other DNA
aaggtcccgcagtcggcgtccagcggctctgcttgttcgtgtgtgtgtcgttgcaggccttattc

SEQ ID NO: 100 - DNA, 65 bp, synthetic construct
  source 1..65: mol_type = other DNA
tggcgaataaggcctgcaacgacacacacacgaacaagcagagccgctggacgccgactgcggga

SEQ ID NO: 101 - DNA, 65 bp, synthetic construct
  source 1..65: mol_type = other DNA
ataggtataaggcctccaacgacactcacacgaactagcagagcccctggacgcccactgcggga

SEQ ID NO: 102 - DNA, 65 bp, synthetic construct
  source 1..65: mol_type = other DNA
tttttcccgcagtgggcgtccaggggctctgctagttcgtgtgagtgtcgttggaggccttatac

SEQ ID NO: 103 - DNA, 65 bp, synthetic construct
  source 1..65: mol_type = other DNA
ataggaataagccctgcaaccacacacactcgaacaaggagagccgcaggacgccgtctgcggga

SEQ ID NO: 104 - DNA, 65 bp, synthetic construct
  source 1..65: mol_type = other DNA
tttttcccgcagacggcgtcctgcggctctccttgttcgagtgtgtgtggttgcagggcttattc

SEQ ID NO: 105 - DNA, 65 bp, synthetic construct
  source 1..65: mol_type = other DNA
ataggaatatggcctgctacgacactcacacgatcaagcagtgccgctgcacgccgagtgcggga

SEQ ID NO: 106 - DNA, 65 bp, synthetic construct
  source 1..65: mol_type = other DNA
tttttcccgcactcggcgtgcagcggcactgcttgatcgtgtgagtgtcgtagcaggccatattc

SEQ ID NO: 107 - DNA, 65 bp, synthetic construct
  source 1..65: mol_type = other DNA
ataggaatatggcctggaacgactcacacaggaacaaccagagcggctggaggccgacagcggga

SEQ ID NO: 108 - DNA, 65 bp, synthetic construct
  source 1..65: mol_type = other DNA
tttttcccgctgtcggcctccagccgctctggttgttcctgtgtgagtcgttccaggccatattc

SEQ ID NO: 109 - DNA, 65 bp, synthetic construct
  source 1..65: mol_type = other DNA
ataggtataagccctgctacgactcacactcgaactagcagtgccgcaggacggcgactccggga

SEQ ID NO: 110 - DNA, 65 bp, synthetic construct
  source 1..65: mol_type = other DNA
tttttcccggagtcgccgtcctgcggcactgctagttcgagtgtgagtcgtagcagggcttatac

SEQ ID NO: 111 - DNA, 65 bp, synthetic construct
  source 1..65: mol_type = other DNA
ataggtataacgcctccaaccacactcacaggaactagcacagcccctggtcgcccactggggga

SEQ ID NO: 112 - DNA, 65 bp, synthetic construct
  source 1..65: mol_type = other DNA
tttttcccccagtgggcgaccaggggctgtgctagttcctgtgagtgtggttggaggcgttatac

SEQ ID NO: 113 - DNA, 65 bp, synthetic construct
  source 1..65: mol_type = other DNA
ataggtatatggcgtgctacgtcactcactcgatcaaccagtgcccctgcacggcgagtgccgga

SEQ ID NO: 114 - DNA, 65 bp, synthetic construct
  source 1..65: mol_type = other DNA
tttttccggcactcgccgtgcaggggcactggttgatcgagtgagtgacgtagcacgccatatac

SEQ ID NO: 115 - DNA, 65 bp, synthetic construct
  source 1..65: mol_type = other DNA
ataggaataacccctgcaacgtgacacacacgttcaagcagaggggctggacgcgcactgcggga

SEQ ID NO: 116 - DNA, 65 bp, synthetic construct
  source 1..65: mol_type = other DNA
tttttcccgcagtgcgcgtccagcccctctgcttgaacgtgtgtgtcacgttgcaggggttattc

SEQ ID NO: 117 - DNA, 65 bp, synthetic construct
  source 1..65: mol_type = other DNA
ataggtttaaggcctcgaacgacactgacacgaacttgcagagcccgtggacgccctctgcggga

SEQ ID NO: 118 - DNA, 65 bp, synthetic construct
  source 1..65: mol_type = other DNA
tttttcccgcagagggcgtccacgggctctgcaagttcgtgtcagtgtcgttcgaggccttaaac

SEQ ID NO: 119 - DNA, 65 bp, synthetic construct
  source 1..65: mol_type = other DNA
ataggaataagcgctgcaacctcacacactggaacaaggtgagccgcacgacgccgtgtgcggga

SEQ ID NO: 120 - DNA, 65 bp, synthetic construct
  source 1..65: mol_type = other DNA
tttttcccgcacacggcgtcgtgcggctcaccttgttccagtgtgtgaggttgcagcgcttattc

SEQ ID NO: 121 - DNA, 65 bp, synthetic construct
  source 1..65: mol_type = other DNA
ataggaatatcgcctgcttcgacactgacacgatgaagcagtcccgctgctcgccgagagcggga

SEQ ID NO: 122 - DNA, 65 bp, synthetic construct
  source 1..65: mol_type = other DNA
tttttcccgctctcggcgagcagcgggactgcttcatcgtgtcagtgtcgaagcaggcgatattc

SEQ ID NO: 123 - DNA, 65 bp, synthetic construct
  source 1..65: mol_type = other DNA
ataggaatatcgcctggtacgactgacacagcaacaacgagagcgcctggagcccgacaccggga

SEQ ID NO: 124 - DNA, 65 bp, synthetic construct
  source 1..65: mol_type = other DNA
tttttcccggtgtcgggctccaggcgctctcgttgttgctgtgtcagtcgtaccaggcgatattc

SEQ ID NO: 125 - DNA, 65 bp, synthetic construct
  source 1..65: mol_type = other DNA
ataggttaaaggcctgcaacctgacacacacgaacttccagagccgctggtgcccgactgcggga

SEQ ID NO: 126 - DNA, 65 bp, synthetic construct
  source 1..65: mol_type = other DNA
tttttcccgcagtcgggcaccagcggctctggaagttcgtgtgtgtcaggttgcaggcctttaac

SEQ ID NO: 127 - DNA, 65 bp, synthetic construct
  source 1..65: mol_type = other DNA
ataggaatatcccctgcaacgactgtcacacgaacaacgtgagccgctggagcgcgactgcggga

SEQ ID NO: 128 - DNA, 65 bp, synthetic construct
  source 1..65: mol_type = other DNA
tttttcccgcagtcgcgctccagcggctcacgttgttcgtgtgacagtcgttgcaggggatattc

SEQ ID NO: 129 - DNA, 65 bp, synthetic construct
  source 1..65: mol_type = other DNA
ataggaataaggcgaccaacgacacagtgacgaacaagctctgccgctggaccgggactgcggga

SEQ ID NO: 130 - DNA, 65 bp, synthetic construct
  source 1..65: mol_type = other DNA
tttttcccgcagtcccggtccagcggcagagcttgttcgtcactgtgtcgttggtcgccttattc

SEQ ID NO: 131 - DNA, 65 bp, synthetic construct
  source 1..65: mol_type = other DNA
ataggttaaaggcctgcttggacacacactgcaacaagcagtcgcgctggacgggcactgcggga

SEQ ID NO: 132 - DNA, 65 bp, synthetic construct
  source 1..65: mol_type = other DNA
tttttcccgcagtgcccgtccagcgcgactgcttgttgcagtgtgtgtccaagcaggcctttaac

SEQ ID NO: 133 - DNA, 65 bp, synthetic construct
  source 1..65: mol_type = other DNA
ataggaataaccgctgcaacgtgtcacacacgttgaagcagagggcctggacgcgctctgcggga

SEQ ID NO: 134 - DNA, 65 bp, synthetic construct
  source 1..65: mol_type = other DNA
tttttcccgcagagcgcgtccaggccctctgcttcaacgtgtgtgacacgttgcagcggttattc

SEQ ID NO: 135 - DNA, 227 bp, synthetic construct
  source 1..227: mol_type = other DNA
taatacgactcactataaggcgagaccaataataataggtctccgccaccatgcgaagagcacaagtttaagctcttcctgataatagccccgcaggtgatgtcaataacacctgcccccaaaaaaaaaaaaaaaaaaaaaaaaaaaaaaaaaaaaaaaaaaaaaaaaaaaaaaaaaaaaaaaaaaaaaaaaaaaaaaaaaaaaaaaaaaaaaaaaaaaaagagacg

SEQ ID NO: 136 - DNA, 1160 bp, synthetic construct
  source 1..1160: mol_type = other DNA
taatacgactcactataagggagaataaactagtattcttctggtccccacagactcagagagaacccgccaccatggatagcactgagaacgtcatcaagcccttcatgcgcttcaaggtgcacatggagggctccgtgaacggccacgagttcgagatcgagggcgtgggcgagggcaagccctacgagggcacccagaccgccaagctgcaagtgaccaagggcggccccctgcccttcgcctgggacatcctgtccccccagttcttctacggctccaaggcgtacatcaagcaccccgccgacatccccgactacctcaagcagtccttccccgagggcttcaagtgggagcgcgtgatgaacttcgaggacggcggcgtggtgaccgtgacccaggactcctccctgcaggacggcaccctcatctaccacgtgaagttcatcggcgtgaacttcccctccgacggccccgtaatgcagaagaaaactctgggctgggagccctccactgagcgcaactacccccgcgacggcgtgctgaagggcgagaaccacatggcgctgaagctgaagggcggcggccactacctgtgtgagttcaagtccatctacatggccaagaagcccgtgaagctgcccggctaccactacgtggactacaagctcgacatcacctcccacaacgaggactacaccgtggtggagcagtacgagcgcgccgaggcccgccaccacctgttccagtgataatagctcgagctggtactgcatgcacgcaatgctagctgcccctttcccgtcctgggtaccccgagtctcccccgacctcgggtcccaggtatgctcccacctccacctgccccactcaccacctctgctagttccagacacctcccaagcacgcagcaatgcagctcaaaacgcttagcctagccacacccccacgggaaacagcagtgattaacctttagcaataaacgaaagtttaactaagctatactaaccccagggttggtcaatttcgtgccagccacaccctggagctagcaaaaaaaaaaaaaaaaaaaaaaaaaaaaaaaaaaaaaaaaaaaaaaaaaaaaaaaaaaaaaaaaaaaaaaaaaaaaaaaaaaaaaaaaaaaaaaaaaaaaagagacg

SEQ ID NO: 137 - DNA, 951 bp, synthetic construct
  source 1..951: mol_type = other DNA
taatacgactcactataagggctctctgctcctcctgttcgacagtcagccgcatcttcttttgcgtcgccagccgagccacatcgctcagccaccatggatagcactgagaacgtcatcaagcccttcatgcgcttcaaggtgcacatggagggctccgtgaacggccacgagttcgagatcgagggcgtgggcgagggcaagccctacgagggcacccagaccgccaagctgcaagtgaccaagggcggccccctgcccttcgcctgggacatcctgtccccccagttcttctacggctccaaggcgtacatcaagcaccccgccgacatccccgactacctcaagcagtccttccccgagggcttcaagtgggagcgcgtgatgaacttcgaggacggcggcgtggtgaccgtgacccaggactcctccctgcaggacggcaccctcatctaccacgtgaagttcatcggcgtgaacttcccctccgacggccccgtaatgcagaagaaaactctgggctgggagccctccactgagcgcaactacccccgcgacggcgtgctgaagggcgagaaccacatggcgctgaagctgaagggcggcggccactacctgtgtgagttcaagtccatctacatggccaagaagcccgtgaagctgcccggctaccactacgtggactacaagctcgacatcacctcccacaacgaggactacaccgtggtggagcagtacgagcgcgccgaggcccgccaccacctgttccagtgataatagatgtggctcggctggcgacgcaaaagaagatgcggctgactgtcgaacaggaggagcagagagcaaaaaaaaaaaaaaaaaaaaaaaaaaaaaaaaaaaaaaaaaaaaaaaaaaaaaaaaaaaaaaaaaaaaaaaaaaaaaaaaaaaaaaaaaaaaaaaaaaaaagagacg

SEQ ID NO: 138 - DNA, 951 bp, synthetic construct
  source 1..951: mol_type = other DNA
taatacgactcactataagggctctctgctcctcctgttcgacagtcagccgcatcttcttttgcgtcgccagccgagccacatcgctcagccaccatggatagcactgagaacgtcatcaagcccttcatgcgcttcaaggtgcacatggagggctccgtgaacggccacgagttcgagatcgagggcgtgggcgagggcaagccctacgagggcacccagaccgccaagctgcaagtgaccaagggcggccccctgcccttcgcctgggacatcctgtccccccagttcttctacggctccaaggcgtacatcaagcaccccgccgacatccccgactacctcaagcagtccttccccgagggcttcaagtgggagcgcgtgatgaacttcgaggacggcggcgtggtgaccgtgacccaggactcctccctgcaggacggcaccctcatctaccacgtgaagttcatcggcgtgaacttcccctccgacggccccgtaatgcagaagaaaactctgggctgggagccctccactgagcgcaactacccccgcgacggcgtgctgaagggcgagaaccacatggcgctgaagctgaagggcggcggccactacctgtgtgagttcaagtccatctacatggccaagaagcccgtgaagctgcccggctaccactacgtggactacaagctcgacatcacctcccacaacgaggactacaccgtggtggagcagtacgagcgcgccgaggcccgccaccacctgttccagtgataatagatgtggctcggctggggacgcaaaagaagatccggctgactgtcgaagaggaggagcagagaggaaaaaaaaaaaaaaaaaaaaaaaaaaaaaaaaaaaaaaaaaaaaaaaaaaaaaaaaaaaaaaaaaaaaaaaaaaaaaaaaaaaaaaaaaaaaaaaaaaaaagagacg

SEQ ID NO: 139 - DNA, 951 bp, synthetic construct
  source 1..951: mol_type = other DNA
taatacgactcactataagggctctctgctcctcctgttcgacagtcagccgcatcttcttttgcgtcgccagccgagccacatcgctcagccaccatggatagcactgagaacgtcatcaagcccttcatgcgcttcaaggtgcacatggagggctccgtgaacggccacgagttcgagatcgagggcgtgggcgagggcaagccctacgagggcacccagaccgccaagctgcaagtgaccaagggcggccccctgcccttcgcctgggacatcctgtccccccagttcttctacggctccaaggcgtacatcaagcaccccgccgacatccccgactacctcaagcagtccttccccgagggcttcaagtgggagcgcgtgatgaacttcgaggacggcggcgtggtgaccgtgacccaggactcctccctgcaggacggcaccctcatctaccacgtgaagttcatcggcgtgaacttcccctccgacggccccgtaatgcagaagaaaactctgggctgggagccctccactgagcgcaactacccccgcgacggcgtgctgaagggcgagaaccacatggcgctgaagctgaagggcggcggccactacctgtgtgagttcaagtccatctacatggccaagaagcccgtgaagctgcccggctaccactacgtggactacaagctcgacatcacctcccacaacgaggactacaccgtggtggagcagtacgagcgcgccgaggcccgccaccacctgttccagtgataatagatgaggcacgggtggggacccaatagatgatccgggtgagtgtggaagaggtggaccagtgaggaaaaaaaaaaaaaaaaaaaaaaaaaaaaaaaaaaaaaaaaaaaaaaaaaaaaaaaaaaaaaaaaaaaaaaaaaaaaaaaaaaaaaaaaaaaaaaaaaaaaagagacg

SEQ ID NO: 140 - DNA, 951 bp, synthetic construct
  source 1..951: mol_type = other DNA
taatacgactcactataagggctctctgctcctcctgttcgacagtcagccgcatcttcttttgcgtcgccagccgagccacatcgctcagccaccatggatagcactgagaacgtcatcaagcccttcatgcgcttcaaggtgcacatggagggctccgtgaacggccacgagttcgagatcgagggcgtgggcgagggcaagccctacgagggcacccagaccgccaagctgcaagtgaccaagggcggccccctgcccttcgcctgggacatcctgtccccccagttcttctacggctccaaggcgtacatcaagcaccccgccgacatccccgactacctcaagcagtccttccccgagggcttcaagtgggagcgcgtgatgaacttcgaggacggcggcgtggtgaccgtgacccaggactcctccctgcaggacggcaccctcatctaccacgtgaagttcatcggcgtgaacttcccctccgacggccccgtaatgcagaagaaaactctgggctgggagccctccactgagcgcaactacccccgcgacggcgtgctgaagggcgagaaccacatggcgctgaagctgaagggcggcggccactacctgtgtgagttcaagtccatctacatggccaagaagcccgtgaagctgcccggctaccactacgtggactacaagctcgacatcacctcccacaacgaggactacaccgtggtggagcagtacgagcgcgccgaggcccgccaccacctgttccagtgataatagatgtgggacggctgcggacgcattagaagaaccggctgtgtgtcgatgaggaggcccagagatgaaaaaaaaaaaaaaaaaaaaaaaaaaaaaaaaaaaaaaaaaaaaaaaaaaaaaaaaaaaaaaaaaaaaaaaaaaaaaaaaaaaaaaaaaaaaaaaaaaaaagagacg

SEQ ID NO: 141 - DNA, 951 bp, synthetic construct
  source 1..951: mol_type = other DNA
taatacgactcactataagggctctctgctcctcctgttcgacagtcagccgcatcttcttttgcgtcgccagccgagccacatcgctcagccaccatggatagcactgagaacgtcatcaagcccttcatgcgcttcaaggtgcacatggagggctccgtgaacggccacgagttcgagatcgagggcgtgggcgagggcaagccctacgagggcacccagaccgccaagctgcaagtgaccaagggcggccccctgcccttcgcctgggacatcctgtccccccagttcttctacggctccaaggcgtacatcaagcaccccgccgacatccccgactacctcaagcagtccttccccgagggcttcaagtgggagcgcgtgatgaacttcgaggacggcggcgtggtgaccgtgacccaggactcctccctgcaggacggcaccctcatctaccacgtgaagttcatcggcgtgaacttcccctccgacggccccgtaatgcagaagaaaactctgggctgggagccctccactgagcgcaactacccccgcgacggcgtgctgaagggcgagaaccacatggcgctgaagctgaagggcggcggccactacctgtgtgagttcaagtccatctacatggccaagaagcccgtgaagctgcccggctaccactacgtggactacaagctcgacatcacctcccacaacgaggactacaccgtggtggagcagtacgagcgcgccgaggcccgccaccacctgttccagtgataatagatgtggctcggcaccggacgcaaaagaactaccggctgactgtccttgaggaggagcagactcgaaaaaaaaaaaaaaaaaaaaaaaaaaaaaaaaaaaaaaaaaaaaaaaaaaaaaaaaaaaaaaaaaaaaaaaaaaaaaaaaaaaaaaaaaaaaaaaaaaaaagagacg

SEQ ID NO: 142 - DNA, 951 bp, synthetic construct
  source 1..951: mol_type = other DNA
taatacgactcactataagggctctctgctcctcctgttcgacagtcagccgcatcttcttttgcgtcgccagccgagccacatcgctcagccaccatggatagcactgagaacgtcatcaagcccttcatgcgcttcaaggtgcacatggagggctccgtgaacggccacgagttcgagatcgagggcgtgggcgagggcaagccctacgagggcacccagaccgccaagctgcaagtgaccaagggcggccccctgcccttcgcctgggacatcctgtccccccagttcttctacggctccaaggcgtacatcaagcaccccgccgacatccccgactacctcaagcagtccttccccgagggcttcaagtgggagcgcgtgatgaacttcgaggacggcggcgtggtgaccgtgacccaggactcctccctgcaggacggcaccctcatctaccacgtgaagttcatcggcgtgaacttcccctccgacggccccgtaatgcagaagaaaactctgggctgggagccctccactgagcgcaactacccccgcgacggcgtgctgaagggcgagaaccacatggcgctgaagctgaagggcggcggccactacctgtgtgagttcaagtccatctacatggccaagaagcccgtgaagctgcccggctaccactacgtggactacaagctcgacatcacctcccacaacgaggactacaccgtggtggagcagtacgagcgcgccgaggcccgccaccacctgttccagtgataatagtacaccgacggctggcgacgcaaaagaagatgcggctgactgtcgaacaggaggaggtctctcgaaaaaaaaaaaaaaaaaaaaaaaaaaaaaaaaaaaaaaaaaaaaaaaaaaaaaaaaaaaaaaaaaaaaaaaaaaaaaaaaaaaaaaaaaaaaaaaaaaaaagagacg

SEQ ID NO: 143 - DNA, 951 bp, synthetic construct
  source 1..951: mol_type = other DNA
taatacgactcactataagggctctctgctcctcctgttcgacagtcagccgcatcttcttttgcgtcgccagccgagccacatcgctcagccaccatggatagcactgagaacgtcatcaagcccttcatgcgcttcaaggtgcacatggagggctccgtgaacggccacgagttcgagatcgagggcgtgggcgagggcaagccctacgagggcacccagaccgccaagctgcaagtgaccaagggcggccccctgcccttcgcctgggacatcctgtccccccagttcttctacggctccaaggcgtacatcaagcaccccgccgacatccccgactacctcaagcagtccttccccgagggcttcaagtgggagcgcgtgatgaacttcgaggacggcggcgtggtgaccgtgacccaggactcctccctgcaggacggcaccctcatctaccacgtgaagttcatcggcgtgaacttcccctccgacggccccgtaatgcagaagaaaactctgggctgggagccctccactgagcgcaactacccccgcgacggcgtgctgaagggcgagaaccacatggcgctgaagctgaagggcggcggccactacctgtgtgagttcaagtccatctacatggccaagaagcccgtgaagctgcccggctaccactacgtggactacaagctcgacatcacctcccacaacgaggactacaccgtggtggagcagtacgagcgcgccgaggcccgccaccacctgttccagtgataatagatgtggctccgctggcgacggaaaagaagatccggctgactgacgaacaggagcagcagagagcaaaaaaaaaaaaaaaaaaaaaaaaaaaaaaaaaaaaaaaaaaaaaaaaaaaaaaaaaaaaaaaaaaaaaaaaaaaaaaaaaaaaaaaaaaaaaaaaaaaaagagacg

SEQ ID NO: 144 - DNA, 951 bp, synthetic construct
  source 1..951: mol_type = other DNA
taatacgactcactataagggctctctgctcctcctgttcgacagtcagccgcatcttcttttgcgtcgccagccgagccacatcgctcagccaccatggatagcactgagaacgtcatcaagcccttcatgcgcttcaaggtgcacatggagggctccgtgaacggccacgagttcgagatcgagggcgtgggcgagggcaagccctacgagggcacccagaccgccaagctgcaagtgaccaagggcggccccctgcccttcgcctgggacatcctgtccccccagttcttctacggctccaaggcgtacatcaagcaccccgccgacatccccgactacctcaagcagtccttccccgagggcttcaagtgggagcgcgtgatgaacttcgaggacggcggcgtggtgaccgtgacccaggactcctccctgcaggacggcaccctcatctaccacgtgaagttcatcggcgtgaacttcccctccgacggccccgtaatgcagaagaaaactctgggctgggagccctccactgagcgcaactacccccgcgacggcgtgctgaagggcgagaaccacatggcgctgaagctgaagggcggcggccactacctgtgtgagttcaagtccatctacatggccaagaagcccgtgaagctgcccggctaccactacgtggactacaagctcgacatcacctcccacaacgaggactacaccgtggtggagcagtacgagcgcgccgaggcccgccaccacctgttccagtgataatagatgtgcctcggctggggacgcaaaacaagatgcgggtgactgtcgtacaggaggtgcagagagcaaaaaaaaaaaaaaaaaaaaaaaaaaaaaaaaaaaaaaaaaaaaaaaaaaaaaaaaaaaaaaaaaaaaaaaaaaaaaaaaaaaaaaaaaaaaaaaaaaaaagagacg

SEQ ID NO: 145 - DNA, 951 bp, synthetic construct
  source 1..951: mol_type = other DNA
taatacgactcactataagggctctctgctcctcctgttcgacagtcagccgcatcttcttttgcgtcgccagccgagccacatcgctcagccaccatggatagcactgagaacgtcatcaagcccttcatgcgcttcaaggtgcacatggagggctccgtgaacggccacgagttcgagatcgagggcgtgggcgagggcaagccctacgagggcacccagaccgccaagctgcaagtgaccaagggcggccccctgcccttcgcctgggacatcctgtccccccagttcttctacggctccaaggcgtacatcaagcaccccgccgacatccccgactacctcaagcagtccttccccgagggcttcaagtgggagcgcgtgatgaacttcgaggacggcggcgtggtgaccgtgacccaggactcctccctgcaggacggcaccctcatctaccacgtgaagttcatcggcgtgaacttcccctccgacggccccgtaatgcagaagaaaactctgggctgggagccctccactgagcgcaactacccccgcgacggcgtgctgaagggcgagaaccacatggcgctgaagctgaagggcggcggccactacctgtgtgagttcaagtccatctacatggccaagaagcccgtgaagctgcccggctaccactacgtggactacaagctcgacatcacctcccacaacgaggactacaccgtggtggagcagtacgagcgcgccgaggcccgccaccacctgttccagtgataatagaagtggctcgcctggcgacccaaaagaacatgcggctcactgtcgatcaggaggaccagagagcaaaaaaaaaaaaaaaaaaaaaaaaaaaaaaaaaaaaaaaaaaaaaaaaaaaaaaaaaaaaaaaaaaaaaaaaaaaaaaaaaaaaaaaaaaaaaaaaaaaaagagacg

SEQ ID NO: 146 - DNA, 951 bp, synthetic construct
  source 1..951: mol_type = other DNA
taatacgactcactataagggctctctgctcctcctgttcgacagtcagccgcatcttcttttgcgtcgccagccgagccacatcgctcagccaccatggatagcactgagaacgtcatcaagcccttcatgcgcttcaaggtgcacatggagggctccgtgaacggccacgagttcgagatcgagggcgtgggcgagggcaagccctacgagggcacccagaccgccaagctgcaagtgaccaagggcggccccctgcccttcgcctgggacatcctgtccccccagttcttctacggctccaaggcgtacatcaagcaccccgccgacatccccgactacctcaagcagtccttccccgagggcttcaagtgggagcgcgtgatgaacttcgaggacggcggcgtggtgaccgtgacccaggactcctccctgcaggacggcaccctcatctaccacgtgaagttcatcggcgtgaacttcccctccgacggccccgtaatgcagaagaaaactctgggctgggagccctccactgagcgcaactacccccgcgacggcgtgctgaagggcgagaaccacatggcgctgaagctgaagggcggcggccactacctgtgtgagttcaagtccatctacatggccaagaagcccgtgaagctgcccggctaccactacgtggactacaagctcgacatcacctcccacaacgaggactacaccgtggtggagcagtacgagcgcgccgaggcccgccaccacctgttccagtgataatagaagtggctccgctggcgtcgcaaaacaagatgccgctgactctcgaacacgaggagctgagagcaaaaaaaaaaaaaaaaaaaaaaaaaaaaaaaaaaaaaaaaaaaaaaaaaaaaaaaaaaaaaaaaaaaaaaaaaaaaaaaaaaaaaaaaaaaaaaaaaaaaagagacg

SEQ ID NO: 147 - DNA, 951 bp, synthetic construct
  source 1..951: mol_type = other DNA
taatacgactcactataagggctctctgctcctcctgttcgacagtcagccgcatcttcttttgcgtcgccagccgagccacatcgctcagccaccatggatagcactgagaacgtcatcaagcccttcatgcgcttcaaggtgcacatggagggctccgtgaacggccacgagttcgagatcgagggcgtgggcgagggcaagccctacgagggcacccagaccgccaagctgcaagtgaccaagggcggccccctgcccttcgcctgggacatcctgtccccccagttcttctacggctccaaggcgtacatcaagcaccccgccgacatccccgactacctcaagcagtccttccccgagggcttcaagtgggagcgcgtgatgaacttcgaggacggcggcgtggtgaccgtgacccaggactcctccctgcaggacggcaccctcatctaccacgtgaagttcatcggcgtgaacttcccctccgacggccccgtaatgcagaagaaaactctgggctgggagccctccactgagcgcaactacccccgcgacggcgtgctgaagggcgagaaccacatggcgctgaagctgaagggcggcggccactacctgtgtgagttcaagtccatctacatggccaagaagcccgtgaagctgcccggctaccactacgtggactacaagctcgacatcacctcccacaacgaggactacaccgtggtggagcagtacgagcgcgccgaggcccgccaccacctgttccagtgataatagaagtggctgggctggggacgcataagaagttgcggcagactgtggaacagcaggagctgagagcaaaaaaaaaaaaaaaaaaaaaaaaaaaaaaaaaaaaaaaaaaaaaaaaaaaaaaaaaaaaaaaaaaaaaaaaaaaaaaaaaaaaaaaaaaaaaaaaaaaaagagacg

SEQ ID NO: 148 - DNA, 951 bp, synthetic construct
  source 1..951: mol_type = other DNA
taatacgactcactataagggctctctgctcctcctgttcgacagtcagccgcatcttcttttgcgtcgccagccgagccacatcgctcagccaccatggatagcactgagaacgtcatcaagcccttcatgcgcttcaaggtgcacatggagggctccgtgaacggccacgagttcgagatcgagggcgtgggcgagggcaagccctacgagggcacccagaccgccaagctgcaagtgaccaagggcggccccctgcccttcgcctgggacatcctgtccccccagttcttctacggctccaaggcgtacatcaagcaccccgccgacatccccgactacctcaagcagtccttccccgagggcttcaagtgggagcgcgtgatgaacttcgaggacggcggcgtggtgaccgtgacccaggactcctccctgcaggacggcaccctcatctaccacgtgaagttcatcggcgtgaacttcccctccgacggccccgtaatgcagaagaaaactctgggctgggagccctccactgagcgcaactacccccgcgacggcgtgctgaagggcgagaaccacatggcgctgaagctgaagggcggcggccactacctgtgtgagttcaagtccatctacatggccaagaagcccgtgaagctgcccggctaccactacgtggactacaagctcgacatcacctcccacaacgaggactacaccgtggtggagcagtacgagcgcgccgaggcccgccaccacctgttccagtgataatagatgtcgctcgcctggccacgcataagaacatgcgcctgacagtcgatcaggacgagcacagagcaaaaaaaaaaaaaaaaaaaaaaaaaaaaaaaaaaaaaaaaaaaaaaaaaaaaaaaaaaaaaaaaaaaaaaaaaaaaaaaaaaaaaaaaaaaaaaaaaaaaagagacg

SEQ ID NO: 149 - DNA, 951 bp, synthetic construct
  source 1..951: mol_type = other DNA
taatacgactcactataagggctctctgctcctcctgttcgacagtcagccgcatcttcttttgcgtcgccagccgagccacatcgctcagccaccatggatagcactgagaacgtcatcaagcccttcatgcgcttcaaggtgcacatggagggctccgtgaacggccacgagttcgagatcgagggcgtgggcgagggcaagccctacgagggcacccagaccgccaagctgcaagtgaccaagggcggccccctgcccttcgcctgggacatcctgtccccccagttcttctacggctccaaggcgtacatcaagcaccccgccgacatccccgactacctcaagcagtccttccccgagggcttcaagtgggagcgcgtgatgaacttcgaggacggcggcgtggtgaccgtgacccaggactcctccctgcaggacggcaccctcatctaccacgtgaagttcatcggcgtgaacttcccctccgacggccccgtaatgcagaagaaaactctgggctgggagccctccactgagcgcaactacccccgcgacggcgtgctgaagggcgagaaccacatggcgctgaagctgaagggcggcggccactacctgtgtgagttcaagtccatctacatggccaagaagcccgtgaagctgcccggctaccactacgtggactacaagctcgacatcacctcccacaacgaggactacaccgtggtggagcagtacgagcgcgccgaggcccgccaccacctgttccagtgataatagatgtcgctccgctgccgacccaaatgaagttgcgcctgagtgtccaacacgaggtgcagtgagcaaaaaaaaaaaaaaaaaaaaaaaaaaaaaaaaaaaaaaaaaaaaaaaaaaaaaaaaaaaaaaaaaaaaaaaaaaaaaaaaaaaaaaaaaaaaaaaaaaaaagagacg

SEQ ID NO: 150 - DNA, 951 bp, synthetic construct
  source 1..951: mol_type = other DNA
taatacgactcactataagggctctctgctcctcctgttcgacagtcagccgcatcttcttttgcgtcgccagccgagccacatcgctcagccaccatggatagcactgagaacgtcatcaagcccttcatgcgcttcaaggtgcacatggagggctccgtgaacggccacgagttcgagatcgagggcgtgggcgagggcaagccctacgagggcacccagaccgccaagctgcaagtgaccaagggcggccccctgcccttcgcctgggacatcctgtccccccagttcttctacggctccaaggcgtacatcaagcaccccgccgacatccccgactacctcaagcagtccttccccgagggcttcaagtgggagcgcgtgatgaacttcgaggacggcggcgtggtgaccgtgacccaggactcctccctgcaggacggcaccctcatctaccacgtgaagttcatcggcgtgaacttcccctccgacggccccgtaatgcagaagaaaactctgggctgggagccctccactgagcgcaactacccccgcgacggcgtgctgaagggcgagaaccacatggcgctgaagctgaagggcggcggccactacctgtgtgagttcaagtccatctacatggccaagaagcccgtgaagctgcccggctaccactacgtggactacaagctcgacatcacctcccacaacgaggactacaccgtggtggagcagtacgagcgcgccgaggcccgccaccacctgttccagtgataatagaagtgcctccgctcgcgtcgctaaacaagttgccgctcactctcgtacacgagcagctgagtgcaaaaaaaaaaaaaaaaaaaaaaaaaaaaaaaaaaaaaaaaaaaaaaaaaaaaaaaaaaaaaaaaaaaaaaaaaaaaaaaaaaaaaaaaaaaaaaaaaaaaagagacg

SEQ ID NO: 151 - DNA, 951 bp, synthetic construct
  source 1..951: mol_type = other DNA
taatacgactcactataagggctctctgctcctcctgttcgacagtcagccgcatcttcttttgcgtcgccagccgagccacatcgctcagccaccatggatagcactgagaacgtcatcaagcccttcatgcgcttcaaggtgcacatggagggctccgtgaacggccacgagttcgagatcgagggcgtgggcgagggcaagccctacgagggcacccagaccgccaagctgcaagtgaccaagggcggccccctgcccttcgcctgggacatcctgtccccccagttcttctacggctccaaggcgtacatcaagcaccccgccgacatccccgactacctcaagcagtccttccccgagggcttcaagtgggagcgcgtgatgaacttcgaggacggcggcgtggtgaccgtgacccaggactcctccctgcaggacggcaccctcatctaccacgtgaagttcatcggcgtgaacttcccctccgacggccccgtaatgcagaagaaaactctgggctgggagccctccactgagcgcaactacccccgcgacggcgtgctgaagggcgagaaccacatggcgctgaagctgaagggcggcggccactacctgtgtgagttcaagtccatctacatggccaagaagcccgtgaagctgcccggctaccactacgtggactacaagctcgacatcacctcccacaacgaggactacaccgtggtggagcagtacgagcgcgccgaggcccgccaccacctgttccagtgataatagatgtccctcggctggcgaccgaaaagaagatgcgcgtgactgtcgaacaccaggagcagagagcaaaaaaaaaaaaaaaaaaaaaaaaaaaaaaaaaaaaaaaaaaaaaaaaaaaaaaaaaaaaaaaaaaaaaaaaaaaaaaaaaaaaaaaaaaaaaaaaaaaaagagacg

SEQ ID NO: 152 - DNA, 951 bp, synthetic construct
  source 1..951: mol_type = other DNA
taatacgactcactataagggctctctgctcctcctgttcgacagtcagccgcatcttcttttgcgtcgccagccgagccacatcgctcagccaccatggatagcactgagaacgtcatcaagcccttcatgcgcttcaaggtgcacatggagggctccgtgaacggccacgagttcgagatcgagggcgtgggcgagggcaagccctacgagggcacccagaccgccaagctgcaagtgaccaagggcggccccctgcccttcgcctgggacatcctgtccccccagttcttctacggctccaaggcgtacatcaagcaccccgccgacatccccgactacctcaagcagtccttccccgagggcttcaagtgggagcgcgtgatgaacttcgaggacggcggcgtggtgaccgtgacccaggactcctccctgcaggacggcaccctcatctaccacgtgaagttcatcggcgtgaacttcccctccgacggccccgtaatgcagaagaaaactctgggctgggagccctccactgagcgcaactacccccgcgacggcgtgctgaagggcgagaaccacatggcgctgaagctgaagggcggcggccactacctgtgtgagttcaagtccatctacatggccaagaagcccgtgaagctgcccggctaccactacgtggactacaagctcgacatcacctcccacaacgaggactacaccgtggtggagcagtacgagcgcgccgaggcccgccaccacctgttccagtgataatagatgtccctcggctggcctcgcaaaagaacttgcggctgacactcgaacaggaccagcagagagcaaaaaaaaaaaaaaaaaaaaaaaaaaaaaaaaaaaaaaaaaaaaaaaaaaaaaaaaaaaaaaaaaaaaaaaaaaaaaaaaaaaaaaaaaaaaaaaaaaaaagagacg

SEQ ID NO: 153 - DNA, 951 bp, synthetic construct
  source 1..951: mol_type = other DNA
taatacgactcactataagggctctctgctcctcctgttcgacagtcagccgcatcttcttttgcgtcgccagccgagccacatcgctcagccaccatggatagcactgagaacgtcatcaagcccttcatgcgcttcaaggtgcacatggagggctccgtgaacggccacgagttcgagatcgagggcgtgggcgagggcaagccctacgagggcacccagaccgccaagctgcaagtgaccaagggcggccccctgcccttcgcctgggacatcctgtccccccagttcttctacggctccaaggcgtacatcaagcaccccgccgacatccccgactacctcaagcagtccttccccgagggcttcaagtgggagcgcgtgatgaacttcgaggacggcggcgtggtgaccgtgacccaggactcctccctgcaggacggcaccctcatctaccacgtgaagttcatcggcgtgaacttcccctccgacggccccgtaatgcagaagaaaactctgggctgggagccctccactgagcgcaactacccccgcgacggcgtgctgaagggcgagaaccacatggcgctgaagctgaagggcggcggccactacctgtgtgagttcaagtccatctacatggccaagaagcccgtgaagctgcccggctaccactacgtggactacaagctcgacatcacctcccacaacgaggactacaccgtggtggagcagtacgagcgcgccgaggcccgccaccacctgttccagtgataatagatgtggctcccctggcgacggtaaagaagatcgggctgactgaggaacaggagctgcagagagcaaaaaaaaaaaaaaaaaaaaaaaaaaaaaaaaaaaaaaaaaaaaaaaaaaaaaaaaaaaaaaaaaaaaaaaaaaaaaaaaaaaaaaaaaaaaaaaaaaaaagagacg

SEQ ID NO: 154 - DNA, 951 bp, synthetic construct
  source 1..951: mol_type = other DNA
taatacgactcactataagggctctctgctcctcctgttcgacagtcagccgcatcttcttttgcgtcgccagccgagccacatcgctcagccaccatggatagcactgagaacgtcatcaagcccttcatgcgcttcaaggtgcacatggagggctccgtgaacggccacgagttcgagatcgagggcgtgggcgagggcaagccctacgagggcacccagaccgccaagctgcaagtgaccaagggcggccccctgcccttcgcctgggacatcctgtccccccagttcttctacggctccaaggcgtacatcaagcaccccgccgacatccccgactacctcaagcagtccttccccgagggcttcaagtgggagcgcgtgatgaacttcgaggacggcggcgtggtgaccgtgacccaggactcctccctgcaggacggcaccctcatctaccacgtgaagttcatcggcgtgaacttcccctccgacggccccgtaatgcagaagaaaactctgggctgggagccctccactgagcgcaactacccccgcgacggcgtgctgaagggcgagaaccacatggcgctgaagctgaagggcggcggccactacctgtgtgagttcaagtccatctacatggccaagaagcccgtgaagctgcccggctaccactacgtggactacaagctcgacatcacctcccacaacgaggactacaccgtggtggagcagtacgagcgcgccgaggcccgccaccacctgttccagtgataatagatgtccctcggctgcggacgcaaatcaagatgcgcgtgactgtcctacaggaggtccagagagcaaaaaaaaaaaaaaaaaaaaaaaaaaaaaaaaaaaaaaaaaaaaaaaaaaaaaaaaaaaaaaaaaaaaaaaaaaaaaaaaaaaaaaaaaaaaaaaaaaaaagagacg

SEQ ID NO: 155 - DNA, 951 bp, synthetic construct
  source 1..951: mol_type = other DNA
taatacgactcactataagggctctctgctcctcctgttcgacagtcagccgcatcttcttttgcgtcgccagccgagccacatcgctcagccaccatggatagcactgagaacgtcatcaagcccttcatgcgcttcaaggtgcacatggagggctccgtgaacggccacgagttcgagatcgagggcgtgggcgagggcaagccctacgagggcacccagaccgccaagctgcaagtgaccaagggcggccccctgcccttcgcctgggacatcctgtccccccagttcttctacggctccaaggcgtacatcaagcaccccgccgacatccccgactacctcaagcagtccttccccgagggcttcaagtgggagcgcgtgatgaacttcgaggacggcggcgtggtgaccgtgacccaggactcctccctgcaggacggcaccctcatctaccacgtgaagttcatcggcgtgaacttcccctccgacggccccgtaatgcagaagaaaactctgggctgggagccctccactgagcgcaactacccccgcgacggcgtgctgaagggcgagaaccacatggcgctgaagctgaagggcggcggccactacctgtgtgagttcaagtccatctacatggccaagaagcccgtgaagctgcccggctaccactacgtggactacaagctcgacatcacctcccacaacgaggactacaccgtggtggagcagtacgagcgcgccgaggcccgccaccacctgttccagtgataatagaactggctcccctggcgtggcaaaactagatgcccctgactcacgaacaccaggagctcagagcaaaaaaaaaaaaaaaaaaaaaaaaaaaaaaaaaaaaaaaaaaaaaaaaaaaaaaaaaaaaaaaaaaaaaaaaaaaaaaaaaaaaaaaaaaaaaaaaaaaaagagacg

SEQ ID NO: 156 - DNA, 951 bp, synthetic construct
  source 1..951: mol_type = other DNA
taatacgactcactataagggctctctgctcctcctgttcgacagtcagccgcatcttcttttgcgtcgccagccgagccacatcgctcagccaccatggatagcactgagaacgtcatcaagcccttcatgcgcttcaaggtgcacatggagggctccgtgaacggccacgagttcgagatcgagggcgtgggcgagggcaagccctacgagggcacccagaccgccaagctgcaagtgaccaagggcggccccctgcccttcgcctgggacatcctgtccccccagttcttctacggctccaaggcgtacatcaagcaccccgccgacatccccgactacctcaagcagtccttccccgagggcttcaagtgggagcgcgtgatgaacttcgaggacggcggcgtggtgaccgtgacccaggactcctccctgcaggacggcaccctcatctaccacgtgaagttcatcggcgtgaacttcccctccgacggccccgtaatgcagaagaaaactctgggctgggagccctccactgagcgcaactacccccgcgacggcgtgctgaagggcgagaaccacatggcgctgaagctgaagggcggcggccactacctgtgtgagttcaagtccatctacatggccaagaagcccgtgaagctgcccggctaccactacgtggactacaagctcgacatcacctcccacaacgaggactacaccgtggtggagcagtacgagcgcgccgaggcccgccaccacctgttccagtgataatagatgtggctcggctggcgagcgaaaagaagatgcggctgactcaggaacaggaggagcagagagcaaaaaaaaaaaaaaaaaaaaaaaaaaaaaaaaaaaaaaaaaaaaaaaaaaaaaaaaaaaaaaaaaaaaaaaaaaaaaaaaaaaaaaaaaaaaaaaaaaaaagagacg

SEQ ID NO: 157 - DNA, 951 bp, synthetic construct
  source 1..951: mol_type = other DNA
taatacgactcactataagggctctctgctcctcctgttcgacagtcagccgcatcttcttttgcgtcgccagccgagccacatcgctcagccaccatggatagcactgagaacgtcatcaagcccttcatgcgcttcaaggtgcacatggagggctccgtgaacggccacgagttcgagatcgagggcgtgggcgagggcaagccctacgagggcacccagaccgccaagctgcaagtgaccaagggcggccccctgcccttcgcctgggacatcctgtccccccagttcttctacggctccaaggcgtacatcaagcaccccgccgacatccccgactacctcaagcagtccttccccgagggcttcaagtgggagcgcgtgatgaacttcgaggacggcggcgtggtgaccgtgacccaggactcctccctgcaggacggcaccctcatctaccacgtgaagttcatcggcgtgaacttcccctccgacggccccgtaatgcagaagaaaactctgggctgggagccctccactgagcgcaactacccccgcgacggcgtgctgaagggcgagaaccacatggcgctgaagctgaagggcggcggccactacctgtgtgagttcaagtccatctacatggccaagaagcccgtgaagctgcccggctaccactacgtggactacaagctcgacatcacctcccacaacgaggactacaccgtggtggagcagtacgagcgcgccgaggcccgccaccacctgttccagtgataatagatgtggctcggctccggacgcaaaagaagaacgggctgactgtcgaagtcgaggagcagagagcaaaaaaaaaaaaaaaaaaaaaaaaaaaaaaaaaaaaaaaaaaaaaaaaaaaaaaaaaaaaaaaaaaaaaaaaaaaaaaaaaaaaaaaaaaaaaaaaaaaaagagacg

SEQ ID NO: 158 - DNA, 951 bp, synthetic construct
  source 1..951: mol_type = other DNA
taatacgactcactataagggctctctgctcctcctgttcgacagtcagccgcatcttcttttgcgtcgccagccgagccacatcgctcagccaccatggatagcactgagaacgtcatcaagcccttcatgcgcttcaaggtgcacatggagggctccgtgaacggccacgagttcgagatcgagggcgtgggcgagggcaagccctacgagggcacccagaccgccaagctgcaagtgaccaagggcggccccctgcccttcgcctgggacatcctgtccccccagttcttctacggctccaaggcgtacatcaagcaccccgccgacatccccgactacctcaagcagtccttccccgagggcttcaagtgggagcgcgtgatgaacttcgaggacggcggcgtggtgaccgtgacccaggactcctccctgcaggacggcaccctcatctaccacgtgaagttcatcggcgtgaacttcccctccgacggccccgtaatgcagaagaaaactctgggctgggagccctccactgagcgcaactacccccgcgacggcgtgctgaagggcgagaaccacatggcgctgaagctgaagggcggcggccactacctgtgtgagttcaagtccatctacatggccaagaagcccgtgaagctgcccggctaccactacgtggactacaagctcgacatcacctcccacaacgaggactacaccgtggtggagcagtacgagcgcgccgaggcccgccaccacctgttccagtgataatagatgtggctgccctggcgacgcatttgaagatgcggcactctgtcgaacagctcgagcagagagcaaaaaaaaaaaaaaaaaaaaaaaaaaaaaaaaaaaaaaaaaaaaaaaaaaaaaaaaaaaaaaaaaaaaaaaaaaaaaaaaaaaaaaaaaaaaaaaaaaaaagagacg

SEQ ID NO: 159 - DNA, 913 bp, synthetic construct
  source 1..913: mol_type = other DNA
taatacgactcactataagggagaataaactagtattcttctggtccccacagactcagagagaacccgccaccatggatagcactgagaacgtcatcaagcccttcatgcgcttcaaggtgcacatggagggctccgtgaacggccacgagttcgagatcgagggcgtgggcgagggcaagccctacgagggcacccagaccgccaagctgcaagtgaccaagggcggccccctgcccttcgcctgggacatcctgtccccccagttcttctacggctccaaggcgtacatcaagcaccccgccgacatccccgactacctcaagcagtccttccccgagggcttcaagtgggagcgcgtgatgaacttcgaggacggcggcgtggtgaccgtgacccaggactcctccctgcaggacggcaccctcatctaccacgtgaagttcatcggcgtgaacttcccctccgacggccccgtaatgcagaagaaaactctgggctgggagccctccactgagcgcaactacccccgcgacggcgtgctgaagggcgagaaccacatggcgctgaagctgaagggcggcggccactacctgtgtgagttcaagtccatctacatggccaagaagcccgtgaagctgcccggctaccactacgtggactacaagctcgacatcacctcccacaacgaggactacaccgtggtggagcagtacgagcgcgccgaggcccgccaccacctgttccagtgataataggggttctctctgagtctgtggggaccagaagaatactagtttattctcaaaaaaaaaaaaaaaaaaaaaaaaaaaaaaaaaaaaaaaaaaaaaaaaaaaaaaaaaaaaaaaaaaaaaaaaaaaaaaaaaaaaaaaaaaaaaaaaaaaaagagacg

SEQ ID NO: 160 - DNA, 913 bp, synthetic construct
  source 1..913: mol_type = other DNA
taatacgactcactataagggagaataaactagtattcttctggtccccacagactcagagagaacccgccaccatggatagcactgagaacgtcatcaagcccttcatgcgcttcaaggtgcacatggagggctccgtgaacggccacgagttcgagatcgagggcgtgggcgagggcaagccctacgagggcacccagaccgccaagctgcaagtgaccaagggcggccccctgcccttcgcctgggacatcctgtccccccagttcttctacggctccaaggcgtacatcaagcaccccgccgacatccccgactacctcaagcagtccttccccgagggcttcaagtgggagcgcgtgatgaacttcgaggacggcggcgtggtgaccgtgacccaggactcctccctgcaggacggcaccctcatctaccacgtgaagttcatcggcgtgaacttcccctccgacggccccgtaatgcagaagaaaactctgggctgggagccctccactgagcgcaactacccccgcgacggcgtgctgaagggcgagaaccacatggcgctgaagctgaagggcggcggccactacctgtgtgagttcaagtccatctacatggccaagaagcccgtgaagctgcccggctaccactacgtggactacaagctcgacatcacctcccacaacgaggactacaccgtggtggagcagtacgagcgcgccgaggcccgccaccacctgttccagtgataataggggttctcactgagtctgaggggaccagtagaatactactttattctcaaaaaaaaaaaaaaaaaaaaaaaaaaaaaaaaaaaaaaaaaaaaaaaaaaaaaaaaaaaaaaaaaaaaaaaaaaaaaaaaaaaaaaaaaaaaaaaaaaaaagagacg

SEQ ID NO: 161 - DNA, 913 bp, synthetic construct
  source 1..913: mol_type = other DNA
taatacgactcactataagggagaataaactagtattcttctggtccccacagactcagagagaacccgccaccatggatagcactgagaacgtcatcaagcccttcatgcgcttcaaggtgcacatggagggctccgtgaacggccacgagttcgagatcgagggcgtgggcgagggcaagccctacgagggcacccagaccgccaagctgcaagtgaccaagggcggccccctgcccttcgcctgggacatcctgtccccccagttcttctacggctccaaggcgtacatcaagcaccccgccgacatccccgactacctcaagcagtccttccccgagggcttcaagtgggagcgcgtgatgaacttcgaggacggcggcgtggtgaccgtgacccaggactcctccctgcaggacggcaccctcatctaccacgtgaagttcatcggcgtgaacttcccctccgacggccccgtaatgcagaagaaaactctgggctgggagccctccactgagcgcaactacccccgcgacggcgtgctgaagggcgagaaccacatggcgctgaagctgaagggcggcggccactacctgtgtgagttcaagtccatctacatggccaagaagcccgtgaagctgcccggctaccactacgtggactacaagctcgacatcacctcccacaacgaggactacaccgtggtggagcagtacgagcgcgccgaggcccgccaccacctgttccagtgataataggggatctctctgtgtctgtggcgaccagaacaatactagattattctcaaaaaaaaaaaaaaaaaaaaaaaaaaaaaaaaaaaaaaaaaaaaaaaaaaaaaaaaaaaaaaaaaaaaaaaaaaaaaaaaaaaaaaaaaaaaaaaaaaaaagagacg

SEQ ID NO: 162 - DNA, 913 bp, synthetic construct
  source 1..913: mol_type = other DNA
taatacgactcactataagggagaataaactagtattcttctggtccccacagactcagagagaacccgccaccatggatagcactgagaacgtcatcaagcccttcatgcgcttcaaggtgcacatggagggctccgtgaacggccacgagttcgagatcgagggcgtgggcgagggcaagccctacgagggcacccagaccgccaagctgcaagtgaccaagggcggccccctgcccttcgcctgggacatcctgtccccccagttcttctacggctccaaggcgtacatcaagcaccccgccgacatccccgactacctcaagcagtccttccccgagggcttcaagtgggagcgcgtgatgaacttcgaggacggcggcgtggtgaccgtgacccaggactcctccctgcaggacggcaccctcatctaccacgtgaagttcatcggcgtgaacttcccctccgacggccccgtaatgcagaagaaaactctgggctgggagccctccactgagcgcaactacccccgcgacggcgtgctgaagggcgagaaccacatggcgctgaagctgaagggcggcggccactacctgtgtgagttcaagtccatctacatggccaagaagcccgtgaagctgcccggctaccactacgtggactacaagctcgacatcacctcccacaacgaggactacaccgtggtggagcagtacgagcgcgccgaggcccgccaccacctgttccagtgataataggcgttctctgtgagtctctggggacgagaagaaaactagttaattctcaaaaaaaaaaaaaaaaaaaaaaaaaaaaaaaaaaaaaaaaaaaaaaaaaaaaaaaaaaaaaaaaaaaaaaaaaaaaaaaaaaaaaaaaaaaaaaaaaaaaagagacg

SEQ ID NO: 163 - DNA, 913 bp, synthetic construct
  source 1..913: mol_type = other DNA
taatacgactcactataagggagaataaactagtattcttctggtccccacagactcagagagaacccgccaccatggatagcactgagaacgtcatcaagcccttcatgcgcttcaaggtgcacatggagggctccgtgaacggccacgagttcgagatcgagggcgtgggcgagggcaagccctacgagggcacccagaccgccaagctgcaagtgaccaagggcggccccctgcccttcgcctgggacatcctgtccccccagttcttctacggctccaaggcgtacatcaagcaccccgccgacatccccgactacctcaagcagtccttccccgagggcttcaagtgggagcgcgtgatgaacttcgaggacggcggcgtggtgaccgtgacccaggactcctccctgcaggacggcaccctcatctaccacgtgaagttcatcggcgtgaacttcccctccgacggccccgtaatgcagaagaaaactctgggctgggagccctccactgagcgcaactacccccgcgacggcgtgctgaagggcgagaaccacatggcgctgaagctgaagggcggcggccactacctgtgtgagttcaagtccatctacatggccaagaagcccgtgaagctgcccggctaccactacgtggactacaagctcgacatcacctcccacaacgaggactacaccgtggtggagcagtacgagcgcgccgaggcccgccaccacctgttccagtgataataggggttcactctgactctgtgcggaccacaagaattctagttaattctcaaaaaaaaaaaaaaaaaaaaaaaaaaaaaaaaaaaaaaaaaaaaaaaaaaaaaaaaaaaaaaaaaaaaaaaaaaaaaaaaaaaaaaaaaaaaaaaaaaaaagagacg

SEQ ID NO: 164 - DNA, 913 bp, synthetic construct
  source 1..913: mol_type = other DNA
taatacgactcactataagggagaataaactagtattcttctggtccccacagactcagagagaacccgccaccatggatagcactgagaacgtcatcaagcccttcatgcgcttcaaggtgcacatggagggctccgtgaacggccacgagttcgagatcgagggcgtgggcgagggcaagccctacgagggcacccagaccgccaagctgcaagtgaccaagggcggccccctgcccttcgcctgggacatcctgtccccccagttcttctacggctccaaggcgtacatcaagcaccccgccgacatccccgactacctcaagcagtccttccccgagggcttcaagtgggagcgcgtgatgaacttcgaggacggcggcgtggtgaccgtgacccaggactcctccctgcaggacggcaccctcatctaccacgtgaagttcatcggcgtgaacttcccctccgacggccccgtaatgcagaagaaaactctgggctgggagccctccactgagcgcaactacccccgcgacggcgtgctgaagggcgagaaccacatggcgctgaagctgaagggcggcggccactacctgtgtgagttcaagtccatctacatggccaagaagcccgtgaagctgcccggctaccactacgtggactacaagctcgacatcacctcccacaacgaggactacaccgtggtggagcagtacgagcgcgccgaggcccgccaccacctgttccagtgataataggcgttctgtctgactctgtcgggacgagaagtatacttgtttaatctcaaaaaaaaaaaaaaaaaaaaaaaaaaaaaaaaaaaaaaaaaaaaaaaaaaaaaaaaaaaaaaaaaaaaaaaaaaaaaaaaaaaaaaaaaaaaaaaaaaaaagagacg

SEQ ID NO: 165 - DNA, 913 bp, synthetic construct
  source 1..913: mol_type = other DNA
taatacgactcactataagggagaataaactagtattcttctggtccccacagactcagagagaacccgccaccatggatagcactgagaacgtcatcaagcccttcatgcgcttcaaggtgcacatggagggctccgtgaacggccacgagttcgagatcgagggcgtgggcgagggcaagccctacgagggcacccagaccgccaagctgcaagtgaccaagggcggccccctgcccttcgcctgggacatcctgtccccccagttcttctacggctccaaggcgtacatcaagcaccccgccgacatccccgactacctcaagcagtccttccccgagggcttcaagtgggagcgcgtgatgaacttcgaggacggcggcgtggtgaccgtgacccaggactcctccctgcaggacggcaccctcatctaccacgtgaagttcatcggcgtgaacttcccctccgacggccccgtaatgcagaagaaaactctgggctgggagccctccactgagcgcaactacccccgcgacggcgtgctgaagggcgagaaccacatggcgctgaagctgaagggcggcggccactacctgtgtgagttcaagtccatctacatggccaagaagcccgtgaagctgcccggctaccactacgtggactacaagctcgacatcacctcccacaacgaggactacaccgtggtggagcagtacgagcgcgccgaggcccgccaccacctgttccagtgataataggggatctcactgactctgaggggtccagtagaaaactactttaatctcaaaaaaaaaaaaaaaaaaaaaaaaaaaaaaaaaaaaaaaaaaaaaaaaaaaaaaaaaaaaaaaaaaaaaaaaaaaaaaaaaaaaaaaaaaaaaaaaaaaaagagacg

SEQ ID NO: 166 - DNA, 913 bp, synthetic construct
  source 1..913: mol_type = other DNA
taatacgactcactataagggagaataaactagtattcttctggtccccacagactcagagagaacccgccaccatggatagcactgagaacgtcatcaagcccttcatgcgcttcaaggtgcacatggagggctccgtgaacggccacgagttcgagatcgagggcgtgggcgagggcaagccctacgagggcacccagaccgccaagctgcaagtgaccaagggcggccccctgcccttcgcctgggacatcctgtccccccagttcttctacggctccaaggcgtacatcaagcaccccgccgacatccccgactacctcaagcagtccttccccgagggcttcaagtgggagcgcgtgatgaacttcgaggacggcggcgtggtgaccgtgacccaggactcctccctgcaggacggcaccctcatctaccacgtgaagttcatcggcgtgaacttcccctccgacggccccgtaatgcagaagaaaactctgggctgggagccctccactgagcgcaactacccccgcgacggcgtgctgaagggcgagaaccacatggcgctgaagctgaagggcggcggccactacctgtgtgagttcaagtccatctacatggccaagaagcccgtgaagctgcccggctaccactacgtggactacaagctcgacatcacctcccacaacgaggactacaccgtggtggagcagtacgagcgcgccgaggcccgccaccacctgttccagtgataataggcgttgtctgtgactctctggcgacgagatgaaaacttgttaattgtcaaaaaaaaaaaaaaaaaaaaaaaaaaaaaaaaaaaaaaaaaaaaaaaaaaaaaaaaaaaaaaaaaaaaaaaaaaaaaaaaaaaaaaaaaaaaaaaaaaaaagagacg

SEQ ID NO: 167 - DNA, 913 bp, synthetic construct
  source 1..913: mol_type = other DNA
taatacgactcactataagggagaataaactagtattcttctggtccccacagactcagagagaacccgccaccatggatagcactgagaacgtcatcaagcccttcatgcgcttcaaggtgcacatggagggctccgtgaacggccacgagttcgagatcgagggcgtgggcgagggcaagccctacgagggcacccagaccgccaagctgcaagtgaccaagggcggccccctgcccttcgcctgggacatcctgtccccccagttcttctacggctccaaggcgtacatcaagcaccccgccgacatccccgactacctcaagcagtccttccccgagggcttcaagtgggagcgcgtgatgaacttcgaggacggcggcgtggtgaccgtgacccaggactcctccctgcaggacggcaccctcatctaccacgtgaagttcatcggcgtgaacttcccctccgacggccccgtaatgcagaagaaaactctgggctgggagccctccactgagcgcaactacccccgcgacggcgtgctgaagggcgagaaccacatggcgctgaagctgaagggcggcggccactacctgtgtgagttcaagtccatctacatggccaagaagcccgtgaagctgcccggctaccactacgtggactacaagctcgacatcacctcccacaacgaggactacaccgtggtggagcagtacgagcgcgccgaggcccgccaccacctgttccagtgataataggggttctctgagagtctgtgggctccagaagaatagaagtttattctcaaaaaaaaaaaaaaaaaaaaaaaaaaaaaaaaaaaaaaaaaaaaaaaaaaaaaaaaaaaaaaaaaaaaaaaaaaaaaaaaaaaaaaaaaaaaaaaaaaaaagagacg

SEQ ID NO: 168 - DNA, 913 bp, synthetic construct
  source 1..913: mol_type = other DNA
taatacgactcactataagggagaataaactagtattcttctggtccccacagactcagagagaacccgccaccatggatagcactgagaacgtcatcaagcccttcatgcgcttcaaggtgcacatggagggctccgtgaacggccacgagttcgagatcgagggcgtgggcgagggcaagccctacgagggcacccagaccgccaagctgcaagtgaccaagggcggccccctgcccttcgcctgggacatcctgtccccccagttcttctacggctccaaggcgtacatcaagcaccccgccgacatccccgactacctcaagcagtccttccccgagggcttcaagtgggagcgcgtgatgaacttcgaggacggcggcgtggtgaccgtgacccaggactcctccctgcaggacggcaccctcatctaccacgtgaagttcatcggcgtgaacttcccctccgacggccccgtaatgcagaagaaaactctgggctgggagccctccactgagcgcaactacccccgcgacggcgtgctgaagggcgagaaccacatggcgctgaagctgaagggcggcggccactacctgtgtgagttcaagtccatctacatggccaagaagcccgtgaagctgcccggctaccactacgtggactacaagctcgacatcacctcccacaacgaggactacaccgtggtggagcagtacgagcgcgccgaggcccgccaccacctgttccagtgataataggccttctctctgacactgtggggacgtgaagaatacttctttattctcaaaaaaaaaaaaaaaaaaaaaaaaaaaaaaaaaaaaaaaaaaaaaaaaaaaaaaaaaaaaaaaaaaaaaaaaaaaaaaaaaaaaaaaaaaaaaaaaaaaaagagacg

SEQ ID NO: 169 - DNA, 913 bp, synthetic construct
  source 1..913: mol_type = other DNA
taatacgactcactataagggagaataaactagtattcttctggtccccacagactcagagagaacccgccaccatggatagcactgagaacgtcatcaagcccttcatgcgcttcaaggtgcacatggagggctccgtgaacggccacgagttcgagatcgagggcgtgggcgagggcaagccctacgagggcacccagaccgccaagctgcaagtgaccaagggcggccccctgcccttcgcctgggacatcctgtccccccagttcttctacggctccaaggcgtacatcaagcaccccgccgacatccccgactacctcaagcagtccttccccgagggcttcaagtgggagcgcgtgatgaacttcgaggacggcggcgtggtgaccgtgacccaggactcctccctgcaggacggcaccctcatctaccacgtgaagttcatcggcgtgaacttcccctccgacggccccgtaatgcagaagaaaactctgggctgggagccctccactgagcgcaactacccccgcgacggcgtgctgaagggcgagaaccacatggcgctgaagctgaagggcggcggccactacctgtgtgagttcaagtccatctacatggccaagaagcccgtgaagctgcccggctaccactacgtggactacaagctcgacatcacctcccacaacgaggactacaccgtggtggagcagtacgagcgcgccgaggcccgccaccacctgttccagtgataataggggtagtctctgagtgagtggggacctcaagaatacttctttattctcaaaaaaaaaaaaaaaaaaaaaaaaaaaaaaaaaaaaaaaaaaaaaaaaaaaaaaaaaaaaaaaaaaaaaaaaaaaaaaaaaaaaaaaaaaaaaaaaaaaaagagacg

SEQ ID NO: 170 - DNA, 913 bp, synthetic construct
  source 1..913: mol_type = other DNA
taatacgactcactataagggagaataaactagtattcttctggtccccacagactcagagagaacccgccaccatggatagcactgagaacgtcatcaagcccttcatgcgcttcaaggtgcacatggagggctccgtgaacggccacgagttcgagatcgagggcgtgggcgagggcaagccctacgagggcacccagaccgccaagctgcaagtgaccaagggcggccccctgcccttcgcctgggacatcctgtccccccagttcttctacggctccaaggcgtacatcaagcaccccgccgacatccccgactacctcaagcagtccttccccgagggcttcaagtgggagcgcgtgatgaacttcgaggacggcggcgtggtgaccgtgacccaggactcctccctgcaggacggcaccctcatctaccacgtgaagttcatcggcgtgaacttcccctccgacggccccgtaatgcagaagaaaactctgggctgggagccctccactgagcgcaactacccccgcgacggcgtgctgaagggcgagaaccacatggcgctgaagctgaagggcggcggccactacctgtgtgagttcaagtccatctacatggccaagaagcccgtgaagctgcccggctaccactacgtggactacaagctcgacatcacctcccacaacgaggactacaccgtggtggagcagtacgagcgcgccgaggcccgccaccacctgttccagtgataataggggttctcagtgagtctgacgggaccagttgaatactacattattctcaaaaaaaaaaaaaaaaaaaaaaaaaaaaaaaaaaaaaaaaaaaaaaaaaaaaaaaaaaaaaaaaaaaaaaaaaaaaaaaaaaaaaaaaaaaaaaaaaaaaagagacg

SEQ ID NO: 171 - DNA, 913 bp, synthetic construct
  source 1..913: mol_type = other DNA
taatacgactcactataagggagaataaactagtattcttctggtccccacagactcagagagaacccgccaccatggatagcactgagaacgtcatcaagcccttcatgcgcttcaaggtgcacatggagggctccgtgaacggccacgagttcgagatcgagggcgtgggcgagggcaagccctacgagggcacccagaccgccaagctgcaagtgaccaagggcggccccctgcccttcgcctgggacatcctgtccccccagttcttctacggctccaaggcgtacatcaagcaccccgccgacatccccgactacctcaagcagtccttccccgagggcttcaagtgggagcgcgtgatgaacttcgaggacggcggcgtggtgaccgtgacccaggactcctccctgcaggacggcaccctcatctaccacgtgaagttcatcggcgtgaacttcccctccgacggccccgtaatgcagaagaaaactctgggctgggagccctccactgagcgcaactacccccgcgacggcgtgctgaagggcgagaaccacatggcgctgaagctgaagggcggcggccactacctgtgtgagttcaagtccatctacatggccaagaagcccgtgaagctgcccggctaccactacgtggactacaagctcgacatcacctcccacaacgaggactacaccgtggtggagcagtacgagcgcgccgaggcccgccaccacctgttccagtgataataggggaactctctgtctctgtggccaccagaactatactagaatattctcaaaaaaaaaaaaaaaaaaaaaaaaaaaaaaaaaaaaaaaaaaaaaaaaaaaaaaaaaaaaaaaaaaaaaaaaaaaaaaaaaaaaaaaaaaaaaaaaaaaaagagacg

SEQ ID NO: 172 - DNA, 913 bp, synthetic construct
  source 1..913: mol_type = other DNA
taatacgactcactataagggagaataaactagtattcttctggtccccacagactcagagagaacccgccaccatggatagcactgagaacgtcatcaagcccttcatgcgcttcaaggtgcacatggagggctccgtgaacggccacgagttcgagatcgagggcgtgggcgagggcaagccctacgagggcacccagaccgccaagctgcaagtgaccaagggcggccccctgcccttcgcctgggacatcctgtccccccagttcttctacggctccaaggcgtacatcaagcaccccgccgacatccccgactacctcaagcagtccttccccgagggcttcaagtgggagcgcgtgatgaacttcgaggacggcggcgtggtgaccgtgacccaggactcctccctgcaggacggcaccctcatctaccacgtgaagttcatcggcgtgaacttcccctccgacggccccgtaatgcagaagaaaactctgggctgggagccctccactgagcgcaactacccccgcgacggcgtgctgaagggcgagaaccacatggcgctgaagctgaagggcggcggccactacctgtgtgagttcaagtccatctacatggccaagaagcccgtgaagctgcccggctaccactacgtggactacaagctcgacatcacctcccacaacgaggactacaccgtggtggagcagtacgagcgcgccgaggcccgccaccacctgttccagtgataataggccttctctgagagtctcaggggacgtgaagaaatctagttatttctcaaaaaaaaaaaaaaaaaaaaaaaaaaaaaaaaaaaaaaaaaaaaaaaaaaaaaaaaaaaaaaaaaaaaaaaaaaaaaaaaaaaaaaaaaaaaaaaaaaaaagagacg

SEQ ID NO: 173 - DNA, 913 bp, synthetic construct
  source 1..913: mol_type = other DNA
taatacgactcactataagggagaataaactagtattcttctggtccccacagactcagagagaacccgccaccatggatagcactgagaacgtcatcaagcccttcatgcgcttcaaggtgcacatggagggctccgtgaacggccacgagttcgagatcgagggcgtgggcgagggcaagccctacgagggcacccagaccgccaagctgcaagtgaccaagggcggccccctgcccttcgcctgggacatcctgtccccccagttcttctacggctccaaggcgtacatcaagcaccccgccgacatccccgactacctcaagcagtccttccccgagggcttcaagtgggagcgcgtgatgaacttcgaggacggcggcgtggtgaccgtgacccaggactcctccctgcaggacggcaccctcatctaccacgtgaagttcatcggcgtgaacttcccctccgacggccccgtaatgcagaagaaaactctgggctgggagccctccactgagcgcaactacccccgcgacggcgtgctgaagggcgagaaccacatggcgctgaagctgaagggcggcggccactacctgtgtgagttcaagtccatctacatggccaagaagcccgtgaagctgcccggctaccactacgtggactacaagctcgacatcacctcccacaacgaggactacaccgtggtggagcagtacgagcgcgccgaggcccgccaccacctgttccagtgataataggccttctcagtgagtgagtgggctccagatcaatacatgtttaaactcaaaaaaaaaaaaaaaaaaaaaaaaaaaaaaaaaaaaaaaaaaaaaaaaaaaaaaaaaaaaaaaaaaaaaaaaaaaaaaaaaaaaaaaaaaaaaaaaaaaaagagacg

SEQ ID NO: 174 - DNA, 913 bp, synthetic construct
  source 1..913: mol_type = other DNA
taatacgactcactataagggagaataaactagtattcttctggtccccacagactcagagagaacccgccaccatggatagcactgagaacgtcatcaagcccttcatgcgcttcaaggtgcacatggagggctccgtgaacggccacgagttcgagatcgagggcgtgggcgagggcaagccctacgagggcacccagaccgccaagctgcaagtgaccaagggcggccccctgcccttcgcctgggacatcctgtccccccagttcttctacggctccaaggcgtacatcaagcaccccgccgacatccccgactacctcaagcagtccttccccgagggcttcaagtgggagcgcgtgatgaacttcgaggacggcggcgtggtgaccgtgacccaggactcctccctgcaggacggcaccctcatctaccacgtgaagttcatcggcgtgaacttcccctccgacggccccgtaatgcagaagaaaactctgggctgggagccctccactgagcgcaactacccccgcgacggcgtgctgaagggcgagaaccacatggcgctgaagctgaagggcggcggccactacctgtgtgagttcaagtccatctacatggccaagaagcccgtgaagctgcccggctaccactacgtggactacaagctcgacatcacctcccacaacgaggactacaccgtggtggagcagtacgagcgcgccgaggcccgccaccacctgttccagtgataataggggaagtctctgagtctgaccggaccagaagaaatgtagtttattctcaaaaaaaaaaaaaaaaaaaaaaaaaaaaaaaaaaaaaaaaaaaaaaaaaaaaaaaaaaaaaaaaaaaaaaaaaaaaaaaaaaaaaaaaaaaaaaaaaaaaagagacg

SEQ ID NO: 175 - DNA, 913 bp, synthetic construct
  source 1..913: mol_type = other DNA
taatacgactcactataagggagaataaactagtattcttctggtccccacagactcagagagaacccgccaccatggatagcactgagaacgtcatcaagcccttcatgcgcttcaaggtgcacatggagggctccgtgaacggccacgagttcgagatcgagggcgtgggcgagggcaagccctacgagggcacccagaccgccaagctgcaagtgaccaagggcggccccctgcccttcgcctgggacatcctgtccccccagttcttctacggctccaaggcgtacatcaagcaccccgccgacatccccgactacctcaagcagtccttccccgagggcttcaagtgggagcgcgtgatgaacttcgaggacggcggcgtggtgaccgtgacccaggactcctccctgcaggacggcaccctcatctaccacgtgaagttcatcggcgtgaacttcccctccgacggccccgtaatgcagaagaaaactctgggctgggagccctccactgagcgcaactacccccgcgacggcgtgctgaagggcgagaaccacatggcgctgaagctgaagggcggcggccactacctgtgtgagttcaagtccatctacatggccaagaagcccgtgaagctgcccggctaccactacgtggactacaagctcgacatcacctcccacaacgaggactacaccgtggtggagcagtacgagcgcgccgaggcccgccaccacctgttccagtgataataggggttctctgacagtctgtgggctgcagaagaatagatgtttattctcaaaaaaaaaaaaaaaaaaaaaaaaaaaaaaaaaaaaaaaaaaaaaaaaaaaaaaaaaaaaaaaaaaaaaaaaaaaaaaaaaaaaaaaaaaaaaaaaaaaaagagacg

SEQ ID NO: 176 - DNA, 913 bp, synthetic construct
  source 1..913: mol_type = other DNA
taatacgactcactataagggagaataaactagtattcttctggtccccacagactcagagagaacccgccaccatggatagcactgagaacgtcatcaagcccttcatgcgcttcaaggtgcacatggagggctccgtgaacggccacgagttcgagatcgagggcgtgggcgagggcaagccctacgagggcacccagaccgccaagctgcaagtgaccaagggcggccccctgcccttcgcctgggacatcctgtccccccagttcttctacggctccaaggcgtacatcaagcaccccgccgacatccccgactacctcaagcagtccttccccgagggcttcaagtgggagcgcgtgatgaacttcgaggacggcggcgtggtgaccgtgacccaggactcctccctgcaggacggcaccctcatctaccacgtgaagttcatcggcgtgaacttcccctccgacggccccgtaatgcagaagaaaactctgggctgggagccctccactgagcgcaactacccccgcgacggcgtgctgaagggcgagaaccacatggcgctgaagctgaagggcggcggccactacctgtgtgagttcaagtccatctacatggccaagaagcccgtgaagctgcccggctaccactacgtggactacaagctcgacatcacctcccacaacgaggactacaccgtggtggagcagtacgagcgcgccgaggcccgccaccacctgttccagtgataataggccatctctctgacagtgtggggacgtcaagaatacttcattattctcaaaaaaaaaaaaaaaaaaaaaaaaaaaaaaaaaaaaaaaaaaaaaaaaaaaaaaaaaaaaaaaaaaaaaaaaaaaaaaaaaaaaaaaaaaaaaaaaaaaaagagacg

SEQ ID NO: 177 - DNA, 913 bp, synthetic construct
  source 1..913: mol_type = other DNA
taatacgactcactataagggagaataaactagtattcttctggtccccacagactcagagagaacccgccaccatggatagcactgagaacgtcatcaagcccttcatgcgcttcaaggtgcacatggagggctccgtgaacggccacgagttcgagatcgagggcgtgggcgagggcaagccctacgagggcacccagaccgccaagctgcaagtgaccaagggcggccccctgcccttcgcctgggacatcctgtccccccagttcttctacggctccaaggcgtacatcaagcaccccgccgacatccccgactacctcaagcagtccttccccgagggcttcaagtgggagcgcgtgatgaacttcgaggacggcggcgtggtgaccgtgacccaggactcctccctgcaggacggcaccctcatctaccacgtgaagttcatcggcgtgaacttcccctccgacggccccgtaatgcagaagaaaactctgggctgggagccctccactgagcgcaactacccccgcgacggcgtgctgaagggcgagaaccacatggcgctgaagctgaagggcggcggccactacctgtgtgagttcaagtccatctacatggccaagaagcccgtgaagctgcccggctaccactacgtggactacaagctcgacatcacctcccacaacgaggactacaccgtggtggagcagtacgagcgcgccgaggcccgccaccacctgttccagtgataataggggtagactctgagtgactggggacctctagaatacttcattattctcaaaaaaaaaaaaaaaaaaaaaaaaaaaaaaaaaaaaaaaaaaaaaaaaaaaaaaaaaaaaaaaaaaaaaaaaaaaaaaaaaaaaaaaaaaaaaaaaaaaaagagacg

SEQ ID NO: 178 - DNA, 939 bp, synthetic construct
  source 1..939: mol_type = other DNA
taatacgactcactataaggtcccgcagtcggcgtccagcggctctgcttgttcgtgtgtgtgtcgttgcaggccttattcgccaccatggatagcactgagaacgtcatcaagcccttcatgcgcttcaaggtgcacatggagggctccgtgaacggccacgagttcgagatcgagggcgtgggcgagggcaagccctacgagggcacccagaccgccaagctgcaagtgaccaagggcggccccctgcccttcgcctgggacatcctgtccccccagttcttctacggctccaaggcgtacatcaagcaccccgccgacatccccgactacctcaagcagtccttccccgagggcttcaagtgggagcgcgtgatgaacttcgaggacggcggcgtggtgaccgtgacccaggactcctccctgcaggacggcaccctcatctaccacgtgaagttcatcggcgtgaacttcccctccgacggccccgtaatgcagaagaaaactctgggctgggagccctccactgagcgcaactacccccgcgacggcgtgctgaagggcgagaaccacatggcgctgaagctgaagggcggcggccactacctgtgtgagttcaagtccatctacatggccaagaagcccgtgaagctgcccggctaccactacgtggactacaagctcgacatcacctcccacaacgaggactacaccgtggtggagcagtacgagcgcgccgaggcccgccaccacctgttccagtgataataggtataaggcctccaacgacactcacacgaactagcagagcccctggacgcccactgcgggaaaaaaaaaaaaaaaaaaaaaaaaaaaaaaaaaaaaaaaaaaaaaaaaaaaaaaaaaaaaaaaaaaaaaaaaaaaaaaaaaaaaaaaaaaaaaaaaaaaaaagagacg

SEQ ID NO: 179 - DNA, 939 bp, synthetic construct
  source 1..939: mol_type = other DNA
taatacgactcactataaggtcccgcagtcggcgtccagcggctctgcttgttcgtgtgtgtgtcgttgcaggccttattcgccaccatggatagcactgagaacgtcatcaagcccttcatgcgcttcaaggtgcacatggagggctccgtgaacggccacgagttcgagatcgagggcgtgggcgagggcaagccctacgagggcacccagaccgccaagctgcaagtgaccaagggcggccccctgcccttcgcctgggacatcctgtccccccagttcttctacggctccaaggcgtacatcaagcaccccgccgacatccccgactacctcaagcagtccttccccgagggcttcaagtgggagcgcgtgatgaacttcgaggacggcggcgtggtgaccgtgacccaggactcctccctgcaggacggcaccctcatctaccacgtgaagttcatcggcgtgaacttcccctccgacggccccgtaatgcagaagaaaactctgggctgggagccctccactgagcgcaactacccccgcgacggcgtgctgaagggcgagaaccacatggcgctgaagctgaagggcggcggccactacctgtgtgagttcaagtccatctacatggccaagaagcccgtgaagctgcccggctaccactacgtggactacaagctcgacatcacctcccacaacgaggactacaccgtggtggagcagtacgagcgcgccgaggcccgccaccacctgttccagtgataataggaataagccctgcaaccacacacactcgaacaaggagagccgcaggacgccgtctgcgggaaaaaaaaaaaaaaaaaaaaaaaaaaaaaaaaaaaaaaaaaaaaaaaaaaaaaaaaaaaaaaaaaaaaaaaaaaaaaaaaaaaaaaaaaaaaaaaaaaaaaagagacg

SEQ ID NO: 180 - DNA, 939 bp, synthetic construct
  source 1..939: mol_type = other DNA
taatacgactcactataaggtcccgcagtcggcgtccagcggctctgcttgttcgtgtgtgtgtcgttgcaggccttattcgccaccatggatagcactgagaacgtcatcaagcccttcatgcgcttcaaggtgcacatggagggctccgtgaacggccacgagttcgagatcgagggcgtgggcgagggcaagccctacgagggcacccagaccgccaagctgcaagtgaccaagggcggccccctgcccttcgcctgggacatcctgtccccccagttcttctacggctccaaggcgtacatcaagcaccccgccgacatccccgactacctcaagcagtccttccccgagggcttcaagtgggagcgcgtgatgaacttcgaggacggcggcgtggtgaccgtgacccaggactcctccctgcaggacggcaccctcatctaccacgtgaagttcatcggcgtgaacttcccctccgacggccccgtaatgcagaagaaaactctgggctgggagccctccactgagcgcaactacccccgcgacggcgtgctgaagggcgagaaccacatggcgctgaagctgaagggcggcggccactacctgtgtgagttcaagtccatctacatggccaagaagcccgtgaagctgcccggctaccactacgtggactacaagctcgacatcacctcccacaacgaggactacaccgtggtggagcagtacgagcgcgccgaggcccgccaccacctgttccagtgataataggaatatggcctgctacgacactcacacgatcaagcagtgccgctgcacgccgagtgcgggaaaaaaaaaaaaaaaaaaaaaaaaaaaaaaaaaaaaaaaaaaaaaaaaaaaaaaaaaaaaaaaaaaaaaaaaaaaaaaaaaaaaaaaaaaaaaaaaaaaaaagagacg

SEQ ID NO: 181 - DNA, 939 bp, synthetic construct
  source 1..939: mol_type = other DNA
taatacgactcactataaggtcccgcagtcggcgtccagcggctctgcttgttcgtgtgtgtgtcgttgcaggccttattcgccaccatggatagcactgagaacgtcatcaagcccttcatgcgcttcaaggtgcacatggagggctccgtgaacggccacgagttcgagatcgagggcgtgggcgagggcaagccctacgagggcacccagaccgccaagctgcaagtgaccaagggcggccccctgcccttcgcctgggacatcctgtccccccagttcttctacggctccaaggcgtacatcaagcaccccgccgacatccccgactacctcaagcagtccttccccgagggcttcaagtgggagcgcgtgatgaacttcgaggacggcggcgtggtgaccgtgacccaggactcctccctgcaggacggcaccctcatctaccacgtgaagttcatcggcgtgaacttcccctccgacggccccgtaatgcagaagaaaactctgggctgggagccctccactgagcgcaactacccccgcgacggcgtgctgaagggcgagaaccacatggcgctgaagctgaagggcggcggccactacctgtgtgagttcaagtccatctacatggccaagaagcccgtgaagctgcccggctaccactacgtggactacaagctcgacatcacctcccacaacgaggactacaccgtggtggagcagtacgagcgcgccgaggcccgccaccacctgttccagtgataataggaatatggcctggaacgactcacacaggaacaaccagagcggctggaggccgacagcgggaaaaaaaaaaaaaaaaaaaaaaaaaaaaaaaaaaaaaaaaaaaaaaaaaaaaaaaaaaaaaaaaaaaaaaaaaaaaaaaaaaaaaaaaaaaaaaaaaaaaaagagacg

SEQ ID NO: 182 - DNA, 939 bp, synthetic construct
  source 1..939: mol_type = other DNA
taatacgactcactataaggtcccgcagtcggcgtccagcggctctgcttgttcgtgtgtgtgtcgttgcaggccttattcgccaccatggatagcactgagaacgtcatcaagcccttcatgcgcttcaaggtgcacatggagggctccgtgaacggccacgagttcgagatcgagggcgtgggcgagggcaagccctacgagggcacccagaccgccaagctgcaagtgaccaagggcggccccctgcccttcgcctgggacatcctgtccccccagttcttctacggctccaaggcgtacatcaagcaccccgccgacatccccgactacctcaagcagtccttccccgagggcttcaagtgggagcgcgtgatgaacttcgaggacggcggcgtggtgaccgtgacccaggactcctccctgcaggacggcaccctcatctaccacgtgaagttcatcggcgtgaacttcccctccgacggccccgtaatgcagaagaaaactctgggctgggagccctccactgagcgcaactacccccgcgacggcgtgctgaagggcgagaaccacatggcgctgaagctgaagggcggcggccactacctgtgtgagttcaagtccatctacatggccaagaagcccgtgaagctgcccggctaccactacgtggactacaagctcgacatcacctcccacaacgaggactacaccgtggtggagcagtacgagcgcgccgaggcccgccaccacctgttccagtgataataggtataagccctgctacgactcacactcgaactagcagtgccgcaggacggcgactccgggaaaaaaaaaaaaaaaaaaaaaaaaaaaaaaaaaaaaaaaaaaaaaaaaaaaaaaaaaaaaaaaaaaaaaaaaaaaaaaaaaaaaaaaaaaaaaaaaaaaaaagagacg

SEQ ID NO: 183 - DNA, 939 bp, synthetic construct
  source 1..939: mol_type = other DNA
taatacgactcactataaggtcccgcagtcggcgtccagcggctctgcttgttcgtgtgtgtgtcgttgcaggccttattcgccaccatggatagcactgagaacgtcatcaagcccttcatgcgcttcaaggtgcacatggagggctccgtgaacggccacgagttcgagatcgagggcgtgggcgagggcaagccctacgagggcacccagaccgccaagctgcaagtgaccaagggcggccccctgcccttcgcctgggacatcctgtccccccagttcttctacggctccaaggcgtacatcaagcaccccgccgacatccccgactacctcaagcagtccttccccgagggcttcaagtgggagcgcgtgatgaacttcgaggacggcggcgtggtgaccgtgacccaggactcctccctgcaggacggcaccctcatctaccacgtgaagttcatcggcgtgaacttcccctccgacggccccgtaatgcagaagaaaactctgggctgggagccctccactgagcgcaactacccccgcgacggcgtgctgaagggcgagaaccacatggcgctgaagctgaagggcggcggccactacctgtgtgagttcaagtccatctacatggccaagaagcccgtgaagctgcccggctaccactacgtggactacaagctcgacatcacctcccacaacgaggactacaccgtggtggagcagtacgagcgcgccgaggcccgccaccacctgttccagtgataataggtataacgcctccaaccacactcacaggaactagcacagcccctggtcgcccactgggggaaaaaaaaaaaaaaaaaaaaaaaaaaaaaaaaaaaaaaaaaaaaaaaaaaaaaaaaaaaaaaaaaaaaaaaaaaaaaaaaaaaaaaaaaaaaaaaaaaaaaagagacg

SEQ ID NO: 184 - DNA, 939 bp, synthetic construct
  source 1..939: mol_type = other DNA
taatacgactcactataaggtcccgcagtcggcgtccagcggctctgcttgttcgtgtgtgtgtcgttgcaggccttattcgccaccatggatagcactgagaacgtcatcaagcccttcatgcgcttcaaggtgcacatggagggctccgtgaacggccacgagttcgagatcgagggcgtgggcgagggcaagccctacgagggcacccagaccgccaagctgcaagtgaccaagggcggccccctgcccttcgcctgggacatcctgtccccccagttcttctacggctccaaggcgtacatcaagcaccccgccgacatccccgactacctcaagcagtccttccccgagggcttcaagtgggagcgcgtgatgaacttcgaggacggcggcgtggtgaccgtgacccaggactcctccctgcaggacggcaccctcatctaccacgtgaagttcatcggcgtgaacttcccctccgacggccccgtaatgcagaagaaaactctgggctgggagccctccactgagcgcaactacccccgcgacggcgtgctgaagggcgagaaccacatggcgctgaagctgaagggcggcggccactacctgtgtgagttcaagtccatctacatggccaagaagcccgtgaagctgcccggctaccactacgtggactacaagctcgacatcacctcccacaacgaggactacaccgtggtggagcagtacgagcgcgccgaggcccgccaccacctgttccagtgataataggtatatggcgtgctacgtcactcactcgatcaaccagtgcccctgcacggcgagtgccggaaaaaaaaaaaaaaaaaaaaaaaaaaaaaaaaaaaaaaaaaaaaaaaaaaaaaaaaaaaaaaaaaaaaaaaaaaaaaaaaaaaaaaaaaaaaaaaaaaaaaagagacg

SEQ ID NO: 185 - DNA, 939 bp, synthetic construct
  source 1..939: mol_type = other DNA
taatacgactcactataaggtcccgcagtcggcgtccagcggctctgcttgttcgtgtgtgtgtcgttgcaggccttattcgccaccatggatagcactgagaacgtcatcaagcccttcatgcgcttcaaggtgcacatggagggctccgtgaacggccacgagttcgagatcgagggcgtgggcgagggcaagccctacgagggcacccagaccgccaagctgcaagtgaccaagggcggccccctgcccttcgcctgggacatcctgtccccccagttcttctacggctccaaggcgtacatcaagcaccccgccgacatccccgactacctcaagcagtccttccccgagggcttcaagtgggagcgcgtgatgaacttcgaggacggcggcgtggtgaccgtgacccaggactcctccctgcaggacggcaccctcatctaccacgtgaagttcatcggcgtgaacttcccctccgacggccccgtaatgcagaagaaaactctgggctgggagccctccactgagcgcaactacccccgcgacggcgtgctgaagggcgagaaccacatggcgctgaagctgaagggcggcggccactacctgtgtgagttcaagtccatctacatggccaagaagcccgtgaagctgcccggctaccactacgtggactacaagctcgacatcacctcccacaacgaggactacaccgtggtggagcagtacgagcgcgccgaggcccgccaccacctgttccagtgataataggaataacccctgcaacgtgacacacacgttcaagcagaggggctggacgcgcactgcgggaaaaaaaaaaaaaaaaaaaaaaaaaaaaaaaaaaaaaaaaaaaaaaaaaaaaaaaaaaaaaaaaaaaaaaaaaaaaaaaaaaaaaaaaaaaaaaaaaaaaaagagacg

SEQ ID NO: 186 - DNA, 939 bp, synthetic construct
  source 1..939: mol_type = other DNA
taatacgactcactataaggtcccgcagtcggcgtccagcggctctgcttgttcgtgtgtgtgtcgttgcaggccttattcgccaccatggatagcactgagaacgtcatcaagcccttcatgcgcttcaaggtgcacatggagggctccgtgaacggccacgagttcgagatcgagggcgtgggcgagggcaagccctacgagggcacccagaccgccaagctgcaagtgaccaagggcggccccctgcccttcgcctgggacatcctgtccccccagttcttctacggctccaaggcgtacatcaagcaccccgccgacatccccgactacctcaagcagtccttccccgagggcttcaagtgggagcgcgtgatgaacttcgaggacggcggcgtggtgaccgtgacccaggactcctccctgcaggacggcaccctcatctaccacgtgaagttcatcggcgtgaacttcccctccgacggccccgtaatgcagaagaaaactctgggctgggagccctccactgagcgcaactacccccgcgacggcgtgctgaagggcgagaaccacatggcgctgaagctgaagggcggcggccactacctgtgtgagttcaagtccatctacatggccaagaagcccgtgaagctgcccggctaccactacgtggactacaagctcgacatcacctcccacaacgaggactacaccgtggtggagcagtacgagcgcgccgaggcccgccaccacctgttccagtgataataggtttaaggcctcgaacgacactgacacgaacttgcagagcccgtggacgccctctgcgggaaaaaaaaaaaaaaaaaaaaaaaaaaaaaaaaaaaaaaaaaaaaaaaaaaaaaaaaaaaaaaaaaaaaaaaaaaaaaaaaaaaaaaaaaaaaaaaaaaaaaagagacg

SEQ ID NO: 187 - DNA, 939 bp, synthetic construct
  source 1..939: mol_type = other DNA
taatacgactcactataaggtcccgcagtcggcgtccagcggctctgcttgttcgtgtgtgtgtcgttgcaggccttattcgccaccatggatagcactgagaacgtcatcaagcccttcatgcgcttcaaggtgcacatggagggctccgtgaacggccacgagttcgagatcgagggcgtgggcgagggcaagccctacgagggcacccagaccgccaagctgcaagtgaccaagggcggccccctgcccttcgcctgggacatcctgtccccccagttcttctacggctccaaggcgtacatcaagcaccccgccgacatccccgactacctcaagcagtccttccccgagggcttcaagtgggagcgcgtgatgaacttcgaggacggcggcgtggtgaccgtgacccaggactcctccctgcaggacggcaccctcatctaccacgtgaagttcatcggcgtgaacttcccctccgacggccccgtaatgcagaagaaaactctgggctgggagccctccactgagcgcaactacccccgcgacggcgtgctgaagggcgagaaccacatggcgctgaagctgaagggcggcggccactacctgtgtgagttcaagtccatctacatggccaagaagcccgtgaagctgcccggctaccactacgtggactacaagctcgacatcacctcccacaacgaggactacaccgtggtggagcagtacgagcgcgccgaggcccgccaccacctgttccagtgataataggaataagcgctgcaacctcacacactggaacaaggtgagccgcacgacgccgtgtgcgggaaaaaaaaaaaaaaaaaaaaaaaaaaaaaaaaaaaaaaaaaaaaaaaaaaaaaaaaaaaaaaaaaaaaaaaaaaaaaaaaaaaaaaaaaaaaaaaaaaaaaagagacg

SEQ ID NO: 188 - DNA, 939 bp, synthetic construct
  source 1..939: mol_type = other DNA
taatacgactcactataaggtcccgcagtcggcgtccagcggctctgcttgttcgtgtgtgtgtcgttgcaggccttattcgccaccatggatagcactgagaacgtcatcaagcccttcatgcgcttcaaggtgcacatggagggctccgtgaacggccacgagttcgagatcgagggcgtgggcgagggcaagccctacgagggcacccagaccgccaagctgcaagtgaccaagggcggccccctgcccttcgcctgggacatcctgtccccccagttcttctacggctccaaggcgtacatcaagcaccccgccgacatccccgactacctcaagcagtccttccccgagggcttcaagtgggagcgcgtgatgaacttcgaggacggcggcgtggtgaccgtgacccaggactcctccctgcaggacggcaccctcatctaccacgtgaagttcatcggcgtgaacttcccctccgacggccccgtaatgcagaagaaaactctgggctgggagccctccactgagcgcaactacccccgcgacggcgtgctgaagggcgagaaccacatggcgctgaagctgaagggcggcggccactacctgtgtgagttcaagtccatctacatggccaagaagcccgtgaagctgcccggctaccactacgtggactacaagctcgacatcacctcccacaacgaggactacaccgtggtggagcagtacgagcgcgccgaggcccgccaccacctgttccagtgataataggaatatcgcctgcttcgacactgacacgatgaagcagtcccgctgctcgccgagagcgggaaaaaaaaaaaaaaaaaaaaaaaaaaaaaaaaaaaaaaaaaaaaaaaaaaaaaaaaaaaaaaaaaaaaaaaaaaaaaaaaaaaaaaaaaaaaaaaaaaaaaagagacg

SEQ ID NO: 189 - DNA, 939 bp, synthetic construct
  source 1..939: mol_type = other DNA
taatacgactcactataaggtcccgcagtcggcgtccagcggctctgcttgttcgtgtgtgtgtcgttgcaggccttattcgccaccatggatagcactgagaacgtcatcaagcccttcatgcgcttcaaggtgcacatggagggctccgtgaacggccacgagttcgagatcgagggcgtgggcgagggcaagccctacgagggcacccagaccgccaagctgcaagtgaccaagggcggccccctgcccttcgcctgggacatcctgtccccccagttcttctacggctccaaggcgtacatcaagcaccccgccgacatccccgactacctcaagcagtccttccccgagggcttcaagtgggagcgcgtgatgaacttcgaggacggcggcgtggtgaccgtgacccaggactcctccctgcaggacggcaccctcatctaccacgtgaagttcatcggcgtgaacttcccctccgacggccccgtaatgcagaagaaaactctgggctgggagccctccactgagcgcaactacccccgcgacggcgtgctgaagggcgagaaccacatggcgctgaagctgaagggcggcggccactacctgtgtgagttcaagtccatctacatggccaagaagcccgtgaagctgcccggctaccactacgtggactacaagctcgacatcacctcccacaacgaggactacaccgtggtggagcagtacgagcgcgccgaggcccgccaccacctgttccagtgataataggaatatcgcctggtacgactgacacagcaacaacgagagcgcctggagcccgacaccgggaaaaaaaaaaaaaaaaaaaaaaaaaaaaaaaaaaaaaaaaaaaaaaaaaaaaaaaaaaaaaaaaaaaaaaaaaaaaaaaaaaaaaaaaaaaaaaaaaaaaaagagacg

SEQ ID NO: 190 - DNA, 939 bp, synthetic construct
  source 1..939: mol_type = other DNA
taatacgactcactataaggtcccgcagtcggcgtccagcggctctgcttgttcgtgtgtgtgtcgttgcaggccttattcgccaccatggatagcactgagaacgtcatcaagcccttcatgcgcttcaaggtgcacatggagggctccgtgaacggccacgagttcgagatcgagggcgtgggcgagggcaagccctacgagggcacccagaccgccaagctgcaagtgaccaagggcggccccctgcccttcgcctgggacatcctgtccccccagttcttctacggctccaaggcgtacatcaagcaccccgccgacatccccgactacctcaagcagtccttccccgagggcttcaagtgggagcgcgtgatgaacttcgaggacggcggcgtggtgaccgtgacccaggactcctccctgcaggacggcaccctcatctaccacgtgaagttcatcggcgtgaacttcccctccgacggccccgtaatgcagaagaaaactctgggctgggagccctccactgagcgcaactacccccgcgacggcgtgctgaagggcgagaaccacatggcgctgaagctgaagggcggcggccactacctgtgtgagttcaagtccatctacatggccaagaagcccgtgaagctgcccggctaccactacgtggactacaagctcgacatcacctcccacaacgaggactacaccgtggtggagcagtacgagcgcgccgaggcccgccaccacctgttccagtgataataggttaaaggcctgcaacctgacacacacgaacttccagagccgctggtgcccgactgcgggaaaaaaaaaaaaaaaaaaaaaaaaaaaaaaaaaaaaaaaaaaaaaaaaaaaaaaaaaaaaaaaaaaaaaaaaaaaaaaaaaaaaaaaaaaaaaaaaaaaaaagagacg

SEQ ID NO: 191 - DNA, 939 bp, synthetic construct
  source 1..939: mol_type = other DNA
taatacgactcactataaggtcccgcagtcggcgtccagcggctctgcttgttcgtgtgtgtgtcgttgcaggccttattcgccaccatggatagcactgagaacgtcatcaagcccttcatgcgcttcaaggtgcacatggagggctccgtgaacggccacgagttcgagatcgagggcgtgggcgagggcaagccctacgagggcacccagaccgccaagctgcaagtgaccaagggcggccccctgcccttcgcctgggacatcctgtccccccagttcttctacggctccaaggcgtacatcaagcaccccgccgacatccccgactacctcaagcagtccttccccgagggcttcaagtgggagcgcgtgatgaacttcgaggacggcggcgtggtgaccgtgacccaggactcctccctgcaggacggcaccctcatctaccacgtgaagttcatcggcgtgaacttcccctccgacggccccgtaatgcagaagaaaactctgggctgggagccctccactgagcgcaactacccccgcgacggcgtgctgaagggcgagaaccacatggcgctgaagctgaagggcggcggccactacctgtgtgagttcaagtccatctacatggccaagaagcccgtgaagctgcccggctaccactacgtggactacaagctcgacatcacctcccacaacgaggactacaccgtggtggagcagtacgagcgcgccgaggcccgccaccacctgttccagtgataataggaatatcccctgcaacgactgtcacacgaacaacgtgagccgctggagcgcgactgcgggaaaaaaaaaaaaaaaaaaaaaaaaaaaaaaaaaaaaaaaaaaaaaaaaaaaaaaaaaaaaaaaaaaaaaaaaaaaaaaaaaaaaaaaaaaaaaaaaaaaaaagagacg

SEQ ID NO: 192 - DNA, 939 bp, synthetic construct
  source 1..939: mol_type = other DNA
taatacgactcactataaggtcccgcagtcggcgtccagcggctctgcttgttcgtgtgtgtgtcgttgcaggccttattcgccaccatggatagcactgagaacgtcatcaagcccttcatgcgcttcaaggtgcacatggagggctccgtgaacggccacgagttcgagatcgagggcgtgggcgagggcaagccctacgagggcacccagaccgccaagctgcaagtgaccaagggcggccccctgcccttcgcctgggacatcctgtccccccagttcttctacggctccaaggcgtacatcaagcaccccgccgacatccccgactacctcaagcagtccttccccgagggcttcaagtgggagcgcgtgatgaacttcgaggacggcggcgtggtgaccgtgacccaggactcctccctgcaggacggcaccctcatctaccacgtgaagttcatcggcgtgaacttcccctccgacggccccgtaatgcagaagaaaactctgggctgggagccctccactgagcgcaactacccccgcgacggcgtgctgaagggcgagaaccacatggcgctgaagctgaagggcggcggccactacctgtgtgagttcaagtccatctacatggccaagaagcccgtgaagctgcccggctaccactacgtggactacaagctcgacatcacctcccacaacgaggactacaccgtggtggagcagtacgagcgcgccgaggcccgccaccacctgttccagtgataataggaataaggcgaccaacgacacagtgacgaacaagctctgccgctggaccgggactgcgggaaaaaaaaaaaaaaaaaaaaaaaaaaaaaaaaaaaaaaaaaaaaaaaaaaaaaaaaaaaaaaaaaaaaaaaaaaaaaaaaaaaaaaaaaaaaaaaaaaaaaagagacg

SEQ ID NO: 193 - DNA, 939 bp, synthetic construct
  source 1..939: mol_type = other DNA
taatacgactcactataaggtcccgcagtcggcgtccagcggctctgcttgttcgtgtgtgtgtcgttgcaggccttattcgccaccatggatagcactgagaacgtcatcaagcccttcatgcgcttcaaggtgcacatggagggctccgtgaacggccacgagttcgagatcgagggcgtgggcgagggcaagccctacgagggcacccagaccgccaagctgcaagtgaccaagggcggccccctgcccttcgcctgggacatcctgtccccccagttcttctacggctccaaggcgtacatcaagcaccccgccgacatccccgactacctcaagcagtccttccccgagggcttcaagtgggagcgcgtgatgaacttcgaggacggcggcgtggtgaccgtgacccaggactcctccctgcaggacggcaccctcatctaccacgtgaagttcatcggcgtgaacttcccctccgacggccccgtaatgcagaagaaaactctgggctgggagccctccactgagcgcaactacccccgcgacggcgtgctgaagggcgagaaccacatggcgctgaagctgaagggcggcggccactacctgtgtgagttcaagtccatctacatggccaagaagcccgtgaagctgcccggctaccactacgtggactacaagctcgacatcacctcccacaacgaggactacaccgtggtggagcagtacgagcgcgccgaggcccgccaccacctgttccagtgataataggttaaaggcctgcttggacacacactgcaacaagcagtcgcgctggacgggcactgcgggaaaaaaaaaaaaaaaaaaaaaaaaaaaaaaaaaaaaaaaaaaaaaaaaaaaaaaaaaaaaaaaaaaaaaaaaaaaaaaaaaaaaaaaaaaaaaaaaaaaaaagagacg

SEQ ID NO: 194 - DNA, 939 bp, synthetic construct
  source 1..939: mol_type = other DNA
taatacgactcactataaggtcccgcagtcggcgtccagcggctctgcttgttcgtgtgtgtgtcgttgcaggccttattcgccaccatggatagcactgagaacgtcatcaagcccttcatgcgcttcaaggtgcacatggagggctccgtgaacggccacgagttcgagatcgagggcgtgggcgagggcaagccctacgagggcacccagaccgccaagctgcaagtgaccaagggcggccccctgcccttcgcctgggacatcctgtccccccagttcttctacggctccaaggcgtacatcaagcaccccgccgacatccccgactacctcaagcagtccttccccgagggcttcaagtgggagcgcgtgatgaacttcgaggacggcggcgtggtgaccgtgacccaggactcctccctgcaggacggcaccctcatctaccacgtgaagttcatcggcgtgaacttcccctccgacggccccgtaatgcagaagaaaactctgggctgggagccctccactgagcgcaactacccccgcgacggcgtgctgaagggcgagaaccacatggcgctgaagctgaagggcggcggccactacctgtgtgagttcaagtccatctacatggccaagaagcccgtgaagctgcccggctaccactacgtggactacaagctcgacatcacctcccacaacgaggactacaccgtggtggagcagtacgagcgcgccgaggcccgccaccacctgttccagtgataataggaataaccgctgcaacgtgtcacacacgttgaagcagagggcctggacgcgctctgcgggaaaaaaaaaaaaaaaaaaaaaaaaaaaaaaaaaaaaaaaaaaaaaaaaaaaaaaaaaaaaaaaaaaaaaaaaaaaaaaaaaaaaaaaaaaaaaaaaaaaaaagagacg

SEQ ID NO: 195 - DNA, 68 bp, synthetic construct
  source 1..68: mol_type = other DNA
atagaagtgggtcgcctgccgacccaatagatgatggggcagacagtcgtacacgagcagcacagacc

SEQ ID NO: 196 - DNA, 68 bp, synthetic construct
  source 1..68: mol_type = other DNA
ttttggtctgtgctgctcgtgtacgactgtctgccccatcatctattgggtcggcaggcgacccactt

SEQ ID NO: 197 - DNA, 68 bp, synthetic construct
  source 1..68: mol_type = other DNA
atagaagtgcctcgcctgccgacccaatagaacatggggctcactctcgatcagcaggaccagtgagc

SEQ ID NO: 198 - DNA, 68 bp, synthetic construct
  source 1..68: mol_type = other DNA
ttttgctcactggtcctgctgatcgagagtgagccccatgttctattgggtcggcaggcgaggcactt

SEQ ID NO: 199 - DNA, 68 bp, synthetic construct
  source 1..68: mol_type = other DNA
atagatgaggctgggcaggcgtcgcataagtagatccggcagacagtcgtacagcaggtgcagtgagc

SEQ ID NO: 200 - DNA, 68 bp, synthetic construct
  source 1..68: mol_type = other DNA
ttttgctcactgcacctgctgtacgactgtctgccggatctacttatgcgacgcctgcccagcctcat

SEQ ID NO: 201 - DNA, 68 bp, synthetic construct
  source 1..68: mol_type = other DNA
atagaagtgcctccgctcgcgtcgctaaacaagttgcgcctgagtgtccaacacgaggtgcagtgagc

SEQ ID NO: 202 - DNA, 68 bp, synthetic construct
  source 1..68: mol_type = other DNA
ttttgctcactgcacctcgtgttggacactcaggcgcaacttgtttagcgacgcgagcggaggcactt

SEQ ID NO: 203 - DNA, 68 bp, synthetic construct
  source 1..68: mol_type = other DNA
atagatctggcacggcaggcgtcgcataagatgatggggcagacagtccaactggacgaggagacagc

SEQ ID NO: 204 - DNA, 68 bp, synthetic construct
  source 1..68: mol_type = other DNA
ttttgctgtctcctcgtccagttggactgtctgccccatcatcttatgcgacgcctgccgtgccagat

SEQ ID NO: 205 - DNA, 68 bp, synthetic construct
  source 1..68: mol_type = other DNA
atagaagtgcctccgctgccgaggcataagatgatccgggtgacagtccaactggagcagctgagtgc

SEQ ID NO: 206 - DNA, 68 bp, synthetic construct
  source 1..68: mol_type = other DNA
ttttgcactcagctgctccagttggactgtcacccggatcatcttatgcctcggcagcggaggcactt

SEQ ID NO: 207 - DNA, 68 bp, synthetic construct
  source 1..68: mol_type = other DNA
atagatctgggtcgggtggggacccaaatgaacatggggctcactctcgtacacgaggtgcacagacc

SEQ ID NO: 208 - DNA, 68 bp, synthetic construct
  source 1..68: mol_type = other DNA
ttttggtctgtgcacctcgtgtacgagagtgagccccatgttcatttgggtccccacccgacccagat

SEQ ID NO: 209 - DNA, 951 bp, synthetic construct
  source 1..951: mol_type = other DNA
taatacgactcactataagggctctctgctcctcctgttcgacagtcagccgcatcttcttttgcgtcgccagccgagccacatcgctcagccaccatggatagcactgagaacgtcatcaagcccttcatgcgcttcaaggtgcacatggagggctccgtgaacggccacgagttcgagatcgagggcgtgggcgagggcaagccctacgagggcacccagaccgccaagctgcaagtgaccaagggcggccccctgcccttcgcctgggacatcctgtccccccagttcttctacggctccaaggcgtacatcaagcaccccgccgacatccccgactacctcaagcagtccttccccgagggcttcaagtgggagcgcgtgatgaacttcgaggacggcggcgtggtgaccgtgacccaggactcctccctgcaggacggcaccctcatctaccacgtgaagttcatcggcgtgaacttcccctccgacggccccgtaatgcagaagaaaactctgggctgggagccctccactgagcgcaactacccccgcgacggcgtgctgaagggcgagaaccacatggcgctgaagctgaagggcggcggccactacctgtgtgagttcaagtccatctacatggccaagaagcccgtgaagctgcccggctaccactacgtggactacaagctcgacatcacctcccacaacgaggactacaccgtggtggagcagtacgagcgcgccgaggcccgccaccacctgttccagtgataatagaagtgggtcgcctgccgacccaatagatgatggggcagacagtcgtacacgagcagcacagaccaaaaaaaaaaaaaaaaaaaaaaaaaaaaaaaaaaaaaaaaaaaaaaaaaaaaaaaaaaaaaaaaaaaaaaaaaaaaaaaaaaaaaaaaaaaaaaaaaaaaagagacg

SEQ ID NO: 210 - DNA, 951 bp, synthetic construct
  source 1..951: mol_type = other DNA
taatacgactcactataagggctctctgctcctcctgttcgacagtcagccgcatcttcttttgcgtcgccagccgagccacatcgctcagccaccatggatagcactgagaacgtcatcaagcccttcatgcgcttcaaggtgcacatggagggctccgtgaacggccacgagttcgagatcgagggcgtgggcgagggcaagccctacgagggcacccagaccgccaagctgcaagtgaccaagggcggccccctgcccttcgcctgggacatcctgtccccccagttcttctacggctccaaggcgtacatcaagcaccccgccgacatccccgactacctcaagcagtccttccccgagggcttcaagtgggagcgcgtgatgaacttcgaggacggcggcgtggtgaccgtgacccaggactcctccctgcaggacggcaccctcatctaccacgtgaagttcatcggcgtgaacttcccctccgacggccccgtaatgcagaagaaaactctgggctgggagccctccactgagcgcaactacccccgcgacggcgtgctgaagggcgagaaccacatggcgctgaagctgaagggcggcggccactacctgtgtgagttcaagtccatctacatggccaagaagcccgtgaagctgcccggctaccactacgtggactacaagctcgacatcacctcccacaacgaggactacaccgtggtggagcagtacgagcgcgccgaggcccgccaccacctgttccagtgataatagaagtgcctcgcctgccgacccaatagaacatggggctcactctcgatcagcaggaccagtgagcaaaaaaaaaaaaaaaaaaaaaaaaaaaaaaaaaaaaaaaaaaaaaaaaaaaaaaaaaaaaaaaaaaaaaaaaaaaaaaaaaaaaaaaaaaaaaaaaaaaaagagacg

SEQ ID NO: 211 - DNA, 951 bp, synthetic construct
  source 1..951: mol_type = other DNA
taatacgactcactataagggctctctgctcctcctgttcgacagtcagccgcatcttcttttgcgtcgccagccgagccacatcgctcagccaccatggatagcactgagaacgtcatcaagcccttcatgcgcttcaaggtgcacatggagggctccgtgaacggccacgagttcgagatcgagggcgtgggcgagggcaagccctacgagggcacccagaccgccaagctgcaagtgaccaagggcggccccctgcccttcgcctgggacatcctgtccccccagttcttctacggctccaaggcgtacatcaagcaccccgccgacatccccgactacctcaagcagtccttccccgagggcttcaagtgggagcgcgtgatgaacttcgaggacggcggcgtggtgaccgtgacccaggactcctccctgcaggacggcaccctcatctaccacgtgaagttcatcggcgtgaacttcccctccgacggccccgtaatgcagaagaaaactctgggctgggagccctccactgagcgcaactacccccgcgacggcgtgctgaagggcgagaaccacatggcgctgaagctgaagggcggcggccactacctgtgtgagttcaagtccatctacatggccaagaagcccgtgaagctgcccggctaccactacgtggactacaagctcgacatcacctcccacaacgaggactacaccgtggtggagcagtacgagcgcgccgaggcccgccaccacctgttccagtgataatagatgaggctgggcaggcgtcgcataagtagatccggcagacagtcgtacagcaggtgcagtgagcaaaaaaaaaaaaaaaaaaaaaaaaaaaaaaaaaaaaaaaaaaaaaaaaaaaaaaaaaaaaaaaaaaaaaaaaaaaaaaaaaaaaaaaaaaaaaaaaaaaaagagacg

SEQ ID NO: 212 - DNA, 951 bp, synthetic construct
  source 1..951: mol_type = other DNA
taatacgactcactataagggctctctgctcctcctgttcgacagtcagccgcatcttcttttgcgtcgccagccgagccacatcgctcagccaccatggatagcactgagaacgtcatcaagcccttcatgcgcttcaaggtgcacatggagggctccgtgaacggccacgagttcgagatcgagggcgtgggcgagggcaagccctacgagggcacccagaccgccaagctgcaagtgaccaagggcggccccctgcccttcgcctgggacatcctgtccccccagttcttctacggctccaaggcgtacatcaagcaccccgccgacatccccgactacctcaagcagtccttccccgagggcttcaagtgggagcgcgtgatgaacttcgaggacggcggcgtggtgaccgtgacccaggactcctccctgcaggacggcaccctcatctaccacgtgaagttcatcggcgtgaacttcccctccgacggccccgtaatgcagaagaaaactctgggctgggagccctccactgagcgcaactacccccgcgacggcgtgctgaagggcgagaaccacatggcgctgaagctgaagggcggcggccactacctgtgtgagttcaagtccatctacatggccaagaagcccgtgaagctgcccggctaccactacgtggactacaagctcgacatcacctcccacaacgaggactacaccgtggtggagcagtacgagcgcgccgaggcccgccaccacctgttccagtgataatagaagtgcctccgctcgcgtcgctaaacaagttgcgcctgagtgtccaacacgaggtgcagtgagcaaaaaaaaaaaaaaaaaaaaaaaaaaaaaaaaaaaaaaaaaaaaaaaaaaaaaaaaaaaaaaaaaaaaaaaaaaaaaaaaaaaaaaaaaaaaaaaaaaaaagagacg

SEQ ID NO: 213 - DNA, 951 bp, synthetic construct
  source 1..951: mol_type = other DNA
taatacgactcactataagggctctctgctcctcctgttcgacagtcagccgcatcttcttttgcgtcgccagccgagccacatcgctcagccaccatggatagcactgagaacgtcatcaagcccttcatgcgcttcaaggtgcacatggagggctccgtgaacggccacgagttcgagatcgagggcgtgggcgagggcaagccctacgagggcacccagaccgccaagctgcaagtgaccaagggcggccccctgcccttcgcctgggacatcctgtccccccagttcttctacggctccaaggcgtacatcaagcaccccgccgacatccccgactacctcaagcagtccttccccgagggcttcaagtgggagcgcgtgatgaacttcgaggacggcggcgtggtgaccgtgacccaggactcctccctgcaggacggcaccctcatctaccacgtgaagttcatcggcgtgaacttcccctccgacggccccgtaatgcagaagaaaactctgggctgggagccctccactgagcgcaactacccccgcgacggcgtgctgaagggcgagaaccacatggcgctgaagctgaagggcggcggccactacctgtgtgagttcaagtccatctacatggccaagaagcccgtgaagctgcccggctaccactacgtggactacaagctcgacatcacctcccacaacgaggactacaccgtggtggagcagtacgagcgcgccgaggcccgccaccacctgttccagtgataatagatctggcacggcaggcgtcgcataagatgatggggcagacagtccaactggacgaggagacagcaaaaaaaaaaaaaaaaaaaaaaaaaaaaaaaaaaaaaaaaaaaaaaaaaaaaaaaaaaaaaaaaaaaaaaaaaaaaaaaaaaaaaaaaaaaaaaaaaaaaagagacg

SEQ ID NO: 214 - DNA, 951 bp, synthetic construct
  source 1..951: mol_type = other DNA
taatacgactcactataagggctctctgctcctcctgttcgacagtcagccgcatcttcttttgcgtcgccagccgagccacatcgctcagccaccatggatagcactgagaacgtcatcaagcccttcatgcgcttcaaggtgcacatggagggctccgtgaacggccacgagttcgagatcgagggcgtgggcgagggcaagccctacgagggcacccagaccgccaagctgcaagtgaccaagggcggccccctgcccttcgcctgggacatcctgtccccccagttcttctacggctccaaggcgtacatcaagcaccccgccgacatccccgactacctcaagcagtccttccccgagggcttcaagtgggagcgcgtgatgaacttcgaggacggcggcgtggtgaccgtgacccaggactcctccctgcaggacggcaccctcatctaccacgtgaagttcatcggcgtgaacttcccctccgacggccccgtaatgcagaagaaaactctgggctgggagccctccactgagcgcaactacccccgcgacggcgtgctgaagggcgagaaccacatggcgctgaagctgaagggcggcggccactacctgtgtgagttcaagtccatctacatggccaagaagcccgtgaagctgcccggctaccactacgtggactacaagctcgacatcacctcccacaacgaggactacaccgtggtggagcagtacgagcgcgccgaggcccgccaccacctgttccagtgataatagaagtgcctccgctgccgaggcataagatgatccgggtgacagtccaactggagcagctgagtgcaaaaaaaaaaaaaaaaaaaaaaaaaaaaaaaaaaaaaaaaaaaaaaaaaaaaaaaaaaaaaaaaaaaaaaaaaaaaaaaaaaaaaaaaaaaaaaaaaaaaagagacg

SEQ ID NO: 215 - DNA, 951 bp, synthetic construct
  source 1..951: mol_type = other DNA
taatacgactcactataagggctctctgctcctcctgttcgacagtcagccgcatcttcttttgcgtcgccagccgagccacatcgctcagccaccatggatagcactgagaacgtcatcaagcccttcatgcgcttcaaggtgcacatggagggctccgtgaacggccacgagttcgagatcgagggcgtgggcgagggcaagccctacgagggcacccagaccgccaagctgcaagtgaccaagggcggccccctgcccttcgcctgggacatcctgtccccccagttcttctacggctccaaggcgtacatcaagcaccccgccgacatccccgactacctcaagcagtccttccccgagggcttcaagtgggagcgcgtgatgaacttcgaggacggcggcgtggtgaccgtgacccaggactcctccctgcaggacggcaccctcatctaccacgtgaagttcatcggcgtgaacttcccctccgacggccccgtaatgcagaagaaaactctgggctgggagccctccactgagcgcaactacccccgcgacggcgtgctgaagggcgagaaccacatggcgctgaagctgaagggcggcggccactacctgtgtgagttcaagtccatctacatggccaagaagcccgtgaagctgcccggctaccactacgtggactacaagctcgacatcacctcccacaacgaggactacaccgtggtggagcagtacgagcgcgccgaggcccgccaccacctgttccagtgataatagatctgggtcgggtggggacccaaatgaacatggggctcactctcgtacacgaggtgcacagaccaaaaaaaaaaaaaaaaaaaaaaaaaaaaaaaaaaaaaaaaaaaaaaaaaaaaaaaaaaaaaaaaaaaaaaaaaaaaaaaaaaaaaaaaaaaaaaaaaaaaagagacg

SEQ ID NO: 216 - DNA, 48 bp, synthetic construct
  source 1..48: mol_type = other DNA
ataggggttctcctgagtctgggggaccagagaatactatttattctc

SEQ ID NO: 217 - DNA, 48 bp, synthetic construct
  source 1..48: mol_type = other DNA
ttttgagaataaatagtattctctggtcccccagactcaggagaaccc

SEQ ID NO: 218 - DNA, 47 bp, synthetic construct
  source 1..47: mol_type = other DNA
ataggggtctctctggtctgtgggaccagaaaatactagttattctc

SEQ ID NO: 219 - DNA, 47 bp, synthetic construct
  source 1..47: mol_type = other DNA
ttttgagaataactagtattttctggtcccacagaccagagagaccc

SEQ ID NO: 220 - DNA, 46 bp, synthetic construct
  source 1..46: mol_type = other DNA
atagggttctcttgagtcttggggacagaagaaactagttattctc

SEQ ID NO: 221 - DNA, 46 bp, synthetic construct
  source 1..46: mol_type = other DNA
ttttgagaataactagtttcttctgtccccaagactcaagagaacc

SEQ ID NO: 222 - DNA, 46 bp, synthetic construct
  source 1..46: mol_type = other DNA
ataggggttcctctgatctgtgggaccaaagaatctagttattctc

SEQ ID NO: 223 - DNA, 46 bp, synthetic construct
  source 1..46: mol_type = other DNA
ttttgagaataactagattctttggtcccacagatcagaggaaccc

SEQ ID NO: 224 - DNA, 44 bp, synthetic construct
  source 1..44: mol_type = other DNA
atagggttcttctgatctgtgggacagaagatactgtttatctc

SEQ ID NO: 225 - DNA, 44 bp, synthetic construct
  source 1..44: mol_type = other DNA
ttttgagataaacagtatcttctgtcccacagatcagaagaacc

SEQ ID NO: 226 - DNA, 43 bp, synthetic construct
  source 1..43: mol_type = other DNA
ataggggtctcctgatctgggggccagagaaactatttatctc

SEQ ID NO: 227 - DNA, 43 bp, synthetic construct
  source 1..43: mol_type = other DNA
ttttgagataaatagtttctctggcccccagatcaggagaccc

SEQ ID NO: 228 - DNA, 40 bp, synthetic construct
  source 1..40: mol_type = other DNA
atagggtttcttgatcttgggacagagaaactgttatttc

SEQ ID NO: 229 - DNA, 40 bp, synthetic construct
  source 1..40: mol_type = other DNA
ttttgaaataacagtttctctgtcccaagatcaagaaacc

SEQ ID NO: 230 - DNA, 46 bp, synthetic construct
  source 1..46: mol_type = other DNA
ataggggttctctgagtctgtgggccagaagaataagtttattctc

SEQ ID NO: 231 - DNA, 46 bp, synthetic construct
  source 1..46: mol_type = other DNA
ttttgagaataaacttattcttctggcccacagactcagagaaccc

SEQ ID NO: 232 - DNA, 44 bp, synthetic construct
  source 1..44: mol_type = other DNA
ataggttctctctgactgtggggacgaagaatacttttattctc

SEQ ID NO: 233 - DNA, 44 bp, synthetic construct
  source 1..44: mol_type = other DNA
ttttgagaataaaagtattcttcgtccccacagtcagagagaac

SEQ ID NO: 234 - DNA, 44 bp, synthetic construct
  source 1..44: mol_type = other DNA
ataggggttctctgagtgtggggaccaagaatacttttattctc

SEQ ID NO: 235 - DNA, 44 bp, synthetic construct
  source 1..44: mol_type = other DNA
ttttgagaataaaagtattcttggtccccacactcagagaaccc

SEQ ID NO: 236 - DNA, 44 bp, synthetic construct
  source 1..44: mol_type = other DNA
ataggggttctctgagtctggggaccaggaatactattattctc

SEQ ID NO: 237 - DNA, 44 bp, synthetic construct
  source 1..44: mol_type = other DNA
ttttgagaataatagtattcctggtccccagactcagagaaccc

SEQ ID NO: 238 - DNA, 42 bp, synthetic construct
  source 1..42: mol_type = other DNA
ataggggctctctgtctgtggaccagaaatactagtattctc

SEQ ID NO: 239 - DNA, 42 bp, synthetic construct
  source 1..42: mol_type = other DNA
ttttgagaatactagtatttctggtccacagacagagagccc

SEQ ID NO: 240 - DNA, 40 bp, synthetic construct
  source 1..40: mol_type = other DNA
ataggttctctgagtctggggacgaagaactagttttctc

SEQ ID NO: 241 - DNA, 40 bp, synthetic construct
  source 1..40: mol_type = other DNA
ttttgagaaaactagttcttcgtccccagactcagagaac

SEQ ID NO: 242 - DNA, 38 bp, synthetic construct
  source 1..38: mol_type = other DNA
ataggttctctgagtgtgggccagaaatacgtttactc

SEQ ID NO: 243 - DNA, 38 bp, synthetic construct
  source 1..38: mol_type = other DNA
ttttgagtaaacgtatttctggcccacactcagagaac

SEQ ID NO: 244 - DNA, 43 bp, synthetic construct
  source 1..43: mol_type = other DNA
ataggggtctctgagtctgggaccagaagaatagtttattctc

SEQ ID NO: 245 - DNA, 43 bp, synthetic construct
  source 1..43: mol_type = other DNA
ttttgagaataaactattcttctggtcccagactcagagaccc

SEQ ID NO: 246 - DNA, 43 bp, synthetic construct
  source 1..43: mol_type = other DNA
ataggggttcctgagtctgtgaccagaagaatagtttattctc

SEQ ID NO: 247 - DNA, 43 bp, synthetic construct
  source 1..43: mol_type = other DNA
ttttgagaataaactattcttctggtcacagactcaggaaccc

SEQ ID NO: 248 - DNA, 43 bp, synthetic construct
  source 1..43: mol_type = other DNA
ataggggttctctagtctgtgggcagaagaatagtttattctc

SEQ ID NO: 249 - DNA, 43 bp, synthetic construct
  source 1..43: mol_type = other DNA
ttttgagaataaactattcttctgcccacagactagagaaccc

SEQ ID NO: 250 - DNA, 40 bp, synthetic construct
  source 1..40: mol_type = other DNA
ataggtctctctgatgtggggacaagaatactttattctc

SEQ ID NO: 251 - DNA, 40 bp, synthetic construct
  source 1..40: mol_type = other DNA
ttttgagaataaagtattcttgtccccacatcagagagac

SEQ ID NO: 252 - DNA, 40 bp, synthetic construct
  source 1..40: mol_type = other DNA
ataggggtctctgagttggggaccagaatactttattctc

SEQ ID NO: 253 - DNA, 40 bp, synthetic construct
  source 1..40: mol_type = other DNA
ttttgagaataaagtattctggtccccaactcagagaccc

SEQ ID NO: 254 - DNA, 46 bp, synthetic construct
  source 1..46: mol_type = other DNA
ataggggttctctctgaggtggggaccagaagactagtttattctc

SEQ ID NO: 255 - DNA, 46 bp, synthetic construct
  source 1..46: mol_type = other DNA
ttttgagaataaactagtcttctggtccccacctcagagagaaccc

SEQ ID NO: 256 - DNA, 43 bp, synthetic construct
  source 1..43: mol_type = other DNA
ataggtctctctgagtctgggaccagaagaatagtttattctc

SEQ ID NO: 257 - DNA, 43 bp, synthetic construct
  source 1..43: mol_type = other DNA
ttttgagaataaactattcttctggtcccagactcagagagac

SEQ ID NO: 258 - DNA, 909 bp, synthetic construct
  source 1..909: mol_type = other DNA
taatacgactcactataagggagaataaactagtattcttctggtccccacagactcagagagaacccgccaccatggatagcactgagaacgtcatcaagcccttcatgcgcttcaaggtgcacatggagggctccgtgaacggccacgagttcgagatcgagggcgtgggcgagggcaagccctacgagggcacccagaccgccaagctgcaagtgaccaagggcggccccctgcccttcgcctgggacatcctgtccccccagttcttctacggctccaaggcgtacatcaagcaccccgccgacatccccgactacctcaagcagtccttccccgagggcttcaagtgggagcgcgtgatgaacttcgaggacggcggcgtggtgaccgtgacccaggactcctccctgcaggacggcaccctcatctaccacgtgaagttcatcggcgtgaacttcccctccgacggccccgtaatgcagaagaaaactctgggctgggagccctccactgagcgcaactacccccgcgacggcgtgctgaagggcgagaaccacatggcgctgaagctgaagggcggcggccactacctgtgtgagttcaagtccatctacatggccaagaagcccgtgaagctgcccggctaccactacgtggactacaagctcgacatcacctcccacaacgaggactacaccgtggtggagcagtacgagcgcgccgaggcccgccaccacctgttccagtgataataggggttctcctgagtctgggggaccagagaatactatttattctcaaaaaaaaaaaaaaaaaaaaaaaaaaaaaaaaaaaaaaaaaaaaaaaaaaaaaaaaaaaaaaaaaaaaaaaaaaaaaaaaaaaaaaaaaaaaaaaaaaaaagagacg

SEQ ID NO: 259 - DNA, 908 bp, synthetic construct
  source 1..908: mol_type = other DNA
taatacgactcactataagggagaataaactagtattcttctggtccccacagactcagagagaacccgccaccatggatagcactgagaacgtcatcaagcccttcatgcgcttcaaggtgcacatggagggctccgtgaacggccacgagttcgagatcgagggcgtgggcgagggcaagccctacgagggcacccagaccgccaagctgcaagtgaccaagggcggccccctgcccttcgcctgggacatcctgtccccccagttcttctacggctccaaggcgtacatcaagcaccccgccgacatccccgactacctcaagcagtccttccccgagggcttcaagtgggagcgcgtgatgaacttcgaggacggcggcgtggtgaccgtgacccaggactcctccctgcaggacggcaccctcatctaccacgtgaagttcatcggcgtgaacttcccctccgacggccccgtaatgcagaagaaaactctgggctgggagccctccactgagcgcaactacccccgcgacggcgtgctgaagggcgagaaccacatggcgctgaagctgaagggcggcggccactacctgtgtgagttcaagtccatctacatggccaagaagcccgtgaagctgcccggctaccactacgtggactacaagctcgacatcacctcccacaacgaggactacaccgtggtggagcagtacgagcgcgccgaggcccgccaccacctgttccagtgataataggggtctctctggtctgtgggaccagaaaatactagttattctcaaaaaaaaaaaaaaaaaaaaaaaaaaaaaaaaaaaaaaaaaaaaaaaaaaaaaaaaaaaaaaaaaaaaaaaaaaaaaaaaaaaaaaaaaaaaaaaaaaaaagagacg

SEQ ID NO: 260 - DNA, 907 bp, synthetic construct
  source 1..907: mol_type = other DNA
taatacgactcactataagggagaataaactagtattcttctggtccccacagactcagagagaacccgccaccatggatagcactgagaacgtcatcaagcccttcatgcgcttcaaggtgcacatggagggctccgtgaacggccacgagttcgagatcgagggcgtgggcgagggcaagccctacgagggcacccagaccgccaagctgcaagtgaccaagggcggccccctgcccttcgcctgggacatcctgtccccccagttcttctacggctccaaggcgtacatcaagcaccccgccgacatccccgactacctcaagcagtccttccccgagggcttcaagtgggagcgcgtgatgaacttcgaggacggcggcgtggtgaccgtgacccaggactcctccctgcaggacggcaccctcatctaccacgtgaagttcatcggcgtgaacttcccctccgacggccccgtaatgcagaagaaaactctgggctgggagccctccactgagcgcaactacccccgcgacggcgtgctgaagggcgagaaccacatggcgctgaagctgaagggcggcggccactacctgtgtgagttcaagtccatctacatggccaagaagcccgtgaagctgcccggctaccactacgtggactacaagctcgacatcacctcccacaacgaggactacaccgtggtggagcagtacgagcgcgccgaggcccgccaccacctgttccagtgataatagggttctcttgagtcttggggacagaagaaactagttattctcaaaaaaaaaaaaaaaaaaaaaaaaaaaaaaaaaaaaaaaaaaaaaaaaaaaaaaaaaaaaaaaaaaaaaaaaaaaaaaaaaaaaaaaaaaaaaaaaaaaaagagacg

SEQ ID NO: 261 - DNA, 907 bp, synthetic construct
  source 1..907: mol_type = other DNA
taatacgactcactataagggagaataaactagtattcttctggtccccacagactcagagagaacccgccaccatggatagcactgagaacgtcatcaagcccttcatgcgcttcaaggtgcacatggagggctccgtgaacggccacgagttcgagatcgagggcgtgggcgagggcaagccctacgagggcacccagaccgccaagctgcaagtgaccaagggcggccccctgcccttcgcctgggacatcctgtccccccagttcttctacggctccaaggcgtacatcaagcaccccgccgacatccccgactacctcaagcagtccttccccgagggcttcaagtgggagcgcgtgatgaacttcgaggacggcggcgtggtgaccgtgacccaggactcctccctgcaggacggcaccctcatctaccacgtgaagttcatcggcgtgaacttcccctccgacggccccgtaatgcagaagaaaactctgggctgggagccctccactgagcgcaactacccccgcgacggcgtgctgaagggcgagaaccacatggcgctgaagctgaagggcggcggccactacctgtgtgagttcaagtccatctacatggccaagaagcccgtgaagctgcccggctaccactacgtggactacaagctcgacatcacctcccacaacgaggactacaccgtggtggagcagtacgagcgcgccgaggcccgccaccacctgttccagtgataataggggttcctctgatctgtgggaccaaagaatctagttattctcaaaaaaaaaaaaaaaaaaaaaaaaaaaaaaaaaaaaaaaaaaaaaaaaaaaaaaaaaaaaaaaaaaaaaaaaaaaaaaaaaaaaaaaaaaaaaaaaaaaaagagacg

SEQ ID NO: 262 - DNA, 905 bp, synthetic construct
  source 1..905: mol_type = other DNA
taatacgactcactataagggagaataaactagtattcttctggtccccacagactcagagagaacccgccaccatggatagcactgagaacgtcatcaagcccttcatgcgcttcaaggtgcacatggagggctccgtgaacggccacgagttcgagatcgagggcgtgggcgagggcaagccctacgagggcacccagaccgccaagctgcaagtgaccaagggcggccccctgcccttcgcctgggacatcctgtccccccagttcttctacggctccaaggcgtacatcaagcaccccgccgacatccccgactacctcaagcagtccttccccgagggcttcaagtgggagcgcgtgatgaacttcgaggacggcggcgtggtgaccgtgacccaggactcctccctgcaggacggcaccctcatctaccacgtgaagttcatcggcgtgaacttcccctccgacggccccgtaatgcagaagaaaactctgggctgggagccctccactgagcgcaactacccccgcgacggcgtgctgaagggcgagaaccacatggcgctgaagctgaagggcggcggccactacctgtgtgagttcaagtccatctacatggccaagaagcccgtgaagctgcccggctaccactacgtggactacaagctcgacatcacctcccacaacgaggactacaccgtggtggagcagtacgagcgcgccgaggcccgccaccacctgttccagtgataatagggttcttctgatctgtgggacagaagatactgtttatctcaaaaaaaaaaaaaaaaaaaaaaaaaaaaaaaaaaaaaaaaaaaaaaaaaaaaaaaaaaaaaaaaaaaaaaaaaaaaaaaaaaaaaaaaaaaaaaaaaaaaagagacg

SEQ ID NO: 263 - DNA, 904 bp, synthetic construct
  source 1..904: mol_type = other DNA
taatacgactcactataagggagaataaactagtattcttctggtccccacagactcagagagaacccgccaccatggatagcactgagaacgtcatcaagcccttcatgcgcttcaaggtgcacatggagggctccgtgaacggccacgagttcgagatcgagggcgtgggcgagggcaagccctacgagggcacccagaccgccaagctgcaagtgaccaagggcggccccctgcccttcgcctgggacatcctgtccccccagttcttctacggctccaaggcgtacatcaagcaccccgccgacatccccgactacctcaagcagtccttccccgagggcttcaagtgggagcgcgtgatgaacttcgaggacggcggcgtggtgaccgtgacccaggactcctccctgcaggacggcaccctcatctaccacgtgaagttcatcggcgtgaacttcccctccgacggccccgtaatgcagaagaaaactctgggctgggagccctccactgagcgcaactacccccgcgacggcgtgctgaagggcgagaaccacatggcgctgaagctgaagggcggcggccactacctgtgtgagttcaagtccatctacatggccaagaagcccgtgaagctgcccggctaccactacgtggactacaagctcgacatcacctcccacaacgaggactacaccgtggtggagcagtacgagcgcgccgaggcccgccaccacctgttccagtgataataggggtctcctgatctgggggccagagaaactatttatctcaaaaaaaaaaaaaaaaaaaaaaaaaaaaaaaaaaaaaaaaaaaaaaaaaaaaaaaaaaaaaaaaaaaaaaaaaaaaaaaaaaaaaaaaaaaaaaaaaaaaagagacg

SEQ ID NO: 264 - DNA, 901 bp, synthetic construct
  source 1..901: mol_type = other DNA
taatacgactcactataagggagaataaactagtattcttctggtccccacagactcagagagaacccgccaccatggatagcactgagaacgtcatcaagcccttcatgcgcttcaaggtgcacatggagggctccgtgaacggccacgagttcgagatcgagggcgtgggcgagggcaagccctacgagggcacccagaccgccaagctgcaagtgaccaagggcggccccctgcccttcgcctgggacatcctgtccccccagttcttctacggctccaaggcgtacatcaagcaccccgccgacatccccgactacctcaagcagtccttccccgagggcttcaagtgggagcgcgtgatgaacttcgaggacggcggcgtggtgaccgtgacccaggactcctccctgcaggacggcaccctcatctaccacgtgaagttcatcggcgtgaacttcccctccgacggccccgtaatgcagaagaaaactctgggctgggagccctccactgagcgcaactacccccgcgacggcgtgctgaagggcgagaaccacatggcgctgaagctgaagggcggcggccactacctgtgtgagttcaagtccatctacatggccaagaagcccgtgaagctgcccggctaccactacgtggactacaagctcgacatcacctcccacaacgaggactacaccgtggtggagcagtacgagcgcgccgaggcccgccaccacctgttccagtgataatagggtttcttgatcttgggacagagaaactgttatttcaaaaaaaaaaaaaaaaaaaaaaaaaaaaaaaaaaaaaaaaaaaaaaaaaaaaaaaaaaaaaaaaaaaaaaaaaaaaaaaaaaaaaaaaaaaaaaaaaaaaagagacg

SEQ ID NO: 265 - DNA, 907 bp, synthetic construct
  source 1..907: mol_type = other DNA
taatacgactcactataagggagaataaactagtattcttctggtccccacagactcagagagaacccgccaccatggatagcactgagaacgtcatcaagcccttcatgcgcttcaaggtgcacatggagggctccgtgaacggccacgagttcgagatcgagggcgtgggcgagggcaagccctacgagggcacccagaccgccaagctgcaagtgaccaagggcggccccctgcccttcgcctgggacatcctgtccccccagttcttctacggctccaaggcgtacatcaagcaccccgccgacatccccgactacctcaagcagtccttccccgagggcttcaagtgggagcgcgtgatgaacttcgaggacggcggcgtggtgaccgtgacccaggactcctccctgcaggacggcaccctcatctaccacgtgaagttcatcggcgtgaacttcccctccgacggccccgtaatgcagaagaaaactctgggctgggagccctccactgagcgcaactacccccgcgacggcgtgctgaagggcgagaaccacatggcgctgaagctgaagggcggcggccactacctgtgtgagttcaagtccatctacatggccaagaagcccgtgaagctgcccggctaccactacgtggactacaagctcgacatcacctcccacaacgaggactacaccgtggtggagcagtacgagcgcgccgaggcccgccaccacctgttccagtgataataggggttctctgagtctgtgggccagaagaataagtttattctcaaaaaaaaaaaaaaaaaaaaaaaaaaaaaaaaaaaaaaaaaaaaaaaaaaaaaaaaaaaaaaaaaaaaaaaaaaaaaaaaaaaaaaaaaaaaaaaaaaaaagagacg

SEQ ID NO: 266 - DNA, 905 bp, synthetic construct
  source 1..905: mol_type = other DNA
taatacgactcactataagggagaataaactagtattcttctggtccccacagactcagagagaacccgccaccatggatagcactgagaacgtcatcaagcccttcatgcgcttcaaggtgcacatggagggctccgtgaacggccacgagttcgagatcgagggcgtgggcgagggcaagccctacgagggcacccagaccgccaagctgcaagtgaccaagggcggccccctgcccttcgcctgggacatcctgtccccccagttcttctacggctccaaggcgtacatcaagcaccccgccgacatccccgactacctcaagcagtccttccccgagggcttcaagtgggagcgcgtgatgaacttcgaggacggcggcgtggtgaccgtgacccaggactcctccctgcaggacggcaccctcatctaccacgtgaagttcatcggcgtgaacttcccctccgacggccccgtaatgcagaagaaaactctgggctgggagccctccactgagcgcaactacccccgcgacggcgtgctgaagggcgagaaccacatggcgctgaagctgaagggcggcggccactacctgtgtgagttcaagtccatctacatggccaagaagcccgtgaagctgcccggctaccactacgtggactacaagctcgacatcacctcccacaacgaggactacaccgtggtggagcagtacgagcgcgccgaggcccgccaccacctgttccagtgataataggttctctctgactgtggggacgaagaatacttttattctcaaaaaaaaaaaaaaaaaaaaaaaaaaaaaaaaaaaaaaaaaaaaaaaaaaaaaaaaaaaaaaaaaaaaaaaaaaaaaaaaaaaaaaaaaaaaaaaaaaaaagagacg

SEQ ID NO: 267 - DNA, 905 bp, synthetic construct
  source 1..905: mol_type = other DNA
taatacgactcactataagggagaataaactagtattcttctggtccccacagactcagagagaacccgccaccatggatagcactgagaacgtcatcaagcccttcatgcgcttcaaggtgcacatggagggctccgtgaacggccacgagttcgagatcgagggcgtgggcgagggcaagccctacgagggcacccagaccgccaagctgcaagtgaccaagggcggccccctgcccttcgcctgggacatcctgtccccccagttcttctacggctccaaggcgtacatcaagcaccccgccgacatccccgactacctcaagcagtccttccccgagggcttcaagtgggagcgcgtgatgaacttcgaggacggcggcgtggtgaccgtgacccaggactcctccctgcaggacggcaccctcatctaccacgtgaagttcatcggcgtgaacttcccctccgacggccccgtaatgcagaagaaaactctgggctgggagccctccactgagcgcaactacccccgcgacggcgtgctgaagggcgagaaccacatggcgctgaagctgaagggcggcggccactacctgtgtgagttcaagtccatctacatggccaagaagcccgtgaagctgcccggctaccactacgtggactacaagctcgacatcacctcccacaacgaggactacaccgtggtggagcagtacgagcgcgccgaggcccgccaccacctgttccagtgataataggggttctctgagtgtggggaccaagaatacttttattctcaaaaaaaaaaaaaaaaaaaaaaaaaaaaaaaaaaaaaaaaaaaaaaaaaaaaaaaaaaaaaaaaaaaaaaaaaaaaaaaaaaaaaaaaaaaaaaaaaaaaagagacg

SEQ ID NO: 268 - DNA, 905 bp, synthetic construct
  source 1..905: mol_type = other DNA
taatacgactcactataagggagaataaactagtattcttctggtccccacagactcagagagaacccgccaccatggatagcactgagaacgtcatcaagcccttcatgcgcttcaaggtgcacatggagggctccgtgaacggccacgagttcgagatcgagggcgtgggcgagggcaagccctacgagggcacccagaccgccaagctgcaagtgaccaagggcggccccctgcccttcgcctgggacatcctgtccccccagttcttctacggctccaaggcgtacatcaagcaccccgccgacatccccgactacctcaagcagtccttccccgagggcttcaagtgggagcgcgtgatgaacttcgaggacggcggcgtggtgaccgtgacccaggactcctccctgcaggacggcaccctcatctaccacgtgaagttcatcggcgtgaacttcccctccgacggccccgtaatgcagaagaaaactctgggctgggagccctccactgagcgcaactacccccgcgacggcgtgctgaagggcgagaaccacatggcgctgaagctgaagggcggcggccactacctgtgtgagttcaagtccatctacatggccaagaagcccgtgaagctgcccggctaccactacgtggactacaagctcgacatcacctcccacaacgaggactacaccgtggtggagcagtacgagcgcgccgaggcccgccaccacctgttccagtgataataggggttctctgagtctggggaccaggaatactattattctcaaaaaaaaaaaaaaaaaaaaaaaaaaaaaaaaaaaaaaaaaaaaaaaaaaaaaaaaaaaaaaaaaaaaaaaaaaaaaaaaaaaaaaaaaaaaaaaaaaaaagagacg

SEQ ID NO: 269 - DNA, 903 bp, synthetic construct
  source 1..903: mol_type = other DNA
taatacgactcactataagggagaataaactagtattcttctggtccccacagactcagagagaacccgccaccatggatagcactgagaacgtcatcaagcccttcatgcgcttcaaggtgcacatggagggctccgtgaacggccacgagttcgagatcgagggcgtgggcgagggcaagccctacgagggcacccagaccgccaagctgcaagtgaccaagggcggccccctgcccttcgcctgggacatcctgtccccccagttcttctacggctccaaggcgtacatcaagcaccccgccgacatccccgactacctcaagcagtccttccccgagggcttcaagtgggagcgcgtgatgaacttcgaggacggcggcgtggtgaccgtgacccaggactcctccctgcaggacggcaccctcatctaccacgtgaagttcatcggcgtgaacttcccctccgacggccccgtaatgcagaagaaaactctgggctgggagccctccactgagcgcaactacccccgcgacggcgtgctgaagggcgagaaccacatggcgctgaagctgaagggcggcggccactacctgtgtgagttcaagtccatctacatggccaagaagcccgtgaagctgcccggctaccactacgtggactacaagctcgacatcacctcccacaacgaggactacaccgtggtggagcagtacgagcgcgccgaggcccgccaccacctgttccagtgataataggggctctctgtctgtggaccagaaatactagtattctcaaaaaaaaaaaaaaaaaaaaaaaaaaaaaaaaaaaaaaaaaaaaaaaaaaaaaaaaaaaaaaaaaaaaaaaaaaaaaaaaaaaaaaaaaaaaaaaaaaaaagagacg

SEQ ID NO: 270 - DNA, 901 bp, synthetic construct
  source 1..901: mol_type = other DNA
taatacgactcactataagggagaataaactagtattcttctggtccccacagactcagagagaacccgccaccatggatagcactgagaacgtcatcaagcccttcatgcgcttcaaggtgcacatggagggctccgtgaacggccacgagttcgagatcgagggcgtgggcgagggcaagccctacgagggcacccagaccgccaagctgcaagtgaccaagggcggccccctgcccttcgcctgggacatcctgtccccccagttcttctacggctccaaggcgtacatcaagcaccccgccgacatccccgactacctcaagcagtccttccccgagggcttcaagtgggagcgcgtgatgaacttcgaggacggcggcgtggtgaccgtgacccaggactcctccctgcaggacggcaccctcatctaccacgtgaagttcatcggcgtgaacttcccctccgacggccccgtaatgcagaagaaaactctgggctgggagccctccactgagcgcaactacccccgcgacggcgtgctgaagggcgagaaccacatggcgctgaagctgaagggcggcggccactacctgtgtgagttcaagtccatctacatggccaagaagcccgtgaagctgcccggctaccactacgtggactacaagctcgacatcacctcccacaacgaggactacaccgtggtggagcagtacgagcgcgccgaggcccgccaccacctgttccagtgataataggttctctgagtctggggacgaagaactagttttctcaaaaaaaaaaaaaaaaaaaaaaaaaaaaaaaaaaaaaaaaaaaaaaaaaaaaaaaaaaaaaaaaaaaaaaaaaaaaaaaaaaaaaaaaaaaaaaaaaaaaagagacg

SEQ ID NO: 271 - DNA, 899 bp, synthetic construct
  source 1..899: mol_type = other DNA
taatacgactcactataagggagaataaactagtattcttctggtccccacagactcagagagaacccgccaccatggatagcactgagaacgtcatcaagcccttcatgcgcttcaaggtgcacatggagggctccgtgaacggccacgagttcgagatcgagggcgtgggcgagggcaagccctacgagggcacccagaccgccaagctgcaagtgaccaagggcggccccctgcccttcgcctgggacatcctgtccccccagttcttctacggctccaaggcgtacatcaagcaccccgccgacatccccgactacctcaagcagtccttccccgagggcttcaagtgggagcgcgtgatgaacttcgaggacggcggcgtggtgaccgtgacccaggactcctccctgcaggacggcaccctcatctaccacgtgaagttcatcggcgtgaacttcccctccgacggccccgtaatgcagaagaaaactctgggctgggagccctccactgagcgcaactacccccgcgacggcgtgctgaagggcgagaaccacatggcgctgaagctgaagggcggcggccactacctgtgtgagttcaagtccatctacatggccaagaagcccgtgaagctgcccggctaccactacgtggactacaagctcgacatcacctcccacaacgaggactacaccgtggtggagcagtacgagcgcgccgaggcccgccaccacctgttccagtgataataggttctctgagtgtgggccagaaatacgtttactcaaaaaaaaaaaaaaaaaaaaaaaaaaaaaaaaaaaaaaaaaaaaaaaaaaaaaaaaaaaaaaaaaaaaaaaaaaaaaaaaaaaaaaaaaaaaaaaaaaaaagagacg

SEQ ID NO: 272 - DNA, 904 bp, synthetic construct
  source 1..904: mol_type = other DNA
taatacgactcactataagggagaataaactagtattcttctggtccccacagactcagagagaacccgccaccatggatagcactgagaacgtcatcaagcccttcatgcgcttcaaggtgcacatggagggctccgtgaacggccacgagttcgagatcgagggcgtgggcgagggcaagccctacgagggcacccagaccgccaagctgcaagtgaccaagggcggccccctgcccttcgcctgggacatcctgtccccccagttcttctacggctccaaggcgtacatcaagcaccccgccgacatccccgactacctcaagcagtccttccccgagggcttcaagtgggagcgcgtgatgaacttcgaggacggcggcgtggtgaccgtgacccaggactcctccctgcaggacggcaccctcatctaccacgtgaagttcatcggcgtgaacttcccctccgacggccccgtaatgcagaagaaaactctgggctgggagccctccactgagcgcaactacccccgcgacggcgtgctgaagggcgagaaccacatggcgctgaagctgaagggcggcggccactacctgtgtgagttcaagtccatctacatggccaagaagcccgtgaagctgcccggctaccactacgtggactacaagctcgacatcacctcccacaacgaggactacaccgtggtggagcagtacgagcgcgccgaggcccgccaccacctgttccagtgataataggggtctctgagtctgggaccagaagaatagtttattctcaaaaaaaaaaaaaaaaaaaaaaaaaaaaaaaaaaaaaaaaaaaaaaaaaaaaaaaaaaaaaaaaaaaaaaaaaaaaaaaaaaaaaaaaaaaaaaaaaaaaagagacg

SEQ ID NO: 273 - DNA, 904 bp, synthetic construct
  source 1..904: mol_type = other DNA
taatacgactcactataagggagaataaactagtattcttctggtccccacagactcagagagaacccgccaccatggatagcactgagaacgtcatcaagcccttcatgcgcttcaaggtgcacatggagggctccgtgaacggccacgagttcgagatcgagggcgtgggcgagggcaagccctacgagggcacccagaccgccaagctgcaagtgaccaagggcggccccctgcccttcgcctgggacatcctgtccccccagttcttctacggctccaaggcgtacatcaagcaccccgccgacatccccgactacctcaagcagtccttccccgagggcttcaagtgggagcgcgtgatgaacttcgaggacggcggcgtggtgaccgtgacccaggactcctccctgcaggacggcaccctcatctaccacgtgaagttcatcggcgtgaacttcccctccgacggccccgtaatgcagaagaaaactctgggctgggagccctccactgagcgcaactacccccgcgacggcgtgctgaagggcgagaaccacatggcgctgaagctgaagggcggcggccactacctgtgtgagttcaagtccatctacatggccaagaagcccgtgaagctgcccggctaccactacgtggactacaagctcgacatcacctcccacaacgaggactacaccgtggtggagcagtacgagcgcgccgaggcccgccaccacctgttccagtgataataggggttcctgagtctgtgaccagaagaatagtttattctcaaaaaaaaaaaaaaaaaaaaaaaaaaaaaaaaaaaaaaaaaaaaaaaaaaaaaaaaaaaaaaaaaaaaaaaaaaaaaaaaaaaaaaaaaaaaaaaaaaaaagagacg

SEQ ID NO: 274 - DNA, 904 bp, synthetic construct
  source 1..904: mol_type = other DNA
taatacgactcactataagggagaataaactagtattcttctggtccccacagactcagagagaacccgccaccatggatagcactgagaacgtcatcaagcccttcatgcgcttcaaggtgcacatggagggctccgtgaacggccacgagttcgagatcgagggcgtgggcgagggcaagccctacgagggcacccagaccgccaagctgcaagtgaccaagggcggccccctgcccttcgcctgggacatcctgtccccccagttcttctacggctccaaggcgtacatcaagcaccccgccgacatccccgactacctcaagcagtccttccccgagggcttcaagtgggagcgcgtgatgaacttcgaggacggcggcgtggtgaccgtgacccaggactcctccctgcaggacggcaccctcatctaccacgtgaagttcatcggcgtgaacttcccctccgacggccccgtaatgcagaagaaaactctgggctgggagccctccactgagcgcaactacccccgcgacggcgtgctgaagggcgagaaccacatggcgctgaagctgaagggcggcggccactacctgtgtgagttcaagtccatctacatggccaagaagcccgtgaagctgcccggctaccactacgtggactacaagctcgacatcacctcccacaacgaggactacaccgtggtggagcagtacgagcgcgccgaggcccgccaccacctgttccagtgataataggggttctctagtctgtgggcagaagaatagtttattctcaaaaaaaaaaaaaaaaaaaaaaaaaaaaaaaaaaaaaaaaaaaaaaaaaaaaaaaaaaaaaaaaaaaaaaaaaaaaaaaaaaaaaaaaaaaaaaaaaaaaagagacg

SEQ ID NO: 275 - DNA, 901 bp, synthetic construct
  source 1..901: mol_type = other DNA
taatacgactcactataagggagaataaactagtattcttctggtccccacagactcagagagaacccgccaccatggatagcactgagaacgtcatcaagcccttcatgcgcttcaaggtgcacatggagggctccgtgaacggccacgagttcgagatcgagggcgtgggcgagggcaagccctacgagggcacccagaccgccaagctgcaagtgaccaagggcggccccctgcccttcgcctgggacatcctgtccccccagttcttctacggctccaaggcgtacatcaagcaccccgccgacatccccgactacctcaagcagtccttccccgagggcttcaagtgggagcgcgtgatgaacttcgaggacggcggcgtggtgaccgtgacccaggactcctccctgcaggacggcaccctcatctaccacgtgaagttcatcggcgtgaacttcccctccgacggccccgtaatgcagaagaaaactctgggctgggagccctccactgagcgcaactacccccgcgacggcgtgctgaagggcgagaaccacatggcgctgaagctgaagggcggcggccactacctgtgtgagttcaagtccatctacatggccaagaagcccgtgaagctgcccggctaccactacgtggactacaagctcgacatcacctcccacaacgaggactacaccgtggtggagcagtacgagcgcgccgaggcccgccaccacctgttccagtgataataggtctctctgatgtggggacaagaatactttattctcaaaaaaaaaaaaaaaaaaaaaaaaaaaaaaaaaaaaaaaaaaaaaaaaaaaaaaaaaaaaaaaaaaaaaaaaaaaaaaaaaaaaaaaaaaaaaaaaaaaaagagacg

SEQ ID NO: 276 - DNA, 901 bp, synthetic construct
  source 1..901: mol_type = other DNA
taatacgactcactataagggagaataaactagtattcttctggtccccacagactcagagagaacccgccaccatggatagcactgagaacgtcatcaagcccttcatgcgcttcaaggtgcacatggagggctccgtgaacggccacgagttcgagatcgagggcgtgggcgagggcaagccctacgagggcacccagaccgccaagctgcaagtgaccaagggcggccccctgcccttcgcctgggacatcctgtccccccagttcttctacggctccaaggcgtacatcaagcaccccgccgacatccccgactacctcaagcagtccttccccgagggcttcaagtgggagcgcgtgatgaacttcgaggacggcggcgtggtgaccgtgacccaggactcctccctgcaggacggcaccctcatctaccacgtgaagttcatcggcgtgaacttcccctccgacggccccgtaatgcagaagaaaactctgggctgggagccctccactgagcgcaactacccccgcgacggcgtgctgaagggcgagaaccacatggcgctgaagctgaagggcggcggccactacctgtgtgagttcaagtccatctacatggccaagaagcccgtgaagctgcccggctaccactacgtggactacaagctcgacatcacctcccacaacgaggactacaccgtggtggagcagtacgagcgcgccgaggcccgccaccacctgttccagtgataataggggtctctgagttggggaccagaatactttattctcaaaaaaaaaaaaaaaaaaaaaaaaaaaaaaaaaaaaaaaaaaaaaaaaaaaaaaaaaaaaaaaaaaaaaaaaaaaaaaaaaaaaaaaaaaaaaaaaaaaaagagacg

SEQ ID NO: 277 - DNA, 907 bp, synthetic construct
  source 1..907: mol_type = other DNA
taatacgactcactataagggagaataaactagtattcttctggtccccacagactcagagagaacccgccaccatggatagcactgagaacgtcatcaagcccttcatgcgcttcaaggtgcacatggagggctccgtgaacggccacgagttcgagatcgagggcgtgggcgagggcaagccctacgagggcacccagaccgccaagctgcaagtgaccaagggcggccccctgcccttcgcctgggacatcctgtccccccagttcttctacggctccaaggcgtacatcaagcaccccgccgacatccccgactacctcaagcagtccttccccgagggcttcaagtgggagcgcgtgatgaacttcgaggacggcggcgtggtgaccgtgacccaggactcctccctgcaggacggcaccctcatctaccacgtgaagttcatcggcgtgaacttcccctccgacggccccgtaatgcagaagaaaactctgggctgggagccctccactgagcgcaactacccccgcgacggcgtgctgaagggcgagaaccacatggcgctgaagctgaagggcggcggccactacctgtgtgagttcaagtccatctacatggccaagaagcccgtgaagctgcccggctaccactacgtggactacaagctcgacatcacctcccacaacgaggactacaccgtggtggagcagtacgagcgcgccgaggcccgccaccacctgttccagtgataataggggttctctctgaggtggggaccagaagactagtttattctcaaaaaaaaaaaaaaaaaaaaaaaaaaaaaaaaaaaaaaaaaaaaaaaaaaaaaaaaaaaaaaaaaaaaaaaaaaaaaaaaaaaaaaaaaaaaaaaaaaaaagagacg

SEQ ID NO: 278 - DNA, 904 bp, synthetic construct
  source 1..904: mol_type = other DNA
taatacgactcactataagggagaataaactagtattcttctggtccccacagactcagagagaacccgccaccatggatagcactgagaacgtcatcaagcccttcatgcgcttcaaggtgcacatggagggctccgtgaacggccacgagttcgagatcgagggcgtgggcgagggcaagccctacgagggcacccagaccgccaagctgcaagtgaccaagggcggccccctgcccttcgcctgggacatcctgtccccccagttcttctacggctccaaggcgtacatcaagcaccccgccgacatccccgactacctcaagcagtccttccccgagggcttcaagtgggagcgcgtgatgaacttcgaggacggcggcgtggtgaccgtgacccaggactcctccctgcaggacggcaccctcatctaccacgtgaagttcatcggcgtgaacttcccctccgacggccccgtaatgcagaagaaaactctgggctgggagccctccactgagcgcaactacccccgcgacggcgtgctgaagggcgagaaccacatggcgctgaagctgaagggcggcggccactacctgtgtgagttcaagtccatctacatggccaagaagcccgtgaagctgcccggctaccactacgtggactacaagctcgacatcacctcccacaacgaggactacaccgtggtggagcagtacgagcgcgccgaggcccgccaccacctgttccagtgataataggtctctctgagtctgggaccagaagaatagtttattctcaaaaaaaaaaaaaaaaaaaaaaaaaaaaaaaaaaaaaaaaaaaaaaaaaaaaaaaaaaaaaaaaaaaaaaaaaaaaaaaaaaaaaaaaaaaaaaaaaaaaagagacg

SEQ ID NO: 279 - DNA, 4725 bp, synthetic construct
  source 1..4725: mol_type = other DNA
taatacgactcactataagggagaataaactagtattcttctggtccccacagactcagagagaacccgccaccatgttcgtgttcctggtgctgctgcctctggtgtccagccagtgtgtgaacctgaccaccagaacacagctgcctccagcctacaccaacagctttaccagaggcgtgtactaccccgacaaggtgttcagatccagcgtgctgcactctacccaggacctgttcctgcctttcttcagcaacgtgacctggttccacgccatccacgtgtccggcaccaatggcaccaagagattcgacaaccccgtgctgcccttcaacgacggggtgtactttgccagcaccgagaagtccaacatcatcagaggctggatcttcggcaccacactggacagcaagacccagagcctgctgatcgtgaacaacgccaccaacgtggtcatcaaagtgtgcgagttccagttctgcaacgaccccttcctgggcgtctactaccacaagaacaacaagagctggatggaaagcgagttccgggtgtacagcagcgccaacaactgcaccttcgagtacgtgtcccagcctttcctgatggacctggaaggcaagcagggcaacttcaagaacctgcgcgagttcgtgtttaagaacatcgacggctacttcaagatctacagcaagcacacccctatcaacctcgtgcgggatctgcctcagggcttctctgctctggaacccctggtggatctgcccatcggcatcaacatcacccggtttcagacactgctggccctgcacagaagctacctgacacctggcgatagcagcagcggatggacagctggtgccgccgcttactatgtgggctacctgcagcctagaaccttcctgctgaagtacaacgagaacggcaccatcaccgacgccgtggattgtgctctggatcctctgagcgagacaaagtgcaccctgaagtccttcaccgtggaaaagggcatctaccagaccagcaacttccgggtgcagcccaccgaatccatcgtgcggttccccaatatcaccaatctgtgccccttcggcgaggtgttcaatgccaccagattcgcctctgtgtacgcctggaaccggaagcggatcagcaattgcgtggccgactactccgtgctgtacaactccgccagcttcagcaccttcaagtgctacggcgtgtcccctaccaagctgaacgacctgtgcttcacaaacgtgtacgccgacagcttcgtgatccggggagatgaagtgcggcagattgcccctggacagacaggcaagatcgccgactacaactacaagctgcccgacgacttcaccggctgtgtgattgcctggaacagcaacaacctggactccaaagtcggcggcaactacaattacctgtaccggctgttccggaagtccaatctgaagcccttcgagcgggacatctccaccgagatctatcaggccggcagcaccccttgtaacggcgtggaaggcttcaactgctacttcccactgcagtcctacggctttcagcccacaaatggcgtgggctatcagccctacagagtggtggtgctgagcttcgaactgctgcatgcccctgccacagtgtgcggccctaagaaaagcaccaatctcgtgaagaacaaatgcgtgaacttcaacttcaacggcctgaccggcaccggcgtgctgacagagagcaacaagaagttcctgccattccagcagtttggccgggatatcgccgataccacagacgccgttagagatccccagacactggaaatcctggacatcaccccttgcagcttcggcggagtgtctgtgatcacccctggcaccaacaccagcaatcaggtggcagtgctgtaccaggacgtgaactgtaccgaagtgcccgtggccattcacgccgatcagctgacacctacatggcgggtgtactccaccggcagcaatgtgtttcagaccagagccggctgtctgatcggagccgagcacgtgaacaatagctacgagtgcgacatccccatcggcgctggaatctgcgccagctaccagacacagacaaacagccctcggagagccagaagcgtggccagccagagcatcattgcctacacaatgtctctgggcgccgagaacagcgtggcctactccaacaactctatcgctatccccaccaacttcaccatcagcgtgaccacagagatcctgcctgtgtccatgaccaagaccagcgtggactgcaccatgtacatctgcggcgattccaccgagtgctccaacctgctgctgcagtacggcagcttctgcacccagctgaatagagccctgacagggatcgccgtggaacaggacaagaacacccaagaggtgttcgcccaagtgaagcagatctacaagacccctcctatcaaggacttcggcggcttcaatttcagccagattctgcccgatcctagcaagcccagcaagcggagcttcatcgaggacctgctgttcaacaaagtgacactggccgacgccggcttcatcaagcagtatggcgattgtctgggcgacattgccgccagggatctgatttgcgcccagaagtttaacggactgacagtgctgcctcctctgctgaccgatgagatgatcgcccagtacacatctgccctgctggccggcacaatcacaagcggctggacatttggagcaggcgccgctctgcagatcccctttgctatgcagatggcctaccggttcaacggcatcggagtgacccagaatgtgctgtacgagaaccagaagctgatcgccaaccagttcaacagcgccatcggcaagatccaggacagcctgagcagcacagcaagcgccctgggaaagctgcaggacgtggtcaaccagaatgcccaggcactgaacaccctggtcaagcagctgtcctccaacttcggcgccatcagctctgtgctgaacgatatcctgagcagactggaccctcctgaggccgaggtgcagatcgacagactgatcacaggcagactgcagagcctccagacatacgtgacccagcagctgatcagagccgccgagattagagcctctgccaatctggccgccaccaagatgtctgagtgtgtgctgggccagagcaagagagtggacttttgcggcaagggctaccacctgatgagcttccctcagtctgcccctcacggcgtggtgtttctgcacgtgacatatgtgcccgctcaagagaagaatttcaccaccgctccagccatctgccacgacggcaaagcccactttcctagagaaggcgtgttcgtgtccaacggcacccattggttcgtgacacagcggaacttctacgagccccagatcatcaccaccgacaacaccttcgtgtctggcaactgcgacgtcgtgatcggcattgtgaacaataccgtgtacgaccctctgcagcccgagctggacagcttcaaagaggaactggacaagtactttaagaaccacacaagccccgacgtggacctgggcgatatcagcggaatcaatgccagcgtcgtgaacatccagaaagagatcgaccggctgaacgaggtggccaagaatctgaacgagagcctgatcgacctgcaagaactggggaagtacgagcagtacatcaagtggccctggtacatctggctgggctttatcgccggactgattgccatcgtgatggtcacaatcatgctgtgttgcatgaccagctgctgtagctgcctgaagggctgttgtagctgtggcagctgctgcaagttcgacgaggacgattctgagcccgtgctgaagggcgtgaaactgcactacacagatagcactgagaacgtcatcaagcccttcatgcgcttcaaggtgcacatggagggctccgtgaacggccacgagttcgagatcgagggcgtgggcgagggcaagccctacgagggcacccagaccgccaagctgcaagtgaccaagggcggccccctgcccttcgcctgggacatcctgtccccccagttcttctacggctccaaggcgtacatcaagcaccccgccgacatccccgactacctcaagcagtccttccccgagggcttcaagtgggagcgcgtgatgaacttcgaggacggcggcgtggtgaccgtgacccaggactcctccctgcaggacggcaccctcatctaccacgtgaagttcatcggcgtgaacttcccctccgacggccccgtaatgcagaagaaaactctgggctgggagccctccactgagcgcaactacccccgcgacggcgtgctgaagggcgagaaccacatggcgctgaagctgaagggcggcggccactacctgtgtgagttcaagtccatctacatggccaagaagcccgtgaagctgcccggctaccactacgtggactacaagctcgacatcacctcccacaacgaggactacaccgtggtggagcagtacgagcgcgccgaggcccgccaccacctgttccagtgataataggggttctcctgagtctgggggaccagagaatactatttattctcaaaaaaaaaaaaaaaaaaaaaaaaaaaaaaaaaaaaaaaaaaaaaaaaaaaaaaaaaaaaaaaaaaaaaaaaaaaaaaaaaaaaaaaaaaaaaaaaaaaaagagacg

SEQ ID NO: 280 - DNA, 4724 bp, synthetic construct
  source 1..4724: mol_type = other DNA
taatacgactcactataagggagaataaactagtattcttctggtccccacagactcagagagaacccgccaccatgttcgtgttcctggtgctgctgcctctggtgtccagccagtgtgtgaacctgaccaccagaacacagctgcctccagcctacaccaacagctttaccagaggcgtgtactaccccgacaaggtgttcagatccagcgtgctgcactctacccaggacctgttcctgcctttcttcagcaacgtgacctggttccacgccatccacgtgtccggcaccaatggcaccaagagattcgacaaccccgtgctgcccttcaacgacggggtgtactttgccagcaccgagaagtccaacatcatcagaggctggatcttcggcaccacactggacagcaagacccagagcctgctgatcgtgaacaacgccaccaacgtggtcatcaaagtgtgcgagttccagttctgcaacgaccccttcctgggcgtctactaccacaagaacaacaagagctggatggaaagcgagttccgggtgtacagcagcgccaacaactgcaccttcgagtacgtgtcccagcctttcctgatggacctggaaggcaagcagggcaacttcaagaacctgcgcgagttcgtgtttaagaacatcgacggctacttcaagatctacagcaagcacacccctatcaacctcgtgcgggatctgcctcagggcttctctgctctggaacccctggtggatctgcccatcggcatcaacatcacccggtttcagacactgctggccctgcacagaagctacctgacacctggcgatagcagcagcggatggacagctggtgccgccgcttactatgtgggctacctgcagcctagaaccttcctgctgaagtacaacgagaacggcaccatcaccgacgccgtggattgtgctctggatcctctgagcgagacaaagtgcaccctgaagtccttcaccgtggaaaagggcatctaccagaccagcaacttccgggtgcagcccaccgaatccatcgtgcggttccccaatatcaccaatctgtgccccttcggcgaggtgttcaatgccaccagattcgcctctgtgtacgcctggaaccggaagcggatcagcaattgcgtggccgactactccgtgctgtacaactccgccagcttcagcaccttcaagtgctacggcgtgtcccctaccaagctgaacgacctgtgcttcacaaacgtgtacgccgacagcttcgtgatccggggagatgaagtgcggcagattgcccctggacagacaggcaagatcgccgactacaactacaagctgcccgacgacttcaccggctgtgtgattgcctggaacagcaacaacctggactccaaagtcggcggcaactacaattacctgtaccggctgttccggaagtccaatctgaagcccttcgagcgggacatctccaccgagatctatcaggccggcagcaccccttgtaacggcgtggaaggcttcaactgctacttcccactgcagtcctacggctttcagcccacaaatggcgtgggctatcagccctacagagtggtggtgctgagcttcgaactgctgcatgcccctgccacagtgtgcggccctaagaaaagcaccaatctcgtgaagaacaaatgcgtgaacttcaacttcaacggcctgaccggcaccggcgtgctgacagagagcaacaagaagttcctgccattccagcagtttggccgggatatcgccgataccacagacgccgttagagatccccagacactggaaatcctggacatcaccccttgcagcttcggcggagtgtctgtgatcacccctggcaccaacaccagcaatcaggtggcagtgctgtaccaggacgtgaactgtaccgaagtgcccgtggccattcacgccgatcagctgacacctacatggcgggtgtactccaccggcagcaatgtgtttcagaccagagccggctgtctgatcggagccgagcacgtgaacaatagctacgagtgcgacatccccatcggcgctggaatctgcgccagctaccagacacagacaaacagccctcggagagccagaagcgtggccagccagagcatcattgcctacacaatgtctctgggcgccgagaacagcgtggcctactccaacaactctatcgctatccccaccaacttcaccatcagcgtgaccacagagatcctgcctgtgtccatgaccaagaccagcgtggactgcaccatgtacatctgcggcgattccaccgagtgctccaacctgctgctgcagtacggcagcttctgcacccagctgaatagagccctgacagggatcgccgtggaacaggacaagaacacccaagaggtgttcgcccaagtgaagcagatctacaagacccctcctatcaaggacttcggcggcttcaatttcagccagattctgcccgatcctagcaagcccagcaagcggagcttcatcgaggacctgctgttcaacaaagtgacactggccgacgccggcttcatcaagcagtatggcgattgtctgggcgacattgccgccagggatctgatttgcgcccagaagtttaacggactgacagtgctgcctcctctgctgaccgatgagatgatcgcccagtacacatctgccctgctggccggcacaatcacaagcggctggacatttggagcaggcgccgctctgcagatcccctttgctatgcagatggcctaccggttcaacggcatcggagtgacccagaatgtgctgtacgagaaccagaagctgatcgccaaccagttcaacagcgccatcggcaagatccaggacagcctgagcagcacagcaagcgccctgggaaagctgcaggacgtggtcaaccagaatgcccaggcactgaacaccctggtcaagcagctgtcctccaacttcggcgccatcagctctgtgctgaacgatatcctgagcagactggaccctcctgaggccgaggtgcagatcgacagactgatcacaggcagactgcagagcctccagacatacgtgacccagcagctgatcagagccgccgagattagagcctctgccaatctggccgccaccaagatgtctgagtgtgtgctgggccagagcaagagagtggacttttgcggcaagggctaccacctgatgagcttccctcagtctgcccctcacggcgtggtgtttctgcacgtgacatatgtgcccgctcaagagaagaatttcaccaccgctccagccatctgccacgacggcaaagcccactttcctagagaaggcgtgttcgtgtccaacggcacccattggttcgtgacacagcggaacttctacgagccccagatcatcaccaccgacaacaccttcgtgtctggcaactgcgacgtcgtgatcggcattgtgaacaataccgtgtacgaccctctgcagcccgagctggacagcttcaaagaggaactggacaagtactttaagaaccacacaagccccgacgtggacctgggcgatatcagcggaatcaatgccagcgtcgtgaacatccagaaagagatcgaccggctgaacgaggtggccaagaatctgaacgagagcctgatcgacctgcaagaactggggaagtacgagcagtacatcaagtggccctggtacatctggctgggctttatcgccggactgattgccatcgtgatggtcacaatcatgctgtgttgcatgaccagctgctgtagctgcctgaagggctgttgtagctgtggcagctgctgcaagttcgacgaggacgattctgagcccgtgctgaagggcgtgaaactgcactacacagatagcactgagaacgtcatcaagcccttcatgcgcttcaaggtgcacatggagggctccgtgaacggccacgagttcgagatcgagggcgtgggcgagggcaagccctacgagggcacccagaccgccaagctgcaagtgaccaagggcggccccctgcccttcgcctgggacatcctgtccccccagttcttctacggctccaaggcgtacatcaagcaccccgccgacatccccgactacctcaagcagtccttccccgagggcttcaagtgggagcgcgtgatgaacttcgaggacggcggcgtggtgaccgtgacccaggactcctccctgcaggacggcaccctcatctaccacgtgaagttcatcggcgtgaacttcccctccgacggccccgtaatgcagaagaaaactctgggctgggagccctccactgagcgcaactacccccgcgacggcgtgctgaagggcgagaaccacatggcgctgaagctgaagggcggcggccactacctgtgtgagttcaagtccatctacatggccaagaagcccgtgaagctgcccggctaccactacgtggactacaagctcgacatcacctcccacaacgaggactacaccgtggtggagcagtacgagcgcgccgaggcccgccaccacctgttccagtgataataggggtctctctggtctgtgggaccagaaaatactagttattctcaaaaaaaaaaaaaaaaaaaaaaaaaaaaaaaaaaaaaaaaaaaaaaaaaaaaaaaaaaaaaaaaaaaaaaaaaaaaaaaaaaaaaaaaaaaaaaaaaaaaagagacg

SEQ ID NO: 281 - DNA, 4723 bp, synthetic construct
  source 1..4723: mol_type = other DNA
taatacgactcactataagggagaataaactagtattcttctggtccccacagactcagagagaacccgccaccatgttcgtgttcctggtgctgctgcctctggtgtccagccagtgtgtgaacctgaccaccagaacacagctgcctccagcctacaccaacagctttaccagaggcgtgtactaccccgacaaggtgttcagatccagcgtgctgcactctacccaggacctgttcctgcctttcttcagcaacgtgacctggttccacgccatccacgtgtccggcaccaatggcaccaagagattcgacaaccccgtgctgcccttcaacgacggggtgtactttgccagcaccgagaagtccaacatcatcagaggctggatcttcggcaccacactggacagcaagacccagagcctgctgatcgtgaacaacgccaccaacgtggtcatcaaagtgtgcgagttccagttctgcaacgaccccttcctgggcgtctactaccacaagaacaacaagagctggatggaaagcgagttccgggtgtacagcagcgccaacaactgcaccttcgagtacgtgtcccagcctttcctgatggacctggaaggcaagcagggcaacttcaagaacctgcgcgagttcgtgtttaagaacatcgacggctacttcaagatctacagcaagcacacccctatcaacctcgtgcgggatctgcctcagggcttctctgctctggaacccctggtggatctgcccatcggcatcaacatcacccggtttcagacactgctggccctgcacagaagctacctgacacctggcgatagcagcagcggatggacagctggtgccgccgcttactatgtgggctacctgcagcctagaaccttcctgctgaagtacaacgagaacggcaccatcaccgacgccgtggattgtgctctggatcctctgagcgagacaaagtgcaccctgaagtccttcaccgtggaaaagggcatctaccagaccagcaacttccgggtgcagcccaccgaatccatcgtgcggttccccaatatcaccaatctgtgccccttcggcgaggtgttcaatgccaccagattcgcctctgtgtacgcctggaaccggaagcggatcagcaattgcgtggccgactactccgtgctgtacaactccgccagcttcagcaccttcaagtgctacggcgtgtcccctaccaagctgaacgacctgtgcttcacaaacgtgtacgccgacagcttcgtgatccggggagatgaagtgcggcagattgcccctggacagacaggcaagatcgccgactacaactacaagctgcccgacgacttcaccggctgtgtgattgcctggaacagcaacaacctggactccaaagtcggcggcaactacaattacctgtaccggctgttccggaagtccaatctgaagcccttcgagcgggacatctccaccgagatctatcaggccggcagcaccccttgtaacggcgtggaaggcttcaactgctacttcccactgcagtcctacggctttcagcccacaaatggcgtgggctatcagccctacagagtggtggtgctgagcttcgaactgctgcatgcccctgccacagtgtgcggccctaagaaaagcaccaatctcgtgaagaacaaatgcgtgaacttcaacttcaacggcctgaccggcaccggcgtgctgacagagagcaacaagaagttcctgccattccagcagtttggccgggatatcgccgataccacagacgccgttagagatccccagacactggaaatcctggacatcaccccttgcagcttcggcggagtgtctgtgatcacccctggcaccaacaccagcaatcaggtggcagtgctgtaccaggacgtgaactgtaccgaagtgcccgtggccattcacgccgatcagctgacacctacatggcgggtgtactccaccggcagcaatgtgtttcagaccagagccggctgtctgatcggagccgagcacgtgaacaatagctacgagtgcgacatccccatcggcgctggaatctgcgccagctaccagacacagacaaacagccctcggagagccagaagcgtggccagccagagcatcattgcctacacaatgtctctgggcgccgagaacagcgtggcctactccaacaactctatcgctatccccaccaacttcaccatcagcgtgaccacagagatcctgcctgtgtccatgaccaagaccagcgtggactgcaccatgtacatctgcggcgattccaccgagtgctccaacctgctgctgcagtacggcagcttctgcacccagctgaatagagccctgacagggatcgccgtggaacaggacaagaacacccaagaggtgttcgcccaagtgaagcagatctacaagacccctcctatcaaggacttcggcggcttcaatttcagccagattctgcccgatcctagcaagcccagcaagcggagcttcatcgaggacctgctgttcaacaaagtgacactggccgacgccggcttcatcaagcagtatggcgattgtctgggcgacattgccgccagggatctgatttgcgcccagaagtttaacggactgacagtgctgcctcctctgctgaccgatgagatgatcgcccagtacacatctgccctgctggccggcacaatcacaagcggctggacatttggagcaggcgccgctctgcagatcccctttgctatgcagatggcctaccggttcaacggcatcggagtgacccagaatgtgctgtacgagaaccagaagctgatcgccaaccagttcaacagcgccatcggcaagatccaggacagcctgagcagcacagcaagcgccctgggaaagctgcaggacgtggtcaaccagaatgcccaggcactgaacaccctggtcaagcagctgtcctccaacttcggcgccatcagctctgtgctgaacgatatcctgagcagactggaccctcctgaggccgaggtgcagatcgacagactgatcacaggcagactgcagagcctccagacatacgtgacccagcagctgatcagagccgccgagattagagcctctgccaatctggccgccaccaagatgtctgagtgtgtgctgggccagagcaagagagtggacttttgcggcaagggctaccacctgatgagcttccctcagtctgcccctcacggcgtggtgtttctgcacgtgacatatgtgcccgctcaagagaagaatttcaccaccgctccagccatctgccacgacggcaaagcccactttcctagagaaggcgtgttcgtgtccaacggcacccattggttcgtgacacagcggaacttctacgagccccagatcatcaccaccgacaacaccttcgtgtctggcaactgcgacgtcgtgatcggcattgtgaacaataccgtgtacgaccctctgcagcccgagctggacagcttcaaagaggaactggacaagtactttaagaaccacacaagccccgacgtggacctgggcgatatcagcggaatcaatgccagcgtcgtgaacatccagaaagagatcgaccggctgaacgaggtggccaagaatctgaacgagagcctgatcgacctgcaagaactggggaagtacgagcagtacatcaagtggccctggtacatctggctgggctttatcgccggactgattgccatcgtgatggtcacaatcatgctgtgttgcatgaccagctgctgtagctgcctgaagggctgttgtagctgtggcagctgctgcaagttcgacgaggacgattctgagcccgtgctgaagggcgtgaaactgcactacacagatagcactgagaacgtcatcaagcccttcatgcgcttcaaggtgcacatggagggctccgtgaacggccacgagttcgagatcgagggcgtgggcgagggcaagccctacgagggcacccagaccgccaagctgcaagtgaccaagggcggccccctgcccttcgcctgggacatcctgtccccccagttcttctacggctccaaggcgtacatcaagcaccccgccgacatccccgactacctcaagcagtccttccccgagggcttcaagtgggagcgcgtgatgaacttcgaggacggcggcgtggtgaccgtgacccaggactcctccctgcaggacggcaccctcatctaccacgtgaagttcatcggcgtgaacttcccctccgacggccccgtaatgcagaagaaaactctgggctgggagccctccactgagcgcaactacccccgcgacggcgtgctgaagggcgagaaccacatggcgctgaagctgaagggcggcggccactacctgtgtgagttcaagtccatctacatggccaagaagcccgtgaagctgcccggctaccactacgtggactacaagctcgacatcacctcccacaacgaggactacaccgtggtggagcagtacgagcgcgccgaggcccgccaccacctgttccagtgataatagggttctcttgagtcttggggacagaagaaactagttattctcaaaaaaaaaaaaaaaaaaaaaaaaaaaaaaaaaaaaaaaaaaaaaaaaaaaaaaaaaaaaaaaaaaaaaaaaaaaaaaaaaaaaaaaaaaaaaaaaaaaaagagacg

SEQ ID NO: 282 - DNA, 4723 bp, synthetic construct
  source 1..4723: mol_type = other DNA
taatacgactcactataagggagaataaactagtattcttctggtccccacagactcagagagaacccgccaccatgttcgtgttcctggtgctgctgcctctggtgtccagccagtgtgtgaacctgaccaccagaacacagctgcctccagcctacaccaacagctttaccagaggcgtgtactaccccgacaaggtgttcagatccagcgtgctgcactctacccaggacctgttcctgcctttcttcagcaacgtgacctggttccacgccatccacgtgtccggcaccaatggcaccaagagattcgacaaccccgtgctgcccttcaacgacggggtgtactttgccagcaccgagaagtccaacatcatcagaggctggatcttcggcaccacactggacagcaagacccagagcctgctgatcgtgaacaacgccaccaacgtggtcatcaaagtgtgcgagttccagttctgcaacgaccccttcctgggcgtctactaccacaagaacaacaagagctggatggaaagcgagttccgggtgtacagcagcgccaacaactgcaccttcgagtacgtgtcccagcctttcctgatggacctggaaggcaagcagggcaacttcaagaacctgcgcgagttcgtgtttaagaacatcgacggctacttcaagatctacagcaagcacacccctatcaacctcgtgcgggatctgcctcagggcttctctgctctggaacccctggtggatctgcccatcggcatcaacatcacccggtttcagacactgctggccctgcacagaagctacctgacacctggcgatagcagcagcggatggacagctggtgccgccgcttactatgtgggctacctgcagcctagaaccttcctgctgaagtacaacgagaacggcaccatcaccgacgccgtggattgtgctctggatcctctgagcgagacaaagtgcaccctgaagtccttcaccgtggaaaagggcatctaccagaccagcaacttccgggtgcagcccaccgaatccatcgtgcggttccccaatatcaccaatctgtgccccttcggcgaggtgttcaatgccaccagattcgcctctgtgtacgcctggaaccggaagcggatcagcaattgcgtggccgactactccgtgctgtacaactccgccagcttcagcaccttcaagtgctacggcgtgtcccctaccaagctgaacgacctgtgcttcacaaacgtgtacgccgacagcttcgtgatccggggagatgaagtgcggcagattgcccctggacagacaggcaagatcgccgactacaactacaagctgcccgacgacttcaccggctgtgtgattgcctggaacagcaacaacctggactccaaagtcggcggcaactacaattacctgtaccggctgttccggaagtccaatctgaagcccttcgagcgggacatctccaccgagatctatcaggccggcagcaccccttgtaacggcgtggaaggcttcaactgctacttcccactgcagtcctacggctttcagcccacaaatggcgtgggctatcagccctacagagtggtggtgctgagcttcgaactgctgcatgcccctgccacagtgtgcggccctaagaaaagcaccaatctcgtgaagaacaaatgcgtgaacttcaacttcaacggcctgaccggcaccggcgtgctgacagagagcaacaagaagttcctgccattccagcagtttggccgggatatcgccgataccacagacgccgttagagatccccagacactggaaatcctggacatcaccccttgcagcttcggcggagtgtctgtgatcacccctggcaccaacaccagcaatcaggtggcagtgctgtaccaggacgtgaactgtaccgaagtgcccgtggccattcacgccgatcagctgacacctacatggcgggtgtactccaccggcagcaatgtgtttcagaccagagccggctgtctgatcggagccgagcacgtgaacaatagctacgagtgcgacatccccatcggcgctggaatctgcgccagctaccagacacagacaaacagccctcggagagccagaagcgtggccagccagagcatcattgcctacacaatgtctctgggcgccgagaacagcgtggcctactccaacaactctatcgctatccccaccaacttcaccatcagcgtgaccacagagatcctgcctgtgtccatgaccaagaccagcgtggactgcaccatgtacatctgcggcgattccaccgagtgctccaacctgctgctgcagtacggcagcttctgcacccagctgaatagagccctgacagggatcgccgtggaacaggacaagaacacccaagaggtgttcgcccaagtgaagcagatctacaagacccctcctatcaaggacttcggcggcttcaatttcagccagattctgcccgatcctagcaagcccagcaagcggagcttcatcgaggacctgctgttcaacaaagtgacactggccgacgccggcttcatcaagcagtatggcgattgtctgggcgacattgccgccagggatctgatttgcgcccagaagtttaacggactgacagtgctgcctcctctgctgaccgatgagatgatcgcccagtacacatctgccctgctggccggcacaatcacaagcggctggacatttggagcaggcgccgctctgcagatcccctttgctatgcagatggcctaccggttcaacggcatcggagtgacccagaatgtgctgtacgagaaccagaagctgatcgccaaccagttcaacagcgccatcggcaagatccaggacagcctgagcagcacagcaagcgccctgggaaagctgcaggacgtggtcaaccagaatgcccaggcactgaacaccctggtcaagcagctgtcctccaacttcggcgccatcagctctgtgctgaacgatatcctgagcagactggaccctcctgaggccgaggtgcagatcgacagactgatcacaggcagactgcagagcctccagacatacgtgacccagcagctgatcagagccgccgagattagagcctctgccaatctggccgccaccaagatgtctgagtgtgtgctgggccagagcaagagagtggacttttgcggcaagggctaccacctgatgagcttccctcagtctgcccctcacggcgtggtgtttctgcacgtgacatatgtgcccgctcaagagaagaatttcaccaccgctccagccatctgccacgacggcaaagcccactttcctagagaaggcgtgttcgtgtccaacggcacccattggttcgtgacacagcggaacttctacgagccccagatcatcaccaccgacaacaccttcgtgtctggcaactgcgacgtcgtgatcggcattgtgaacaataccgtgtacgaccctctgcagcccgagctggacagcttcaaagaggaactggacaagtactttaagaaccacacaagccccgacgtggacctgggcgatatcagcggaatcaatgccagcgtcgtgaacatccagaaagagatcgaccggctgaacgaggtggccaagaatctgaacgagagcctgatcgacctgcaagaactggggaagtacgagcagtacatcaagtggccctggtacatctggctgggctttatcgccggactgattgccatcgtgatggtcacaatcatgctgtgttgcatgaccagctgctgtagctgcctgaagggctgttgtagctgtggcagctgctgcaagttcgacgaggacgattctgagcccgtgctgaagggcgtgaaactgcactacacagatagcactgagaacgtcatcaagcccttcatgcgcttcaaggtgcacatggagggctccgtgaacggccacgagttcgagatcgagggcgtgggcgagggcaagccctacgagggcacccagaccgccaagctgcaagtgaccaagggcggccccctgcccttcgcctgggacatcctgtccccccagttcttctacggctccaaggcgtacatcaagcaccccgccgacatccccgactacctcaagcagtccttccccgagggcttcaagtgggagcgcgtgatgaacttcgaggacggcggcgtggtgaccgtgacccaggactcctccctgcaggacggcaccctcatctaccacgtgaagttcatcggcgtgaacttcccctccgacggccccgtaatgcagaagaaaactctgggctgggagccctccactgagcgcaactacccccgcgacggcgtgctgaagggcgagaaccacatggcgctgaagctgaagggcggcggccactacctgtgtgagttcaagtccatctacatggccaagaagcccgtgaagctgcccggctaccactacgtggactacaagctcgacatcacctcccacaacgaggactacaccgtggtggagcagtacgagcgcgccgaggcccgccaccacctgttccagtgataataggggttcctctgatctgtgggaccaaagaatctagttattctcaaaaaaaaaaaaaaaaaaaaaaaaaaaaaaaaaaaaaaaaaaaaaaaaaaaaaaaaaaaaaaaaaaaaaaaaaaaaaaaaaaaaaaaaaaaaaaaaaaaaagagacg

SEQ ID NO: 283 - DNA, 4721 bp, synthetic construct
  source 1..4721: mol_type = other DNA
taatacgactcactataagggagaataaactagtattcttctggtccccacagactcagagagaacccgccaccatgttcgtgttcctggtgctgctgcctctggtgtccagccagtgtgtgaacctgaccaccagaacacagctgcctccagcctacaccaacagctttaccagaggcgtgtactaccccgacaaggtgttcagatccagcgtgctgcactctacccaggacctgttcctgcctttcttcagcaacgtgacctggttccacgccatccacgtgtccggcaccaatggcaccaagagattcgacaaccccgtgctgcccttcaacgacggggtgtactttgccagcaccgagaagtccaacatcatcagaggctggatcttcggcaccacactggacagcaagacccagagcctgctgatcgtgaacaacgccaccaacgtggtcatcaaagtgtgcgagttccagttctgcaacgaccccttcctgggcgtctactaccacaagaacaacaagagctggatggaaagcgagttccgggtgtacagcagcgccaacaactgcaccttcgagtacgtgtcccagcctttcctgatggacctggaaggcaagcagggcaacttcaagaacctgcgcgagttcgtgtttaagaacatcgacggctacttcaagatctacagcaagcacacccctatcaacctcgtgcgggatctgcctcagggcttctctgctctggaacccctggtggatctgcccatcggcatcaacatcacccggtttcagacactgctggccctgcacagaagctacctgacacctggcgatagcagcagcggatggacagctggtgccgccgcttactatgtgggctacctgcagcctagaaccttcctgctgaagtacaacgagaacggcaccatcaccgacgccgtggattgtgctctggatcctctgagcgagacaaagtgcaccctgaagtccttcaccgtggaaaagggcatctaccagaccagcaacttccgggtgcagcccaccgaatccatcgtgcggttccccaatatcaccaatctgtgccccttcggcgaggtgttcaatgccaccagattcgcctctgtgtacgcctggaaccggaagcggatcagcaattgcgtggccgactactccgtgctgtacaactccgccagcttcagcaccttcaagtgctacggcgtgtcccctaccaagctgaacgacctgtgcttcacaaacgtgtacgccgacagcttcgtgatccggggagatgaagtgcggcagattgcccctggacagacaggcaagatcgccgactacaactacaagctgcccgacgacttcaccggctgtgtgattgcctggaacagcaacaacctggactccaaagtcggcggcaactacaattacctgtaccggctgttccggaagtccaatctgaagcccttcgagcgggacatctccaccgagatctatcaggccggcagcaccccttgtaacggcgtggaaggcttcaactgctacttcccactgcagtcctacggctttcagcccacaaatggcgtgggctatcagccctacagagtggtggtgctgagcttcgaactgctgcatgcccctgccacagtgtgcggccctaagaaaagcaccaatctcgtgaagaacaaatgcgtgaacttcaacttcaacggcctgaccggcaccggcgtgctgacagagagcaacaagaagttcctgccattccagcagtttggccgggatatcgccgataccacagacgccgttagagatccccagacactggaaatcctggacatcaccccttgcagcttcggcggagtgtctgtgatcacccctggcaccaacaccagcaatcaggtggcagtgctgtaccaggacgtgaactgtaccgaagtgcccgtggccattcacgccgatcagctgacacctacatggcgggtgtactccaccggcagcaatgtgtttcagaccagagccggctgtctgatcggagccgagcacgtgaacaatagctacgagtgcgacatccccatcggcgctggaatctgcgccagctaccagacacagacaaacagccctcggagagccagaagcgtggccagccagagcatcattgcctacacaatgtctctgggcgccgagaacagcgtggcctactccaacaactctatcgctatccccaccaacttcaccatcagcgtgaccacagagatcctgcctgtgtccatgaccaagaccagcgtggactgcaccatgtacatctgcggcgattccaccgagtgctccaacctgctgctgcagtacggcagcttctgcacccagctgaatagagccctgacagggatcgccgtggaacaggacaagaacacccaagaggtgttcgcccaagtgaagcagatctacaagacccctcctatcaaggacttcggcggcttcaatttcagccagattctgcccgatcctagcaagcccagcaagcggagcttcatcgaggacctgctgttcaacaaagtgacactggccgacgccggcttcatcaagcagtatggcgattgtctgggcgacattgccgccagggatctgatttgcgcccagaagtttaacggactgacagtgctgcctcctctgctgaccgatgagatgatcgcccagtacacatctgccctgctggccggcacaatcacaagcggctggacatttggagcaggcgccgctctgcagatcccctttgctatgcagatggcctaccggttcaacggcatcggagtgacccagaatgtgctgtacgagaaccagaagctgatcgccaaccagttcaacagcgccatcggcaagatccaggacagcctgagcagcacagcaagcgccctgggaaagctgcaggacgtggtcaaccagaatgcccaggcactgaacaccctggtcaagcagctgtcctccaacttcggcgccatcagctctgtgctgaacgatatcctgagcagactggaccctcctgaggccgaggtgcagatcgacagactgatcacaggcagactgcagagcctccagacatacgtgacccagcagctgatcagagccgccgagattagagcctctgccaatctggccgccaccaagatgtctgagtgtgtgctgggccagagcaagagagtggacttttgcggcaagggctaccacctgatgagcttccctcagtctgcccctcacggcgtggtgtttctgcacgtgacatatgtgcccgctcaagagaagaatttcaccaccgctccagccatctgccacgacggcaaagcccactttcctagagaaggcgtgttcgtgtccaacggcacccattggttcgtgacacagcggaacttctacgagccccagatcatcaccaccgacaacaccttcgtgtctggcaactgcgacgtcgtgatcggcattgtgaacaataccgtgtacgaccctctgcagcccgagctggacagcttcaaagaggaactggacaagtactttaagaaccacacaagccccgacgtggacctgggcgatatcagcggaatcaatgccagcgtcgtgaacatccagaaagagatcgaccggctgaacgaggtggccaagaatctgaacgagagcctgatcgacctgcaagaactggggaagtacgagcagtacatcaagtggccctggtacatctggctgggctttatcgccggactgattgccatcgtgatggtcacaatcatgctgtgttgcatgaccagctgctgtagctgcctgaagggctgttgtagctgtggcagctgctgcaagttcgacgaggacgattctgagcccgtgctgaagggcgtgaaactgcactacacagatagcactgagaacgtcatcaagcccttcatgcgcttcaaggtgcacatggagggctccgtgaacggccacgagttcgagatcgagggcgtgggcgagggcaagccctacgagggcacccagaccgccaagctgcaagtgaccaagggcggccccctgcccttcgcctgggacatcctgtccccccagttcttctacggctccaaggcgtacatcaagcaccccgccgacatccccgactacctcaagcagtccttccccgagggcttcaagtgggagcgcgtgatgaacttcgaggacggcggcgtggtgaccgtgacccaggactcctccctgcaggacggcaccctcatctaccacgtgaagttcatcggcgtgaacttcccctccgacggccccgtaatgcagaagaaaactctgggctgggagccctccactgagcgcaactacccccgcgacggcgtgctgaagggcgagaaccacatggcgctgaagctgaagggcggcggccactacctgtgtgagttcaagtccatctacatggccaagaagcccgtgaagctgcccggctaccactacgtggactacaagctcgacatcacctcccacaacgaggactacaccgtggtggagcagtacgagcgcgccgaggcccgccaccacctgttccagtgataatagggttcttctgatctgtgggacagaagatactgtttatctcaaaaaaaaaaaaaaaaaaaaaaaaaaaaaaaaaaaaaaaaaaaaaaaaaaaaaaaaaaaaaaaaaaaaaaaaaaaaaaaaaaaaaaaaaaaaaaaaaaaaagagacg

SEQ ID NO: 284 - DNA, 4720 bp, synthetic construct
  source 1..4720: mol_type = other DNA
taatacgactcactataagggagaataaactagtattcttctggtccccacagactcagagagaacccgccaccatgttcgtgttcctggtgctgctgcctctggtgtccagccagtgtgtgaacctgaccaccagaacacagctgcctccagcctacaccaacagctttaccagaggcgtgtactaccccgacaaggtgttcagatccagcgtgctgcactctacccaggacctgttcctgcctttcttcagcaacgtgacctggttccacgccatccacgtgtccggcaccaatggcaccaagagattcgacaaccccgtgctgcccttcaacgacggggtgtactttgccagcaccgagaagtccaacatcatcagaggctggatcttcggcaccacactggacagcaagacccagagcctgctgatcgtgaacaacgccaccaacgtggtcatcaaagtgtgcgagttccagttctgcaacgaccccttcctgggcgtctactaccacaagaacaacaagagctggatggaaagcgagttccgggtgtacagcagcgccaacaactgcaccttcgagtacgtgtcccagcctttcctgatggacctggaaggcaagcagggcaacttcaagaacctgcgcgagttcgtgtttaagaacatcgacggctacttcaagatctacagcaagcacacccctatcaacctcgtgcgggatctgcctcagggcttctctgctctggaacccctggtggatctgcccatcggcatcaacatcacccggtttcagacactgctggccctgcacagaagctacctgacacctggcgatagcagcagcggatggacagctggtgccgccgcttactatgtgggctacctgcagcctagaaccttcctgctgaagtacaacgagaacggcaccatcaccgacgccgtggattgtgctctggatcctctgagcgagacaaagtgcaccctgaagtccttcaccgtggaaaagggcatctaccagaccagcaacttccgggtgcagcccaccgaatccatcgtgcggttccccaatatcaccaatctgtgccccttcggcgaggtgttcaatgccaccagattcgcctctgtgtacgcctggaaccggaagcggatcagcaattgcgtggccgactactccgtgctgtacaactccgccagcttcagcaccttcaagtgctacggcgtgtcccctaccaagctgaacgacctgtgcttcacaaacgtgtacgccgacagcttcgtgatccggggagatgaagtgcggcagattgcccctggacagacaggcaagatcgccgactacaactacaagctgcccgacgacttcaccggctgtgtgattgcctggaacagcaacaacctggactccaaagtcggcggcaactacaattacctgtaccggctgttccggaagtccaatctgaagcccttcgagcgggacatctccaccgagatctatcaggccggcagcaccccttgtaacggcgtggaaggcttcaactgctacttcccactgcagtcctacggctttcagcccacaaatggcgtgggctatcagccctacagagtggtggtgctgagcttcgaactgctgcatgcccctgccacagtgtgcggccctaagaaaagcaccaatctcgtgaagaacaaatgcgtgaacttcaacttcaacggcctgaccggcaccggcgtgctgacagagagcaacaagaagttcctgccattccagcagtttggccgggatatcgccgataccacagacgccgttagagatccccagacactggaaatcctggacatcaccccttgcagcttcggcggagtgtctgtgatcacccctggcaccaacaccagcaatcaggtggcagtgctgtaccaggacgtgaactgtaccgaagtgcccgtggccattcacgccgatcagctgacacctacatggcgggtgtactccaccggcagcaatgtgtttcagaccagagccggctgtctgatcggagccgagcacgtgaacaatagctacgagtgcgacatccccatcggcgctggaatctgcgccagctaccagacacagacaaacagccctcggagagccagaagcgtggccagccagagcatcattgcctacacaatgtctctgggcgccgagaacagcgtggcctactccaacaactctatcgctatccccaccaacttcaccatcagcgtgaccacagagatcctgcctgtgtccatgaccaagaccagcgtggactgcaccatgtacatctgcggcgattccaccgagtgctccaacctgctgctgcagtacggcagcttctgcacccagctgaatagagccctgacagggatcgccgtggaacaggacaagaacacccaagaggtgttcgcccaagtgaagcagatctacaagacccctcctatcaaggacttcggcggcttcaatttcagccagattctgcccgatcctagcaagcccagcaagcggagcttcatcgaggacctgctgttcaacaaagtgacactggccgacgccggcttcatcaagcagtatggcgattgtctgggcgacattgccgccagggatctgatttgcgcccagaagtttaacggactgacagtgctgcctcctctgctgaccgatgagatgatcgcccagtacacatctgccctgctggccggcacaatcacaagcggctggacatttggagcaggcgccgctctgcagatcccctttgctatgcagatggcctaccggttcaacggcatcggagtgacccagaatgtgctgtacgagaaccagaagctgatcgccaaccagttcaacagcgccatcggcaagatccaggacagcctgagcagcacagcaagcgccctgggaaagctgcaggacgtggtcaaccagaatgcccaggcactgaacaccctggtcaagcagctgtcctccaacttcggcgccatcagctctgtgctgaacgatatcctgagcagactggaccctcctgaggccgaggtgcagatcgacagactgatcacaggcagactgcagagcctccagacatacgtgacccagcagctgatcagagccgccgagattagagcctctgccaatctggccgccaccaagatgtctgagtgtgtgctgggccagagcaagagagtggacttttgcggcaagggctaccacctgatgagcttccctcagtctgcccctcacggcgtggtgtttctgcacgtgacatatgtgcccgctcaagagaagaatttcaccaccgctccagccatctgccacgacggcaaagcccactttcctagagaaggcgtgttcgtgtccaacggcacccattggttcgtgacacagcggaacttctacgagccccagatcatcaccaccgacaacaccttcgtgtctggcaactgcgacgtcgtgatcggcattgtgaacaataccgtgtacgaccctctgcagcccgagctggacagcttcaaagaggaactggacaagtactttaagaaccacacaagccccgacgtggacctgggcgatatcagcggaatcaatgccagcgtcgtgaacatccagaaagagatcgaccggctgaacgaggtggccaagaatctgaacgagagcctgatcgacctgcaagaactggggaagtacgagcagtacatcaagtggccctggtacatctggctgggctttatcgccggactgattgccatcgtgatggtcacaatcatgctgtgttgcatgaccagctgctgtagctgcctgaagggctgttgtagctgtggcagctgctgcaagttcgacgaggacgattctgagcccgtgctgaagggcgtgaaactgcactacacagatagcactgagaacgtcatcaagcccttcatgcgcttcaaggtgcacatggagggctccgtgaacggccacgagttcgagatcgagggcgtgggcgagggcaagccctacgagggcacccagaccgccaagctgcaagtgaccaagggcggccccctgcccttcgcctgggacatcctgtccccccagttcttctacggctccaaggcgtacatcaagcaccccgccgacatccccgactacctcaagcagtccttccccgagggcttcaagtgggagcgcgtgatgaacttcgaggacggcggcgtggtgaccgtgacccaggactcctccctgcaggacggcaccctcatctaccacgtgaagttcatcggcgtgaacttcccctccgacggccccgtaatgcagaagaaaactctgggctgggagccctccactgagcgcaactacccccgcgacggcgtgctgaagggcgagaaccacatggcgctgaagctgaagggcggcggccactacctgtgtgagttcaagtccatctacatggccaagaagcccgtgaagctgcccggctaccactacgtggactacaagctcgacatcacctcccacaacgaggactacaccgtggtggagcagtacgagcgcgccgaggcccgccaccacctgttccagtgataataggggtctcctgatctgggggccagagaaactatttatctcaaaaaaaaaaaaaaaaaaaaaaaaaaaaaaaaaaaaaaaaaaaaaaaaaaaaaaaaaaaaaaaaaaaaaaaaaaaaaaaaaaaaaaaaaaaaaaaaaaaaagagacg

SEQ ID NO: 285 - DNA, 4717 bp, synthetic construct
  source 1..4717: mol_type = other DNA
taatacgactcactataagggagaataaactagtattcttctggtccccacagactcagagagaacccgccaccatgttcgtgttcctggtgctgctgcctctggtgtccagccagtgtgtgaacctgaccaccagaacacagctgcctccagcctacaccaacagctttaccagaggcgtgtactaccccgacaaggtgttcagatccagcgtgctgcactctacccaggacctgttcctgcctttcttcagcaacgtgacctggttccacgccatccacgtgtccggcaccaatggcaccaagagattcgacaaccccgtgctgcccttcaacgacggggtgtactttgccagcaccgagaagtccaacatcatcagaggctggatcttcggcaccacactggacagcaagacccagagcctgctgatcgtgaacaacgccaccaacgtggtcatcaaagtgtgcgagttccagttctgcaacgaccccttcctgggcgtctactaccacaagaacaacaagagctggatggaaagcgagttccgggtgtacagcagcgccaacaactgcaccttcgagtacgtgtcccagcctttcctgatggacctggaaggcaagcagggcaacttcaagaacctgcgcgagttcgtgtttaagaacatcgacggctacttcaagatctacagcaagcacacccctatcaacctcgtgcgggatctgcctcagggcttctctgctctggaacccctggtggatctgcccatcggcatcaacatcacccggtttcagacactgctggccctgcacagaagctacctgacacctggcgatagcagcagcggatggacagctggtgccgccgcttactatgtgggctacctgcagcctagaaccttcctgctgaagtacaacgagaacggcaccatcaccgacgccgtggattgtgctctggatcctctgagcgagacaaagtgcaccctgaagtccttcaccgtggaaaagggcatctaccagaccagcaacttccgggtgcagcccaccgaatccatcgtgcggttccccaatatcaccaatctgtgccccttcggcgaggtgttcaatgccaccagattcgcctctgtgtacgcctggaaccggaagcggatcagcaattgcgtggccgactactccgtgctgtacaactccgccagcttcagcaccttcaagtgctacggcgtgtcccctaccaagctgaacgacctgtgcttcacaaacgtgtacgccgacagcttcgtgatccggggagatgaagtgcggcagattgcccctggacagacaggcaagatcgccgactacaactacaagctgcccgacgacttcaccggctgtgtgattgcctggaacagcaacaacctggactccaaagtcggcggcaactacaattacctgtaccggctgttccggaagtccaatctgaagcccttcgagcgggacatctccaccgagatctatcaggccggcagcaccccttgtaacggcgtggaaggcttcaactgctacttcccactgcagtcctacggctttcagcccacaaatggcgtgggctatcagccctacagagtggtggtgctgagcttcgaactgctgcatgcccctgccacagtgtgcggccctaagaaaagcaccaatctcgtgaagaacaaatgcgtgaacttcaacttcaacggcctgaccggcaccggcgtgctgacagagagcaacaagaagttcctgccattccagcagtttggccgggatatcgccgataccacagacgccgttagagatccccagacactggaaatcctggacatcaccccttgcagcttcggcggagtgtctgtgatcacccctggcaccaacaccagcaatcaggtggcagtgctgtaccaggacgtgaactgtaccgaagtgcccgtggccattcacgccgatcagctgacacctacatggcgggtgtactccaccggcagcaatgtgtttcagaccagagccggctgtctgatcggagccgagcacgtgaacaatagctacgagtgcgacatccccatcggcgctggaatctgcgccagctaccagacacagacaaacagccctcggagagccagaagcgtggccagccagagcatcattgcctacacaatgtctctgggcgccgagaacagcgtggcctactccaacaactctatcgctatccccaccaacttcaccatcagcgtgaccacagagatcctgcctgtgtccatgaccaagaccagcgtggactgcaccatgtacatctgcggcgattccaccgagtgctccaacctgctgctgcagtacggcagcttctgcacccagctgaatagagccctgacagggatcgccgtggaacaggacaagaacacccaagaggtgttcgcccaagtgaagcagatctacaagacccctcctatcaaggacttcggcggcttcaatttcagccagattctgcccgatcctagcaagcccagcaagcggagcttcatcgaggacctgctgttcaacaaagtgacactggccgacgccggcttcatcaagcagtatggcgattgtctgggcgacattgccgccagggatctgatttgcgcccagaagtttaacggactgacagtgctgcctcctctgctgaccgatgagatgatcgcccagtacacatctgccctgctggccggcacaatcacaagcggctggacatttggagcaggcgccgctctgcagatcccctttgctatgcagatggcctaccggttcaacggcatcggagtgacccagaatgtgctgtacgagaaccagaagctgatcgccaaccagttcaacagcgccatcggcaagatccaggacagcctgagcagcacagcaagcgccctgggaaagctgcaggacgtggtcaaccagaatgcccaggcactgaacaccctggtcaagcagctgtcctccaacttcggcgccatcagctctgtgctgaacgatatcctgagcagactggaccctcctgaggccgaggtgcagatcgacagactgatcacaggcagactgcagagcctccagacatacgtgacccagcagctgatcagagccgccgagattagagcctctgccaatctggccgccaccaagatgtctgagtgtgtgctgggccagagcaagagagtggacttttgcggcaagggctaccacctgatgagcttccctcagtctgcccctcacggcgtggtgtttctgcacgtgacatatgtgcccgctcaagagaagaatttcaccaccgctccagccatctgccacgacggcaaagcccactttcctagagaaggcgtgttcgtgtccaacggcacccattggttcgtgacacagcggaacttctacgagccccagatcatcaccaccgacaacaccttcgtgtctggcaactgcgacgtcgtgatcggcattgtgaacaataccgtgtacgaccctctgcagcccgagctggacagcttcaaagaggaactggacaagtactttaagaaccacacaagccccgacgtggacctgggcgatatcagcggaatcaatgccagcgtcgtgaacatccagaaagagatcgaccggctgaacgaggtggccaagaatctgaacgagagcctgatcgacctgcaagaactggggaagtacgagcagtacatcaagtggccctggtacatctggctgggctttatcgccggactgattgccatcgtgatggtcacaatcatgctgtgttgcatgaccagctgctgtagctgcctgaagggctgttgtagctgtggcagctgctgcaagttcgacgaggacgattctgagcccgtgctgaagggcgtgaaactgcactacacagatagcactgagaacgtcatcaagcccttcatgcgcttcaaggtgcacatggagggctccgtgaacggccacgagttcgagatcgagggcgtgggcgagggcaagccctacgagggcacccagaccgccaagctgcaagtgaccaagggcggccccctgcccttcgcctgggacatcctgtccccccagttcttctacggctccaaggcgtacatcaagcaccccgccgacatccccgactacctcaagcagtccttccccgagggcttcaagtgggagcgcgtgatgaacttcgaggacggcggcgtggtgaccgtgacccaggactcctccctgcaggacggcaccctcatctaccacgtgaagttcatcggcgtgaacttcccctccgacggccccgtaatgcagaagaaaactctgggctgggagccctccactgagcgcaactacccccgcgacggcgtgctgaagggcgagaaccacatggcgctgaagctgaagggcggcggccactacctgtgtgagttcaagtccatctacatggccaagaagcccgtgaagctgcccggctaccactacgtggactacaagctcgacatcacctcccacaacgaggactacaccgtggtggagcagtacgagcgcgccgaggcccgccaccacctgttccagtgataatagggtttcttgatcttgggacagagaaactgttatttcaaaaaaaaaaaaaaaaaaaaaaaaaaaaaaaaaaaaaaaaaaaaaaaaaaaaaaaaaaaaaaaaaaaaaaaaaaaaaaaaaaaaaaaaaaaaaaaaaaaaagagacg

SEQ ID NO: 286 - DNA, 4723 bp, synthetic construct
  source 1..4723: mol_type = other DNA
taatacgactcactataagggagaataaactagtattcttctggtccccacagactcagagagaacccgccaccatgttcgtgttcctggtgctgctgcctctggtgtccagccagtgtgtgaacctgaccaccagaacacagctgcctccagcctacaccaacagctttaccagaggcgtgtactaccccgacaaggtgttcagatccagcgtgctgcactctacccaggacctgttcctgcctttcttcagcaacgtgacctggttccacgccatccacgtgtccggcaccaatggcaccaagagattcgacaaccccgtgctgcccttcaacgacggggtgtactttgccagcaccgagaagtccaacatcatcagaggctggatcttcggcaccacactggacagcaagacccagagcctgctgatcgtgaacaacgccaccaacgtggtcatcaaagtgtgcgagttccagttctgcaacgaccccttcctgggcgtctactaccacaagaacaacaagagctggatggaaagcgagttccgggtgtacagcagcgccaacaactgcaccttcgagtacgtgtcccagcctttcctgatggacctggaaggcaagcagggcaacttcaagaacctgcgcgagttcgtgtttaagaacatcgacggctacttcaagatctacagcaagcacacccctatcaacctcgtgcgggatctgcctcagggcttctctgctctggaacccctggtggatctgcccatcggcatcaacatcacccggtttcagacactgctggccctgcacagaagctacctgacacctggcgatagcagcagcggatggacagctggtgccgccgcttactatgtgggctacctgcagcctagaaccttcctgctgaagtacaacgagaacggcaccatcaccgacgccgtggattgtgctctggatcctctgagcgagacaaagtgcaccctgaagtccttcaccgtggaaaagggcatctaccagaccagcaacttccgggtgcagcccaccgaatccatcgtgcggttccccaatatcaccaatctgtgccccttcggcgaggtgttcaatgccaccagattcgcctctgtgtacgcctggaaccggaagcggatcagcaattgcgtggccgactactccgtgctgtacaactccgccagcttcagcaccttcaagtgctacggcgtgtcccctaccaagctgaacgacctgtgcttcacaaacgtgtacgccgacagcttcgtgatccggggagatgaagtgcggcagattgcccctggacagacaggcaagatcgccgactacaactacaagctgcccgacgacttcaccggctgtgtgattgcctggaacagcaacaacctggactccaaagtcggcggcaactacaattacctgtaccggctgttccggaagtccaatctgaagcccttcgagcgggacatctccaccgagatctatcaggccggcagcaccccttgtaacggcgtggaaggcttcaactgctacttcccactgcagtcctacggctttcagcccacaaatggcgtgggctatcagccctacagagtggtggtgctgagcttcgaactgctgcatgcccctgccacagtgtgcggccctaagaaaagcaccaatctcgtgaagaacaaatgcgtgaacttcaacttcaacggcctgaccggcaccggcgtgctgacagagagcaacaagaagttcctgccattccagcagtttggccgggatatcgccgataccacagacgccgttagagatccccagacactggaaatcctggacatcaccccttgcagcttcggcggagtgtctgtgatcacccctggcaccaacaccagcaatcaggtggcagtgctgtaccaggacgtgaactgtaccgaagtgcccgtggccattcacgccgatcagctgacacctacatggcgggtgtactccaccggcagcaatgtgtttcagaccagagccggctgtctgatcggagccgagcacgtgaacaatagctacgagtgcgacatccccatcggcgctggaatctgcgccagctaccagacacagacaaacagccctcggagagccagaagcgtggccagccagagcatcattgcctacacaatgtctctgggcgccgagaacagcgtggcctactccaacaactctatcgctatccccaccaacttcaccatcagcgtgaccacagagatcctgcctgtgtccatgaccaagaccagcgtggactgcaccatgtacatctgcggcgattccaccgagtgctccaacctgctgctgcagtacggcagcttctgcacccagctgaatagagccctgacagggatcgccgtggaacaggacaagaacacccaagaggtgttcgcccaagtgaagcagatctacaagacccctcctatcaaggacttcggcggcttcaatttcagccagattctgcccgatcctagcaagcccagcaagcggagcttcatcgaggacctgctgttcaacaaagtgacactggccgacgccggcttcatcaagcagtatggcgattgtctgggcgacattgccgccagggatctgatttgcgcccagaagtttaacggactgacagtgctgcctcctctgctgaccgatgagatgatcgcccagtacacatctgccctgctggccggcacaatcacaagcggctggacatttggagcaggcgccgctctgcagatcccctttgctatgcagatggcctaccggttcaacggcatcggagtgacccagaatgtgctgtacgagaaccagaagctgatcgccaaccagttcaacagcgccatcggcaagatccaggacagcctgagcagcacagcaagcgccctgggaaagctgcaggacgtggtcaaccagaatgcccaggcactgaacaccctggtcaagcagctgtcctccaacttcggcgccatcagctctgtgctgaacgatatcctgagcagactggaccctcctgaggccgaggtgcagatcgacagactgatcacaggcagactgcagagcctccagacatacgtgacccagcagctgatcagagccgccgagattagagcctctgccaatctggccgccaccaagatgtctgagtgtgtgctgggccagagcaagagagtggacttttgcggcaagggctaccacctgatgagcttccctcagtctgcccctcacggcgtggtgtttctgcacgtgacatatgtgcccgctcaagagaagaatttcaccaccgctccagccatctgccacgacggcaaagcccactttcctagagaaggcgtgttcgtgtccaacggcacccattggttcgtgacacagcggaacttctacgagccccagatcatcaccaccgacaacaccttcgtgtctggcaactgcgacgtcgtgatcggcattgtgaacaataccgtgtacgaccctctgcagcccgagctggacagcttcaaagaggaactggacaagtactttaagaaccacacaagccccgacgtggacctgggcgatatcagcggaatcaatgccagcgtcgtgaacatccagaaagagatcgaccggctgaacgaggtggccaagaatctgaacgagagcctgatcgacctgcaagaactggggaagtacgagcagtacatcaagtggccctggtacatctggctgggctttatcgccggactgattgccatcgtgatggtcacaatcatgctgtgttgcatgaccagctgctgtagctgcctgaagggctgttgtagctgtggcagctgctgcaagttcgacgaggacgattctgagcccgtgctgaagggcgtgaaactgcactacacagatagcactgagaacgtcatcaagcccttcatgcgcttcaaggtgcacatggagggctccgtgaacggccacgagttcgagatcgagggcgtgggcgagggcaagccctacgagggcacccagaccgccaagctgcaagtgaccaagggcggccccctgcccttcgcctgggacatcctgtccccccagttcttctacggctccaaggcgtacatcaagcaccccgccgacatccccgactacctcaagcagtccttccccgagggcttcaagtgggagcgcgtgatgaacttcgaggacggcggcgtggtgaccgtgacccaggactcctccctgcaggacggcaccctcatctaccacgtgaagttcatcggcgtgaacttcccctccgacggccccgtaatgcagaagaaaactctgggctgggagccctccactgagcgcaactacccccgcgacggcgtgctgaagggcgagaaccacatggcgctgaagctgaagggcggcggccactacctgtgtgagttcaagtccatctacatggccaagaagcccgtgaagctgcccggctaccactacgtggactacaagctcgacatcacctcccacaacgaggactacaccgtggtggagcagtacgagcgcgccgaggcccgccaccacctgttccagtgataataggggttctctgagtctgtgggccagaagaataagtttattctcaaaaaaaaaaaaaaaaaaaaaaaaaaaaaaaaaaaaaaaaaaaaaaaaaaaaaaaaaaaaaaaaaaaaaaaaaaaaaaaaaaaaaaaaaaaaaaaaaaaaagagacg

SEQ ID NO: 287 - DNA, 4721 bp, synthetic construct
  source 1..4721: mol_type = other DNA
taatacgactcactataagggagaataaactagtattcttctggtccccacagactcagagagaacccgccaccatgttcgtgttcctggtgctgctgcctctggtgtccagccagtgtgtgaacctgaccaccagaacacagctgcctccagcctacaccaacagctttaccagaggcgtgtactaccccgacaaggtgttcagatccagcgtgctgcactctacccaggacctgttcctgcctttcttcagcaacgtgacctggttccacgccatccacgtgtccggcaccaatggcaccaagagattcgacaaccccgtgctgcccttcaacgacggggtgtactttgccagcaccgagaagtccaacatcatcagaggctggatcttcggcaccacactggacagcaagacccagagcctgctgatcgtgaacaacgccaccaacgtggtcatcaaagtgtgcgagttccagttctgcaacgaccccttcctgggcgtctactaccacaagaacaacaagagctggatggaaagcgagttccgggtgtacagcagcgccaacaactgcaccttcgagtacgtgtcccagcctttcctgatggacctggaaggcaagcagggcaacttcaagaacctgcgcgagttcgtgtttaagaacatcgacggctacttcaagatctacagcaagcacacccctatcaacctcgtgcgggatctgcctcagggcttctctgctctggaacccctggtggatctgcccatcggcatcaacatcacccggtttcagacactgctggccctgcacagaagctacctgacacctggcgatagcagcagcggatggacagctggtgccgccgcttactatgtgggctacctgcagcctagaaccttcctgctgaagtacaacgagaacggcaccatcaccgacgccgtggattgtgctctggatcctctgagcgagacaaagtgcaccctgaagtccttcaccgtggaaaagggcatctaccagaccagcaacttccgggtgcagcccaccgaatccatcgtgcggttccccaatatcaccaatctgtgccccttcggcgaggtgttcaatgccaccagattcgcctctgtgtacgcctggaaccggaagcggatcagcaattgcgtggccgactactccgtgctgtacaactccgccagcttcagcaccttcaagtgctacggcgtgtcccctaccaagctgaacgacctgtgcttcacaaacgtgtacgccgacagcttcgtgatccggggagatgaagtgcggcagattgcccctggacagacaggcaagatcgccgactacaactacaagctgcccgacgacttcaccggctgtgtgattgcctggaacagcaacaacctggactccaaagtcggcggcaactacaattacctgtaccggctgttccggaagtccaatctgaagcccttcgagcgggacatctccaccgagatctatcaggccggcagcaccccttgtaacggcgtggaaggcttcaactgctacttcccactgcagtcctacggctttcagcccacaaatggcgtgggctatcagccctacagagtggtggtgctgagcttcgaactgctgcatgcccctgccacagtgtgcggccctaagaaaagcaccaatctcgtgaagaacaaatgcgtgaacttcaacttcaacggcctgaccggcaccggcgtgctgacagagagcaacaagaagttcctgccattccagcagtttggccgggatatcgccgataccacagacgccgttagagatccccagacactggaaatcctggacatcaccccttgcagcttcggcggagtgtctgtgatcacccctggcaccaacaccagcaatcaggtggcagtgctgtaccaggacgtgaactgtaccgaagtgcccgtggccattcacgccgatcagctgacacctacatggcgggtgtactccaccggcagcaatgtgtttcagaccagagccggctgtctgatcggagccgagcacgtgaacaatagctacgagtgcgacatccccatcggcgctggaatctgcgccagctaccagacacagacaaacagccctcggagagccagaagcgtggccagccagagcatcattgcctacacaatgtctctgggcgccgagaacagcgtggcctactccaacaactctatcgctatccccaccaacttcaccatcagcgtgaccacagagatcctgcctgtgtccatgaccaagaccagcgtggactgcaccatgtacatctgcggcgattccaccgagtgctccaacctgctgctgcagtacggcagcttctgcacccagctgaatagagccctgacagggatcgccgtggaacaggacaagaacacccaagaggtgttcgcccaagtgaagcagatctacaagacccctcctatcaaggacttcggcggcttcaatttcagccagattctgcccgatcctagcaagcccagcaagcggagcttcatcgaggacctgctgttcaacaaagtgacactggccgacgccggcttcatcaagcagtatggcgattgtctgggcgacattgccgccagggatctgatttgcgcccagaagtttaacggactgacagtgctgcctcctctgctgaccgatgagatgatcgcccagtacacatctgccctgctggccggcacaatcacaagcggctggacatttggagcaggcgccgctctgcagatcccctttgctatgcagatggcctaccggttcaacggcatcggagtgacccagaatgtgctgtacgagaaccagaagctgatcgccaaccagttcaacagcgccatcggcaagatccaggacagcctgagcagcacagcaagcgccctgggaaagctgcaggacgtggtcaaccagaatgcccaggcactgaacaccctggtcaagcagctgtcctccaacttcggcgccatcagctctgtgctgaacgatatcctgagcagactggaccctcctgaggccgaggtgcagatcgacagactgatcacaggcagactgcagagcctccagacatacgtgacccagcagctgatcagagccgccgagattagagcctctgccaatctggccgccaccaagatgtctgagtgtgtgctgggccagagcaagagagtggacttttgcggcaagggctaccacctgatgagcttccctcagtctgcccctcacggcgtggtgtttctgcacgtgacatatgtgcccgctcaagagaagaatttcaccaccgctccagccatctgccacgacggcaaagcccactttcctagagaaggcgtgttcgtgtccaacggcacccattggttcgtgacacagcggaacttctacgagccccagatcatcaccaccgacaacaccttcgtgtctggcaactgcgacgtcgtgatcggcattgtgaacaataccgtgtacgaccctctgcagcccgagctggacagcttcaaagaggaactggacaagtactttaagaaccacacaagccccgacgtggacctgggcgatatcagcggaatcaatgccagcgtcgtgaacatccagaaagagatcgaccggctgaacgaggtggccaagaatctgaacgagagcctgatcgacctgcaagaactggggaagtacgagcagtacatcaagtggccctggtacatctggctgggctttatcgccggactgattgccatcgtgatggtcacaatcatgctgtgttgcatgaccagctgctgtagctgcctgaagggctgttgtagctgtggcagctgctgcaagttcgacgaggacgattctgagcccgtgctgaagggcgtgaaactgcactacacagatagcactgagaacgtcatcaagcccttcatgcgcttcaaggtgcacatggagggctccgtgaacggccacgagttcgagatcgagggcgtgggcgagggcaagccctacgagggcacccagaccgccaagctgcaagtgaccaagggcggccccctgcccttcgcctgggacatcctgtccccccagttcttctacggctccaaggcgtacatcaagcaccccgccgacatccccgactacctcaagcagtccttccccgagggcttcaagtgggagcgcgtgatgaacttcgaggacggcggcgtggtgaccgtgacccaggactcctccctgcaggacggcaccctcatctaccacgtgaagttcatcggcgtgaacttcccctccgacggccccgtaatgcagaagaaaactctgggctgggagccctccactgagcgcaactacccccgcgacggcgtgctgaagggcgagaaccacatggcgctgaagctgaagggcggcggccactacctgtgtgagttcaagtccatctacatggccaagaagcccgtgaagctgcccggctaccactacgtggactacaagctcgacatcacctcccacaacgaggactacaccgtggtggagcagtacgagcgcgccgaggcccgccaccacctgttccagtgataataggttctctctgactgtggggacgaagaatacttttattctcaaaaaaaaaaaaaaaaaaaaaaaaaaaaaaaaaaaaaaaaaaaaaaaaaaaaaaaaaaaaaaaaaaaaaaaaaaaaaaaaaaaaaaaaaaaaaaaaaaaaagagacg

SEQ ID NO: 288 - DNA, 4721 bp, synthetic construct
  source 1..4721: mol_type = other DNA
taatacgactcactataagggagaataaactagtattcttctggtccccacagactcagagagaacccgccaccatgttcgtgttcctggtgctgctgcctctggtgtccagccagtgtgtgaacctgaccaccagaacacagctgcctccagcctacaccaacagctttaccagaggcgtgtactaccccgacaaggtgttcagatccagcgtgctgcactctacccaggacctgttcctgcctttcttcagcaacgtgacctggttccacgccatccacgtgtccggcaccaatggcaccaagagattcgacaaccccgtgctgcccttcaacgacggggtgtactttgccagcaccgagaagtccaacatcatcagaggctggatcttcggcaccacactggacagcaagacccagagcctgctgatcgtgaacaacgccaccaacgtggtcatcaaagtgtgcgagttccagttctgcaacgaccccttcctgggcgtctactaccacaagaacaacaagagctggatggaaagcgagttccgggtgtacagcagcgccaacaactgcaccttcgagtacgtgtcccagcctttcctgatggacctggaaggcaagcagggcaacttcaagaacctgcgcgagttcgtgtttaagaacatcgacggctacttcaagatctacagcaagcacacccctatcaacctcgtgcgggatctgcctcagggcttctctgctctggaacccctggtggatctgcccatcggcatcaacatcacccggtttcagacactgctggccctgcacagaagctacctgacacctggcgatagcagcagcggatggacagctggtgccgccgcttactatgtgggctacctgcagcctagaaccttcctgctgaagtacaacgagaacggcaccatcaccgacgccgtggattgtgctctggatcctctgagcgagacaaagtgcaccctgaagtccttcaccgtggaaaagggcatctaccagaccagcaacttccgggtgcagcccaccgaatccatcgtgcggttccccaatatcaccaatctgtgccccttcggcgaggtgttcaatgccaccagattcgcctctgtgtacgcctggaaccggaagcggatcagcaattgcgtggccgactactccgtgctgtacaactccgccagcttcagcaccttcaagtgctacggcgtgtcccctaccaagctgaacgacctgtgcttcacaaacgtgtacgccgacagcttcgtgatccggggagatgaagtgcggcagattgcccctggacagacaggcaagatcgccgactacaactacaagctgcccgacgacttcaccggctgtgtgattgcctggaacagcaacaacctggactccaaagtcggcggcaactacaattacctgtaccggctgttccggaagtccaatctgaagcccttcgagcgggacatctccaccgagatctatcaggccggcagcaccccttgtaacggcgtggaaggcttcaactgctacttcccactgcagtcctacggctttcagcccacaaatggcgtgggctatcagccctacagagtggtggtgctgagcttcgaactgctgcatgcccctgccacagtgtgcggccctaagaaaagcaccaatctcgtgaagaacaaatgcgtgaacttcaacttcaacggcctgaccggcaccggcgtgctgacagagagcaacaagaagttcctgccattccagcagtttggccgggatatcgccgataccacagacgccgttagagatccccagacactggaaatcctggacatcaccccttgcagcttcggcggagtgtctgtgatcacccctggcaccaacaccagcaatcaggtggcagtgctgtaccaggacgtgaactgtaccgaagtgcccgtggccattcacgccgatcagctgacacctacatggcgggtgtactccaccggcagcaatgtgtttcagaccagagccggctgtctgatcggagccgagcacgtgaacaatagctacgagtgcgacatccccatcggcgctggaatctgcgccagctaccagacacagacaaacagccctcggagagccagaagcgtggccagccagagcatcattgcctacacaatgtctctgggcgccgagaacagcgtggcctactccaacaactctatcgctatccccaccaacttcaccatcagcgtgaccacagagatcctgcctgtgtccatgaccaagaccagcgtggactgcaccatgtacatctgcggcgattccaccgagtgctccaacctgctgctgcagtacggcagcttctgcacccagctgaatagagccctgacagggatcgccgtggaacaggacaagaacacccaagaggtgttcgcccaagtgaagcagatctacaagacccctcctatcaaggacttcggcggcttcaatttcagccagattctgcccgatcctagcaagcccagcaagcggagcttcatcgaggacctgctgttcaacaaagtgacactggccgacgccggcttcatcaagcagtatggcgattgtctgggcgacattgccgccagggatctgatttgcgcccagaagtttaacggactgacagtgctgcctcctctgctgaccgatgagatgatcgcccagtacacatctgccctgctggccggcacaatcacaagcggctggacatttggagcaggcgccgctctgcagatcccctttgctatgcagatggcctaccggttcaacggcatcggagtgacccagaatgtgctgtacgagaaccagaagctgatcgccaaccagttcaacagcgccatcggcaagatccaggacagcctgagcagcacagcaagcgccctgggaaagctgcaggacgtggtcaaccagaatgcccaggcactgaacaccctggtcaagcagctgtcctccaacttcggcgccatcagctctgtgctgaacgatatcctgagcagactggaccctcctgaggccgaggtgcagatcgacagactgatcacaggcagactgcagagcctccagacatacgtgacccagcagctgatcagagccgccgagattagagcctctgccaatctggccgccaccaagatgtctgagtgtgtgctgggccagagcaagagagtggacttttgcggcaagggctaccacctgatgagcttccctcagtctgcccctcacggcgtggtgtttctgcacgtgacatatgtgcccgctcaagagaagaatttcaccaccgctccagccatctgccacgacggcaaagcccactttcctagagaaggcgtgttcgtgtccaacggcacccattggttcgtgacacagcggaacttctacgagccccagatcatcaccaccgacaacaccttcgtgtctggcaactgcgacgtcgtgatcggcattgtgaacaataccgtgtacgaccctctgcagcccgagctggacagcttcaaagaggaactggacaagtactttaagaaccacacaagccccgacgtggacctgggcgatatcagcggaatcaatgccagcgtcgtgaacatccagaaagagatcgaccggctgaacgaggtggccaagaatctgaacgagagcctgatcgacctgcaagaactggggaagtacgagcagtacatcaagtggccctggtacatctggctgggctttatcgccggactgattgccatcgtgatggtcacaatcatgctgtgttgcatgaccagctgctgtagctgcctgaagggctgttgtagctgtggcagctgctgcaagttcgacgaggacgattctgagcccgtgctgaagggcgtgaaactgcactacacagatagcactgagaacgtcatcaagcccttcatgcgcttcaaggtgcacatggagggctccgtgaacggccacgagttcgagatcgagggcgtgggcgagggcaagccctacgagggcacccagaccgccaagctgcaagtgaccaagggcggccccctgcccttcgcctgggacatcctgtccccccagttcttctacggctccaaggcgtacatcaagcaccccgccgacatccccgactacctcaagcagtccttccccgagggcttcaagtgggagcgcgtgatgaacttcgaggacggcggcgtggtgaccgtgacccaggactcctccctgcaggacggcaccctcatctaccacgtgaagttcatcggcgtgaacttcccctccgacggccccgtaatgcagaagaaaactctgggctgggagccctccactgagcgcaactacccccgcgacggcgtgctgaagggcgagaaccacatggcgctgaagctgaagggcggcggccactacctgtgtgagttcaagtccatctacatggccaagaagcccgtgaagctgcccggctaccactacgtggactacaagctcgacatcacctcccacaacgaggactacaccgtggtggagcagtacgagcgcgccgaggcccgccaccacctgttccagtgataataggggttctctgagtgtggggaccaagaatacttttattctcaaaaaaaaaaaaaaaaaaaaaaaaaaaaaaaaaaaaaaaaaaaaaaaaaaaaaaaaaaaaaaaaaaaaaaaaaaaaaaaaaaaaaaaaaaaaaaaaaaaaagagacg

SEQ ID NO: 289 - DNA, 4721 bp, synthetic construct
  source 1..4721: mol_type = other DNA
taatacgactcactataagggagaataaactagtattcttctggtccccacagactcagagagaacccgccaccatgttcgtgttcctggtgctgctgcctctggtgtccagccagtgtgtgaacctgaccaccagaacacagctgcctccagcctacaccaacagctttaccagaggcgtgtactaccccgacaaggtgttcagatccagcgtgctgcactctacccaggacctgttcctgcctttcttcagcaacgtgacctggttccacgccatccacgtgtccggcaccaatggcaccaagagattcgacaaccccgtgctgcccttcaacgacggggtgtactttgccagcaccgagaagtccaacatcatcagaggctggatcttcggcaccacactggacagcaagacccagagcctgctgatcgtgaacaacgccaccaacgtggtcatcaaagtgtgcgagttccagttctgcaacgaccccttcctgggcgtctactaccacaagaacaacaagagctggatggaaagcgagttccgggtgtacagcagcgccaacaactgcaccttcgagtacgtgtcccagcctttcctgatggacctggaaggcaagcagggcaacttcaagaacctgcgcgagttcgtgtttaagaacatcgacggctacttcaagatctacagcaagcacacccctatcaacctcgtgcgggatctgcctcagggcttctctgctctggaacccctggtggatctgcccatcggcatcaacatcacccggtttcagacactgctggccctgcacagaagctacctgacacctggcgatagcagcagcggatggacagctggtgccgccgcttactatgtgggctacctgcagcctagaaccttcctgctgaagtacaacgagaacggcaccatcaccgacgccgtggattgtgctctggatcctctgagcgagacaaagtgcaccctgaagtccttcaccgtggaaaagggcatctaccagaccagcaacttccgggtgcagcccaccgaatccatcgtgcggttccccaatatcaccaatctgtgccccttcggcgaggtgttcaatgccaccagattcgcctctgtgtacgcctggaaccggaagcggatcagcaattgcgtggccgactactccgtgctgtacaactccgccagcttcagcaccttcaagtgctacggcgtgtcccctaccaagctgaacgacctgtgcttcacaaacgtgtacgccgacagcttcgtgatccggggagatgaagtgcggcagattgcccctggacagacaggcaagatcgccgactacaactacaagctgcccgacgacttcaccggctgtgtgattgcctggaacagcaacaacctggactccaaagtcggcggcaactacaattacctgtaccggctgttccggaagtccaatctgaagcccttcgagcgggacatctccaccgagatctatcaggccggcagcaccccttgtaacggcgtggaaggcttcaactgctacttcccactgcagtcctacggctttcagcccacaaatggcgtgggctatcagccctacagagtggtggtgctgagcttcgaactgctgcatgcccctgccacagtgtgcggccctaagaaaagcaccaatctcgtgaagaacaaatgcgtgaacttcaacttcaacggcctgaccggcaccggcgtgctgacagagagcaacaagaagttcctgccattccagcagtttggccgggatatcgccgataccacagacgccgttagagatccccagacactggaaatcctggacatcaccccttgcagcttcggcggagtgtctgtgatcacccctggcaccaacaccagcaatcaggtggcagtgctgtaccaggacgtgaactgtaccgaagtgcccgtggccattcacgccgatcagctgacacctacatggcgggtgtactccaccggcagcaatgtgtttcagaccagagccggctgtctgatcggagccgagcacgtgaacaatagctacgagtgcgacatccccatcggcgctggaatctgcgccagctaccagacacagacaaacagccctcggagagccagaagcgtggccagccagagcatcattgcctacacaatgtctctgggcgccgagaacagcgtggcctactccaacaactctatcgctatccccaccaacttcaccatcagcgtgaccacagagatcctgcctgtgtccatgaccaagaccagcgtggactgcaccatgtacatctgcggcgattccaccgagtgctccaacctgctgctgcagtacggcagcttctgcacccagctgaatagagccctgacagggatcgccgtggaacaggacaagaacacccaagaggtgttcgcccaagtgaagcagatctacaagacccctcctatcaaggacttcggcggcttcaatttcagccagattctgcccgatcctagcaagcccagcaagcggagcttcatcgaggacctgctgttcaacaaagtgacactggccgacgccggcttcatcaagcagtatggcgattgtctgggcgacattgccgccagggatctgatttgcgcccagaagtttaacggactgacagtgctgcctcctctgctgaccgatgagatgatcgcccagtacacatctgccctgctggccggcacaatcacaagcggctggacatttggagcaggcgccgctctgcagatcccctttgctatgcagatggcctaccggttcaacggcatcggagtgacccagaatgtgctgtacgagaaccagaagctgatcgccaaccagttcaacagcgccatcggcaagatccaggacagcctgagcagcacagcaagcgccctgggaaagctgcaggacgtggtcaaccagaatgcccaggcactgaacaccctggtcaagcagctgtcctccaacttcggcgccatcagctctgtgctgaacgatatcctgagcagactggaccctcctgaggccgaggtgcagatcgacagactgatcacaggcagactgcagagcctccagacatacgtgacccagcagctgatcagagccgccgagattagagcctctgccaatctggccgccaccaagatgtctgagtgtgtgctgggccagagcaagagagtggacttttgcggcaagggctaccacctgatgagcttccctcagtctgcccctcacggcgtggtgtttctgcacgtgacatatgtgcccgctcaagagaagaatttcaccaccgctccagccatctgccacgacggcaaagcccactttcctagagaaggcgtgttcgtgtccaacggcacccattggttcgtgacacagcggaacttctacgagccccagatcatcaccaccgacaacaccttcgtgtctggcaactgcgacgtcgtgatcggcattgtgaacaataccgtgtacgaccctctgcagcccgagctggacagcttcaaagaggaactggacaagtactttaagaaccacacaagccccgacgtggacctgggcgatatcagcggaatcaatgccagcgtcgtgaacatccagaaagagatcgaccggctgaacgaggtggccaagaatctgaacgagagcctgatcgacctgcaagaactggggaagtacgagcagtacatcaagtggccctggtacatctggctgggctttatcgccggactgattgccatcgtgatggtcacaatcatgctgtgttgcatgaccagctgctgtagctgcctgaagggctgttgtagctgtggcagctgctgcaagttcgacgaggacgattctgagcccgtgctgaagggcgtgaaactgcactacacagatagcactgagaacgtcatcaagcccttcatgcgcttcaaggtgcacatggagggctccgtgaacggccacgagttcgagatcgagggcgtgggcgagggcaagccctacgagggcacccagaccgccaagctgcaagtgaccaagggcggccccctgcccttcgcctgggacatcctgtccccccagttcttctacggctccaaggcgtacatcaagcaccccgccgacatccccgactacctcaagcagtccttccccgagggcttcaagtgggagcgcgtgatgaacttcgaggacggcggcgtggtgaccgtgacccaggactcctccctgcaggacggcaccctcatctaccacgtgaagttcatcggcgtgaacttcccctccgacggccccgtaatgcagaagaaaactctgggctgggagccctccactgagcgcaactacccccgcgacggcgtgctgaagggcgagaaccacatggcgctgaagctgaagggcggcggccactacctgtgtgagttcaagtccatctacatggccaagaagcccgtgaagctgcccggctaccactacgtggactacaagctcgacatcacctcccacaacgaggactacaccgtggtggagcagtacgagcgcgccgaggcccgccaccacctgttccagtgataataggggttctctgagtctggggaccaggaatactattattctcaaaaaaaaaaaaaaaaaaaaaaaaaaaaaaaaaaaaaaaaaaaaaaaaaaaaaaaaaaaaaaaaaaaaaaaaaaaaaaaaaaaaaaaaaaaaaaaaaaaaagagacg

SEQ ID NO: 290 - DNA, 4719 bp, synthetic construct
  source 1..4719: mol_type = other DNA
taatacgactcactataagggagaataaactagtattcttctggtccccacagactcagagagaacccgccaccatgttcgtgttcctggtgctgctgcctctggtgtccagccagtgtgtgaacctgaccaccagaacacagctgcctccagcctacaccaacagctttaccagaggcgtgtactaccccgacaaggtgttcagatccagcgtgctgcactctacccaggacctgttcctgcctttcttcagcaacgtgacctggttccacgccatccacgtgtccggcaccaatggcaccaagagattcgacaaccccgtgctgcccttcaacgacggggtgtactttgccagcaccgagaagtccaacatcatcagaggctggatcttcggcaccacactggacagcaagacccagagcctgctgatcgtgaacaacgccaccaacgtggtcatcaaagtgtgcgagttccagttctgcaacgaccccttcctgggcgtctactaccacaagaacaacaagagctggatggaaagcgagttccgggtgtacagcagcgccaacaactgcaccttcgagtacgtgtcccagcctttcctgatggacctggaaggcaagcagggcaacttcaagaacctgcgcgagttcgtgtttaagaacatcgacggctacttcaagatctacagcaagcacacccctatcaacctcgtgcgggatctgcctcagggcttctctgctctggaacccctggtggatctgcccatcggcatcaacatcacccggtttcagacactgctggccctgcacagaagctacctgacacctggcgatagcagcagcggatggacagctggtgccgccgcttactatgtgggctacctgcagcctagaaccttcctgctgaagtacaacgagaacggcaccatcaccgacgccgtggattgtgctctggatcctctgagcgagacaaagtgcaccctgaagtccttcaccgtggaaaagggcatctaccagaccagcaacttccgggtgcagcccaccgaatccatcgtgcggttccccaatatcaccaatctgtgccccttcggcgaggtgttcaatgccaccagattcgcctctgtgtacgcctggaaccggaagcggatcagcaattgcgtggccgactactccgtgctgtacaactccgccagcttcagcaccttcaagtgctacggcgtgtcccctaccaagctgaacgacctgtgcttcacaaacgtgtacgccgacagcttcgtgatccggggagatgaagtgcggcagattgcccctggacagacaggcaagatcgccgactacaactacaagctgcccgacgacttcaccggctgtgtgattgcctggaacagcaacaacctggactccaaagtcggcggcaactacaattacctgtaccggctgttccggaagtccaatctgaagcccttcgagcgggacatctccaccgagatctatcaggccggcagcaccccttgtaacggcgtggaaggcttcaactgctacttcccactgcagtcctacggctttcagcccacaaatggcgtgggctatcagccctacagagtggtggtgctgagcttcgaactgctgcatgcccctgccacagtgtgcggccctaagaaaagcaccaatctcgtgaagaacaaatgcgtgaacttcaacttcaacggcctgaccggcaccggcgtgctgacagagagcaacaagaagttcctgccattccagcagtttggccgggatatcgccgataccacagacgccgttagagatccccagacactggaaatcctggacatcaccccttgcagcttcggcggagtgtctgtgatcacccctggcaccaacaccagcaatcaggtggcagtgctgtaccaggacgtgaactgtaccgaagtgcccgtggccattcacgccgatcagctgacacctacatggcgggtgtactccaccggcagcaatgtgtttcagaccagagccggctgtctgatcggagccgagcacgtgaacaatagctacgagtgcgacatccccatcggcgctggaatctgcgccagctaccagacacagacaaacagccctcggagagccagaagcgtggccagccagagcatcattgcctacacaatgtctctgggcgccgagaacagcgtggcctactccaacaactctatcgctatccccaccaacttcaccatcagcgtgaccacagagatcctgcctgtgtccatgaccaagaccagcgtggactgcaccatgtacatctgcggcgattccaccgagtgctccaacctgctgctgcagtacggcagcttctgcacccagctgaatagagccctgacagggatcgccgtggaacaggacaagaacacccaagaggtgttcgcccaagtgaagcagatctacaagacccctcctatcaaggacttcggcggcttcaatttcagccagattctgcccgatcctagcaagcccagcaagcggagcttcatcgaggacctgctgttcaacaaagtgacactggccgacgccggcttcatcaagcagtatggcgattgtctgggcgacattgccgccagggatctgatttgcgcccagaagtttaacggactgacagtgctgcctcctctgctgaccgatgagatgatcgcccagtacacatctgccctgctggccggcacaatcacaagcggctggacatttggagcaggcgccgctctgcagatcccctttgctatgcagatggcctaccggttcaacggcatcggagtgacccagaatgtgctgtacgagaaccagaagctgatcgccaaccagttcaacagcgccatcggcaagatccaggacagcctgagcagcacagcaagcgccctgggaaagctgcaggacgtggtcaaccagaatgcccaggcactgaacaccctggtcaagcagctgtcctccaacttcggcgccatcagctctgtgctgaacgatatcctgagcagactggaccctcctgaggccgaggtgcagatcgacagactgatcacaggcagactgcagagcctccagacatacgtgacccagcagctgatcagagccgccgagattagagcctctgccaatctggccgccaccaagatgtctgagtgtgtgctgggccagagcaagagagtggacttttgcggcaagggctaccacctgatgagcttccctcagtctgcccctcacggcgtggtgtttctgcacgtgacatatgtgcccgctcaagagaagaatttcaccaccgctccagccatctgccacgacggcaaagcccactttcctagagaaggcgtgttcgtgtccaacggcacccattggttcgtgacacagcggaacttctacgagccccagatcatcaccaccgacaacaccttcgtgtctggcaactgcgacgtcgtgatcggcattgtgaacaataccgtgtacgaccctctgcagcccgagctggacagcttcaaagaggaactggacaagtactttaagaaccacacaagccccgacgtggacctgggcgatatcagcggaatcaatgccagcgtcgtgaacatccagaaagagatcgaccggctgaacgaggtggccaagaatctgaacgagagcctgatcgacctgcaagaactggggaagtacgagcagtacatcaagtggccctggtacatctggctgggctttatcgccggactgattgccatcgtgatggtcacaatcatgctgtgttgcatgaccagctgctgtagctgcctgaagggctgttgtagctgtggcagctgctgcaagttcgacgaggacgattctgagcccgtgctgaagggcgtgaaactgcactacacagatagcactgagaacgtcatcaagcccttcatgcgcttcaaggtgcacatggagggctccgtgaacggccacgagttcgagatcgagggcgtgggcgagggcaagccctacgagggcacccagaccgccaagctgcaagtgaccaagggcggccccctgcccttcgcctgggacatcctgtccccccagttcttctacggctccaaggcgtacatcaagcaccccgccgacatccccgactacctcaagcagtccttccccgagggcttcaagtgggagcgcgtgatgaacttcgaggacggcggcgtggtgaccgtgacccaggactcctccctgcaggacggcaccctcatctaccacgtgaagttcatcggcgtgaacttcccctccgacggccccgtaatgcagaagaaaactctgggctgggagccctccactgagcgcaactacccccgcgacggcgtgctgaagggcgagaaccacatggcgctgaagctgaagggcggcggccactacctgtgtgagttcaagtccatctacatggccaagaagcccgtgaagctgcccggctaccactacgtggactacaagctcgacatcacctcccacaacgaggactacaccgtggtggagcagtacgagcgcgccgaggcccgccaccacctgttccagtgataataggggctctctgtctgtggaccagaaatactagtattctcaaaaaaaaaaaaaaaaaaaaaaaaaaaaaaaaaaaaaaaaaaaaaaaaaaaaaaaaaaaaaaaaaaaaaaaaaaaaaaaaaaaaaaaaaaaaaaaaaaaaagagacg

SEQ ID NO: 291 - DNA, 4717 bp, synthetic construct
  source 1..4717: mol_type = other DNA
taatacgactcactataagggagaataaactagtattcttctggtccccacagactcagagagaacccgccaccatgttcgtgttcctggtgctgctgcctctggtgtccagccagtgtgtgaacctgaccaccagaacacagctgcctccagcctacaccaacagctttaccagaggcgtgtactaccccgacaaggtgttcagatccagcgtgctgcactctacccaggacctgttcctgcctttcttcagcaacgtgacctggttccacgccatccacgtgtccggcaccaatggcaccaagagattcgacaaccccgtgctgcccttcaacgacggggtgtactttgccagcaccgagaagtccaacatcatcagaggctggatcttcggcaccacactggacagcaagacccagagcctgctgatcgtgaacaacgccaccaacgtggtcatcaaagtgtgcgagttccagttctgcaacgaccccttcctgggcgtctactaccacaagaacaacaagagctggatggaaagcgagttccgggtgtacagcagcgccaacaactgcaccttcgagtacgtgtcccagcctttcctgatggacctggaaggcaagcagggcaacttcaagaacctgcgcgagttcgtgtttaagaacatcgacggctacttcaagatctacagcaagcacacccctatcaacctcgtgcgggatctgcctcagggcttctctgctctggaacccctggtggatctgcccatcggcatcaacatcacccggtttcagacactgctggccctgcacagaagctacctgacacctggcgatagcagcagcggatggacagctggtgccgccgcttactatgtgggctacctgcagcctagaaccttcctgctgaagtacaacgagaacggcaccatcaccgacgccgtggattgtgctctggatcctctgagcgagacaaagtgcaccctgaagtccttcaccgtggaaaagggcatctaccagaccagcaacttccgggtgcagcccaccgaatccatcgtgcggttccccaatatcaccaatctgtgccccttcggcgaggtgttcaatgccaccagattcgcctctgtgtacgcctggaaccggaagcggatcagcaattgcgtggccgactactccgtgctgtacaactccgccagcttcagcaccttcaagtgctacggcgtgtcccctaccaagctgaacgacctgtgcttcacaaacgtgtacgccgacagcttcgtgatccggggagatgaagtgcggcagattgcccctggacagacaggcaagatcgccgactacaactacaagctgcccgacgacttcaccggctgtgtgattgcctggaacagcaacaacctggactccaaagtcggcggcaactacaattacctgtaccggctgttccggaagtccaatctgaagcccttcgagcgggacatctccaccgagatctatcaggccggcagcaccccttgtaacggcgtggaaggcttcaactgctacttcccactgcagtcctacggctttcagcccacaaatggcgtgggctatcagccctacagagtggtggtgctgagcttcgaactgctgcatgcccctgccacagtgtgcggccctaagaaaagcaccaatctcgtgaagaacaaatgcgtgaacttcaacttcaacggcctgaccggcaccggcgtgctgacagagagcaacaagaagttcctgccattccagcagtttggccgggatatcgccgataccacagacgccgttagagatccccagacactggaaatcctggacatcaccccttgcagcttcggcggagtgtctgtgatcacccctggcaccaacaccagcaatcaggtggcagtgctgtaccaggacgtgaactgtaccgaagtgcccgtggccattcacgccgatcagctgacacctacatggcgggtgtactccaccggcagcaatgtgtttcagaccagagccggctgtctgatcggagccgagcacgtgaacaatagctacgagtgcgacatccccatcggcgctggaatctgcgccagctaccagacacagacaaacagccctcggagagccagaagcgtggccagccagagcatcattgcctacacaatgtctctgggcgccgagaacagcgtggcctactccaacaactctatcgctatccccaccaacttcaccatcagcgtgaccacagagatcctgcctgtgtccatgaccaagaccagcgtggactgcaccatgtacatctgcggcgattccaccgagtgctccaacctgctgctgcagtacggcagcttctgcacccagctgaatagagccctgacagggatcgccgtggaacaggacaagaacacccaagaggtgttcgcccaagtgaagcagatctacaagacccctcctatcaaggacttcggcggcttcaatttcagccagattctgcccgatcctagcaagcccagcaagcggagcttcatcgaggacctgctgttcaacaaagtgacactggccgacgccggcttcatcaagcagtatggcgattgtctgggcgacattgccgccagggatctgatttgcgcccagaagtttaacggactgacagtgctgcctcctctgctgaccgatgagatgatcgcccagtacacatctgccctgctggccggcacaatcacaagcggctggacatttggagcaggcgccgctctgcagatcccctttgctatgcagatggcctaccggttcaacggcatcggagtgacccagaatgtgctgtacgagaaccagaagctgatcgccaaccagttcaacagcgccatcggcaagatccaggacagcctgagcagcacagcaagcgccctgggaaagctgcaggacgtggtcaaccagaatgcccaggcactgaacaccctggtcaagcagctgtcctccaacttcggcgccatcagctctgtgctgaacgatatcctgagcagactggaccctcctgaggccgaggtgcagatcgacagactgatcacaggcagactgcagagcctccagacatacgtgacccagcagctgatcagagccgccgagattagagcctctgccaatctggccgccaccaagatgtctgagtgtgtgctgggccagagcaagagagtggacttttgcggcaagggctaccacctgatgagcttccctcagtctgcccctcacggcgtggtgtttctgcacgtgacatatgtgcccgctcaagagaagaatttcaccaccgctccagccatctgccacgacggcaaagcccactttcctagagaaggcgtgttcgtgtccaacggcacccattggttcgtgacacagcggaacttctacgagccccagatcatcaccaccgacaacaccttcgtgtctggcaactgcgacgtcgtgatcggcattgtgaacaataccgtgtacgaccctctgcagcccgagctggacagcttcaaagaggaactggacaagtactttaagaaccacacaagccccgacgtggacctgggcgatatcagcggaatcaatgccagcgtcgtgaacatccagaaagagatcgaccggctgaacgaggtggccaagaatctgaacgagagcctgatcgacctgcaagaactggggaagtacgagcagtacatcaagtggccctggtacatctggctgggctttatcgccggactgattgccatcgtgatggtcacaatcatgctgtgttgcatgaccagctgctgtagctgcctgaagggctgttgtagctgtggcagctgctgcaagttcgacgaggacgattctgagcccgtgctgaagggcgtgaaactgcactacacagatagcactgagaacgtcatcaagcccttcatgcgcttcaaggtgcacatggagggctccgtgaacggccacgagttcgagatcgagggcgtgggcgagggcaagccctacgagggcacccagaccgccaagctgcaagtgaccaagggcggccccctgcccttcgcctgggacatcctgtccccccagttcttctacggctccaaggcgtacatcaagcaccccgccgacatccccgactacctcaagcagtccttccccgagggcttcaagtgggagcgcgtgatgaacttcgaggacggcggcgtggtgaccgtgacccaggactcctccctgcaggacggcaccctcatctaccacgtgaagttcatcggcgtgaacttcccctccgacggccccgtaatgcagaagaaaactctgggctgggagccctccactgagcgcaactacccccgcgacggcgtgctgaagggcgagaaccacatggcgctgaagctgaagggcggcggccactacctgtgtgagttcaagtccatctacatggccaagaagcccgtgaagctgcccggctaccactacgtggactacaagctcgacatcacctcccacaacgaggactacaccgtggtggagcagtacgagcgcgccgaggcccgccaccacctgttccagtgataataggttctctgagtctggggacgaagaactagttttctcaaaaaaaaaaaaaaaaaaaaaaaaaaaaaaaaaaaaaaaaaaaaaaaaaaaaaaaaaaaaaaaaaaaaaaaaaaaaaaaaaaaaaaaaaaaaaaaaaaaaagagacg

SEQ ID NO: 292 - DNA, 4715 bp, synthetic construct
  source 1..4715: mol_type = other DNA
taatacgactcactataagggagaataaactagtattcttctggtccccacagactcagagagaacccgccaccatgttcgtgttcctggtgctgctgcctctggtgtccagccagtgtgtgaacctgaccaccagaacacagctgcctccagcctacaccaacagctttaccagaggcgtgtactaccccgacaaggtgttcagatccagcgtgctgcactctacccaggacctgttcctgcctttcttcagcaacgtgacctggttccacgccatccacgtgtccggcaccaatggcaccaagagattcgacaaccccgtgctgcccttcaacgacggggtgtactttgccagcaccgagaagtccaacatcatcagaggctggatcttcggcaccacactggacagcaagacccagagcctgctgatcgtgaacaacgccaccaacgtggtcatcaaagtgtgcgagttccagttctgcaacgaccccttcctgggcgtctactaccacaagaacaacaagagctggatggaaagcgagttccgggtgtacagcagcgccaacaactgcaccttcgagtacgtgtcccagcctttcctgatggacctggaaggcaagcagggcaacttcaagaacctgcgcgagttcgtgtttaagaacatcgacggctacttcaagatctacagcaagcacacccctatcaacctcgtgcgggatctgcctcagggcttctctgctctggaacccctggtggatctgcccatcggcatcaacatcacccggtttcagacactgctggccctgcacagaagctacctgacacctggcgatagcagcagcggatggacagctggtgccgccgcttactatgtgggctacctgcagcctagaaccttcctgctgaagtacaacgagaacggcaccatcaccgacgccgtggattgtgctctggatcctctgagcgagacaaagtgcaccctgaagtccttcaccgtggaaaagggcatctaccagaccagcaacttccgggtgcagcccaccgaatccatcgtgcggttccccaatatcaccaatctgtgccccttcggcgaggtgttcaatgccaccagattcgcctctgtgtacgcctggaaccggaagcggatcagcaattgcgtggccgactactccgtgctgtacaactccgccagcttcagcaccttcaagtgctacggcgtgtcccctaccaagctgaacgacctgtgcttcacaaacgtgtacgccgacagcttcgtgatccggggagatgaagtgcggcagattgcccctggacagacaggcaagatcgccgactacaactacaagctgcccgacgacttcaccggctgtgtgattgcctggaacagcaacaacctggactccaaagtcggcggcaactacaattacctgtaccggctgttccggaagtccaatctgaagcccttcgagcgggacatctccaccgagatctatcaggccggcagcaccccttgtaacggcgtggaaggcttcaactgctacttcccactgcagtcctacggctttcagcccacaaatggcgtgggctatcagccctacagagtggtggtgctgagcttcgaactgctgcatgcccctgccacagtgtgcggccctaagaaaagcaccaatctcgtgaagaacaaatgcgtgaacttcaacttcaacggcctgaccggcaccggcgtgctgacagagagcaacaagaagttcctgccattccagcagtttggccgggatatcgccgataccacagacgccgttagagatccccagacactggaaatcctggacatcaccccttgcagcttcggcggagtgtctgtgatcacccctggcaccaacaccagcaatcaggtggcagtgctgtaccaggacgtgaactgtaccgaagtgcccgtggccattcacgccgatcagctgacacctacatggcgggtgtactccaccggcagcaatgtgtttcagaccagagccggctgtctgatcggagccgagcacgtgaacaatagctacgagtgcgacatccccatcggcgctggaatctgcgccagctaccagacacagacaaacagccctcggagagccagaagcgtggccagccagagcatcattgcctacacaatgtctctgggcgccgagaacagcgtggcctactccaacaactctatcgctatccccaccaacttcaccatcagcgtgaccacagagatcctgcctgtgtccatgaccaagaccagcgtggactgcaccatgtacatctgcggcgattccaccgagtgctccaacctgctgctgcagtacggcagcttctgcacccagctgaatagagccctgacagggatcgccgtggaacaggacaagaacacccaagaggtgttcgcccaagtgaagcagatctacaagacccctcctatcaaggacttcggcggcttcaatttcagccagattctgcccgatcctagcaagcccagcaagcggagcttcatcgaggacctgctgttcaacaaagtgacactggccgacgccggcttcatcaagcagtatggcgattgtctgggcgacattgccgccagggatctgatttgcgcccagaagtttaacggactgacagtgctgcctcctctgctgaccgatgagatgatcgcccagtacacatctgccctgctggccggcacaatcacaagcggctggacatttggagcaggcgccgctctgcagatcccctttgctatgcagatggcctaccggttcaacggcatcggagtgacccagaatgtgctgtacgagaaccagaagctgatcgccaaccagttcaacagcgccatcggcaagatccaggacagcctgagcagcacagcaagcgccctgggaaagctgcaggacgtggtcaaccagaatgcccaggcactgaacaccctggtcaagcagctgtcctccaacttcggcgccatcagctctgtgctgaacgatatcctgagcagactggaccctcctgaggccgaggtgcagatcgacagactgatcacaggcagactgcagagcctccagacatacgtgacccagcagctgatcagagccgccgagattagagcctctgccaatctggccgccaccaagatgtctgagtgtgtgctgggccagagcaagagagtggacttttgcggcaagggctaccacctgatgagcttccctcagtctgcccctcacggcgtggtgtttctgcacgtgacatatgtgcccgctcaagagaagaatttcaccaccgctccagccatctgccacgacggcaaagcccactttcctagagaaggcgtgttcgtgtccaacggcacccattggttcgtgacacagcggaacttctacgagccccagatcatcaccaccgacaacaccttcgtgtctggcaactgcgacgtcgtgatcggcattgtgaacaataccgtgtacgaccctctgcagcccgagctggacagcttcaaagaggaactggacaagtactttaagaaccacacaagccccgacgtggacctgggcgatatcagcggaatcaatgccagcgtcgtgaacatccagaaagagatcgaccggctgaacgaggtggccaagaatctgaacgagagcctgatcgacctgcaagaactggggaagtacgagcagtacatcaagtggccctggtacatctggctgggctttatcgccggactgattgccatcgtgatggtcacaatcatgctgtgttgcatgaccagctgctgtagctgcctgaagggctgttgtagctgtggcagctgctgcaagttcgacgaggacgattctgagcccgtgctgaagggcgtgaaactgcactacacagatagcactgagaacgtcatcaagcccttcatgcgcttcaaggtgcacatggagggctccgtgaacggccacgagttcgagatcgagggcgtgggcgagggcaagccctacgagggcacccagaccgccaagctgcaagtgaccaagggcggccccctgcccttcgcctgggacatcctgtccccccagttcttctacggctccaaggcgtacatcaagcaccccgccgacatccccgactacctcaagcagtccttccccgagggcttcaagtgggagcgcgtgatgaacttcgaggacggcggcgtggtgaccgtgacccaggactcctccctgcaggacggcaccctcatctaccacgtgaagttcatcggcgtgaacttcccctccgacggccccgtaatgcagaagaaaactctgggctgggagccctccactgagcgcaactacccccgcgacggcgtgctgaagggcgagaaccacatggcgctgaagctgaagggcggcggccactacctgtgtgagttcaagtccatctacatggccaagaagcccgtgaagctgcccggctaccactacgtggactacaagctcgacatcacctcccacaacgaggactacaccgtggtggagcagtacgagcgcgccgaggcccgccaccacctgttccagtgataataggttctctgagtgtgggccagaaatacgtttactcaaaaaaaaaaaaaaaaaaaaaaaaaaaaaaaaaaaaaaaaaaaaaaaaaaaaaaaaaaaaaaaaaaaaaaaaaaaaaaaaaaaaaaaaaaaaaaaaaaaaagagacg

SEQ ID NO: 293 - DNA, 4720 bp, synthetic construct
  source 1..4720: mol_type = other DNA
taatacgactcactataagggagaataaactagtattcttctggtccccacagactcagagagaacccgccaccatgttcgtgttcctggtgctgctgcctctggtgtccagccagtgtgtgaacctgaccaccagaacacagctgcctccagcctacaccaacagctttaccagaggcgtgtactaccccgacaaggtgttcagatccagcgtgctgcactctacccaggacctgttcctgcctttcttcagcaacgtgacctggttccacgccatccacgtgtccggcaccaatggcaccaagagattcgacaaccccgtgctgcccttcaacgacggggtgtactttgccagcaccgagaagtccaacatcatcagaggctggatcttcggcaccacactggacagcaagacccagagcctgctgatcgtgaacaacgccaccaacgtggtcatcaaagtgtgcgagttccagttctgcaacgaccccttcctgggcgtctactaccacaagaacaacaagagctggatggaaagcgagttccgggtgtacagcagcgccaacaactgcaccttcgagtacgtgtcccagcctttcctgatggacctggaaggcaagcagggcaacttcaagaacctgcgcgagttcgtgtttaagaacatcgacggctacttcaagatctacagcaagcacacccctatcaacctcgtgcgggatctgcctcagggcttctctgctctggaacccctggtggatctgcccatcggcatcaacatcacccggtttcagacactgctggccctgcacagaagctacctgacacctggcgatagcagcagcggatggacagctggtgccgccgcttactatgtgggctacctgcagcctagaaccttcctgctgaagtacaacgagaacggcaccatcaccgacgccgtggattgtgctctggatcctctgagcgagacaaagtgcaccctgaagtccttcaccgtggaaaagggcatctaccagaccagcaacttccgggtgcagcccaccgaatccatcgtgcggttccccaatatcaccaatctgtgccccttcggcgaggtgttcaatgccaccagattcgcctctgtgtacgcctggaaccggaagcggatcagcaattgcgtggccgactactccgtgctgtacaactccgccagcttcagcaccttcaagtgctacggcgtgtcccctaccaagctgaacgacctgtgcttcacaaacgtgtacgccgacagcttcgtgatccggggagatgaagtgcggcagattgcccctggacagacaggcaagatcgccgactacaactacaagctgcccgacgacttcaccggctgtgtgattgcctggaacagcaacaacctggactccaaagtcggcggcaactacaattacctgtaccggctgttccggaagtccaatctgaagcccttcgagcgggacatctccaccgagatctatcaggccggcagcaccccttgtaacggcgtggaaggcttcaactgctacttcccactgcagtcctacggctttcagcccacaaatggcgtgggctatcagccctacagagtggtggtgctgagcttcgaactgctgcatgcccctgccacagtgtgcggccctaagaaaagcaccaatctcgtgaagaacaaatgcgtgaacttcaacttcaacggcctgaccggcaccggcgtgctgacagagagcaacaagaagttcctgccattccagcagtttggccgggatatcgccgataccacagacgccgttagagatccccagacactggaaatcctggacatcaccccttgcagcttcggcggagtgtctgtgatcacccctggcaccaacaccagcaatcaggtggcagtgctgtaccaggacgtgaactgtaccgaagtgcccgtggccattcacgccgatcagctgacacctacatggcgggtgtactccaccggcagcaatgtgtttcagaccagagccggctgtctgatcggagccgagcacgtgaacaatagctacgagtgcgacatccccatcggcgctggaatctgcgccagctaccagacacagacaaacagccctcggagagccagaagcgtggccagccagagcatcattgcctacacaatgtctctgggcgccgagaacagcgtggcctactccaacaactctatcgctatccccaccaacttcaccatcagcgtgaccacagagatcctgcctgtgtccatgaccaagaccagcgtggactgcaccatgtacatctgcggcgattccaccgagtgctccaacctgctgctgcagtacggcagcttctgcacccagctgaatagagccctgacagggatcgccgtggaacaggacaagaacacccaagaggtgttcgcccaagtgaagcagatctacaagacccctcctatcaaggacttcggcggcttcaatttcagccagattctgcccgatcctagcaagcccagcaagcggagcttcatcgaggacctgctgttcaacaaagtgacactggccgacgccggcttcatcaagcagtatggcgattgtctgggcgacattgccgccagggatctgatttgcgcccagaagtttaacggactgacagtgctgcctcctctgctgaccgatgagatgatcgcccagtacacatctgccctgctggccggcacaatcacaagcggctggacatttggagcaggcgccgctctgcagatcccctttgctatgcagatggcctaccggttcaacggcatcggagtgacccagaatgtgctgtacgagaaccagaagctgatcgccaaccagttcaacagcgccatcggcaagatccaggacagcctgagcagcacagcaagcgccctgggaaagctgcaggacgtggtcaaccagaatgcccaggcactgaacaccctggtcaagcagctgtcctccaacttcggcgccatcagctctgtgctgaacgatatcctgagcagactggaccctcctgaggccgaggtgcagatcgacagactgatcacaggcagactgcagagcctccagacatacgtgacccagcagctgatcagagccgccgagattagagcctctgccaatctggccgccaccaagatgtctgagtgtgtgctgggccagagcaagagagtggacttttgcggcaagggctaccacctgatgagcttccctcagtctgcccctcacggcgtggtgtttctgcacgtgacatatgtgcccgctcaagagaagaatttcaccaccgctccagccatctgccacgacggcaaagcccactttcctagagaaggcgtgttcgtgtccaacggcacccattggttcgtgacacagcggaacttctacgagccccagatcatcaccaccgacaacaccttcgtgtctggcaactgcgacgtcgtgatcggcattgtgaacaataccgtgtacgaccctctgcagcccgagctggacagcttcaaagaggaactggacaagtactttaagaaccacacaagccccgacgtggacctgggcgatatcagcggaatcaatgccagcgtcgtgaacatccagaaagagatcgaccggctgaacgaggtggccaagaatctgaacgagagcctgatcgacctgcaagaactggggaagtacgagcagtacatcaagtggccctggtacatctggctgggctttatcgccggactgattgccatcgtgatggtcacaatcatgctgtgttgcatgaccagctgctgtagctgcctgaagggctgttgtagctgtggcagctgctgcaagttcgacgaggacgattctgagcccgtgctgaagggcgtgaaactgcactacacagatagcactgagaacgtcatcaagcccttcatgcgcttcaaggtgcacatggagggctccgtgaacggccacgagttcgagatcgagggcgtgggcgagggcaagccctacgagggcacccagaccgccaagctgcaagtgaccaagggcggccccctgcccttcgcctgggacatcctgtccccccagttcttctacggctccaaggcgtacatcaagcaccccgccgacatccccgactacctcaagcagtccttccccgagggcttcaagtgggagcgcgtgatgaacttcgaggacggcggcgtggtgaccgtgacccaggactcctccctgcaggacggcaccctcatctaccacgtgaagttcatcggcgtgaacttcccctccgacggccccgtaatgcagaagaaaactctgggctgggagccctccactgagcgcaactacccccgcgacggcgtgctgaagggcgagaaccacatggcgctgaagctgaagggcggcggccactacctgtgtgagttcaagtccatctacatggccaagaagcccgtgaagctgcccggctaccactacgtggactacaagctcgacatcacctcccacaacgaggactacaccgtggtggagcagtacgagcgcgccgaggcccgccaccacctgttccagtgataataggggtctctgagtctgggaccagaagaatagtttattctcaaaaaaaaaaaaaaaaaaaaaaaaaaaaaaaaaaaaaaaaaaaaaaaaaaaaaaaaaaaaaaaaaaaaaaaaaaaaaaaaaaaaaaaaaaaaaaaaaaaaagagacg

SEQ ID NO: 294 - DNA, 4720 bp, synthetic construct
  source 1..4720: mol_type = other DNA
taatacgactcactataagggagaataaactagtattcttctggtccccacagactcagagagaacccgccaccatgttcgtgttcctggtgctgctgcctctggtgtccagccagtgtgtgaacctgaccaccagaacacagctgcctccagcctacaccaacagctttaccagaggcgtgtactaccccgacaaggtgttcagatccagcgtgctgcactctacccaggacctgttcctgcctttcttcagcaacgtgacctggttccacgccatccacgtgtccggcaccaatggcaccaagagattcgacaaccccgtgctgcccttcaacgacggggtgtactttgccagcaccgagaagtccaacatcatcagaggctggatcttcggcaccacactggacagcaagacccagagcctgctgatcgtgaacaacgccaccaacgtggtcatcaaagtgtgcgagttccagttctgcaacgaccccttcctgggcgtctactaccacaagaacaacaagagctggatggaaagcgagttccgggtgtacagcagcgccaacaactgcaccttcgagtacgtgtcccagcctttcctgatggacctggaaggcaagcagggcaacttcaagaacctgcgcgagttcgtgtttaagaacatcgacggctacttcaagatctacagcaagcacacccctatcaacctcgtgcgggatctgcctcagggcttctctgctctggaacccctggtggatctgcccatcggcatcaacatcacccggtttcagacactgctggccctgcacagaagctacctgacacctggcgatagcagcagcggatggacagctggtgccgccgcttactatgtgggctacctgcagcctagaaccttcctgctgaagtacaacgagaacggcaccatcaccgacgccgtggattgtgctctggatcctctgagcgagacaaagtgcaccctgaagtccttcaccgtggaaaagggcatctaccagaccagcaacttccgggtgcagcccaccgaatccatcgtgcggttccccaatatcaccaatctgtgccccttcggcgaggtgttcaatgccaccagattcgcctctgtgtacgcctggaaccggaagcggatcagcaattgcgtggccgactactccgtgctgtacaactccgccagcttcagcaccttcaagtgctacggcgtgtcccctaccaagctgaacgacctgtgcttcacaaacgtgtacgccgacagcttcgtgatccggggagatgaagtgcggcagattgcccctggacagacaggcaagatcgccgactacaactacaagctgcccgacgacttcaccggctgtgtgattgcctggaacagcaacaacctggactccaaagtcggcggcaactacaattacctgtaccggctgttccggaagtccaatctgaagcccttcgagcgggacatctccaccgagatctatcaggccggcagcaccccttgtaacggcgtggaaggcttcaactgctacttcccactgcagtcctacggctttcagcccacaaatggcgtgggctatcagccctacagagtggtggtgctgagcttcgaactgctgcatgcccctgccacagtgtgcggccctaagaaaagcaccaatctcgtgaagaacaaatgcgtgaacttcaacttcaacggcctgaccggcaccggcgtgctgacagagagcaacaagaagttcctgccattccagcagtttggccgggatatcgccgataccacagacgccgttagagatccccagacactggaaatcctggacatcaccccttgcagcttcggcggagtgtctgtgatcacccctggcaccaacaccagcaatcaggtggcagtgctgtaccaggacgtgaactgtaccgaagtgcccgtggccattcacgccgatcagctgacacctacatggcgggtgtactccaccggcagcaatgtgtttcagaccagagccggctgtctgatcggagccgagcacgtgaacaatagctacgagtgcgacatccccatcggcgctggaatctgcgccagctaccagacacagacaaacagccctcggagagccagaagcgtggccagccagagcatcattgcctacacaatgtctctgggcgccgagaacagcgtggcctactccaacaactctatcgctatccccaccaacttcaccatcagcgtgaccacagagatcctgcctgtgtccatgaccaagaccagcgtggactgcaccatgtacatctgcggcgattccaccgagtgctccaacctgctgctgcagtacggcagcttctgcacccagctgaatagagccctgacagggatcgccgtggaacaggacaagaacacccaagaggtgttcgcccaagtgaagcagatctacaagacccctcctatcaaggacttcggcggcttcaatttcagccagattctgcccgatcctagcaagcccagcaagcggagcttcatcgaggacctgctgttcaacaaagtgacactggccgacgccggcttcatcaagcagtatggcgattgtctgggcgacattgccgccagggatctgatttgcgcccagaagtttaacggactgacagtgctgcctcctctgctgaccgatgagatgatcgcccagtacacatctgccctgctggccggcacaatcacaagcggctggacatttggagcaggcgccgctctgcagatcccctttgctatgcagatggcctaccggttcaacggcatcggagtgacccagaatgtgctgtacgagaaccagaagctgatcgccaaccagttcaacagcgccatcggcaagatccaggacagcctgagcagcacagcaagcgccctgggaaagctgcaggacgtggtcaaccagaatgcccaggcactgaacaccctggtcaagcagctgtcctccaacttcggcgccatcagctctgtgctgaacgatatcctgagcagactggaccctcctgaggccgaggtgcagatcgacagactgatcacaggcagactgcagagcctccagacatacgtgacccagcagctgatcagagccgccgagattagagcctctgccaatctggccgccaccaagatgtctgagtgtgtgctgggccagagcaagagagtggacttttgcggcaagggctaccacctgatgagcttccctcagtctgcccctcacggcgtggtgtttctgcacgtgacatatgtgcccgctcaagagaagaatttcaccaccgctccagccatctgccacgacggcaaagcccactttcctagagaaggcgtgttcgtgtccaacggcacccattggttcgtgacacagcggaacttctacgagccccagatcatcaccaccgacaacaccttcgtgtctggcaactgcgacgtcgtgatcggcattgtgaacaataccgtgtacgaccctctgcagcccgagctggacagcttcaaagaggaactggacaagtactttaagaaccacacaagccccgacgtggacctgggcgatatcagcggaatcaatgccagcgtcgtgaacatccagaaagagatcgaccggctgaacgaggtggccaagaatctgaacgagagcctgatcgacctgcaagaactggggaagtacgagcagtacatcaagtggccctggtacatctggctgggctttatcgccggactgattgccatcgtgatggtcacaatcatgctgtgttgcatgaccagctgctgtagctgcctgaagggctgttgtagctgtggcagctgctgcaagttcgacgaggacgattctgagcccgtgctgaagggcgtgaaactgcactacacagatagcactgagaacgtcatcaagcccttcatgcgcttcaaggtgcacatggagggctccgtgaacggccacgagttcgagatcgagggcgtgggcgagggcaagccctacgagggcacccagaccgccaagctgcaagtgaccaagggcggccccctgcccttcgcctgggacatcctgtccccccagttcttctacggctccaaggcgtacatcaagcaccccgccgacatccccgactacctcaagcagtccttccccgagggcttcaagtgggagcgcgtgatgaacttcgaggacggcggcgtggtgaccgtgacccaggactcctccctgcaggacggcaccctcatctaccacgtgaagttcatcggcgtgaacttcccctccgacggccccgtaatgcagaagaaaactctgggctgggagccctccactgagcgcaactacccccgcgacggcgtgctgaagggcgagaaccacatggcgctgaagctgaagggcggcggccactacctgtgtgagttcaagtccatctacatggccaagaagcccgtgaagctgcccggctaccactacgtggactacaagctcgacatcacctcccacaacgaggactacaccgtggtggagcagtacgagcgcgccgaggcccgccaccacctgttccagtgataataggggttcctgagtctgtgaccagaagaatagtttattctcaaaaaaaaaaaaaaaaaaaaaaaaaaaaaaaaaaaaaaaaaaaaaaaaaaaaaaaaaaaaaaaaaaaaaaaaaaaaaaaaaaaaaaaaaaaaaaaaaaaaagagacg

SEQ ID NO: 295 - DNA, 4720 bp, synthetic construct
  source 1..4720: mol_type = other DNA
taatacgactcactataagggagaataaactagtattcttctggtccccacagactcagagagaacccgccaccatgttcgtgttcctggtgctgctgcctctggtgtccagccagtgtgtgaacctgaccaccagaacacagctgcctccagcctacaccaacagctttaccagaggcgtgtactaccccgacaaggtgttcagatccagcgtgctgcactctacccaggacctgttcctgcctttcttcagcaacgtgacctggttccacgccatccacgtgtccggcaccaatggcaccaagagattcgacaaccccgtgctgcccttcaacgacggggtgtactttgccagcaccgagaagtccaacatcatcagaggctggatcttcggcaccacactggacagcaagacccagagcctgctgatcgtgaacaacgccaccaacgtggtcatcaaagtgtgcgagttccagttctgcaacgaccccttcctgggcgtctactaccacaagaacaacaagagctggatggaaagcgagttccgggtgtacagcagcgccaacaactgcaccttcgagtacgtgtcccagcctttcctgatggacctggaaggcaagcagggcaacttcaagaacctgcgcgagttcgtgtttaagaacatcgacggctacttcaagatctacagcaagcacacccctatcaacctcgtgcgggatctgcctcagggcttctctgctctggaacccctggtggatctgcccatcggcatcaacatcacccggtttcagacactgctggccctgcacagaagctacctgacacctggcgatagcagcagcggatggacagctggtgccgccgcttactatgtgggctacctgcagcctagaaccttcctgctgaagtacaacgagaacggcaccatcaccgacgccgtggattgtgctctggatcctctgagcgagacaaagtgcaccctgaagtccttcaccgtggaaaagggcatctaccagaccagcaacttccgggtgcagcccaccgaatccatcgtgcggttccccaatatcaccaatctgtgccccttcggcgaggtgttcaatgccaccagattcgcctctgtgtacgcctggaaccggaagcggatcagcaattgcgtggccgactactccgtgctgtacaactccgccagcttcagcaccttcaagtgctacggcgtgtcccctaccaagctgaacgacctgtgcttcacaaacgtgtacgccgacagcttcgtgatccggggagatgaagtgcggcagattgcccctggacagacaggcaagatcgccgactacaactacaagctgcccgacgacttcaccggctgtgtgattgcctggaacagcaacaacctggactccaaagtcggcggcaactacaattacctgtaccggctgttccggaagtccaatctgaagcccttcgagcgggacatctccaccgagatctatcaggccggcagcaccccttgtaacggcgtggaaggcttcaactgctacttcccactgcagtcctacggctttcagcccacaaatggcgtgggctatcagccctacagagtggtggtgctgagcttcgaactgctgcatgcccctgccacagtgtgcggccctaagaaaagcaccaatctcgtgaagaacaaatgcgtgaacttcaacttcaacggcctgaccggcaccggcgtgctgacagagagcaacaagaagttcctgccattccagcagtttggccgggatatcgccgataccacagacgccgttagagatccccagacactggaaatcctggacatcaccccttgcagcttcggcggagtgtctgtgatcacccctggcaccaacaccagcaatcaggtggcagtgctgtaccaggacgtgaactgtaccgaagtgcccgtggccattcacgccgatcagctgacacctacatggcgggtgtactccaccggcagcaatgtgtttcagaccagagccggctgtctgatcggagccgagcacgtgaacaatagctacgagtgcgacatccccatcggcgctggaatctgcgccagctaccagacacagacaaacagccctcggagagccagaagcgtggccagccagagcatcattgcctacacaatgtctctgggcgccgagaacagcgtggcctactccaacaactctatcgctatccccaccaacttcaccatcagcgtgaccacagagatcctgcctgtgtccatgaccaagaccagcgtggactgcaccatgtacatctgcggcgattccaccgagtgctccaacctgctgctgcagtacggcagcttctgcacccagctgaatagagccctgacagggatcgccgtggaacaggacaagaacacccaagaggtgttcgcccaagtgaagcagatctacaagacccctcctatcaaggacttcggcggcttcaatttcagccagattctgcccgatcctagcaagcccagcaagcggagcttcatcgaggacctgctgttcaacaaagtgacactggccgacgccggcttcatcaagcagtatggcgattgtctgggcgacattgccgccagggatctgatttgcgcccagaagtttaacggactgacagtgctgcctcctctgctgaccgatgagatgatcgcccagtacacatctgccctgctggccggcacaatcacaagcggctggacatttggagcaggcgccgctctgcagatcccctttgctatgcagatggcctaccggttcaacggcatcggagtgacccagaatgtgctgtacgagaaccagaagctgatcgccaaccagttcaacagcgccatcggcaagatccaggacagcctgagcagcacagcaagcgccctgggaaagctgcaggacgtggtcaaccagaatgcccaggcactgaacaccctggtcaagcagctgtcctccaacttcggcgccatcagctctgtgctgaacgatatcctgagcagactggaccctcctgaggccgaggtgcagatcgacagactgatcacaggcagactgcagagcctccagacatacgtgacccagcagctgatcagagccgccgagattagagcctctgccaatctggccgccaccaagatgtctgagtgtgtgctgggccagagcaagagagtggacttttgcggcaagggctaccacctgatgagcttccctcagtctgcccctcacggcgtggtgtttctgcacgtgacatatgtgcccgctcaagagaagaatttcaccaccgctccagccatctgccacgacggcaaagcccactttcctagagaaggcgtgttcgtgtccaacggcacccattggttcgtgacacagcggaacttctacgagccccagatcatcaccaccgacaacaccttcgtgtctggcaactgcgacgtcgtgatcggcattgtgaacaataccgtgtacgaccctctgcagcccgagctggacagcttcaaagaggaactggacaagtactttaagaaccacacaagccccgacgtggacctgggcgatatcagcggaatcaatgccagcgtcgtgaacatccagaaagagatcgaccggctgaacgaggtggccaagaatctgaacgagagcctgatcgacctgcaagaactggggaagtacgagcagtacatcaagtggccctggtacatctggctgggctttatcgccggactgattgccatcgtgatggtcacaatcatgctgtgttgcatgaccagctgctgtagctgcctgaagggctgttgtagctgtggcagctgctgcaagttcgacgaggacgattctgagcccgtgctgaagggcgtgaaactgcactacacagatagcactgagaacgtcatcaagcccttcatgcgcttcaaggtgcacatggagggctccgtgaacggccacgagttcgagatcgagggcgtgggcgagggcaagccctacgagggcacccagaccgccaagctgcaagtgaccaagggcggccccctgcccttcgcctgggacatcctgtccccccagttcttctacggctccaaggcgtacatcaagcaccccgccgacatccccgactacctcaagcagtccttccccgagggcttcaagtgggagcgcgtgatgaacttcgaggacggcggcgtggtgaccgtgacccaggactcctccctgcaggacggcaccctcatctaccacgtgaagttcatcggcgtgaacttcccctccgacggccccgtaatgcagaagaaaactctgggctgggagccctccactgagcgcaactacccccgcgacggcgtgctgaagggcgagaaccacatggcgctgaagctgaagggcggcggccactacctgtgtgagttcaagtccatctacatggccaagaagcccgtgaagctgcccggctaccactacgtggactacaagctcgacatcacctcccacaacgaggactacaccgtggtggagcagtacgagcgcgccgaggcccgccaccacctgttccagtgataataggggttctctagtctgtgggcagaagaatagtttattctcaaaaaaaaaaaaaaaaaaaaaaaaaaaaaaaaaaaaaaaaaaaaaaaaaaaaaaaaaaaaaaaaaaaaaaaaaaaaaaaaaaaaaaaaaaaaaaaaaaaaagagacg

SEQ ID NO: 296 - DNA, 4717 bp, synthetic construct
  source 1..4717: mol_type = other DNA
taatacgactcactataagggagaataaactagtattcttctggtccccacagactcagagagaacccgccaccatgttcgtgttcctggtgctgctgcctctggtgtccagccagtgtgtgaacctgaccaccagaacacagctgcctccagcctacaccaacagctttaccagaggcgtgtactaccccgacaaggtgttcagatccagcgtgctgcactctacccaggacctgttcctgcctttcttcagcaacgtgacctggttccacgccatccacgtgtccggcaccaatggcaccaagagattcgacaaccccgtgctgcccttcaacgacggggtgtactttgccagcaccgagaagtccaacatcatcagaggctggatcttcggcaccacactggacagcaagacccagagcctgctgatcgtgaacaacgccaccaacgtggtcatcaaagtgtgcgagttccagttctgcaacgaccccttcctgggcgtctactaccacaagaacaacaagagctggatggaaagcgagttccgggtgtacagcagcgccaacaactgcaccttcgagtacgtgtcccagcctttcctgatggacctggaaggcaagcagggcaacttcaagaacctgcgcgagttcgtgtttaagaacatcgacggctacttcaagatctacagcaagcacacccctatcaacctcgtgcgggatctgcctcagggcttctctgctctggaacccctggtggatctgcccatcggcatcaacatcacccggtttcagacactgctggccctgcacagaagctacctgacacctggcgatagcagcagcggatggacagctggtgccgccgcttactatgtgggctacctgcagcctagaaccttcctgctgaagtacaacgagaacggcaccatcaccgacgccgtggattgtgctctggatcctctgagcgagacaaagtgcaccctgaagtccttcaccgtggaaaagggcatctaccagaccagcaacttccgggtgcagcccaccgaatccatcgtgcggttccccaatatcaccaatctgtgccccttcggcgaggtgttcaatgccaccagattcgcctctgtgtacgcctggaaccggaagcggatcagcaattgcgtggccgactactccgtgctgtacaactccgccagcttcagcaccttcaagtgctacggcgtgtcccctaccaagctgaacgacctgtgcttcacaaacgtgtacgccgacagcttcgtgatccggggagatgaagtgcggcagattgcccctggacagacaggcaagatcgccgactacaactacaagctgcccgacgacttcaccggctgtgtgattgcctggaacagcaacaacctggactccaaagtcggcggcaactacaattacctgtaccggctgttccggaagtccaatctgaagcccttcgagcgggacatctccaccgagatctatcaggccggcagcaccccttgtaacggcgtggaaggcttcaactgctacttcccactgcagtcctacggctttcagcccacaaatggcgtgggctatcagccctacagagtggtggtgctgagcttcgaactgctgcatgcccctgccacagtgtgcggccctaagaaaagcaccaatctcgtgaagaacaaatgcgtgaacttcaacttcaacggcctgaccggcaccggcgtgctgacagagagcaacaagaagttcctgccattccagcagtttggccgggatatcgccgataccacagacgccgttagagatccccagacactggaaatcctggacatcaccccttgcagcttcggcggagtgtctgtgatcacccctggcaccaacaccagcaatcaggtggcagtgctgtaccaggacgtgaactgtaccgaagtgcccgtggccattcacgccgatcagctgacacctacatggcgggtgtactccaccggcagcaatgtgtttcagaccagagccggctgtctgatcggagccgagcacgtgaacaatagctacgagtgcgacatccccatcggcgctggaatctgcgccagctaccagacacagacaaacagccctcggagagccagaagcgtggccagccagagcatcattgcctacacaatgtctctgggcgccgagaacagcgtggcctactccaacaactctatcgctatccccaccaacttcaccatcagcgtgaccacagagatcctgcctgtgtccatgaccaagaccagcgtggactgcaccatgtacatctgcggcgattccaccgagtgctccaacctgctgctgcagtacggcagcttctgcacccagctgaatagagccctgacagggatcgccgtggaacaggacaagaacacccaagaggtgttcgcccaagtgaagcagatctacaagacccctcctatcaaggacttcggcggcttcaatttcagccagattctgcccgatcctagcaagcccagcaagcggagcttcatcgaggacctgctgttcaacaaagtgacactggccgacgccggcttcatcaagcagtatggcgattgtctgggcgacattgccgccagggatctgatttgcgcccagaagtttaacggactgacagtgctgcctcctctgctgaccgatgagatgatcgcccagtacacatctgccctgctggccggcacaatcacaagcggctggacatttggagcaggcgccgctctgcagatcccctttgctatgcagatggcctaccggttcaacggcatcggagtgacccagaatgtgctgtacgagaaccagaagctgatcgccaaccagttcaacagcgccatcggcaagatccaggacagcctgagcagcacagcaagcgccctgggaaagctgcaggacgtggtcaaccagaatgcccaggcactgaacaccctggtcaagcagctgtcctccaacttcggcgccatcagctctgtgctgaacgatatcctgagcagactggaccctcctgaggccgaggtgcagatcgacagactgatcacaggcagactgcagagcctccagacatacgtgacccagcagctgatcagagccgccgagattagagcctctgccaatctggccgccaccaagatgtctgagtgtgtgctgggccagagcaagagagtggacttttgcggcaagggctaccacctgatgagcttccctcagtctgcccctcacggcgtggtgtttctgcacgtgacatatgtgcccgctcaagagaagaatttcaccaccgctccagccatctgccacgacggcaaagcccactttcctagagaaggcgtgttcgtgtccaacggcacccattggttcgtgacacagcggaacttctacgagccccagatcatcaccaccgacaacaccttcgtgtctggcaactgcgacgtcgtgatcggcattgtgaacaataccgtgtacgaccctctgcagcccgagctggacagcttcaaagaggaactggacaagtactttaagaaccacacaagccccgacgtggacctgggcgatatcagcggaatcaatgccagcgtcgtgaacatccagaaagagatcgaccggctgaacgaggtggccaagaatctgaacgagagcctgatcgacctgcaagaactggggaagtacgagcagtacatcaagtggccctggtacatctggctgggctttatcgccggactgattgccatcgtgatggtcacaatcatgctgtgttgcatgaccagctgctgtagctgcctgaagggctgttgtagctgtggcagctgctgcaagttcgacgaggacgattctgagcccgtgctgaagggcgtgaaactgcactacacagatagcactgagaacgtcatcaagcccttcatgcgcttcaaggtgcacatggagggctccgtgaacggccacgagttcgagatcgagggcgtgggcgagggcaagccctacgagggcacccagaccgccaagctgcaagtgaccaagggcggccccctgcccttcgcctgggacatcctgtccccccagttcttctacggctccaaggcgtacatcaagcaccccgccgacatccccgactacctcaagcagtccttccccgagggcttcaagtgggagcgcgtgatgaacttcgaggacggcggcgtggtgaccgtgacccaggactcctccctgcaggacggcaccctcatctaccacgtgaagttcatcggcgtgaacttcccctccgacggccccgtaatgcagaagaaaactctgggctgggagccctccactgagcgcaactacccccgcgacggcgtgctgaagggcgagaaccacatggcgctgaagctgaagggcggcggccactacctgtgtgagttcaagtccatctacatggccaagaagcccgtgaagctgcccggctaccactacgtggactacaagctcgacatcacctcccacaacgaggactacaccgtggtggagcagtacgagcgcgccgaggcccgccaccacctgttccagtgataataggtctctctgatgtggggacaagaatactttattctcaaaaaaaaaaaaaaaaaaaaaaaaaaaaaaaaaaaaaaaaaaaaaaaaaaaaaaaaaaaaaaaaaaaaaaaaaaaaaaaaaaaaaaaaaaaaaaaaaaaaagagacg

SEQ ID NO: 297 - DNA, 4717 bp, synthetic construct
  source 1..4717: mol_type = other DNA
taatacgactcactataagggagaataaactagtattcttctggtccccacagactcagagagaacccgccaccatgttcgtgttcctggtgctgctgcctctggtgtccagccagtgtgtgaacctgaccaccagaacacagctgcctccagcctacaccaacagctttaccagaggcgtgtactaccccgacaaggtgttcagatccagcgtgctgcactctacccaggacctgttcctgcctttcttcagcaacgtgacctggttccacgccatccacgtgtccggcaccaatggcaccaagagattcgacaaccccgtgctgcccttcaacgacggggtgtactttgccagcaccgagaagtccaacatcatcagaggctggatcttcggcaccacactggacagcaagacccagagcctgctgatcgtgaacaacgccaccaacgtggtcatcaaagtgtgcgagttccagttctgcaacgaccccttcctgggcgtctactaccacaagaacaacaagagctggatggaaagcgagttccgggtgtacagcagcgccaacaactgcaccttcgagtacgtgtcccagcctttcctgatggacctggaaggcaagcagggcaacttcaagaacctgcgcgagttcgtgtttaagaacatcgacggctacttcaagatctacagcaagcacacccctatcaacctcgtgcgggatctgcctcagggcttctctgctctggaacccctggtggatctgcccatcggcatcaacatcacccggtttcagacactgctggccctgcacagaagctacctgacacctggcgatagcagcagcggatggacagctggtgccgccgcttactatgtgggctacctgcagcctagaaccttcctgctgaagtacaacgagaacggcaccatcaccgacgccgtggattgtgctctggatcctctgagcgagacaaagtgcaccctgaagtccttcaccgtggaaaagggcatctaccagaccagcaacttccgggtgcagcccaccgaatccatcgtgcggttccccaatatcaccaatctgtgccccttcggcgaggtgttcaatgccaccagattcgcctctgtgtacgcctggaaccggaagcggatcagcaattgcgtggccgactactccgtgctgtacaactccgccagcttcagcaccttcaagtgctacggcgtgtcccctaccaagctgaacgacctgtgcttcacaaacgtgtacgccgacagcttcgtgatccggggagatgaagtgcggcagattgcccctggacagacaggcaagatcgccgactacaactacaagctgcccgacgacttcaccggctgtgtgattgcctggaacagcaacaacctggactccaaagtcggcggcaactacaattacctgtaccggctgttccggaagtccaatctgaagcccttcgagcgggacatctccaccgagatctatcaggccggcagcaccccttgtaacggcgtggaaggcttcaactgctacttcccactgcagtcctacggctttcagcccacaaatggcgtgggctatcagccctacagagtggtggtgctgagcttcgaactgctgcatgcccctgccacagtgtgcggccctaagaaaagcaccaatctcgtgaagaacaaatgcgtgaacttcaacttcaacggcctgaccggcaccggcgtgctgacagagagcaacaagaagttcctgccattccagcagtttggccgggatatcgccgataccacagacgccgttagagatccccagacactggaaatcctggacatcaccccttgcagcttcggcggagtgtctgtgatcacccctggcaccaacaccagcaatcaggtggcagtgctgtaccaggacgtgaactgtaccgaagtgcccgtggccattcacgccgatcagctgacacctacatggcgggtgtactccaccggcagcaatgtgtttcagaccagagccggctgtctgatcggagccgagcacgtgaacaatagctacgagtgcgacatccccatcggcgctggaatctgcgccagctaccagacacagacaaacagccctcggagagccagaagcgtggccagccagagcatcattgcctacacaatgtctctgggcgccgagaacagcgtggcctactccaacaactctatcgctatccccaccaacttcaccatcagcgtgaccacagagatcctgcctgtgtccatgaccaagaccagcgtggactgcaccatgtacatctgcggcgattccaccgagtgctccaacctgctgctgcagtacggcagcttctgcacccagctgaatagagccctgacagggatcgccgtggaacaggacaagaacacccaagaggtgttcgcccaagtgaagcagatctacaagacccctcctatcaaggacttcggcggcttcaatttcagccagattctgcccgatcctagcaagcccagcaagcggagcttcatcgaggacctgctgttcaacaaagtgacactggccgacgccggcttcatcaagcagtatggcgattgtctgggcgacattgccgccagggatctgatttgcgcccagaagtttaacggactgacagtgctgcctcctctgctgaccgatgagatgatcgcccagtacacatctgccctgctggccggcacaatcacaagcggctggacatttggagcaggcgccgctctgcagatcccctttgctatgcagatggcctaccggttcaacggcatcggagtgacccagaatgtgctgtacgagaaccagaagctgatcgccaaccagttcaacagcgccatcggcaagatccaggacagcctgagcagcacagcaagcgccctgggaaagctgcaggacgtggtcaaccagaatgcccaggcactgaacaccctggtcaagcagctgtcctccaacttcggcgccatcagctctgtgctgaacgatatcctgagcagactggaccctcctgaggccgaggtgcagatcgacagactgatcacaggcagactgcagagcctccagacatacgtgacccagcagctgatcagagccgccgagattagagcctctgccaatctggccgccaccaagatgtctgagtgtgtgctgggccagagcaagagagtggacttttgcggcaagggctaccacctgatgagcttccctcagtctgcccctcacggcgtggtgtttctgcacgtgacatatgtgcccgctcaagagaagaatttcaccaccgctccagccatctgccacgacggcaaagcccactttcctagagaaggcgtgttcgtgtccaacggcacccattggttcgtgacacagcggaacttctacgagccccagatcatcaccaccgacaacaccttcgtgtctggcaactgcgacgtcgtgatcggcattgtgaacaataccgtgtacgaccctctgcagcccgagctggacagcttcaaagaggaactggacaagtactttaagaaccacacaagccccgacgtggacctgggcgatatcagcggaatcaatgccagcgtcgtgaacatccagaaagagatcgaccggctgaacgaggtggccaagaatctgaacgagagcctgatcgacctgcaagaactggggaagtacgagcagtacatcaagtggccctggtacatctggctgggctttatcgccggactgattgccatcgtgatggtcacaatcatgctgtgttgcatgaccagctgctgtagctgcctgaagggctgttgtagctgtggcagctgctgcaagttcgacgaggacgattctgagcccgtgctgaagggcgtgaaactgcactacacagatagcactgagaacgtcatcaagcccttcatgcgcttcaaggtgcacatggagggctccgtgaacggccacgagttcgagatcgagggcgtgggcgagggcaagccctacgagggcacccagaccgccaagctgcaagtgaccaagggcggccccctgcccttcgcctgggacatcctgtccccccagttcttctacggctccaaggcgtacatcaagcaccccgccgacatccccgactacctcaagcagtccttccccgagggcttcaagtgggagcgcgtgatgaacttcgaggacggcggcgtggtgaccgtgacccaggactcctccctgcaggacggcaccctcatctaccacgtgaagttcatcggcgtgaacttcccctccgacggccccgtaatgcagaagaaaactctgggctgggagccctccactgagcgcaactacccccgcgacggcgtgctgaagggcgagaaccacatggcgctgaagctgaagggcggcggccactacctgtgtgagttcaagtccatctacatggccaagaagcccgtgaagctgcccggctaccactacgtggactacaagctcgacatcacctcccacaacgaggactacaccgtggtggagcagtacgagcgcgccgaggcccgccaccacctgttccagtgataataggggtctctgagttggggaccagaatactttattctcaaaaaaaaaaaaaaaaaaaaaaaaaaaaaaaaaaaaaaaaaaaaaaaaaaaaaaaaaaaaaaaaaaaaaaaaaaaaaaaaaaaaaaaaaaaaaaaaaaaaagagacg

SEQ ID NO: 298 - DNA, 4723 bp, synthetic construct
  source 1..4723: mol_type = other DNA
taatacgactcactataagggagaataaactagtattcttctggtccccacagactcagagagaacccgccaccatgttcgtgttcctggtgctgctgcctctggtgtccagccagtgtgtgaacctgaccaccagaacacagctgcctccagcctacaccaacagctttaccagaggcgtgtactaccccgacaaggtgttcagatccagcgtgctgcactctacccaggacctgttcctgcctttcttcagcaacgtgacctggttccacgccatccacgtgtccggcaccaatggcaccaagagattcgacaaccccgtgctgcccttcaacgacggggtgtactttgccagcaccgagaagtccaacatcatcagaggctggatcttcggcaccacactggacagcaagacccagagcctgctgatcgtgaacaacgccaccaacgtggtcatcaaagtgtgcgagttccagttctgcaacgaccccttcctgggcgtctactaccacaagaacaacaagagctggatggaaagcgagttccgggtgtacagcagcgccaacaactgcaccttcgagtacgtgtcccagcctttcctgatggacctggaaggcaagcagggcaacttcaagaacctgcgcgagttcgtgtttaagaacatcgacggctacttcaagatctacagcaagcacacccctatcaacctcgtgcgggatctgcctcagggcttctctgctctggaacccctggtggatctgcccatcggcatcaacatcacccggtttcagacactgctggccctgcacagaagctacctgacacctggcgatagcagcagcggatggacagctggtgccgccgcttactatgtgggctacctgcagcctagaaccttcctgctgaagtacaacgagaacggcaccatcaccgacgccgtggattgtgctctggatcctctgagcgagacaaagtgcaccctgaagtccttcaccgtggaaaagggcatctaccagaccagcaacttccgggtgcagcccaccgaatccatcgtgcggttccccaatatcaccaatctgtgccccttcggcgaggtgttcaatgccaccagattcgcctctgtgtacgcctggaaccggaagcggatcagcaattgcgtggccgactactccgtgctgtacaactccgccagcttcagcaccttcaagtgctacggcgtgtcccctaccaagctgaacgacctgtgcttcacaaacgtgtacgccgacagcttcgtgatccggggagatgaagtgcggcagattgcccctggacagacaggcaagatcgccgactacaactacaagctgcccgacgacttcaccggctgtgtgattgcctggaacagcaacaacctggactccaaagtcggcggcaactacaattacctgtaccggctgttccggaagtccaatctgaagcccttcgagcgggacatctccaccgagatctatcaggccggcagcaccccttgtaacggcgtggaaggcttcaactgctacttcccactgcagtcctacggctttcagcccacaaatggcgtgggctatcagccctacagagtggtggtgctgagcttcgaactgctgcatgcccctgccacagtgtgcggccctaagaaaagcaccaatctcgtgaagaacaaatgcgtgaacttcaacttcaacggcctgaccggcaccggcgtgctgacagagagcaacaagaagttcctgccattccagcagtttggccgggatatcgccgataccacagacgccgttagagatccccagacactggaaatcctggacatcaccccttgcagcttcggcggagtgtctgtgatcacccctggcaccaacaccagcaatcaggtggcagtgctgtaccaggacgtgaactgtaccgaagtgcccgtggccattcacgccgatcagctgacacctacatggcgggtgtactccaccggcagcaatgtgtttcagaccagagccggctgtctgatcggagccgagcacgtgaacaatagctacgagtgcgacatccccatcggcgctggaatctgcgccagctaccagacacagacaaacagccctcggagagccagaagcgtggccagccagagcatcattgcctacacaatgtctctgggcgccgagaacagcgtggcctactccaacaactctatcgctatccccaccaacttcaccatcagcgtgaccacagagatcctgcctgtgtccatgaccaagaccagcgtggactgcaccatgtacatctgcggcgattccaccgagtgctccaacctgctgctgcagtacggcagcttctgcacccagctgaatagagccctgacagggatcgccgtggaacaggacaagaacacccaagaggtgttcgcccaagtgaagcagatctacaagacccctcctatcaaggacttcggcggcttcaatttcagccagattctgcccgatcctagcaagcccagcaagcggagcttcatcgaggacctgctgttcaacaaagtgacactggccgacgccggcttcatcaagcagtatggcgattgtctgggcgacattgccgccagggatctgatttgcgcccagaagtttaacggactgacagtgctgcctcctctgctgaccgatgagatgatcgcccagtacacatctgccctgctggccggcacaatcacaagcggctggacatttggagcaggcgccgctctgcagatcccctttgctatgcagatggcctaccggttcaacggcatcggagtgacccagaatgtgctgtacgagaaccagaagctgatcgccaaccagttcaacagcgccatcggcaagatccaggacagcctgagcagcacagcaagcgccctgggaaagctgcaggacgtggtcaaccagaatgcccaggcactgaacaccctggtcaagcagctgtcctccaacttcggcgccatcagctctgtgctgaacgatatcctgagcagactggaccctcctgaggccgaggtgcagatcgacagactgatcacaggcagactgcagagcctccagacatacgtgacccagcagctgatcagagccgccgagattagagcctctgccaatctggccgccaccaagatgtctgagtgtgtgctgggccagagcaagagagtggacttttgcggcaagggctaccacctgatgagcttccctcagtctgcccctcacggcgtggtgtttctgcacgtgacatatgtgcccgctcaagagaagaatttcaccaccgctccagccatctgccacgacggcaaagcccactttcctagagaaggcgtgttcgtgtccaacggcacccattggttcgtgacacagcggaacttctacgagccccagatcatcaccaccgacaacaccttcgtgtctggcaactgcgacgtcgtgatcggcattgtgaacaataccgtgtacgaccctctgcagcccgagctggacagcttcaaagaggaactggacaagtactttaagaaccacacaagccccgacgtggacctgggcgatatcagcggaatcaatgccagcgtcgtgaacatccagaaagagatcgaccggctgaacgaggtggccaagaatctgaacgagagcctgatcgacctgcaagaactggggaagtacgagcagtacatcaagtggccctggtacatctggctgggctttatcgccggactgattgccatcgtgatggtcacaatcatgctgtgttgcatgaccagctgctgtagctgcctgaagggctgttgtagctgtggcagctgctgcaagttcgacgaggacgattctgagcccgtgctgaagggcgtgaaactgcactacacagatagcactgagaacgtcatcaagcccttcatgcgcttcaaggtgcacatggagggctccgtgaacggccacgagttcgagatcgagggcgtgggcgagggcaagccctacgagggcacccagaccgccaagctgcaagtgaccaagggcggccccctgcccttcgcctgggacatcctgtccccccagttcttctacggctccaaggcgtacatcaagcaccccgccgacatccccgactacctcaagcagtccttccccgagggcttcaagtgggagcgcgtgatgaacttcgaggacggcggcgtggtgaccgtgacccaggactcctccctgcaggacggcaccctcatctaccacgtgaagttcatcggcgtgaacttcccctccgacggccccgtaatgcagaagaaaactctgggctgggagccctccactgagcgcaactacccccgcgacggcgtgctgaagggcgagaaccacatggcgctgaagctgaagggcggcggccactacctgtgtgagttcaagtccatctacatggccaagaagcccgtgaagctgcccggctaccactacgtggactacaagctcgacatcacctcccacaacgaggactacaccgtggtggagcagtacgagcgcgccgaggcccgccaccacctgttccagtgataataggggttctctctgaggtggggaccagaagactagtttattctcaaaaaaaaaaaaaaaaaaaaaaaaaaaaaaaaaaaaaaaaaaaaaaaaaaaaaaaaaaaaaaaaaaaaaaaaaaaaaaaaaaaaaaaaaaaaaaaaaaaaagagacg

SEQ ID NO: 299 - DNA, 4720 bp, synthetic construct
  source 1..4720: mol_type = other DNA
taatacgactcactataagggagaataaactagtattcttctggtccccacagactcagagagaacccgccaccatgttcgtgttcctggtgctgctgcctctggtgtccagccagtgtgtgaacctgaccaccagaacacagctgcctccagcctacaccaacagctttaccagaggcgtgtactaccccgacaaggtgttcagatccagcgtgctgcactctacccaggacctgttcctgcctttcttcagcaacgtgacctggttccacgccatccacgtgtccggcaccaatggcaccaagagattcgacaaccccgtgctgcccttcaacgacggggtgtactttgccagcaccgagaagtccaacatcatcagaggctggatcttcggcaccacactggacagcaagacccagagcctgctgatcgtgaacaacgccaccaacgtggtcatcaaagtgtgcgagttccagttctgcaacgaccccttcctgggcgtctactaccacaagaacaacaagagctggatggaaagcgagttccgggtgtacagcagcgccaacaactgcaccttcgagtacgtgtcccagcctttcctgatggacctggaaggcaagcagggcaacttcaagaacctgcgcgagttcgtgtttaagaacatcgacggctacttcaagatctacagcaagcacacccctatcaacctcgtgcgggatctgcctcagggcttctctgctctggaacccctggtggatctgcccatcggcatcaacatcacccggtttcagacactgctggccctgcacagaagctacctgacacctggcgatagcagcagcggatggacagctggtgccgccgcttactatgtgggctacctgcagcctagaaccttcctgctgaagtacaacgagaacggcaccatcaccgacgccgtggattgtgctctggatcctctgagcgagacaaagtgcaccctgaagtccttcaccgtggaaaagggcatctaccagaccagcaacttccgggtgcagcccaccgaatccatcgtgcggttccccaatatcaccaatctgtgccccttcggcgaggtgttcaatgccaccagattcgcctctgtgtacgcctggaaccggaagcggatcagcaattgcgtggccgactactccgtgctgtacaactccgccagcttcagcaccttcaagtgctacggcgtgtcccctaccaagctgaacgacctgtgcttcacaaacgtgtacgccgacagcttcgtgatccggggagatgaagtgcggcagattgcccctggacagacaggcaagatcgccgactacaactacaagctgcccgacgacttcaccggctgtgtgattgcctggaacagcaacaacctggactccaaagtcggcggcaactacaattacctgtaccggctgttccggaagtccaatctgaagcccttcgagcgggacatctccaccgagatctatcaggccggcagcaccccttgtaacggcgtggaaggcttcaactgctacttcccactgcagtcctacggctttcagcccacaaatggcgtgggctatcagccctacagagtggtggtgctgagcttcgaactgctgcatgcccctgccacagtgtgcggccctaagaaaagcaccaatctcgtgaagaacaaatgcgtgaacttcaacttcaacggcctgaccggcaccggcgtgctgacagagagcaacaagaagttcctgccattccagcagtttggccgggatatcgccgataccacagacgccgttagagatccccagacactggaaatcctggacatcaccccttgcagcttcggcggagtgtctgtgatcacccctggcaccaacaccagcaatcaggtggcagtgctgtaccaggacgtgaactgtaccgaagtgcccgtggccattcacgccgatcagctgacacctacatggcgggtgtactccaccggcagcaatgtgtttcagaccagagccggctgtctgatcggagccgagcacgtgaacaatagctacgagtgcgacatccccatcggcgctggaatctgcgccagctaccagacacagacaaacagccctcggagagccagaagcgtggccagccagagcatcattgcctacacaatgtctctgggcgccgagaacagcgtggcctactccaacaactctatcgctatccccaccaacttcaccatcagcgtgaccacagagatcctgcctgtgtccatgaccaagaccagcgtggactgcaccatgtacatctgcggcgattccaccgagtgctccaacctgctgctgcagtacggcagcttctgcacccagctgaatagagccctgacagggatcgccgtggaacaggacaagaacacccaagaggtgttcgcccaagtgaagcagatctacaagacccctcctatcaaggacttcggcggcttcaatttcagccagattctgcccgatcctagcaagcccagcaagcggagcttcatcgaggacctgctgttcaacaaagtgacactggccgacgccggcttcatcaagcagtatggcgattgtctgggcgacattgccgccagggatctgatttgcgcccagaagtttaacggactgacagtgctgcctcctctgctgaccgatgagatgatcgcccagtacacatctgccctgctggccggcacaatcacaagcggctggacatttggagcaggcgccgctctgcagatcccctttgctatgcagatggcctaccggttcaacggcatcggagtgacccagaatgtgctgtacgagaaccagaagctgatcgccaaccagttcaacagcgccatcggcaagatccaggacagcctgagcagcacagcaagcgccctgggaaagctgcaggacgtggtcaaccagaatgcccaggcactgaacaccctggtcaagcagctgtcctccaacttcggcgccatcagctctgtgctgaacgatatcctgagcagactggaccctcctgaggccgaggtgcagatcgacagactgatcacaggcagactgcagagcctccagacatacgtgacccagcagctgatcagagccgccgagattagagcctctgccaatctggccgccaccaagatgtctgagtgtgtgctgggccagagcaagagagtggacttttgcggcaagggctaccacctgatgagcttccctcagtctgcccctcacggcgtggtgtttctgcacgtgacatatgtgcccgctcaagagaagaatttcaccaccgctccagccatctgccacgacggcaaagcccactttcctagagaaggcgtgttcgtgtccaacggcacccattggttcgtgacacagcggaacttctacgagccccagatcatcaccaccgacaacaccttcgtgtctggcaactgcgacgtcgtgatcggcattgtgaacaataccgtgtacgaccctctgcagcccgagctggacagcttcaaagaggaactggacaagtactttaagaaccacacaagccccgacgtggacctgggcgatatcagcggaatcaatgccagcgtcgtgaacatccagaaagagatcgaccggctgaacgaggtggccaagaatctgaacgagagcctgatcgacctgcaagaactggggaagtacgagcagtacatcaagtggccctggtacatctggctgggctttatcgccggactgattgccatcgtgatggtcacaatcatgctgtgttgcatgaccagctgctgtagctgcctgaagggctgttgtagctgtggcagctgctgcaagttcgacgaggacgattctgagcccgtgctgaagggcgtgaaactgcactacacagatagcactgagaacgtcatcaagcccttcatgcgcttcaaggtgcacatggagggctccgtgaacggccacgagttcgagatcgagggcgtgggcgagggcaagccctacgagggcacccagaccgccaagctgcaagtgaccaagggcggccccctgcccttcgcctgggacatcctgtccccccagttcttctacggctccaaggcgtacatcaagcaccccgccgacatccccgactacctcaagcagtccttccccgagggcttcaagtgggagcgcgtgatgaacttcgaggacggcggcgtggtgaccgtgacccaggactcctccctgcaggacggcaccctcatctaccacgtgaagttcatcggcgtgaacttcccctccgacggccccgtaatgcagaagaaaactctgggctgggagccctccactgagcgcaactacccccgcgacggcgtgctgaagggcgagaaccacatggcgctgaagctgaagggcggcggccactacctgtgtgagttcaagtccatctacatggccaagaagcccgtgaagctgcccggctaccactacgtggactacaagctcgacatcacctcccacaacgaggactacaccgtggtggagcagtacgagcgcgccgaggcccgccaccacctgttccagtgataataggtctctctgagtctgggaccagaagaatagtttattctcaaaaaaaaaaaaaaaaaaaaaaaaaaaaaaaaaaaaaaaaaaaaaaaaaaaaaaaaaaaaaaaaaaaaaaaaaaaaaaaaaaaaaaaaaaaaaaaaaaaaagagacg

SEQ ID NO: 300 - DNA, 4976 bp, synthetic construct
  source 1..4976: mol_type = other DNA
taatacgactcactataagggagaataaactagtattcttctggtccccacagactcagagagaacccgccaccatgttcgtgttcctggtgctgctgcctctggtgtccagccagtgtgtgaacctgaccaccagaacacagctgcctccagcctacaccaacagctttaccagaggcgtgtactaccccgacaaggtgttcagatccagcgtgctgcactctacccaggacctgttcctgcctttcttcagcaacgtgacctggttccacgccatccacgtgtccggcaccaatggcaccaagagattcgacaaccccgtgctgcccttcaacgacggggtgtactttgccagcaccgagaagtccaacatcatcagaggctggatcttcggcaccacactggacagcaagacccagagcctgctgatcgtgaacaacgccaccaacgtggtcatcaaagtgtgcgagttccagttctgcaacgaccccttcctgggcgtctactaccacaagaacaacaagagctggatggaaagcgagttccgggtgtacagcagcgccaacaactgcaccttcgagtacgtgtcccagcctttcctgatggacctggaaggcaagcagggcaacttcaagaacctgcgcgagttcgtgtttaagaacatcgacggctacttcaagatctacagcaagcacacccctatcaacctcgtgcgggatctgcctcagggcttctctgctctggaacccctggtggatctgcccatcggcatcaacatcacccggtttcagacactgctggccctgcacagaagctacctgacacctggcgatagcagcagcggatggacagctggtgccgccgcttactatgtgggctacctgcagcctagaaccttcctgctgaagtacaacgagaacggcaccatcaccgacgccgtggattgtgctctggatcctctgagcgagacaaagtgcaccctgaagtccttcaccgtggaaaagggcatctaccagaccagcaacttccgggtgcagcccaccgaatccatcgtgcggttccccaatatcaccaatctgtgccccttcggcgaggtgttcaatgccaccagattcgcctctgtgtacgcctggaaccggaagcggatcagcaattgcgtggccgactactccgtgctgtacaactccgccagcttcagcaccttcaagtgctacggcgtgtcccctaccaagctgaacgacctgtgcttcacaaacgtgtacgccgacagcttcgtgatccggggagatgaagtgcggcagattgcccctggacagacaggcaagatcgccgactacaactacaagctgcccgacgacttcaccggctgtgtgattgcctggaacagcaacaacctggactccaaagtcggcggcaactacaattacctgtaccggctgttccggaagtccaatctgaagcccttcgagcgggacatctccaccgagatctatcaggccggcagcaccccttgtaacggcgtggaaggcttcaactgctacttcccactgcagtcctacggctttcagcccacaaatggcgtgggctatcagccctacagagtggtggtgctgagcttcgaactgctgcatgcccctgccacagtgtgcggccctaagaaaagcaccaatctcgtgaagaacaaatgcgtgaacttcaacttcaacggcctgaccggcaccggcgtgctgacagagagcaacaagaagttcctgccattccagcagtttggccgggatatcgccgataccacagacgccgttagagatccccagacactggaaatcctggacatcaccccttgcagcttcggcggagtgtctgtgatcacccctggcaccaacaccagcaatcaggtggcagtgctgtaccaggacgtgaactgtaccgaagtgcccgtggccattcacgccgatcagctgacacctacatggcgggtgtactccaccggcagcaatgtgtttcagaccagagccggctgtctgatcggagccgagcacgtgaacaatagctacgagtgcgacatccccatcggcgctggaatctgcgccagctaccagacacagacaaacagccctcggagagccagaagcgtggccagccagagcatcattgcctacacaatgtctctgggcgccgagaacagcgtggcctactccaacaactctatcgctatccccaccaacttcaccatcagcgtgaccacagagatcctgcctgtgtccatgaccaagaccagcgtggactgcaccatgtacatctgcggcgattccaccgagtgctccaacctgctgctgcagtacggcagcttctgcacccagctgaatagagccctgacagggatcgccgtggaacaggacaagaacacccaagaggtgttcgcccaagtgaagcagatctacaagacccctcctatcaaggacttcggcggcttcaatttcagccagattctgcccgatcctagcaagcccagcaagcggagcttcatcgaggacctgctgttcaacaaagtgacactggccgacgccggcttcatcaagcagtatggcgattgtctgggcgacattgccgccagggatctgatttgcgcccagaagtttaacggactgacagtgctgcctcctctgctgaccgatgagatgatcgcccagtacacatctgccctgctggccggcacaatcacaagcggctggacatttggagcaggcgccgctctgcagatcccctttgctatgcagatggcctaccggttcaacggcatcggagtgacccagaatgtgctgtacgagaaccagaagctgatcgccaaccagttcaacagcgccatcggcaagatccaggacagcctgagcagcacagcaagcgccctgggaaagctgcaggacgtggtcaaccagaatgcccaggcactgaacaccctggtcaagcagctgtcctccaacttcggcgccatcagctctgtgctgaacgatatcctgagcagactggaccctcctgaggccgaggtgcagatcgacagactgatcacaggcagactgcagagcctccagacatacgtgacccagcagctgatcagagccgccgagattagagcctctgccaatctggccgccaccaagatgtctgagtgtgtgctgggccagagcaagagagtggacttttgcggcaagggctaccacctgatgagcttccctcagtctgcccctcacggcgtggtgtttctgcacgtgacatatgtgcccgctcaagagaagaatttcaccaccgctccagccatctgccacgacggcaaagcccactttcctagagaaggcgtgttcgtgtccaacggcacccattggttcgtgacacagcggaacttctacgagccccagatcatcaccaccgacaacaccttcgtgtctggcaactgcgacgtcgtgatcggcattgtgaacaataccgtgtacgaccctctgcagcccgagctggacagcttcaaagaggaactggacaagtactttaagaaccacacaagccccgacgtggacctgggcgatatcagcggaatcaatgccagcgtcgtgaacatccagaaagagatcgaccggctgaacgaggtggccaagaatctgaacgagagcctgatcgacctgcaagaactggggaagtacgagcagtacatcaagtggccctggtacatctggctgggctttatcgccggactgattgccatcgtgatggtcacaatcatgctgtgttgcatgaccagctgctgtagctgcctgaagggctgttgtagctgtggcagctgctgcaagttcgacgaggacgattctgagcccgtgctgaagggcgtgaaactgcactacacagatagcactgagaacgtcatcaagcccttcatgcgcttcaaggtgcacatggagggctccgtgaacggccacgagttcgagatcgagggcgtgggcgagggcaagccctacgagggcacccagaccgccaagctgcaagtgaccaagggcggccccctgcccttcgcctgggacatcctgtccccccagttcttctacggctccaaggcgtacatcaagcaccccgccgacatccccgactacctcaagcagtccttccccgagggcttcaagtgggagcgcgtgatgaacttcgaggacggcggcgtggtgaccgtgacccaggactcctccctgcaggacggcaccctcatctaccacgtgaagttcatcggcgtgaacttcccctccgacggccccgtaatgcagaagaaaactctgggctgggagccctccactgagcgcaactacccccgcgacggcgtgctgaagggcgagaaccacatggcgctgaagctgaagggcggcggccactacctgtgtgagttcaagtccatctacatggccaagaagcccgtgaagctgcccggctaccactacgtggactacaagctcgacatcacctcccacaacgaggactacaccgtggtggagcagtacgagcgcgccgaggcccgccaccacctgttccagtgataatagctcgagctggtactgcatgcacgcaatgctagctgcccctttcccgtcctgggtaccccgagtctcccccgacctcgggtcccaggtatgctcccacctccacctgccccactcaccacctctgctagttccagacacctcccaagcacgcagcaatgcagctcaaaacgcttagcctagccacacccccacgggaaacagcagtgattaacctttagcaataaacgaaagtttaactaagctatactaaccccagggttggtcaatttcgtgccagccacaccctggagctagcaaaaaaaaaaaaaaaaaaaaaaaaaaaaaaaaaaaaaaaaaaaaaaaaaaaaaaaaaaaaaaaaaaaaaaaaaaaaaaaaaaaaaaaaaaaaaaaaaaaaagagacg

SEQ ID NO: 301 - DNA, 905 bp, synthetic construct
  source 1..905: mol_type = other DNA
taatacgactcactataagggagaataatagtattcctggtccccagactcagagaacccgccaccatggatagcactgagaacgtcatcaagcccttcatgcgcttcaaggtgcacatggagggctccgtgaacggccacgagttcgagatcgagggcgtgggcgagggcaagccctacgagggcacccagaccgccaagctgcaagtgaccaagggcggccccctgcccttcgcctgggacatcctgtccccccagttcttctacggctccaaggcgtacatcaagcaccccgccgacatccccgactacctcaagcagtccttccccgagggcttcaagtgggagcgcgtgatgaacttcgaggacggcggcgtggtgaccgtgacccaggactcctccctgcaggacggcaccctcatctaccacgtgaagttcatcggcgtgaacttcccctccgacggccccgtaatgcagaagaaaactctgggctgggagccctccactgagcgcaactacccccgcgacggcgtgctgaagggcgagaaccacatggcgctgaagctgaagggcggcggccactacctgtgtgagttcaagtccatctacatggccaagaagcccgtgaagctgcccggctaccactacgtggactacaagctcgacatcacctcccacaacgaggactacaccgtggtggagcagtacgagcgcgccgaggcccgccaccacctgttccagtgataataggggttctctctgagtctgtggggaccagaagaatactagtttattctcaaaaaaaaaaaaaaaaaaaaaaaaaaaaaaaaaaaaaaaaaaaaaaaaaaaaaaaaaaaaaaaaaaaaaaaaaaaaaaaaaaaaaaaaaaaaaaaaaaaaagagacg

SEQ ID NO: 302 - DNA, 907 bp, synthetic construct
  source 1..907: mol_type = other DNA
taatacgactcactataagggagaataaactagtattcttctggtccccacagactcagagagaacccgccaccatggatagcactgagaacgtcatcaagcccttcatgcgcttcaaggtgcacatggagggctccgtgaacggccacgagttcgagatcgagggcgtgggcgagggcaagccctacgagggcacccagaccgccaagctgcaagtgaccaagggcggccccctgcccttcgcctgggacatcctgtccccccagttcttctacggctccaaggcgtacatcaagcaccccgccgacatccccgactacctcaagcagtccttccccgagggcttcaagtgggagcgcgtgatgaacttcgaggacggcggcgtggtgaccgtgacccaggactcctccctgcaggacggcaccctcatctaccacgtgaagttcatcggcgtgaacttcccctccgacggccccgtaatgcagaagaaaactctgggctgggagccctccactgagcgcaactacccccgcgacggcgtgctgaagggcgagaaccacatggcgctgaagctgaagggcggcggccactacctgtgtgagttcaagtccatctacatggccaagaagcccgtgaagctgcccggctaccactacgtggactacaagctcgacatcacctcccacaacgaggactacaccgtggtggagcagtacgagcgcgccgaggcccgccaccacctgttccagtgataataggggttctctgagtctggggaccaggaatactagtttattctcaaaaaaaaaaaaaaaaaaaaaaaaaaaaaaaaaaaaaaaaaaaaaaaaaaaaaaaaaaaaaaaaaaaaaaaaaaaaaaaaaaaaaaaaaaaaaaaaaaaaagagacg

SEQ ID NO: 303 - DNA, 907 bp, synthetic construct
  source 1..907: mol_type = other DNA
taatacgactcactataagggagaataaactagtattcttctggtccccacagactcagagagaacccgccaccatggatagcactgagaacgtcatcaagcccttcatgcgcttcaaggtgcacatggagggctccgtgaacggccacgagttcgagatcgagggcgtgggcgagggcaagccctacgagggcacccagaccgccaagctgcaagtgaccaagggcggccccctgcccttcgcctgggacatcctgtccccccagttcttctacggctccaaggcgtacatcaagcaccccgccgacatccccgactacctcaagcagtccttccccgagggcttcaagtgggagcgcgtgatgaacttcgaggacggcggcgtggtgaccgtgacccaggactcctccctgcaggacggcaccctcatctaccacgtgaagttcatcggcgtgaacttcccctccgacggccccgtaatgcagaagaaaactctgggctgggagccctccactgagcgcaactacccccgcgacggcgtgctgaagggcgagaaccacatggcgctgaagctgaagggcggcggccactacctgtgtgagttcaagtccatctacatggccaagaagcccgtgaagctgcccggctaccactacgtggactacaagctcgacatcacctcccacaacgaggactacaccgtggtggagcagtacgagcgcgccgaggcccgccaccacctgttccagtgataataggggttctctgagtctggggaccagaagaatactattattctcaaaaaaaaaaaaaaaaaaaaaaaaaaaaaaaaaaaaaaaaaaaaaaaaaaaaaaaaaaaaaaaaaaaaaaaaaaaaaaaaaaaaaaaaaaaaaaaaaaaaagagacg

SEQ ID NO: 304 - DNA, 907 bp, synthetic construct
  source 1..907: mol_type = other DNA
taatacgactcactataagggagaataaactagtattcttctggtccccacagactcagagagaacccgccaccatggatagcactgagaacgtcatcaagcccttcatgcgcttcaaggtgcacatggagggctccgtgaacggccacgagttcgagatcgagggcgtgggcgagggcaagccctacgagggcacccagaccgccaagctgcaagtgaccaagggcggccccctgcccttcgcctgggacatcctgtccccccagttcttctacggctccaaggcgtacatcaagcaccccgccgacatccccgactacctcaagcagtccttccccgagggcttcaagtgggagcgcgtgatgaacttcgaggacggcggcgtggtgaccgtgacccaggactcctccctgcaggacggcaccctcatctaccacgtgaagttcatcggcgtgaacttcccctccgacggccccgtaatgcagaagaaaactctgggctgggagccctccactgagcgcaactacccccgcgacggcgtgctgaagggcgagaaccacatggcgctgaagctgaagggcggcggccactacctgtgtgagttcaagtccatctacatggccaagaagcccgtgaagctgcccggctaccactacgtggactacaagctcgacatcacctcccacaacgaggactacaccgtggtggagcagtacgagcgcgccgaggcccgccaccacctgttccagtgataataggggttctctgagtctgtggggaccaggaatactattattctcaaaaaaaaaaaaaaaaaaaaaaaaaaaaaaaaaaaaaaaaaaaaaaaaaaaaaaaaaaaaaaaaaaaaaaaaaaaaaaaaaaaaaaaaaaaaaaaaaaaaagagacg

SEQ ID NO: 305 - DNA, 907 bp, synthetic construct
  source 1..907: mol_type = other DNA
taatacgactcactataagggagaataaactagtattcttctggtccccacagactcagagagaacccgccaccatggatagcactgagaacgtcatcaagcccttcatgcgcttcaaggtgcacatggagggctccgtgaacggccacgagttcgagatcgagggcgtgggcgagggcaagccctacgagggcacccagaccgccaagctgcaagtgaccaagggcggccccctgcccttcgcctgggacatcctgtccccccagttcttctacggctccaaggcgtacatcaagcaccccgccgacatccccgactacctcaagcagtccttccccgagggcttcaagtgggagcgcgtgatgaacttcgaggacggcggcgtggtgaccgtgacccaggactcctccctgcaggacggcaccctcatctaccacgtgaagttcatcggcgtgaacttcccctccgacggccccgtaatgcagaagaaaactctgggctgggagccctccactgagcgcaactacccccgcgacggcgtgctgaagggcgagaaccacatggcgctgaagctgaagggcggcggccactacctgtgtgagttcaagtccatctacatggccaagaagcccgtgaagctgcccggctaccactacgtggactacaagctcgacatcacctcccacaacgaggactacaccgtggtggagcagtacgagcgcgccgaggcccgccaccacctgttccagtgataataggggttctctctgagtctggggaccaggaatactattattctcaaaaaaaaaaaaaaaaaaaaaaaaaaaaaaaaaaaaaaaaaaaaaaaaaaaaaaaaaaaaaaaaaaaaaaaaaaaaaaaaaaaaaaaaaaaaaaaaaaaaagagacg

SEQ ID NO: 306 - DNA, 907 bp, synthetic construct
  source 1..907: mol_type = other DNA
taatacgactcactataagggagaataaactagtattcctggtccccagactcagagaacccgccaccatggatagcactgagaacgtcatcaagcccttcatgcgcttcaaggtgcacatggagggctccgtgaacggccacgagttcgagatcgagggcgtgggcgagggcaagccctacgagggcacccagaccgccaagctgcaagtgaccaagggcggccccctgcccttcgcctgggacatcctgtccccccagttcttctacggctccaaggcgtacatcaagcaccccgccgacatccccgactacctcaagcagtccttccccgagggcttcaagtgggagcgcgtgatgaacttcgaggacggcggcgtggtgaccgtgacccaggactcctccctgcaggacggcaccctcatctaccacgtgaagttcatcggcgtgaacttcccctccgacggccccgtaatgcagaagaaaactctgggctgggagccctccactgagcgcaactacccccgcgacggcgtgctgaagggcgagaaccacatggcgctgaagctgaagggcggcggccactacctgtgtgagttcaagtccatctacatggccaagaagcccgtgaagctgcccggctaccactacgtggactacaagctcgacatcacctcccacaacgaggactacaccgtggtggagcagtacgagcgcgccgaggcccgccaccacctgttccagtgataataggggttctctctgagtctgtggggaccagaagaatactagtttattctcaaaaaaaaaaaaaaaaaaaaaaaaaaaaaaaaaaaaaaaaaaaaaaaaaaaaaaaaaaaaaaaaaaaaaaaaaaaaaaaaaaaaaaaaaaaaaaaaaaaaagagacg

SEQ ID NO: 307 - DNA, 907 bp, synthetic construct
  source 1..907: mol_type = other DNA
taatacgactcactataagggagaataatagtattcttctggtccccagactcagagaacccgccaccatggatagcactgagaacgtcatcaagcccttcatgcgcttcaaggtgcacatggagggctccgtgaacggccacgagttcgagatcgagggcgtgggcgagggcaagccctacgagggcacccagaccgccaagctgcaagtgaccaagggcggccccctgcccttcgcctgggacatcctgtccccccagttcttctacggctccaaggcgtacatcaagcaccccgccgacatccccgactacctcaagcagtccttccccgagggcttcaagtgggagcgcgtgatgaacttcgaggacggcggcgtggtgaccgtgacccaggactcctccctgcaggacggcaccctcatctaccacgtgaagttcatcggcgtgaacttcccctccgacggccccgtaatgcagaagaaaactctgggctgggagccctccactgagcgcaactacccccgcgacggcgtgctgaagggcgagaaccacatggcgctgaagctgaagggcggcggccactacctgtgtgagttcaagtccatctacatggccaagaagcccgtgaagctgcccggctaccactacgtggactacaagctcgacatcacctcccacaacgaggactacaccgtggtggagcagtacgagcgcgccgaggcccgccaccacctgttccagtgataataggggttctctctgagtctgtggggaccagaagaatactagtttattctcaaaaaaaaaaaaaaaaaaaaaaaaaaaaaaaaaaaaaaaaaaaaaaaaaaaaaaaaaaaaaaaaaaaaaaaaaaaaaaaaaaaaaaaaaaaaaaaaaaaaagagacg

SEQ ID NO: 308 - DNA, 907 bp, synthetic construct
  source 1..907: mol_type = other DNA
taatacgactcactataagggagaataatagtattcctggtccccacagactcagagaacccgccaccatggatagcactgagaacgtcatcaagcccttcatgcgcttcaaggtgcacatggagggctccgtgaacggccacgagttcgagatcgagggcgtgggcgagggcaagccctacgagggcacccagaccgccaagctgcaagtgaccaagggcggccccctgcccttcgcctgggacatcctgtccccccagttcttctacggctccaaggcgtacatcaagcaccccgccgacatccccgactacctcaagcagtccttccccgagggcttcaagtgggagcgcgtgatgaacttcgaggacggcggcgtggtgaccgtgacccaggactcctccctgcaggacggcaccctcatctaccacgtgaagttcatcggcgtgaacttcccctccgacggccccgtaatgcagaagaaaactctgggctgggagccctccactgagcgcaactacccccgcgacggcgtgctgaagggcgagaaccacatggcgctgaagctgaagggcggcggccactacctgtgtgagttcaagtccatctacatggccaagaagcccgtgaagctgcccggctaccactacgtggactacaagctcgacatcacctcccacaacgaggactacaccgtggtggagcagtacgagcgcgccgaggcccgccaccacctgttccagtgataataggggttctctctgagtctgtggggaccagaagaatactagtttattctcaaaaaaaaaaaaaaaaaaaaaaaaaaaaaaaaaaaaaaaaaaaaaaaaaaaaaaaaaaaaaaaaaaaaaaaaaaaaaaaaaaaaaaaaaaaaaaaaaaaaagagacg

SEQ ID NO: 309 - DNA, 907 bp, synthetic construct
  source 1..907: mol_type = other DNA
taatacgactcactataagggagaataatagtattcctggtccccagactcagagagaacccgccaccatggatagcactgagaacgtcatcaagcccttcatgcgcttcaaggtgcacatggagggctccgtgaacggccacgagttcgagatcgagggcgtgggcgagggcaagccctacgagggcacccagaccgccaagctgcaagtgaccaagggcggccccctgcccttcgcctgggacatcctgtccccccagttcttctacggctccaaggcgtacatcaagcaccccgccgacatccccgactacctcaagcagtccttccccgagggcttcaagtgggagcgcgtgatgaacttcgaggacggcggcgtggtgaccgtgacccaggactcctccctgcaggacggcaccctcatctaccacgtgaagttcatcggcgtgaacttcccctccgacggccccgtaatgcagaagaaaactctgggctgggagccctccactgagcgcaactacccccgcgacggcgtgctgaagggcgagaaccacatggcgctgaagctgaagggcggcggccactacctgtgtgagttcaagtccatctacatggccaagaagcccgtgaagctgcccggctaccactacgtggactacaagctcgacatcacctcccacaacgaggactacaccgtggtggagcagtacgagcgcgccgaggcccgccaccacctgttccagtgataataggggttctctctgagtctgtggggaccagaagaatactagtttattctcaaaaaaaaaaaaaaaaaaaaaaaaaaaaaaaaaaaaaaaaaaaaaaaaaaaaaaaaaaaaaaaaaaaaaaaaaaaaaaaaaaaaaaaaaaaaaaaaaaaaagagacg

SEQ ID NO: 310 - DNA, 909 bp, synthetic construct
  source 1..909: mol_type = other DNA
taatacgactcactataagggagaataatagtattcttctggtccccacagactcagagagaacccgccaccatggatagcactgagaacgtcatcaagcccttcatgcgcttcaaggtgcacatggagggctccgtgaacggccacgagttcgagatcgagggcgtgggcgagggcaagccctacgagggcacccagaccgccaagctgcaagtgaccaagggcggccccctgcccttcgcctgggacatcctgtccccccagttcttctacggctccaaggcgtacatcaagcaccccgccgacatccccgactacctcaagcagtccttccccgagggcttcaagtgggagcgcgtgatgaacttcgaggacggcggcgtggtgaccgtgacccaggactcctccctgcaggacggcaccctcatctaccacgtgaagttcatcggcgtgaacttcccctccgacggccccgtaatgcagaagaaaactctgggctgggagccctccactgagcgcaactacccccgcgacggcgtgctgaagggcgagaaccacatggcgctgaagctgaagggcggcggccactacctgtgtgagttcaagtccatctacatggccaagaagcccgtgaagctgcccggctaccactacgtggactacaagctcgacatcacctcccacaacgaggactacaccgtggtggagcagtacgagcgcgccgaggcccgccaccacctgttccagtgataataggggttctctctgagtctgtggggaccaggaatactagtttattctcaaaaaaaaaaaaaaaaaaaaaaaaaaaaaaaaaaaaaaaaaaaaaaaaaaaaaaaaaaaaaaaaaaaaaaaaaaaaaaaaaaaaaaaaaaaaaaaaaaaaagagacg

SEQ ID NO: 311 - DNA, 909 bp, synthetic construct
  source 1..909: mol_type = other DNA
taatacgactcactataagggagaataatagtattcttctggtccccacagactcagagagaacccgccaccatggatagcactgagaacgtcatcaagcccttcatgcgcttcaaggtgcacatggagggctccgtgaacggccacgagttcgagatcgagggcgtgggcgagggcaagccctacgagggcacccagaccgccaagctgcaagtgaccaagggcggccccctgcccttcgcctgggacatcctgtccccccagttcttctacggctccaaggcgtacatcaagcaccccgccgacatccccgactacctcaagcagtccttccccgagggcttcaagtgggagcgcgtgatgaacttcgaggacggcggcgtggtgaccgtgacccaggactcctccctgcaggacggcaccctcatctaccacgtgaagttcatcggcgtgaacttcccctccgacggccccgtaatgcagaagaaaactctgggctgggagccctccactgagcgcaactacccccgcgacggcgtgctgaagggcgagaaccacatggcgctgaagctgaagggcggcggccactacctgtgtgagttcaagtccatctacatggccaagaagcccgtgaagctgcccggctaccactacgtggactacaagctcgacatcacctcccacaacgaggactacaccgtggtggagcagtacgagcgcgccgaggcccgccaccacctgttccagtgataataggggttctctctgagtctggggaccagaagaatactagtttattctcaaaaaaaaaaaaaaaaaaaaaaaaaaaaaaaaaaaaaaaaaaaaaaaaaaaaaaaaaaaaaaaaaaaaaaaaaaaaaaaaaaaaaaaaaaaaaaaaaaaaagagacg

SEQ ID NO: 312 - DNA, 909 bp, synthetic construct
  source 1..909: mol_type = other DNA
taatacgactcactataagggagaataatagtattcttctggtccccacagactcagagagaacccgccaccatggatagcactgagaacgtcatcaagcccttcatgcgcttcaaggtgcacatggagggctccgtgaacggccacgagttcgagatcgagggcgtgggcgagggcaagccctacgagggcacccagaccgccaagctgcaagtgaccaagggcggccccctgcccttcgcctgggacatcctgtccccccagttcttctacggctccaaggcgtacatcaagcaccccgccgacatccccgactacctcaagcagtccttccccgagggcttcaagtgggagcgcgtgatgaacttcgaggacggcggcgtggtgaccgtgacccaggactcctccctgcaggacggcaccctcatctaccacgtgaagttcatcggcgtgaacttcccctccgacggccccgtaatgcagaagaaaactctgggctgggagccctccactgagcgcaactacccccgcgacggcgtgctgaagggcgagaaccacatggcgctgaagctgaagggcggcggccactacctgtgtgagttcaagtccatctacatggccaagaagcccgtgaagctgcccggctaccactacgtggactacaagctcgacatcacctcccacaacgaggactacaccgtggtggagcagtacgagcgcgccgaggcccgccaccacctgttccagtgataataggggttctctgagtctgtggggaccagaagaatactagtttattctcaaaaaaaaaaaaaaaaaaaaaaaaaaaaaaaaaaaaaaaaaaaaaaaaaaaaaaaaaaaaaaaaaaaaaaaaaaaaaaaaaaaaaaaaaaaaaaaaaaaaagagacg

SEQ ID NO: 313 - DNA, 909 bp, synthetic construct
  source 1..909: mol_type = other DNA
taatacgactcactataagggagaataaactagtattcctggtccccacagactcagagagaacccgccaccatggatagcactgagaacgtcatcaagcccttcatgcgcttcaaggtgcacatggagggctccgtgaacggccacgagttcgagatcgagggcgtgggcgagggcaagccctacgagggcacccagaccgccaagctgcaagtgaccaagggcggccccctgcccttcgcctgggacatcctgtccccccagttcttctacggctccaaggcgtacatcaagcaccccgccgacatccccgactacctcaagcagtccttccccgagggcttcaagtgggagcgcgtgatgaacttcgaggacggcggcgtggtgaccgtgacccaggactcctccctgcaggacggcaccctcatctaccacgtgaagttcatcggcgtgaacttcccctccgacggccccgtaatgcagaagaaaactctgggctgggagccctccactgagcgcaactacccccgcgacggcgtgctgaagggcgagaaccacatggcgctgaagctgaagggcggcggccactacctgtgtgagttcaagtccatctacatggccaagaagcccgtgaagctgcccggctaccactacgtggactacaagctcgacatcacctcccacaacgaggactacaccgtggtggagcagtacgagcgcgccgaggcccgccaccacctgttccagtgataataggggttctctctgagtctggggaccagaagaatactagtttattctcaaaaaaaaaaaaaaaaaaaaaaaaaaaaaaaaaaaaaaaaaaaaaaaaaaaaaaaaaaaaaaaaaaaaaaaaaaaaaaaaaaaaaaaaaaaaaaaaaaaaagagacg

SEQ ID NO: 314 - DNA, 909 bp, synthetic construct
  source 1..909: mol_type = other DNA
taatacgactcactataagggagaataaactagtattcctggtccccacagactcagagagaacccgccaccatggatagcactgagaacgtcatcaagcccttcatgcgcttcaaggtgcacatggagggctccgtgaacggccacgagttcgagatcgagggcgtgggcgagggcaagccctacgagggcacccagaccgccaagctgcaagtgaccaagggcggccccctgcccttcgcctgggacatcctgtccccccagttcttctacggctccaaggcgtacatcaagcaccccgccgacatccccgactacctcaagcagtccttccccgagggcttcaagtgggagcgcgtgatgaacttcgaggacggcggcgtggtgaccgtgacccaggactcctccctgcaggacggcaccctcatctaccacgtgaagttcatcggcgtgaacttcccctccgacggccccgtaatgcagaagaaaactctgggctgggagccctccactgagcgcaactacccccgcgacggcgtgctgaagggcgagaaccacatggcgctgaagctgaagggcggcggccactacctgtgtgagttcaagtccatctacatggccaagaagcccgtgaagctgcccggctaccactacgtggactacaagctcgacatcacctcccacaacgaggactacaccgtggtggagcagtacgagcgcgccgaggcccgccaccacctgttccagtgataataggggttctctgagtctgtggggaccagaagaatactagtttattctcaaaaaaaaaaaaaaaaaaaaaaaaaaaaaaaaaaaaaaaaaaaaaaaaaaaaaaaaaaaaaaaaaaaaaaaaaaaaaaaaaaaaaaaaaaaaaaaaaaaaagagacg

SEQ ID NO: 315 - DNA, 909 bp, synthetic construct
  source 1..909: mol_type = other DNA
taatacgactcactataagggagaataaactagtattcttctggtccccagactcagagagaacccgccaccatggatagcactgagaacgtcatcaagcccttcatgcgcttcaaggtgcacatggagggctccgtgaacggccacgagttcgagatcgagggcgtgggcgagggcaagccctacgagggcacccagaccgccaagctgcaagtgaccaagggcggccccctgcccttcgcctgggacatcctgtccccccagttcttctacggctccaaggcgtacatcaagcaccccgccgacatccccgactacctcaagcagtccttccccgagggcttcaagtgggagcgcgtgatgaacttcgaggacggcggcgtggtgaccgtgacccaggactcctccctgcaggacggcaccctcatctaccacgtgaagttcatcggcgtgaacttcccctccgacggccccgtaatgcagaagaaaactctgggctgggagccctccactgagcgcaactacccccgcgacggcgtgctgaagggcgagaaccacatggcgctgaagctgaagggcggcggccactacctgtgtgagttcaagtccatctacatggccaagaagcccgtgaagctgcccggctaccactacgtggactacaagctcgacatcacctcccacaacgaggactacaccgtggtggagcagtacgagcgcgccgaggcccgccaccacctgttccagtgataataggggttctctgagtctgtggggaccagaagaatactagtttattctcaaaaaaaaaaaaaaaaaaaaaaaaaaaaaaaaaaaaaaaaaaaaaaaaaaaaaaaaaaaaaaaaaaaaaaaaaaaaaaaaaaaaaaaaaaaaaaaaaaaaagagacg

SEQ ID NO: 316 - DNA, 913 bp, synthetic construct
  source 1..913: mol_type = other DNA
taatacgactcactataagggagaataaactagtattcttctggtccccacagactcagagagaacccgccaccatggatagcactgagaacgtcatcaagcccttcatgcgcttcaaggtgcacatggagggctccgtgaacggccacgagttcgagatcgagggcgtgggcgagggcaagccctacgagggcacccagaccgccaagctgcaagtgaccaagggcggccccctgcccttcgcctgggacatcctgtccccccagttcttctacggctccaaggcgtacatcaagcaccccgccgacatccccgactacctcaagcagtccttccccgagggcttcaagtgggagcgcgtgatgaacttcgaggacggcggcgtggtgaccgtgacccaggactcctccctgcaggacggcaccctcatctaccacgtgaagttcatcggcgtgaacttcccctccgacggccccgtaatgcagaagaaaactctgggctgggagccctccactgagcgcaactacccccgcgacggcgtgctgaagggcgagaaccacatggcgctgaagctgaagggcggcggccactacctgtgtgagttcaagtccatctacatggccaagaagcccgtgaagctgcccggctaccactacgtggactacaagctcgacatcacctcccacaacgaggactacaccgtggtggagcagtacgagcgcgccgaggcccgccaccacctgttccagtgataataggccttctctgagagtctcaggggacgagatgaaaacttgttaattgtcaaaaaaaaaaaaaaaaaaaaaaaaaaaaaaaaaaaaaaaaaaaaaaaaaaaaaaaaaaaaaaaaaaaaaaaaaaaaaaaaaaaaaaaaaaaaaaaaaaaaagagacg

SEQ ID NO: 317 - DNA, 913 bp, synthetic construct
  source 1..913: mol_type = other DNA
taatacgactcactataagggagaataaactagtattcttctggtccccacagactcagagagaacccgccaccatggatagcactgagaacgtcatcaagcccttcatgcgcttcaaggtgcacatggagggctccgtgaacggccacgagttcgagatcgagggcgtgggcgagggcaagccctacgagggcacccagaccgccaagctgcaagtgaccaagggcggccccctgcccttcgcctgggacatcctgtccccccagttcttctacggctccaaggcgtacatcaagcaccccgccgacatccccgactacctcaagcagtccttccccgagggcttcaagtgggagcgcgtgatgaacttcgaggacggcggcgtggtgaccgtgacccaggactcctccctgcaggacggcaccctcatctaccacgtgaagttcatcggcgtgaacttcccctccgacggccccgtaatgcagaagaaaactctgggctgggagccctccactgagcgcaactacccccgcgacggcgtgctgaagggcgagaaccacatggcgctgaagctgaagggcggcggccactacctgtgtgagttcaagtccatctacatggccaagaagcccgtgaagctgcccggctaccactacgtggactacaagctcgacatcacctcccacaacgaggactacaccgtggtggagcagtacgagcgcgccgaggcccgccaccacctgttccagtgataataggcgttgtctgtgactctctggcgacgtgaagaaatctagttatttctcaaaaaaaaaaaaaaaaaaaaaaaaaaaaaaaaaaaaaaaaaaaaaaaaaaaaaaaaaaaaaaaaaaaaaaaaaaaaaaaaaaaaaaaaaaaaaaaaaaaaagagacg

SEQ ID NO: 318 - DNA, 913 bp, synthetic construct
  source 1..913: mol_type = other DNA
taatacgactcactataagggagaataaactagtattcttctggtccccacagactcagagagaacccgccaccatggatagcactgagaacgtcatcaagcccttcatgcgcttcaaggtgcacatggagggctccgtgaacggccacgagttcgagatcgagggcgtgggcgagggcaagccctacgagggcacccagaccgccaagctgcaagtgaccaagggcggccccctgcccttcgcctgggacatcctgtccccccagttcttctacggctccaaggcgtacatcaagcaccccgccgacatccccgactacctcaagcagtccttccccgagggcttcaagtgggagcgcgtgatgaacttcgaggacggcggcgtggtgaccgtgacccaggactcctccctgcaggacggcaccctcatctaccacgtgaagttcatcggcgtgaacttcccctccgacggccccgtaatgcagaagaaaactctgggctgggagccctccactgagcgcaactacccccgcgacggcgtgctgaagggcgagaaccacatggcgctgaagctgaagggcggcggccactacctgtgtgagttcaagtccatctacatggccaagaagcccgtgaagctgcccggctaccactacgtggactacaagctcgacatcacctcccacaacgaggactacaccgtggtggagcagtacgagcgcgccgaggcccgccaccacctgttccagtgataataggccatctctctgacagtgtggggacgtgaagaaatctagttatttctcaaaaaaaaaaaaaaaaaaaaaaaaaaaaaaaaaaaaaaaaaaaaaaaaaaaaaaaaaaaaaaaaaaaaaaaaaaaaaaaaaaaaaaaaaaaaaaaaaaaaagagacg

SEQ ID NO: 319 - DNA, 913 bp, synthetic construct
  source 1..913: mol_type = other DNA
taatacgactcactataagggagaataaactagtattcttctggtccccacagactcagagagaacccgccaccatggatagcactgagaacgtcatcaagcccttcatgcgcttcaaggtgcacatggagggctccgtgaacggccacgagttcgagatcgagggcgtgggcgagggcaagccctacgagggcacccagaccgccaagctgcaagtgaccaagggcggccccctgcccttcgcctgggacatcctgtccccccagttcttctacggctccaaggcgtacatcaagcaccccgccgacatccccgactacctcaagcagtccttccccgagggcttcaagtgggagcgcgtgatgaacttcgaggacggcggcgtggtgaccgtgacccaggactcctccctgcaggacggcaccctcatctaccacgtgaagttcatcggcgtgaacttcccctccgacggccccgtaatgcagaagaaaactctgggctgggagccctccactgagcgcaactacccccgcgacggcgtgctgaagggcgagaaccacatggcgctgaagctgaagggcggcggccactacctgtgtgagttcaagtccatctacatggccaagaagcccgtgaagctgcccggctaccactacgtggactacaagctcgacatcacctcccacaacgaggactacaccgtggtggagcagtacgagcgcgccgaggcccgccaccacctgttccagtgataataggccttctctgagagtctcaggggacgtcaagaatacttcattattctcaaaaaaaaaaaaaaaaaaaaaaaaaaaaaaaaaaaaaaaaaaaaaaaaaaaaaaaaaaaaaaaaaaaaaaaaaaaaaaaaaaaaaaaaaaaaaaaaaaaaagagacg

SEQ ID NO: 320 - DNA, 913 bp, synthetic construct
  source 1..913: mol_type = other DNA
taatacgactcactataagggagaataaactagtattcttctggtccccacagactcagagagaacccgccaccatggatagcactgagaacgtcatcaagcccttcatgcgcttcaaggtgcacatggagggctccgtgaacggccacgagttcgagatcgagggcgtgggcgagggcaagccctacgagggcacccagaccgccaagctgcaagtgaccaagggcggccccctgcccttcgcctgggacatcctgtccccccagttcttctacggctccaaggcgtacatcaagcaccccgccgacatccccgactacctcaagcagtccttccccgagggcttcaagtgggagcgcgtgatgaacttcgaggacggcggcgtggtgaccgtgacccaggactcctccctgcaggacggcaccctcatctaccacgtgaagttcatcggcgtgaacttcccctccgacggccccgtaatgcagaagaaaactctgggctgggagccctccactgagcgcaactacccccgcgacggcgtgctgaagggcgagaaccacatggcgctgaagctgaagggcggcggccactacctgtgtgagttcaagtccatctacatggccaagaagcccgtgaagctgcccggctaccactacgtggactacaagctcgacatcacctcccacaacgaggactacaccgtggtggagcagtacgagcgcgccgaggcccgccaccacctgttccagtgataataggccatctctctgacagtgtggggacgagatgaaaacttgttaattgtcaaaaaaaaaaaaaaaaaaaaaaaaaaaaaaaaaaaaaaaaaaaaaaaaaaaaaaaaaaaaaaaaaaaaaaaaaaaaaaaaaaaaaaaaaaaaaaaaaaaaagagacg

SEQ ID NO: 321 - DNA, 913 bp, synthetic construct
  source 1..913: mol_type = other DNA
taatacgactcactataagggagaataaactagtattcttctggtccccacagactcagagagaacccgccaccatggatagcactgagaacgtcatcaagcccttcatgcgcttcaaggtgcacatggagggctccgtgaacggccacgagttcgagatcgagggcgtgggcgagggcaagccctacgagggcacccagaccgccaagctgcaagtgaccaagggcggccccctgcccttcgcctgggacatcctgtccccccagttcttctacggctccaaggcgtacatcaagcaccccgccgacatccccgactacctcaagcagtccttccccgagggcttcaagtgggagcgcgtgatgaacttcgaggacggcggcgtggtgaccgtgacccaggactcctccctgcaggacggcaccctcatctaccacgtgaagttcatcggcgtgaacttcccctccgacggccccgtaatgcagaagaaaactctgggctgggagccctccactgagcgcaactacccccgcgacggcgtgctgaagggcgagaaccacatggcgctgaagctgaagggcggcggccactacctgtgtgagttcaagtccatctacatggccaagaagcccgtgaagctgcccggctaccactacgtggactacaagctcgacatcacctcccacaacgaggactacaccgtggtggagcagtacgagcgcgccgaggcccgccaccacctgttccagtgataataggcgttgtctgtgactctctggcgacgtcaagaatacttcattattctcaaaaaaaaaaaaaaaaaaaaaaaaaaaaaaaaaaaaaaaaaaaaaaaaaaaaaaaaaaaaaaaaaaaaaaaaaaaaaaaaaaaaaaaaaaaaaaaaaaaaagagacg

SEQ ID NO: 322 - DNA, 909 bp, synthetic construct
  source 1..909: mol_type = other DNA
taatacgactcactataagggagaataaactagtattcttctggtccccacagactcagagagaacccgccaccatggatagcactgagaacgtcatcaagcccttcatgcgcttcaaggtgcacatggagggctccgtgaacggccacgagttcgagatcgagggcgtgggcgagggcaagccctacgagggcacccagaccgccaagctgcaagtgaccaagggcggccccctgcccttcgcctgggacatcctgtccccccagttcttctacggctccaaggcgtacatcaagcaccccgccgacatccccgactacctcaagcagtccttccccgagggcttcaagtgggagcgcgtgatgaacttcgaggacggcggcgtggtgaccgtgacccaggactcctccctgcaggacggcaccctcatctaccacgtgaagttcatcggcgtgaacttcccctccgacggccccgtaatgcagaagaaaactctgggctgggagccctccactgagcgcaactacccccgcgacggcgtgctgaagggcgagaaccacatggcgctgaagctgaagggcggcggccactacctgtgtgagttcaagtccatctacatggccaagaagcccgtgaagctgcccggctaccactacgtggactacaagctcgacatcacctcccacaacgaggactacaccgtggtggagcagtacgagcgcgccgaggcccgccaccacctgttccagtgataataggcatctctctgaagtgtggggactcaagaatactcattattctcaaaaaaaaaaaaaaaaaaaaaaaaaaaaaaaaaaaaaaaaaaaaaaaaaaaaaaaaaaaaaaaaaaaaaaaaaaaaaaaaaaaaaaaaaaaaaaaaaaaaagagacg

SEQ ID NO: 323 - DNA, 909 bp, synthetic construct
  source 1..909: mol_type = other DNA
taatacgactcactataagggagaataaacagtattcttctgtccccacagatcagagagaaccgccaccatggatagcactgagaacgtcatcaagcccttcatgcgcttcaaggtgcacatggagggctccgtgaacggccacgagttcgagatcgagggcgtgggcgagggcaagccctacgagggcacccagaccgccaagctgcaagtgaccaagggcggccccctgcccttcgcctgggacatcctgtccccccagttcttctacggctccaaggcgtacatcaagcaccccgccgacatccccgactacctcaagcagtccttccccgagggcttcaagtgggagcgcgtgatgaacttcgaggacggcggcgtggtgaccgtgacccaggactcctccctgcaggacggcaccctcatctaccacgtgaagttcatcggcgtgaacttcccctccgacggccccgtaatgcagaagaaaactctgggctgggagccctccactgagcgcaactacccccgcgacggcgtgctgaagggcgagaaccacatggcgctgaagctgaagggcggcggccactacctgtgtgagttcaagtccatctacatggccaagaagcccgtgaagctgcccggctaccactacgtggactacaagctcgacatcacctcccacaacgaggactacaccgtggtggagcagtacgagcgcgccgaggcccgccaccacctgttccagtgataataggccatctctctgacagtgtggggacgtcaagaatacttcattattctcaaaaaaaaaaaaaaaaaaaaaaaaaaaaaaaaaaaaaaaaaaaaaaaaaaaaaaaaaaaaaaaaaaaaaaaaaaaaaaaaaaaaaaaaaaaaaaaaaaaaagagacg

SEQ ID NO: 324 - DNA, 905 bp, synthetic construct
  source 1..905: mol_type = other DNA
taatacgactcactataagggagaataaactagtattcttctggtccccacagactcagagagaacccgccaccatggatagcactgagaacgtcatcaagcccttcatgcgcttcaaggtgcacatggagggctccgtgaacggccacgagttcgagatcgagggcgtgggcgagggcaagccctacgagggcacccagaccgccaagctgcaagtgaccaagggcggccccctgcccttcgcctgggacatcctgtccccccagttcttctacggctccaaggcgtacatcaagcaccccgccgacatccccgactacctcaagcagtccttccccgagggcttcaagtgggagcgcgtgatgaacttcgaggacggcggcgtggtgaccgtgacccaggactcctccctgcaggacggcaccctcatctaccacgtgaagttcatcggcgtgaacttcccctccgacggccccgtaatgcagaagaaaactctgggctgggagccctccactgagcgcaactacccccgcgacggcgtgctgaagggcgagaaccacatggcgctgaagctgaagggcggcggccactacctgtgtgagttcaagtccatctacatggccaagaagcccgtgaagctgcccggctaccactacgtggactacaagctcgacatcacctcccacaacgaggactacaccgtggtggagcagtacgagcgcgccgaggcccgccaccacctgttccagtgataataggatctctctgagtgtggggaccaagaatactattattctcaaaaaaaaaaaaaaaaaaaaaaaaaaaaaaaaaaaaaaaaaaaaaaaaaaaaaaaaaaaaaaaaaaaaaaaaaaaaaaaaaaaaaaaaaaaaaaaaaaaaagagacg

SEQ ID NO: 325 - DNA, 905 bp, synthetic construct
  source 1..905: mol_type = other DNA
taatacgactcactataagggagaataaaagtattcttcgtccccacagtcagagagaacgccaccatggatagcactgagaacgtcatcaagcccttcatgcgcttcaaggtgcacatggagggctccgtgaacggccacgagttcgagatcgagggcgtgggcgagggcaagccctacgagggcacccagaccgccaagctgcaagtgaccaagggcggccccctgcccttcgcctgggacatcctgtccccccagttcttctacggctccaaggcgtacatcaagcaccccgccgacatccccgactacctcaagcagtccttccccgagggcttcaagtgggagcgcgtgatgaacttcgaggacggcggcgtggtgaccgtgacccaggactcctccctgcaggacggcaccctcatctaccacgtgaagttcatcggcgtgaacttcccctccgacggccccgtaatgcagaagaaaactctgggctgggagccctccactgagcgcaactacccccgcgacggcgtgctgaagggcgagaaccacatggcgctgaagctgaagggcggcggccactacctgtgtgagttcaagtccatctacatggccaagaagcccgtgaagctgcccggctaccactacgtggactacaagctcgacatcacctcccacaacgaggactacaccgtggtggagcagtacgagcgcgccgaggcccgccaccacctgttccagtgataataggccatctctctgacagtgtggggacgtcaagaatacttcattattctcaaaaaaaaaaaaaaaaaaaaaaaaaaaaaaaaaaaaaaaaaaaaaaaaaaaaaaaaaaaaaaaaaaaaaaaaaaaaaaaaaaaaaaaaaaaaaaaaaaaaagagacg

SEQ ID NO: 326 - DNA, 909 bp, synthetic construct
  source 1..909: mol_type = other DNA
taatacgactcactataagggagaataaactagtattcttctggtccccacagactcagagagaacccgccaccatggatagcactgagaacgtcatcaagcccttcatgcgcttcaaggtgcacatggagggctccgtgaacggccacgagttcgagatcgagggcgtgggcgagggcaagccctacgagggcacccagaccgccaagctgcaagtgaccaagggcggccccctgcccttcgcctgggacatcctgtccccccagttcttctacggctccaaggcgtacatcaagcaccccgccgacatccccgactacctcaagcagtccttccccgagggcttcaagtgggagcgcgtgatgaacttcgaggacggcggcgtggtgaccgtgacccaggactcctccctgcaggacggcaccctcatctaccacgtgaagttcatcggcgtgaacttcccctccgacggccccgtaatgcagaagaaaactctgggctgggagccctccactgagcgcaactacccccgcgacggcgtgctgaagggcgagaaccacatggcgctgaagctgaagggcggcggccactacctgtgtgagttcaagtccatctacatggccaagaagcccgtgaagctgcccggctaccactacgtggactacaagctcgacatcacctcccacaacgaggactacaccgtggtggagcagtacgagcgcgccgaggcccgccaccacctgttccagtgataataggggttctcgtgagtctgcgggaccagtgaatactaattattctcaaaaaaaaaaaaaaaaaaaaaaaaaaaaaaaaaaaaaaaaaaaaaaaaaaaaaaaaaaaaaaaaaaaaaaaaaaaaaaaaaaaaaaaaaaaaaaaaaaaaagagacg

SEQ ID NO: 327 - DNA, 909 bp, synthetic construct
  source 1..909: mol_type = other DNA
taatacgactcactataagggagaataattagtattcactggtcccgcagactcacgagaacccgccaccatggatagcactgagaacgtcatcaagcccttcatgcgcttcaaggtgcacatggagggctccgtgaacggccacgagttcgagatcgagggcgtgggcgagggcaagccctacgagggcacccagaccgccaagctgcaagtgaccaagggcggccccctgcccttcgcctgggacatcctgtccccccagttcttctacggctccaaggcgtacatcaagcaccccgccgacatccccgactacctcaagcagtccttccccgagggcttcaagtgggagcgcgtgatgaacttcgaggacggcggcgtggtgaccgtgacccaggactcctccctgcaggacggcaccctcatctaccacgtgaagttcatcggcgtgaacttcccctccgacggccccgtaatgcagaagaaaactctgggctgggagccctccactgagcgcaactacccccgcgacggcgtgctgaagggcgagaaccacatggcgctgaagctgaagggcggcggccactacctgtgtgagttcaagtccatctacatggccaagaagcccgtgaagctgcccggctaccactacgtggactacaagctcgacatcacctcccacaacgaggactacaccgtggtggagcagtacgagcgcgccgaggcccgccaccacctgttccagtgataataggggttctctctgagtctgtggggaccagaagaatactagtttattctcaaaaaaaaaaaaaaaaaaaaaaaaaaaaaaaaaaaaaaaaaaaaaaaaaaaaaaaaaaaaaaaaaaaaaaaaaaaaaaaaaaaaaaaaaaaaaaaaaaaaagagacg

SEQ ID NO: 328 - DNA, 909 bp, synthetic construct
  source 1..909: mol_type = other DNA
taatacgactcactataagggagaataaactagtattcttctggtccccacagatcagagagaaccgccaccatggatagcactgagaacgtcatcaagcccttcatgcgcttcaaggtgcacatggagggctccgtgaacggccacgagttcgagatcgagggcgtgggcgagggcaagccctacgagggcacccagaccgccaagctgcaagtgaccaagggcggccccctgcccttcgcctgggacatcctgtccccccagttcttctacggctccaaggcgtacatcaagcaccccgccgacatccccgactacctcaagcagtccttccccgagggcttcaagtgggagcgcgtgatgaacttcgaggacggcggcgtggtgaccgtgacccaggactcctccctgcaggacggcaccctcatctaccacgtgaagttcatcggcgtgaacttcccctccgacggccccgtaatgcagaagaaaactctgggctgggagccctccactgagcgcaactacccccgcgacggcgtgctgaagggcgagaaccacatggcgctgaagctgaagggcggcggccactacctgtgtgagttcaagtccatctacatggccaagaagcccgtgaagctgcccggctaccactacgtggactacaagctcgacatcacctcccacaacgaggactacaccgtggtggagcagtacgagcgcgccgaggcccgccaccacctgttccagtgataataggccatctctctgacagtgtggggactcaagaatactcattattctcaaaaaaaaaaaaaaaaaaaaaaaaaaaaaaaaaaaaaaaaaaaaaaaaaaaaaaaaaaaaaaaaaaaaaaaaaaaaaaaaaaaaaaaaaaaaaaaaaaaaagagacg

SEQ ID NO: 329 - DNA, 909 bp, synthetic construct
  source 1..909: mol_type = other DNA
taatacgactcactataagggagaataaacagtattcttctgtccccacagactcagagagaacccgccaccatggatagcactgagaacgtcatcaagcccttcatgcgcttcaaggtgcacatggagggctccgtgaacggccacgagttcgagatcgagggcgtgggcgagggcaagccctacgagggcacccagaccgccaagctgcaagtgaccaagggcggccccctgcccttcgcctgggacatcctgtccccccagttcttctacggctccaaggcgtacatcaagcaccccgccgacatccccgactacctcaagcagtccttccccgagggcttcaagtgggagcgcgtgatgaacttcgaggacggcggcgtggtgaccgtgacccaggactcctccctgcaggacggcaccctcatctaccacgtgaagttcatcggcgtgaacttcccctccgacggccccgtaatgcagaagaaaactctgggctgggagccctccactgagcgcaactacccccgcgacggcgtgctgaagggcgagaaccacatggcgctgaagctgaagggcggcggccactacctgtgtgagttcaagtccatctacatggccaagaagcccgtgaagctgcccggctaccactacgtggactacaagctcgacatcacctcccacaacgaggactacaccgtggtggagcagtacgagcgcgccgaggcccgccaccacctgttccagtgataataggcatctctctgaagtgtggggacgtcaagaatacttcattattctcaaaaaaaaaaaaaaaaaaaaaaaaaaaaaaaaaaaaaaaaaaaaaaaaaaaaaaaaaaaaaaaaaaaaaaaaaaaaaaaaaaaaaaaaaaaaaaaaaaaaagagacg

SEQ ID NO: 330 - DNA, 905 bp, synthetic construct
  source 1..905: mol_type = other DNA
taatacgactcactataagggagaataaactagtattcttctggtccccacagtcagagagaacgccaccatggatagcactgagaacgtcatcaagcccttcatgcgcttcaaggtgcacatggagggctccgtgaacggccacgagttcgagatcgagggcgtgggcgagggcaagccctacgagggcacccagaccgccaagctgcaagtgaccaagggcggccccctgcccttcgcctgggacatcctgtccccccagttcttctacggctccaaggcgtacatcaagcaccccgccgacatccccgactacctcaagcagtccttccccgagggcttcaagtgggagcgcgtgatgaacttcgaggacggcggcgtggtgaccgtgacccaggactcctccctgcaggacggcaccctcatctaccacgtgaagttcatcggcgtgaacttcccctccgacggccccgtaatgcagaagaaaactctgggctgggagccctccactgagcgcaactacccccgcgacggcgtgctgaagggcgagaaccacatggcgctgaagctgaagggcggcggccactacctgtgtgagttcaagtccatctacatggccaagaagcccgtgaagctgcccggctaccactacgtggactacaagctcgacatcacctcccacaacgaggactacaccgtggtggagcagtacgagcgcgccgaggcccgccaccacctgttccagtgataataggccatctctctgacagtgtggggaccaagaatactattattctcaaaaaaaaaaaaaaaaaaaaaaaaaaaaaaaaaaaaaaaaaaaaaaaaaaaaaaaaaaaaaaaaaaaaaaaaaaaaaaaaaaaaaaaaaaaaaaaaaaaaagagacg

SEQ ID NO: 331 - DNA, 905 bp, synthetic construct
  source 1..905: mol_type = other DNA
taatacgactcactataagggagaataaaagtattcttcgtccccacagactcagagagaacccgccaccatggatagcactgagaacgtcatcaagcccttcatgcgcttcaaggtgcacatggagggctccgtgaacggccacgagttcgagatcgagggcgtgggcgagggcaagccctacgagggcacccagaccgccaagctgcaagtgaccaagggcggccccctgcccttcgcctgggacatcctgtccccccagttcttctacggctccaaggcgtacatcaagcaccccgccgacatccccgactacctcaagcagtccttccccgagggcttcaagtgggagcgcgtgatgaacttcgaggacggcggcgtggtgaccgtgacccaggactcctccctgcaggacggcaccctcatctaccacgtgaagttcatcggcgtgaacttcccctccgacggccccgtaatgcagaagaaaactctgggctgggagccctccactgagcgcaactacccccgcgacggcgtgctgaagggcgagaaccacatggcgctgaagctgaagggcggcggccactacctgtgtgagttcaagtccatctacatggccaagaagcccgtgaagctgcccggctaccactacgtggactacaagctcgacatcacctcccacaacgaggactacaccgtggtggagcagtacgagcgcgccgaggcccgccaccacctgttccagtgataataggatctctctgagtgtggggacgtcaagaatacttcattattctcaaaaaaaaaaaaaaaaaaaaaaaaaaaaaaaaaaaaaaaaaaaaaaaaaaaaaaaaaaaaaaaaaaaaaaaaaaaaaaaaaaaaaaaaaaaaaaaaaaaaagagacg

SEQ ID NO: 332 - DNA, 909 bp, synthetic construct
  source 1..909: mol_type = other DNA
taatacgactcactataagggagaataaactagtattcttctggtcccgcagactcacgagaacccgccaccatggatagcactgagaacgtcatcaagcccttcatgcgcttcaaggtgcacatggagggctccgtgaacggccacgagttcgagatcgagggcgtgggcgagggcaagccctacgagggcacccagaccgccaagctgcaagtgaccaagggcggccccctgcccttcgcctgggacatcctgtccccccagttcttctacggctccaaggcgtacatcaagcaccccgccgacatccccgactacctcaagcagtccttccccgagggcttcaagtgggagcgcgtgatgaacttcgaggacggcggcgtggtgaccgtgacccaggactcctccctgcaggacggcaccctcatctaccacgtgaagttcatcggcgtgaacttcccctccgacggccccgtaatgcagaagaaaactctgggctgggagccctccactgagcgcaactacccccgcgacggcgtgctgaagggcgagaaccacatggcgctgaagctgaagggcggcggccactacctgtgtgagttcaagtccatctacatggccaagaagcccgtgaagctgcccggctaccactacgtggactacaagctcgacatcacctcccacaacgaggactacaccgtggtggagcagtacgagcgcgccgaggcccgccaccacctgttccagtgataataggggttctctctgagtctgtggggaccagtgaatactaattattctcaaaaaaaaaaaaaaaaaaaaaaaaaaaaaaaaaaaaaaaaaaaaaaaaaaaaaaaaaaaaaaaaaaaaaaaaaaaaaaaaaaaaaaaaaaaaaaaaaaaaagagacg

SEQ ID NO: 333 - DNA, 909 bp, synthetic construct
  source 1..909: mol_type = other DNA
taatacgactcactataagggagaataattagtattcactggtccccacagactcagagagaacccgccaccatggatagcactgagaacgtcatcaagcccttcatgcgcttcaaggtgcacatggagggctccgtgaacggccacgagttcgagatcgagggcgtgggcgagggcaagccctacgagggcacccagaccgccaagctgcaagtgaccaagggcggccccctgcccttcgcctgggacatcctgtccccccagttcttctacggctccaaggcgtacatcaagcaccccgccgacatccccgactacctcaagcagtccttccccgagggcttcaagtgggagcgcgtgatgaacttcgaggacggcggcgtggtgaccgtgacccaggactcctccctgcaggacggcaccctcatctaccacgtgaagttcatcggcgtgaacttcccctccgacggccccgtaatgcagaagaaaactctgggctgggagccctccactgagcgcaactacccccgcgacggcgtgctgaagggcgagaaccacatggcgctgaagctgaagggcggcggccactacctgtgtgagttcaagtccatctacatggccaagaagcccgtgaagctgcccggctaccactacgtggactacaagctcgacatcacctcccacaacgaggactacaccgtggtggagcagtacgagcgcgccgaggcccgccaccacctgttccagtgataataggggttctcgtgagtctgcgggaccagaagaatactagtttattctcaaaaaaaaaaaaaaaaaaaaaaaaaaaaaaaaaaaaaaaaaaaaaaaaaaaaaaaaaaaaaaaaaaaaaaaaaaaaaaaaaaaaaaaaaaaaaaaaaaaaagagacg

SEQ ID NO: 334 - DNA, 918 bp, synthetic construct
  source 1..918: mol_type = other DNA
taatacgactcactataagggagaataaactagtattcttctggtccccacagactcagagagaacccgccaccatggatagcactgagaacgtcatcaagcccttcatgcgcttcaaggtgcacatggagggctccgtgaacggccacgagttcgagatcgagggcgtgggcgagggcaagccctacgagggcacccagaccgccaagctgcaagtgaccaagggcggccccctgcccttcgcctgggacatcctgtccccccagttcttctacggctccaaggcgtacatcaagcaccccgccgacatccccgactacctcaagcagtccttccccgagggcttcaagtgggagcgcgtgatgaacttcgaggacggcggcgtggtgaccgtgacccaggactcctccctgcaggacggcaccctcatctaccacgtgaagttcatcggcgtgaacttcccctccgacggccccgtaatgcagaagaaaactctgggctgggagccctccactgagcgcaactacccccgcgacggcgtgctgaagggcgagaaccacatggcgctgaagctgaagggcggcggccactacctgtgtgagttcaagtccatctacatggccaagaagcccgtgaagctgcccggctaccactacgtggactacaagctcgacatcacctcccacaacgaggactacaccgtggtggagcagtacgagcgcgccgaggcccgccaccacctgttccagtgataataggggttctcatctgagtcctgtggggagccagaagatatactagtattattctcaaaaaaaaaaaaaaaaaaaaaaaaaaaaaaaaaaaaaaaaaaaaaaaaaaaaaaaaaaaaaaaaaaaaaaaaaaaaaaaaaaaaaaaaaaaaaaaaaaaaagagacg

SEQ ID NO: 335 - DNA, 923 bp, synthetic construct
  source 1..923: mol_type = other DNA
taatacgactcactataagggagaataaactagtattcttctggtccccacagactcagagagaacccgccaccatggatagcactgagaacgtcatcaagcccttcatgcgcttcaaggtgcacatggagggctccgtgaacggccacgagttcgagatcgagggcgtgggcgagggcaagccctacgagggcacccagaccgccaagctgcaagtgaccaagggcggccccctgcccttcgcctgggacatcctgtccccccagttcttctacggctccaaggcgtacatcaagcaccccgccgacatccccgactacctcaagcagtccttccccgagggcttcaagtgggagcgcgtgatgaacttcgaggacggcggcgtggtgaccgtgacccaggactcctccctgcaggacggcaccctcatctaccacgtgaagttcatcggcgtgaacttcccctccgacggccccgtaatgcagaagaaaactctgggctgggagccctccactgagcgcaactacccccgcgacggcgtgctgaagggcgagaaccacatggcgctgaagctgaagggcggcggccactacctgtgtgagttcaagtccatctacatggccaagaagcccgtgaagctgcccggctaccactacgtggactacaagctcgacatcacctcccacaacgaggactacaccgtggtggagcagtacgagcgcgccgaggcccgccaccacctgttccagtgataataggggttctcgttctgagtcattgtggggagaccagaagacgatactagttattattctcaaaaaaaaaaaaaaaaaaaaaaaaaaaaaaaaaaaaaaaaaaaaaaaaaaaaaaaaaaaaaaaaaaaaaaaaaaaaaaaaaaaaaaaaaaaaaaaaaaaaagagacg

SEQ ID NO: 336 - DNA, 928 bp, synthetic construct
  source 1..928: mol_type = other DNA
taatacgactcactataagggagaataaactagtattcttctggtccccacagactcagagagaacccgccaccatggatagcactgagaacgtcatcaagcccttcatgcgcttcaaggtgcacatggagggctccgtgaacggccacgagttcgagatcgagggcgtgggcgagggcaagccctacgagggcacccagaccgccaagctgcaagtgaccaagggcggccccctgcccttcgcctgggacatcctgtccccccagttcttctacggctccaaggcgtacatcaagcaccccgccgacatccccgactacctcaagcagtccttccccgagggcttcaagtgggagcgcgtgatgaacttcgaggacggcggcgtggtgaccgtgacccaggactcctccctgcaggacggcaccctcatctaccacgtgaagttcatcggcgtgaacttcccctccgacggccccgtaatgcagaagaaaactctgggctgggagccctccactgagcgcaactacccccgcgacggcgtgctgaagggcgagaaccacatggcgctgaagctgaagggcggcggccactacctgtgtgagttcaagtccatctacatggccaagaagcccgtgaagctgcccggctaccactacgtggactacaagctcgacatcacctcccacaacgaggactacaccgtggtggagcagtacgagcgcgccgaggcccgccaccacctgttccagtgataataggggttctccgatctgagtcgtctgtggggaagtccagaagactaatactagttagttattctcaaaaaaaaaaaaaaaaaaaaaaaaaaaaaaaaaaaaaaaaaaaaaaaaaaaaaaaaaaaaaaaaaaaaaaaaaaaaaaaaaaaaaaaaaaaaaaaaaaaaagagacg

SEQ ID NO: 337 - DNA, 918 bp, synthetic construct
  source 1..918: mol_type = other DNA
taatacgactcactataagggagaataaaactagtatttcttctgggtccccacacgactcagaagagaacccgccaccatggatagcactgagaacgtcatcaagcccttcatgcgcttcaaggtgcacatggagggctccgtgaacggccacgagttcgagatcgagggcgtgggcgagggcaagccctacgagggcacccagaccgccaagctgcaagtgaccaagggcggccccctgcccttcgcctgggacatcctgtccccccagttcttctacggctccaaggcgtacatcaagcaccccgccgacatccccgactacctcaagcagtccttccccgagggcttcaagtgggagcgcgtgatgaacttcgaggacggcggcgtggtgaccgtgacccaggactcctccctgcaggacggcaccctcatctaccacgtgaagttcatcggcgtgaacttcccctccgacggccccgtaatgcagaagaaaactctgggctgggagccctccactgagcgcaactacccccgcgacggcgtgctgaagggcgagaaccacatggcgctgaagctgaagggcggcggccactacctgtgtgagttcaagtccatctacatggccaagaagcccgtgaagctgcccggctaccactacgtggactacaagctcgacatcacctcccacaacgaggactacaccgtggtggagcagtacgagcgcgccgaggcccgccaccacctgttccagtgataataggggttctctctgagtctgtggggaccagaagaatactagtttattctcaaaaaaaaaaaaaaaaaaaaaaaaaaaaaaaaaaaaaaaaaaaaaaaaaaaaaaaaaaaaaaaaaaaaaaaaaaaaaaaaaaaaaaaaaaaaaaaaaaaaagagacg

SEQ ID NO: 338 - DNA, 923 bp, synthetic construct
  source 1..923: mol_type = other DNA
taatacgactcactataagggagaataaatactagtatgctcttctggagtccccacatagactcagatggagaacccgccaccatggatagcactgagaacgtcatcaagcccttcatgcgcttcaaggtgcacatggagggctccgtgaacggccacgagttcgagatcgagggcgtgggcgagggcaagccctacgagggcacccagaccgccaagctgcaagtgaccaagggcggccccctgcccttcgcctgggacatcctgtccccccagttcttctacggctccaaggcgtacatcaagcaccccgccgacatccccgactacctcaagcagtccttccccgagggcttcaagtgggagcgcgtgatgaacttcgaggacggcggcgtggtgaccgtgacccaggactcctccctgcaggacggcaccctcatctaccacgtgaagttcatcggcgtgaacttcccctccgacggccccgtaatgcagaagaaaactctgggctgggagccctccactgagcgcaactacccccgcgacggcgtgctgaagggcgagaaccacatggcgctgaagctgaagggcggcggccactacctgtgtgagttcaagtccatctacatggccaagaagcccgtgaagctgcccggctaccactacgtggactacaagctcgacatcacctcccacaacgaggactacaccgtggtggagcagtacgagcgcgccgaggcccgccaccacctgttccagtgataataggggttctctctgagtctgtggggaccagaagaatactagtttattctcaaaaaaaaaaaaaaaaaaaaaaaaaaaaaaaaaaaaaaaaaaaaaaaaaaaaaaaaaaaaaaaaaaaaaaaaaaaaaaaaaaaaaaaaaaaaaaaaaaaaagagacg

SEQ ID NO: 339 - DNA, 928 bp, synthetic construct
  source 1..928: mol_type = other DNA
taatacgactcactataagggagaataagatactagtatatctcttctggtgatccccacactggactcagaagcgagaacccgccaccatggatagcactgagaacgtcatcaagcccttcatgcgcttcaaggtgcacatggagggctccgtgaacggccacgagttcgagatcgagggcgtgggcgagggcaagccctacgagggcacccagaccgccaagctgcaagtgaccaagggcggccccctgcccttcgcctgggacatcctgtccccccagttcttctacggctccaaggcgtacatcaagcaccccgccgacatccccgactacctcaagcagtccttccccgagggcttcaagtgggagcgcgtgatgaacttcgaggacggcggcgtggtgaccgtgacccaggactcctccctgcaggacggcaccctcatctaccacgtgaagttcatcggcgtgaacttcccctccgacggccccgtaatgcagaagaaaactctgggctgggagccctccactgagcgcaactacccccgcgacggcgtgctgaagggcgagaaccacatggcgctgaagctgaagggcggcggccactacctgtgtgagttcaagtccatctacatggccaagaagcccgtgaagctgcccggctaccactacgtggactacaagctcgacatcacctcccacaacgaggactacaccgtggtggagcagtacgagcgcgccgaggcccgccaccacctgttccagtgataataggggttctctctgagtctgtggggaccagaagaatactagtttattctcaaaaaaaaaaaaaaaaaaaaaaaaaaaaaaaaaaaaaaaaaaaaaaaaaaaaaaaaaaaaaaaaaaaaaaaaaaaaaaaaaaaaaaaaaaaaaaaaaaaaagagacg